European Patent Specification EP 3 458 466 B1, published August 7, 2024. Title: DIAGNOSIS OF INFLAMMATORY BOWEL DISEASE BASED ON GENES. Applicant: CEDARS-SINAI MEDICAL CENTER MCGOVERN, Dermot P. LI, Dalin. The sequence listing filed with the application follows.

SEQUENCE LISTING (341 sequences)

SEQ ID NO: 1 - DNA, 1001 bp, Homo sapiens
cctaaggaagttctagactagtgtttcatggagcccattcttttaaattaaaagtagccatttaaaaaaattaaagtcccagaaaatgaccattagaatatgcaatttaaaaatagcaaataaaacaaactaaggtttttttgaacagatatatagaaacaaaatttcacttagtttacaatataaacatgcatttcacattagcattaaaatgctattgtgatttatctctctttcaaatactattgcctctacttacacaatcatatttgtcctttcgccacaatctgcctatttcagcaaactgcatcagcattccctttaagtttcccaatgctaaagctgccaggacggactgtgaaaaacacaaacatcagatgtactttaagttaatgaaataaaccacagggaagcaaaggtgaaggctatagataagtgtgtgctttaaagggcctcaaagcaaatcaaagcattacacccttttccggtgtgcgatgccaygcaagacacaccagaactgggactctgacctgttcctatgaatgactttgtccccacaacagtgacaaggcctaggctgctcttgtgattatgagatagatgatctgatggcgtttagtagcctgcaccttgggacagagaaaggcagaccttcagacctatgacagactaacatttggaataaattcctcccaagcagagacagtctaatgtgtgtttgtttattggagtcaaggagatgggggttgctctttgttaaaaaaaaaaatagcttgggaagcttgaggtcctggaatgagatgacttgaggcgggctttctgggacagcatgaaacatatctatctagttcctgctatatccccagaacctactatgttaaatgcatacaggaggggctttaaaattagtcagtgaatgagtggctgagccaatgaatgaatatttcccaggccagtactaatccctacagccaagcttcagacttccaattcttccacag

SEQ ID NO: 2 - DNA, 1001 bp, Homo sapiens
ttgtttattggagtcaaggagatgggggttgctctttgttaaaaaaaaaaatagcttgggaagcttgaggtcctggaatgagatgacttgaggcgggctttctgggacagcatgaaacatatctatctagttcctgctatatccccagaacctactatgttaaatgcatacaggaggggctttaaaattagtcagtgaatgagtggctgagccaatgaatgaatatttcccaggccagtactaatccctacagccaagcttcagacttccaattcttccacagccagaatgtgatcttttatcttgcaggaattgtgatagttaaggtgaaaaatgctgaatagctaagtatattctcttcattctttggattttatcgtaattgtaggaacatgcccctcaccgtcctgttccccctgccaatttattttattctgaatggagtatggaatttgtatactgctataccatgaaaacacagtgtacaaagaaaagccaaahacagtttttatttttatatcttgaggacagttgaactgatctgcctatttctaattttcacaggtaatccttataatataatatctaagcaattaattttactaactgtgagaatagaggtcacagtttagaagaaatatggtcttaagtgacttttaaaaaatttggcacacaagtgaatgccagttaaaaaatggtgaaaattgaataaagtctgtaatctacttaacatactatactaatgtatagtactgatattgtactacagctgtgtaagatgtcaccattgtggtagctaggcaaagaagtcagaggactgtacaacgggcctctccattttgcaggacttttaattctctaagtataaaatatgtcaagagacacctgtgcgaagagactttttttttccattgggcattatttcccacctagtcagtattctacggaaaaacaatttgaagtaatttacgatgacatacatatacaacagattactttta

SEQ ID NO: 3 - DNA, 1001 bp, Homo sapiens
tcttagatattgaattatatgctaaggttctttggaactagcttcctgaattttacacagttgacatattttcattggaacaatcataaaacgaaagatcattaaaatattaaggaaacaaaggttaaagagggaaacgctgatttctttactgtaaatagatcccaatttgcatcttttaaatccttttggatttccccatctggtcccctccctgttataggcactaaataaatattagaaaacagtcccttcaaaacatgtagtcctttccttatttgccctgcctctcttctaaaaaaaaagaaaaacagaactaactagagattattggctgcacaaacccatcagcacctgccagtttttaaatttcattttggaaaatcagccatcacttaagggacttgtccataatagcttcattaaagctttgttttttatcaaaagggggccacatatgtaaacttgtggaagtaatttacctcctctactcttgtcttyttatttgattgcaaaagttaatgttattaaagttgctatggaagcattaatgttcagcctgaacaagagcttgacgaacttctttatacaagcaataacactctgcaaccccattttatgagatatttttcatgatgtagacatttactttcttagcacaagtgatctcttaagattaatttcttttccattttccttcagttttaaatgatgtaatatagtaatctttataacatgatcagccaagtataatttgagaagtcagttctgttggcaaatatctgaaggacaaaaccaaagccaccctagctgaggtttttgtcccttccttctttcatttaccaaaaaccttaattgggttaacagtaggggaattttagaaatcatgttttcctaatgtaacctgtgaaacaaaagcaaaatagattaaggcaaggggaaaaatgaacttaccaagagtgttctttttcctaagtaaaaaccacaaattttatagtttt

SEQ ID NO: 4 - DNA, 1001 bp, Homo sapiens
gatttcctggtggattttttggcttgatcagcttaagaaaaatggagttgtcattaactgaggtagaaaaaatgctggtagagcagattaggggaagatcagcagatcagccttgacatgttgaaatccagaggaagatgctagaaacatgaattaaatatccctcttttatattcttgttcatgcagtgtagggtcagccatttaaaaaatttcatttacatttctaagtggtaagttcctgtgtttagacaaaaatatgtatcaagtgcttaaataacttacaaaataattttaaagatacactgctcaacatgtattactttcacactttatgaatttctgtaatgtatttgtctcttcacaagttgttctgtctcccagttgcctcctctcccctccaatcttgttctggtttatatacgtttatttttatcttccaacatggtctcttgacttcttcctaaattagggatcagattttggtactaggaaatttccratatgtgctctgaggcaggcaagtagaggctcagccccatgtattcccattactagaagcatacccaaccttagtggcctacaagaaagaaaacatttaaggataaggataagtaaacctctaaggtgttaaggttgaatgtactgtgatgtgggcacaagaattggagtgcttgtgcttgtttcttgagttttttgtttttgtttggtttggtttggtttggttggcaagaagagtgcagagggcacctttgcttgggaagatggagacctcagcgacaatcctatatataaggcatttgcctcaacttcaagccaaatgattgagtaaataggctcctgttttcaatttcgacttcctactctttttagaggagaagttcttaacccaagatttgtgaggcattttatatgtaaattgtgtgtgtgtgtgtgtgtgtgtgtgtgtgtgtgtgtgtgtgtgtgtgtattttttcccccaaagtccatagggtgtatgag

SEQ ID NO: 5 - DNA, 1001 bp, Homo sapiens
aattgagtcattattaaaatgtccaatcgtcccataaatgccttaattaaaaaacaatttattcaaatcaggagttataccacctacttttgatatttttctttcatctgtaggtcactgaatttaaaaactaccaagtagcaaggtataaggtatacattcctcatgctaagatttttgtaaaaactagctccaggcttgtattgccaaaatatactcagtgtgtttatcttctttaaagaaaataataataataaggcgcctggattaggagtctgaaaagtaatctccatttagagactccacatccatcagtctctggctggaccagaaaataggtttttgtgtaggaatattttttcagaggattaaaaatgtgagcgaggggtgggacacttaatcctgtgttctctagaagagtgcatttaaaaggatagatacagttcttggcaaaagcatggtaagcacttcagggttattattttccaggaaatacttatyctttttccaaatagttataaacatcagcagaatccagttcataactttgtgatttgcaaattggttgtgactgagattggattgaaaacccagttttcttgctttttgacagttgttcaagaaagagagcctttggtgtgctaaagactcttgtgcccatcttggagtggctccccaaataccgagtcaaggaatggctgcttagtgacgtcatttcgggagttagtactgggctagtggccacgctgcaaggtaagatgttggcagattgagagttctggtctccagcaggagtttaacacttctccccagctaccataggtctgtgacagatggttgcttacccttcaaggcctgtatctttcctgtagagccccttagtggagagagtcacctctcttctccccttccttagagttctcttcctgggaaactgctgccccactaggtgcagaggtccaatttagaggcatatactaggcagtggcttctcaattttt

SEQ ID NO: 6 - DNA, 1001 bp, Homo sapiens
tcaggctaatatctcagagagtagttaaactttaggctcttgattggggttccagggcaggactctgtcactgaaagggaatcctagttctcagcatactaggaaaaatagccaagagaggaacttatgccctaaagaacaaggcatgaatctaattagcagcactggggtccaagatagagctggacaaacaacaaggataactcatcccaaattctggagtgcttatccagaacttgctaagtgctacttcctaaagaccagaacctccaggcagatttgcaagtagggggaaagtctaataaaactttaggtaattctgatggaaaaaggcaagaataacattcctgtgtttgaatttataatacagcctaagacataaagaagtcattattgacaatgggaaggaaagtaatttaatatgcaacataactcaatccatgaaataaatatttatttatgtaatacaatttgctaaacaccaccattattaaggagagyactaggaaaaactaccaaacacagcatgtgaaacagttgggcacggtggtaaagggcacagactctggagccacagccggctaatacactgcaatattttatgtttagcaaattatagctggtctgtgtataaccagaagagcggtatctgggggatcaggatatctaaattctagacttacagcctggccctgaatctaactatcaatgttgccttggaaaaactgctcaaacttttgatgtctaaagtttcagacttgtaaacttgagagggttgaggtccaaggtcccttaaatgtaaactttaaaatgcttttttgggaatctttcaaatcttcaagctcttcaaagtgcaaccagactttctccttactatacagtctgaacaactttgagaatcactgtattatcttagtttatatagtaatcctgacctaaattttattattctcattttggagacaaggaaatagaggcctaggctagcatggctaaataag

SEQ ID NO: 7 - DNA, 1001 bp, Homo sapiens
actttctccacaaaaccaggtgaccacaccttcccctcctaccctaccgaaccacgggacctaggtccccaggaacagctgtatgtgtaagagaaagccacttggaggggctaccgtgctgggagtgtgggtgcgcgtgggtcccggggagctatctgcaggctcgaagtccactttcacccaagcccctggcaactggctgtccgggctgcttcctcacaccccggtgtcttcctattttgccccgattgtcagactccacgtagctagatcataatggggccctgggcagtgggtccaagcttagaagctcccgggcctgacagatctcaggaaatgacagctacacatagaagcgagagctaccaggggccaatgtacttgagaggccagtgaaactgagatcttcagtgggtctggggtctggggggcagtaagagcagggaccagggtcgggatcccaggagttcgaggctgtgggcagaagacagggagagaacyggaacttgggtagagccataagctgggaatgaagggggacaccggcccagggctgtgaacaggggacagtggccactaactcaggtacaggattggctctctggctctgcaactccctgcaaaatgtggtcactgcagtgcccatcttagagagcttctgaggattaaatgagatcatctttgcacagacagcacgaagtctagcctagcaaatgtgcactgaacagtagctagagtgacggaagaaaaagctaggaagcagtcttgtcgggagctggtgcttcagcctgagggcagatcaggctggggaaggctgagaggggccacagttccatgcctgcatggagggaggagaaaggcacaagagactagaaatttcctgtttgcctgtgtttccagaaattcattgtacaacacacgaaccccttcaatacctggataggtctcacggacagtgatggctcttggaaatgggtggatggcacagactataggcacaa

SEQ ID NO: 8 - DNA, 1001 bp, Homo sapiens
tactaaaaatacaaaaattagccaggcatggtggcgggcgcctatagtcccagctactcaggaggctgaggcagaattgcttgaacccgggaggcggaggttgcagtgaggggagatcatgccactgtactccagcctgggcgacagagcgagactccacctcaaaataaaaaaaaaagaaaaaatacacccagaatctgacctcctctcaccatcccattcaaccaccccaagcctgcaatgctgtgtgactggcctcaggctccaatgcctgggcctgtctgtcctctgcagccgccacagcgatgctctgtgaagtatcagccagcacctggcactgtcctgctctgaacacttcgcagcctctctcaagcagggttccagagcctgaggccctaatgctctcaggcagccagtgtatgcaactaaggagctgctctcccaggatgaggtgcctcccatccctgggagaactgaacaaataatcactctagtcacttmtgccttccagggctcaggtgagccccaatgagaaaggctcctccacaggcttccaactaagagtaaggcaaaatctctccgtgaccttccagactctccatgagccagcccctccgttatttcttggaactcatctaccatcttctctccctcagtaactgcactggccacacggcttctgtgcaatcctgcatttgtcctagctggccccgatactcagaatgtccttcttggctgggtgtgatggctcacgcctataatcccagcgctttgggaggccaaagcaggagaatagcttgagcccaggagttcgagaccagcttgggcaacacaaagagaccccgcctctacaaaaaatacaaaagttagccagttgtggtggtgcatgcatgtagtcccagctactcaggaggctgatatgggaggactgcttgagcctgggaggcggaggttgcagtgaacgaagatcgtaccactgcactccagcatggacgacagag

SEQ ID NO: 9 - DNA, 1001 bp, Homo sapiens
gccaggctaagggctgtgttgggcatatgggcacaatcagagtaatagcgaagggagggacaagagaaggctggggccggggcatacgatgaccccccgactcaacacccagtgccagtaccagtaggacccagagggttggcacagcacaagcacccatgaaggcaggccctggggtctgttccccgagtgggtggccatgccccaatccacagtgctaatgggaggccccaggagctgcctttgaagcccttccccaaacaccacttgccatgtgagtgtcaaccaggaagtctttattgagccagaagagcaccccaaccccccaaatccttgagaggctaatggagaacaggggtggggtctctaagggggggggcgtagacaggtggggaggaggctgaatgggcagagcagacagtggaggtgaggacctgccagaaaccgaggaagcccctgctcctcgtcagggccaggtggtcactggtcctgcctgctcarccaccccaaggctccagaatcacccctcccctcttccttccctgtcggctttgccccagccccccacctgggcctcccccgagcctccgatccattctccatatagcagcctgaagggtgttttggaaagctcagacctgacttgcctcccagagaccctcaagaaacaaggtcaaattcccacctcggcctgcgagactcctgtgtgggcaggccccaggggcacctttcccaatggcgacagcctgacctcctcccttgaccaggccccctccttcgtcccctaggtccagaaccagccagcaagcacctccctcggtccctgcagtctcctgctgctgccgcctactcatccttccttggtctcagcctgagtgtcccctttttcgggaagtcttccctgatgtcccacacccaggctgggttacatggcccctctgggctgcccagtcccaggccacccctctcagttgttactggccagggacttcttgtctctc

SEQ ID NO: 10 - DNA, 1001 bp, Homo sapiens
agaggactcaccggggctgagtgacagggataatgggctctggcctcctcttggcctgcggtgcctcttcctccaggggggacatggagctcagggaacccaccaccgagatggcttggccctgggctgacaggcgccgcttgatcaggacgctctctgtcttcaccaccttctcctccttgggctcctccttgcactgtttggtctgctctacacctgagggggaggcagcaaacagacacccagtgcgtcagacccacctgctccaacccgaggacctcctgtgtgcctggctctgttctgagccctgtacacacaaaacctcgtttaaatccacacaacactgtcctggagtgggtactctttttatccccacttttcaatacaactgaggctcaaactagaaatgccattcattgctggggggagcagcaaatgctacagccactttggaaacatgatgagcagtttttgttttttagactgggtgtcactctgtcrcccaggctggagtacggtggtgcaatcagggctcactgcagtcttgacctcctgggctcaagcaatcctcctgcctcagcctctcagcctcccaactagctgggactacaggcgcatgccaacatacctagctaatttttgtatttttttgtagagatgaggtctccatatgttgcccagcttagtcttgaactcctgggctcaagcgatcctcccgccttggacttccaaagtgctgggattacaggtatgagccactgtgcccagccctcagctgttttttttggagacggagtctcactccatcaccaaggctggagtgcagtggcttgatcctgactcgctgcagcctccacctcctgggtccaagccattttcccacctcagcttctggagtagctgggattatagacacccactgccacacccagctaatttttttgttttcagtagagacggggtttcaccacattggccaggctggtcttgaactgctgacc

SEQ ID NO: 11 - DNA, 1001 bp, Homo sapiens
ccccgagccttgacactgggagaaagaccttgccaagaccatgcccaaatcccaccatccaagattcctctggatgggcaacaagcagccccgacctccctccagaggcctttgtcttcccgatccaggcggctggaccacgagggcaacttgggaagggggtggaagaaaactcagccgccttttaccagagctccccctgggccaggcccaggctaagtgctgcgggagcacctctcatgacattctcacggcagcctccagggggcgaaattacccctgctaaacagcggaggtccgtgccggtgccgggacctgtcctgggtcacatgtacattctcaccgcagcctccagggggcgacattagtcctgcggggtttggtttttttgttctcttttttttttttttttttttttttttttgagagatggtcttactctgccgcccaggctagagtgcagtgagtggcgcgtttcttcctcactgcagccccaaactyctgggctcaagcagtcctcctgtctcggcctcccaaagagttggcattacaggtgtgaaccatcacacctggccttatcgtggtatttctaaagcccaaatttctagcacctcttaaaaaactgggccatttttcagctctgggatgcatcctggccgggcacacagcggtggagggtgaggagcagccatgcctctcccgggtgcacaccccttgagggttaccacagctcctaccacccagctgccctccctcatcacctgggagctggcccagtcatacaccctggagcactgctattttcttggcaggaggcagagcagagcctgctgtcctccaccgggctccctccggggtcagacgggggaaggggagggcaagcaggctagaagctgctgtctgcagcctggaggcggggtggccggggatgggttacctgcttcatgatgaggcgggacaggatgttcatgacgaagccccccaggcgggggtacatggtc

SEQ ID NO: 12 - DNA, 1001 bp, Homo sapiens
gaccccacattaagaactccagctcttggctgggagtggtggctcacgcctgtaatcctaatactttgggaggccgaggcaggaggatggcttgaggccaagagttcaagaccaacccggccaacatagcaagacccccatctcaattatttttatttatttatttatttttatttatttatttttttgagacagagtctcgctctgttgcccaggctggagtgcagtggtgtgatctcggctcactgccaagctccgcctcctgggttcatgccattctcctgcctcagcctccggagtagctgggactgcatgtgcctgctgccacgcttggctaatttcttatatttttagtagagacggggtttcatcatgttagcaaagatggtcttgatctcctgacctcgtgatctgcccacctcggcctcccaaagtgctgaggttacagatgtaagccaccccatcctgccaagactgaagttgttttgtgactggattgtscaatgctgtctttcgcctccaggccttggcacaggctgtgccctaagtatgcttgggcccccactgaccctgatgcccacctctcctgactggctcactcaccacctcctcctccatctcctgttcgccttcagtgccgcctccactccgggtgaacagcgccttctgtttctccgccatcttgtaggtgggctgcatctcggggtcgtcccgcagcgtgtccagcttggggtggaaccactcccactgcgtggtgcggttcagagactccaggacagacaaggggtcctcaggccgctggttcaggatcttggtcagcagattcaccaggtgctcgtacctgcctcccgcaggaggagtgggaggagagggacctcactcactcagctcactgagctggctcccatgtgcctggccctgtgcctggtgctggggacacagtagggaactgaaaaggtccctgcccaggtgtagctgacatttatttatttatttttatt

SEQ ID NO: 13 - DNA, 1001 bp, Homo sapiens
gttaacaggtgtgaaccaccgtgcctggccaacatttgtattttttgtattttttttttgagacagggtctcactttgtcactcaggctggagtgcagtggctcggtcttggctcactgcaacctctggttcccgggttcaagtgattctcccacctcagactccccagagctgggattacacgtgtgccaacatgcctggctaatttttgtactttttgtagagatggggttttgccatgttgcccaggctggtctcaaactcctggactcaagtgatctgcctgcctcagcctccccaactgctgggattacaggcgtgagccaccaggcccggccacagtcagcctttgaaaccaagttggtctgatttccaagcatgtatgtgtcaccttttgctttgcggaagctgttttgttggcagtcttgggtgtggtgttgggccatcatggaagttgggaagggtaagaagaggtgagactttggctagggcttctcaggragagagcctgaagctctgaagagctggcacttggggaatagccagaggttaattctgactagattctaggatccgaggaaggagcaggtagtgactagaaatcaagtttggtcagcggccaggggctgaaccacgtaaggccttttgtttgttggtttgtttgagacagagtctcgctctgttgctcaggctggagtgcactggcacgatcttggctcactgcagcctctgcctcccggttcaagtgattctcctgcctcagcctcccgagtagctgagatcacaggcgtgtgccaccacgcctggctaactttttgtatttttagtagagacagggttttgccatgttggccaggctggtcttgaactcctgacttcgagttatctgtctgcctcagcctcccaaagtgctgggatcacaggcatgagcaaggccttatatgtctcaggccaggagccttgaaggttgtggtgaggagtctgagcttccccctgtgggc

SEQ ID NO: 14 - DNA, 1001 bp, Homo sapiens
gttcactggtgaagatgtttctggctccacccacctgcttcgtgactcggtttctcaggcgcagctggcttggctgcgagcccagaccaggctccacctgctgctgcttcctgagcctgctctgcggtgaatgccaaacaggagccagggccaggctccacctctgcccagtaacgtttacgctcctgactaaaaccgactgtctctgccctcgagaagctcacagccctgccagataacttttctgcaaagtgagatcacttttccacagctggaccaccttgagaatggggctaaaaatctgtttcctcccaactacaagcctgttatccccattttccaggtaagggccccactgaacccaaatggcagataggtggggattaacatacacttctctctcccgtttatcacgaaaatgttctgtaatccaaaaatgtcaggggcagaaagaaaaaaagtggtttcaaatcctgctgcaaactggaagagcagaccttytaatctcaggtgctagtctgtcactgagctgcttctcatgtgggcagacctgtgcctctagagagaggggcaggaaggacttatgtttatgtaatgacagctaaagagtcccgttagcaacactgggaaggccagctcataaagtgacagtaacacagaggtttatgtgcctgagttcatggactccttgcatcagcgtggagggactggaacgtcttccccatttttactgacgggcccaaggtcgcagtgagaaagcgagaagtgaacgcgaacccaggtctatcagctccaggctcctaactgccgggccacttgacgtttcctcaggagtgacatgcggaccgcctgcaagctacacagcctgggtcggcccggggtgaccacccttcgggcttggcacactctgaggtggagcaggttggggaagagctggagctggggacacagccttgcccgtgggtgggcagggcctggtgggctcaggggcctcaccggct

SEQ ID NO: 15 - DNA, 1001 bp, Homo sapiens
aggcagcagtgagggaggcctggaggggcatgaggggaactatagccaccaacagctcgggctgcggtgtttgaaccctcgctgcagaccacacacacacacacacacacacacacacacacacacacacacactctctctctctctctcgctctcttttttttttttttggagacagagtctcgtcgctttgtcactcaggctgcagtgcagtggtgtgagctcgactcactgcaacctctgcctcccaggttcaaacgactctccttcctcaacctcccgagtagctgggattacaggcatgcaccaccacgcccggctaatttttgtatttttagtagagacagggtttcaccatgttggccaagctggtctcgaactcctgacctcaggtgatccacccgcctcagccccccaaagtgctgggattacaggcgtgagccacctcgcctggcctggaccactctttctctatgtggccccaggaagccagttcacctrtctgagcctcagtggctgcacccaggaaatggggagactcatctggcctttgttgcagggtggcagtgaagcctggtgacaaggtctgcagcacacctgctgcagtgcctggcgcccagcagggcctccagactgggaagccactgtgattccactcccgagttggtcatcggtttggaccagggtgcagagggaagggcacaggctggcaggatctggcttcaaatccaggacctgtcccctggcccactcctagcctctctctccacttccctccgggtgcctgaggccccaaccttaaaaaattcctgtccattcatccaaaatccagctccaggttgggcacagtggctcctgcctgtaatcccagcactttgggaggccgagtaaggtggatcacttgaggccaggagttcgagatcagcctggccaacatggtgaaaccccatctccactaaaaatacaaaagttatctgggcgtggtggcacacgcctgcaat

SEQ ID NO: 16 - DNA, 1001 bp, Homo sapiens
tcgctttgtcactcaggctgcagtgcagtggtgtgagctcgactcactgcaacctctgcctcccaggttcaaacgactctccttcctcaacctcccgagtagctgggattacaggcatgcaccaccacgcccggctaatttttgtatttttagtagagacagggtttcaccatgttggccaagctggtctcgaactcctgacctcaggtgatccacccgcctcagccccccaaagtgctgggattacaggcgtgagccacctcgcctggcctggaccactctttctctatgtggccccaggaagccagttcacctgtctgagcctcagtggctgcacccaggaaatggggagactcatctggcctttgttgcagggtggcagtgaagcctggtgacaaggtctgcagcacacctgctgcagtgcctggcgcccagcagggcctccagactgggaagccactgtgattccactcccgagttggtcatcggtttggaccaggktgcagagggaagggcacaggctggcaggatctggcttcaaatccaggacctgtcccctggcccactcctagcctctctctccacttccctccgggtgcctgaggccccaaccttaaaaaattcctgtccattcatccaaaatccagctccaggttgggcacagtggctcctgcctgtaatcccagcactttgggaggccgagtaaggtggatcacttgaggccaggagttcgagatcagcctggccaacatggtgaaaccccatctccactaaaaatacaaaagttatctgggcgtggtggcacacgcctgcaatccagctactcaggaggctgagacgggagaattgcaggaacccgagaggttgaggttgcagtgagccaagattgcaccactacaccctagcctgggtgacagagctggactccatctcaaaacaacaacaatgacaacaacaccaccaccaccacacacacacacacacacatacacacacatgca

SEQ ID NO: 17 - DNA, 1001 bp, Homo sapiens
tctgattttcctgtcgcttggccacctcgactcccccgaatcctgtcccctccaccttcaaggagctgccacctgccctggctcctgactttgaacacatcccagagcccttggccgagtcccatcttactgactgggacttggtggacccaaggctcgcccaatagaggctaaaacggtggcccaggcccctgcggggacacaggattgggagtggtacagggatgcccgggaggcgagtgaggaagccaggccatcctgccaccgtctccccagcaccaaggctcgcaggttcagccgccagcacaaccgcatcgtgaagcaggacggctccagcagcgaggctgaggactgggagacgccaaagcccttctaccagctgctggccgagaaggccttgccgctgcccccgcacctccagtgagagggcggcccctcgcctcgctcccctcacccctcatggcaaccgcggctcttgctggaagccaggacccatcgatkaacttgtccctcctgggcctccagcccctgagaatgcaggtcccatgggactggggaggggggcactgattagccccaaccgctgggcacatttgcctggagcaccagagtcacccacagctgccttgattctcccccaggcttaggaaggaaacccaaaatgaaatgcggggtgtcggaaggtgaagtttacccacccctctccccttcccttccccaccccagagccactcggttgcaaccctgttcatgctcacctcaccctactcctccctctcctgttctatttttagactatttattgttttaaataaaataaagcaagtggaacctttgttaccagcaagagagacaagggcaggccctcctgcgtccccctgctgccccactggggtgctccgtccaccctcatctggaggcctgtggcttgcaagaggcctcagtgccaccccctccccagccactctgtgcatctgaatgcaaacccctcttcccctcgg

SEQ ID NO: 18 - DNA, 1001 bp, Homo sapiens
gcctggcccacataacataatctataatataatcttagtaaatacaaattcagcatagtttaaggtaaataatgaaacatttcagcatggtctgcctgccccaccccaccagcccctctcacccagcttcatcttcttgagtgtggagtccgagtcatcgcggggccgcttgcgggtgtccttgctgctcggcatgttgcgggcgatctcggcctgaggtgtgcccaggtccaccagcagggtggtgatctgggcctggaactccaaggaagccgggtgcttcagcacactcaacaggtgcagcttcagattcttacgcacactgctcacctgcgatttggccagcgtcgggggcaggttggctgtgaggaaagtggcaggagctgtgtcttgtggaagatctcatggcatgctgccagtcttaattctcaaccccaaacttgggcagtggtcttgcaggcatctactagaaaagttccttcaccctcagatctaacgtghggctttccgccttacaagctgatgcttcaaaccctgggggtctccatcagtatcagtcaatcttaaagagaaaaactcaccctctcttttagtaaatacatacaatttcgtcctcctccatctctggtctggaaattcacatatgcttcgcttggggagggttataatcaccacttttgcctccagaaacccccaactgaactgctgcaacagctcactgctagtctccctgacgccaggatgactttctaatggtcaccctgataagtgagcctcccctgttccacagtgaaaaaggatgcctgtaattctgcctgcctagcatccactgccccttcctcagccaacaacacaacccactctccgttaagggagaccccccttctccagtctccttccgagtgggcatgagacctggggccagtgagaataccacattcccttggccactgtaattggctcagagactggctcataatctctgctcagccaatcagaaa

SEQ ID NO: 19 - DNA, 1001 bp, Homo sapiens
ttgcagtgagccgaaattgcgccactgcactccagcctgggtgacagagcaagactccgtctcaaaaaaaaaaaaaaaaagaaggggatggatgggaaggagtttggaaaagcacaaggagctgttagctattgtgttgatcggcacaaatgaatcaataaatttgctcttccccaactctccacccctcaccaacaccctattgcaatattctcaattcccttcccaagggcctcgggcaaaaatggagccctcctggctagactccatctcccagcgcgcccagcggggaagcaccctgcgcttgcgctgccaagtcctccccggctttgtctcccgggagttcgagtcgttcttttcctccgcccgcctaatttgcttcctaccccacctccaagcttgaccgtgctgccttctgggggatgtagtccgtggctgcccggacttcaattcccagcgggcttcgggacgagaacccggaaggggaggctggagaggagygagtgggggaaacccgcgtagccgagggagatgcagcgcgcggcgatggtgagagcccaggcgcgggccgggggcgctggagagtcgggacgggggttcgggaccgggtgacgagggggaagaggcaggggcgaaagaaggggctgggtgaggggagattgcctgggggagaggactgggaggaatgggagccggaggtagtagtagaagaatggtggcttggggaggggtcttggaggtggggtgggagtggagctttggaattgattgtaaaggggctcagagctggggaagtgggccccgagttggagactgggctggacatccaggtagaggccctgaaggggtcgatttcgatgggggcttaacctgcggcgagggtatgaggatcagggttaggatgagtgagggggtctggaagctccaagggacaggcgaacggtggacgcaatgggttggggcctctggatcggattgggggcaggaaggcaagttgagga

SEQ ID NO: 20 - DNA, 1001 bp, Homo sapiens
cactcctggggagagactccccgcccctgccacaagagccccaggtctgcagtgtgcccctcagttgagtgggcagggccgggggtggtccagccctcgcccggcccccaccccagctgcccttgctattgtctgtgcttttgaagagtgttaaattatggaagcccctcaggttcctccctgtcccgcaggacctcttatttatactaaagttccctgttttctcagcgggtctgtccccttcggaggagatgatgtagaggacctgtgtgtgtactctgtggttctaggcagtccgctttccccagaggaggagtgcaggcctgctcccagcccagcgcctcccaccccttttcatagcaggaaaagccggagcccagggagggaacggacctgcgagtcacacaactggtgacccacaccagcggctggagcaggaccctcttggggagaagagcatcctgcccgcagccagggcccctcatcaaagtcctcggtgtkttttaaattatcagaactgcccaggaccacgtttcccaggccctgcccagctgggactcctcggtccttgcctcctagtttctcaggcctggccctctcaaggcccaggcaccccaggccggttggaggccccgacttccactctggagaaccgtccaccctggaaagaagagctcagattcctcttggctctcggagccgcagggagtgtgtcttcccgcgccaccctccaccccccgaaatgtttctgtttctaatcccagcctgggcaggaatgtggctccccggccaggggccaaggagctattttggggtctcgtttgcccagggagggcttggctccaccactttcctcccccagcctttgggcagcaggtcacccctgttcaggctctgagggtgccccctcctggtcctgtcctcaccaccccttccccacctcctgggaaaaaaaaaaaaaaaaaaaaaaaaagctggtataaagcagagagcctgagggc

SEQ ID NO: 21 - DNA, 1001 bp, Homo sapiens
tcaggtgcattggagattcttaggagtgtctcttgggggtaatattttattttttaaaaaatgaggatgtcactcttacccaggttggtcttgaactcctgggctcaagcaatcctcccaccacgggtctctcaaagtgctgggattacaggcgtgagccaccgcacccggcttttttttttttttttaaacggagtctcactctgtcacccaggctggagtgcagtggtgcaatttcagctcactgcaccctccacctcccgagttcaagcctcccgggtagctgggattacaggcaccgccaccatgcctggctaatttttgcattttcagtagagatagggtttctccatgttggccaggctggtctcgaactcctgacctcaagtgatccacccacctcagcctcccaaagtgctgggattacaggcataagccaccatgcccggcccaaatgggctaatgttttaaacagatccttcttgtctgccctgtaggagkacaaattatcaggggcaggggtggaagctggagcccagaaaggaggggactgcaggtgggaagtgatggtggctggaccaggatggaggccactgaggggtatgaagcagtcggatttgaagctgtttaaaaggtggaggtgagaggatttcatgaaggagcacatgaggacacagcagcagagaggactccttggctttggatggtggagagactaaagatagagagattgggttcgggtagggggagaaccacgtgtgctctttggaaaggttaggctggcagtgtttgtaggacatgacaggacactgagtgtaagggtctggagctctcaggagaggggcgagctggagatagtaatgtgagaggcactgggtcctgagagggtgatttggtgtggaccggagcacaggtgaggcaaggcaggcctcgcagctgaaactttatatccagagcagccagggccactgctggctgcggagtgaggacgcatatcccca

SEQ ID NO: 22 - DNA, 1001 bp, Homo sapiens
ctcaggcagggaggtttagttgcaggataagagggtctcaggagggctgggcacggtggttcatgcctgcaatcctagcactttgggaggctgagatgggcggatcacttgaggtcgagtttgagactagcctgggcaacatggtgaaatcttgcctctactaaaaatacaaaaattagctgggtgaagtggagcgcgcctgtaaccccaactactcgggaggctgaagcagaagaatcacttgaacttgggaaggagaggttgccctaagccaagaccacgccactgtgctccagcctgggtgacagggtgagactatgtctgggggaaaaaaaaagcaagagggcttggggagccaaatcacgtgttctggaatcctgactctgccatatcctagctgtgtagttttgggtaagcgacccaacttctctgtgtctcggtctcctcctctgtaaagtaggatgagctgatgtgctcatctccggtgagaattaggtgagdgtgtgcagtgccagcacatgtctgggaagtgaatgctagctgttgttggcattgattccgactcagctgaattagagtcactggttttccatgagggatgatcccttgtctgactgactgaggcaggcacttcgggtggggcccctccctgcctgggtcccccacccgccccactcctagcccctgctcacaggctgaggtcgcaattgatgctggtctgcagcaggtaggccttggcgttctgcacggccagctccagaggctcgggctcaggcacctgggcactgtagtgtgggaagcccagctcagagggcaagaactgaagggcagggtcatcccttatgtaaggcccgtgctgggcaccttcagagaactggtctgtctggtagaggttgaactggcccaaggggttgactgggggctcctggaaggtggggtccagttgctggaacaggctgctttggccctgctggagccgctgcagcattaggctggtggtg

SEQ ID NO: 23 - DNA, 1001 bp, Homo sapiens
gtcacacagcaagcggaggaactaggatttgaatcccagtctttctgcttcaaaaactggagcttatatatcaacctttatgccacctcctgggactgtcccctgctttgtcccactttggggcagctcttactcttacatccctacacactattaaaacaaatgaaggccgggcacggaggctcacgcctgtaatcccaaaactttgggaggccaaggcggatagatcacgaggtcaggagattgagaccatcctggccaacatggtgaaaccccgtctctactaaaaatacaaaaaattagccaggtgtggtggcacatgcctgtaatctcagctactcaggaggctgaggcaggagaatcgcttgaacccaggagacggaggttgcagtgagccgagatcgtgccactgtactccagcctgggcaacaaggcgagactccatctcaataataataataataataataataataataataataataataataacaatgrtaataaagtaactagggtatgttcaggttgattagctcagggaaaaggaaacttgagaattaggttcatatgccactttagaagtctgagcagctatcccaagacctttcagtattcattaattcaataattctttattgagcacccactaagtgttaggcattattccaggacttaagggatataaccagcgcagcattatggcttctgtgggccctatacaattttaccttcttgatccccttcttccatagaaaaatattaacgctgggtgcggtggctcacgcctgtaatcccagcactttaggaggccaaggcgggcagatcacgaggtcaggagttcgagaccagtctggccaacatggtgaaaccccgtctctactaaaaatacaaaaattgggaggcatggtggcgggcacctgcaatcccagctacttgggttgctgatgcagaagaatcgcttgaatctgggaggcggagatttcagtgagctgagatcg

SEQ ID NO: 24 - DNA, 1001 bp, Homo sapiens
ggaagtggaggttgcaatgagtcgagatcataccactgcactccagcctgagcaacagagtaagaccctgtcttttttttttttttgagacggagtcccgctctgtaccccaggctggagtgcagtggcaccatctcggctcactgcaagctctgcctcctgggttcacgccattctcctgcctcagcctcctgagtggctgggactacaggtgcccgccaccacgcccggccaattagtttttgtatttttagtaaagacagggtttcaccgtgttagccaggatgacctcgatctcctgacttcgtgatccacccgcctcgggctctgaaagtgctgggattacaggcgtgagccaccgcgcctggccatgagaccccatcttaaaagaaatagagtcagatgtatctcactccaaaggctcttgccttcaaccattctgtcactcaaggttcaatagatgtttgttgaatgactgaatgagctccctttgttgggacrgttacaggacctgttgatcttaccttcagaaggtctttgagagtccagactctggtgtagcccccaagctaaccttcctgaagtttcaattactgaggcatctgtcttgaaatctgggatgatgcccaattgctttctacatacaacctttatactagtaataataagtaacatttatatattacttcatggtttataaggactttttcttagcgagtgccaaccatatgctccaagcctggtattagagataataagcttaaaaagactgaggctggctgggtgcagtggctcacacatgtaatcccagcactttgggaggccgaggtgggtggatcacttgaggtcggtagttcgagaccaacctggccaacatggtgaaaccttgtctctactaaaaatacaaaaattagccaagcgtggtggcacattcctgtagcccctgctactcaggaggttgaggtgggagaatcgcttgaacctgggagtcagaggctgca

SEQ ID NO: 25 - DNA, 1001 bp, Homo sapiens
gcaaagtgagatcacttttccacagctggaccaccttgagaatggggctaaaaatctgtttcctcccaactacaagcctgttatccccattttccaggtaagggccccactgaacccaaatggcagataggtggggattaacatacacttctctctcccgtttatcacgaaaatgttctgtaatccaaaaatgtcaggggcagaaagaaaaaaagtggtttcaaatcctgctgcaaactggaagagcagaccttctaatctcaggtgctagtctgtcactgagctgcttctcatgtgggcagacctgtgcctctagagagaggggcaggaaggacttatgtttatgtaatgacagctaaagagtcccgttagcaacactgggaaggccagctcataaagtgacagtaacacagaggtttatgtgcctgagttcatggactccttgcatcagcgtggagggactggaacgtcttccccatttttactgacgggcccaaggtygcagtgagaaagcgagaagtgaacgcgaacccaggtctatcagctccaggctcctaactgccgggccacttgacgtttcctcaggagtgacatgcggaccgcctgcaagctacacagcctgggtcggcccggggtgaccacccttcgggcttggcacactctgaggtggagcaggttggggaagagctggagctggggacacagccttgcccgtgggtgggcagggcctggtgggctcaggggcctcaccggctgctcaatgaccctcagcaccgtccgcttgatgtcggcgatggcttcagtgtacacggccgccagttcgtggatcagcttgtggttctgaggcaggagggccaggtagaggtacagacactgcttcactgtctcctccgtccagggtgctgccacctctgacagggcaggagcgggcatcagattggcccacactcttctccaaccccctcggaccctcaggaatgtcccttcttgggcagtggagc

SEQ ID NO: 26 - DNA, 1943 bp, Homo sapiens
gctaaggggaggtgggaaacgggctgacagaactgctgtgttgaggtgaggactcctgactgtgcgacccccattcatgcattcattcactcattgaatttttttttttttttttttttgagatggagttttactctgtggcccaggctggagtgcagtggcacaatcttggctcactgcaacctctgcctcccggtttaagtgattctcctgcgtcagcctcctgagtagctgggattacaggtgcctgacaccacgcctggctaatttttgtattttttagtagagacggggtttcaccaagttggccaggctggtctcgaactcctgacctcaaatgatccacccgccttggcctcccaaagtgctgggattacaggtgcgagccattgcacctggcccactcattgattcttttcttttttttttttgagatggagtctggctctgtcgcccaggctgaagtgcagtggctcactgaaagctccgcctcctgggttcacgccattctcctacctcagcctcccaagcagtggcttacgcctgtaatcccagcactttgggaggctgaggcgggcggatcacgaggtcaggagatagagaccatcctggctaacacggtgaaaccccatctctactaaaactacaaaaaaaatagccgggcatggtggcgggcgcctgtagtcccagctactcaggaggctgaggcaggagaatggcgtgaacctaggaggcagagcttgcagtgagccgagatcacgccactgcactccagcctgggcaatagagcgagactccgtctcagaaaaaaaaaaaaaaaaagccaggcatagttgtggtggtatgtgcctgtagtcctaactactcgggaggctaaggtgggaggattgcttgagccctggaggtcagggtagcagtgagttatgatctcatcactgcacgccagcctgggcaacaaagcaagttgctatgtcttaaaagaaaaaaaaagctgggcatggtggctcatgcctgtaatcccagcactttgagaggctgaggcgggcagatcacctgaggtcaggagtttgagaccagcctgaccaacatgaagaaaccctgtctctcctaaaagtacaaaattagttgggcgtgatggcacatgcctgtaatcccagctacttgggaggctgaggtgggagaattcgcttgaactagggaggcggaggttgcggtgagccgagatcacgccattgtactccagcctgggcaacaagagcgaaattctgtctcaaaaagaaaagaaaagaaaaaaaaaaaaaaccagccagggcgcagtggctcatgtctataatcctagcactttgggaggccaaggtaggcagattgtctgagctcaggactttgagaccagcttgggcaacacagtgaaacctcatctctactaaaatacaaaaaattagccaggtgtggcagcgtgtgcctgtaatcccagctactcaggaggctgaggcgggacaatcgcttgaacccaggaggtggaggttgcagtgagccgagatcgtaccactgcactccatcctgggtgacaagagcgagactctgtctcaaaaaaaaaaaaagaaaagaaaagaaaagaaaaagaaaaaaaagaagaaagaaagaaaagaaaaaaaaatgcctctgtccccaaaggtttctgatgggattatccgctaatatctgttgaaccaatgaatggatggatgaatgaacgaatgaatrttagttgcccagcagagagtaagagcttgatgtcagtattgcagggtcatgcgtgagccccctgctcctgccgtttgtgagaggcgggagtcccggcgctcacctgcggcaggatgtgctgtgtgtgatgcacccagttggccatggagtcgaccagctccagcacggggatgccctcgaagtccgggttctcctcgtag

SEQ ID NO: 27 - DNA, 1001 bp, Homo sapiens
aacactcttcactgaacctctttttgctttctttctttctttctttctttctttatgaatgagatggagtcttgctctgtcacccaggctggagtgcagtagcgcgatctcggctcactgcaactgctgccgcctggattcaagcaattatcctgcctcagcctcccgagtagctgggattacaggcacatgctgctgcgccaggctaatttttgtatttttagtagagacagggtttcaccatgttggccaggctggtcttgggctcctgacctcaagtgatctacctgccttagcctctcaaagtgctgggattgcaggcatgacccactgcacctggcctcttttgttctctggacagggtgccagctctgctgcttcttagccttctcccatggtgtttctctacggggaatacacacccctcccacctcaaaaccttgtcctgtattatgctgactcctgccctcccctcagttctcagcctaggtgcttcttgcrcagggagcccttgccttgcctggctcctgctgtggctcacagtgcccttcatgttaccctctcaagcactacactatataattatttgttttctctgtgacttccagaagaggctgggccccaggagagcaggcccaagtcggtcttaggcactgccatttccccagtattggcatgggcatggaaagaatgcttcttgagttaatgattaaggagaggctctcttcctgggcatcccacaggtcctcatcagcatggtgtacctacccgaggccatgccagcctccttccaggccatctacacccccgtggagtcagcaggcacggaagcccagatcaagcacctggctcggctcatggccacacagatgacagctgccggactgggaccaggtgagtgtgtcctggccctaacctgggccagggattggcacttgtggcttctgggttctccttactggaagagcaacttctcgtggtgcagttgaaaatcatgtggg

SEQ ID NO: 28 - DNA, 1001 bp, Homo sapiens
cccaacctaatcttttccatagtattgggcttgaaccagagacttacagtgtgcaggatcctaataatccagcccaccagcagtcctcttcttataaagacacctcttctcataaggacaccataatcagtaatcaggttttgctggctgtggaagtactctggacagattagataacagtatgtatcaatgtaaatttttgaagctgatactgtgtaaatgtaagggaatatctatttttagaacatacacactgaaatgtttaggaccatattataagtaagtacttataaatgtactttaggaccatattataagtaagtacttataaatgtactttaggaccatattataagtaagtgcttataaatggctcagaacaaacaattatgtatatatatctgtaaatatacacatggagagagtgagcatacatgcacactgtgcaaatgatgaatggggtaaaatgttaacagtgaatctcggtgacggatgtatgcrtgttccttgtgcctttttctttgcaagtttctttaagtttggggttatttctaaagttaggatttttttcaagagtaataattaggattcacttatatcttttaggtttttaagaacctacaactatttatggagaacaagcagcccgaggatgatctttttgatagactcaatgtgagtagatgaagcacacaatgttgaagggagtcccagccagagcctcacagtacctaaaggggagggttgctggcagatgacttgggctctccctttagcctggcctgctctgtggcatcccatacactctctcttcctccctctgagtccacggtgaatctgtagtcaagagaagacacatctgctgcagaacaactgctaaagcactcagggtggggggtagatgagccctaccttttatccttccctgctcctgcagagctttcccttcactgaatgcccagccacccctgctggagacccaaaacctgtccctgatatct

SEQ ID NO: 29 - DNA, 801 bp, Homo sapiens
acaacctttatatcaactttttttcctctaacaatgaacaatgaaaacaatttgtgctccatctttaaaaatgtgtgacacaaaaattttttaaataaaaataaatatgtgataaacattcctgaatgcctagtgtgtgccctggcgctgtgctctgcatttaatttggatcagcagttctcagccttgtttgtacattacaaccaactggagaggtttttaaactcccagtatccggggcatcagtattcgtctagggcacagtgattctaacacacagtcaaggttgagaaccacttatttaattcatcctgtaaatcctcacaatagaatcctgcaaggtagcttttatcaccacctttgccgatgaaattgaggctcaaagaggtaaattgatttcrgcatctgtagccccaacctgtgacctctccttccttccttctcgggctcccttcagggatttcctgatgttacagaaaatggtatgtatgacgctgccctcctggccaccttgacatagctctgctcccaacagggctcttctgagatagcagccagacactacctgggatcaggactgatactaaatgacttctgccaaaatgaggacaactgaggccagtcacttccaaacaggttctgtcaccctgagtcagaataatggcagctacctctcctcctcaccgcccagtcgtttctaagcctggctcgtcgccgttgctgctccgccaagcctttcctcggtgccctctctcttttagaacaaattacttcatctccaggcccttctcagggcagctt

SEQ ID NO: 30 - DNA, 1001 bp, Homo sapiens
cttcttgttcatcataaataatgattaacttagaatgtacttctcccctctcttaaaatgaccaatataaaagactacttattaaaagaatatatattataaaaatacaagagtaataagttcacagcagcacaggataaacaggaaagacaccatcagaatagcatgaggacttctgggccaaagggaggggaaatgccatcaggactgactgaatgacagcaatactaagacgtaaaggaaatttcaatttgaaccaagcaaaagaaggaaactctaaaactgtgaatataaccatagaaccctaggggggaacaaactcaaattcagagataagtgaagctggatgtagaagtagaagtgagcccaggactgtcaggagaataattagaggcctatggaacagctgcatcctccagtgttctcagaaaggctaaggtgtgagaacagctctctgtaataaagtggaggatcagctgtgggggaaccacccacacaggygctgggactacagaatgaagaaacagcaccacaaatgacaatgcacacacccacccagaaggcagctgactgaatccctggacgtatatccctggtacttagcaggaccagcactcctgtactctgaatttacttctggaagaataattcccacttgtgctgagagaacccactacagttaccactcggatcacacaaagagttctcaatcctggatgcacatcagaatcatctgctgagctttttagaaataccaattgcctgggccccaccgcaatgcaactgaatcagtatttatagagggaagagggatctaggcatttgtatttaaatattctccagataatttaatgtgcccttaagtaataacaaataaaaacagcaaaggaagcagaaaataattgtagtattctctgaaagatctattaagataccatttcaaagatctatggagatactaagggagaggaacaatactaaaaagttattagtggggaata

SEQ ID NO: 31 - DNA, 1093 bp, Homo sapiens
cagtgatgtctctgagcatcagtggtgtctcttctcagtggcttacagctccagacatcacatgcagacgtgacaatgtctaatggagaaggggcacattctctcccaattctactcaatgagaaaccctttccttcctggaggtccttcagcggccattcacacagatcccactggcaagactggatcccatgctgttcttacaccagccatttccaagagaatgaggccaccataactggcttaggccaattggtaggacccttcaggaggcagaacctgggaacctaggcagggctctgcccacaggaagaagcaggtgagcgtgtgggggtggcggrtggttgtcaaaacccaatatacagggaacattacaggaagagtcacttactttacaatcatgtcatttcataaacatttcttgacataattagggaacaagaggcagcatgaaggagcacagcttccctgccattccccccgccacagtgagacgcctgcaaggacacagacacagcctttccatcagccttcctctgtggatcccccatccacactgagccagcaggtcaatggggacaggttccatgctgttcagagaaaccagcactgtacacagtggggccctgcatccactgcaggggtggacgcctcagccagcccaggactgtgccgtcatccctgagactcactgatcctgatgtgagactctccccgacaggggcttccaggcatggctctatgcagggtcatttgtggccacactatgacgtgggcgatcccatttctacacatctaaattccccagggcaggcagcatgtggtatctcactccctcggctctaacctggttatgggaagttgctaggtaactgcttcccacactggaggaggcttagttaccatggaaagtccagatgggtgggggggcacagaggaagggagcactggctggggggtctgcagctgggattctgtccccactctctcctgagcccctggacctaaggggagtctctcaacccctctgggcctcagtttcctcctagtaaaatgaaggaaaggctgggtcacttcttgctctaaaccactg

SEQ ID NO: 32 - DNA, 1001 bp, Homo sapiens
ataataataatagcccacattattgatactgacatgtagataggtgaatccaatataaaatgataggaggtatgaaagaagttggtgagtttggaatattatttgactggctataatatagagtaatggggtgggagccagagggaaatcgaaaaggtgacctggaaaacattgttcagggccttgaatgctatgttgaggtattttgactttataaaatagtgggggacaaactacaagtattttatacattgaggtatagtttatgaagtttttttatatgtatagcttatgtaaatctcaaaggaatgctgagaagtaggcgttattatcccattgtacaggtgagaaagctgagtttgtggaatatgcatacattctacattattgagcacctgctatttgccaagcactatgctgagctatgagactagaaggaagttgtagtttaatactctaatagaggaaacaggaataaatcagcaattgtaagtagttgcyataataaaggcaaacaatgttacgggagtgaaagggggacttgtctatatttgcatagtcagggaaggcttcctggaggaggtgagcttaaactgagtttggagaaacaaatagattacagtaattgcccagagatatttaactaggaagcagtttacctgaaacttgaacccaaatctcctgtgtctagctctttcccctactccaaggaccaatctttggtccttgattttaagctctatcagcaactcagtcacaagtggacttgttatgtttggagaaggtcagagattccaattttttatttttaaattcattcattttctccttttaaaatctctgtgtgtgctcaaagagtagattggaagcagaggaactggaagaagaacagaatgttctgatagttcaggcaataagtgatgaaggccataactaaggcagaggtcatgggcatagtgtgaatctccactctgttcactctcctcacacatatactttta

SEQ ID NO: 33 - DNA, 2093 bp, Homo sapiens
tggttttctcctttaattttttgaacttgaggttctataaaagtgaacacagtttgcttcacctgacttcccggacaccatttctccttctcatctccttgactcatccgttctcaattctatgacctctcaactttgaaggagcccattctctaacctcttgtcttctctatctatattcactccacaggtagtgttatccacttgcaaagcggtaaatactcttcgattctgacaactctcaaggttttctcttcagcttctcctgacctccaaactcgtgtatctaactaccttgacctctactcctggtcttgccttccaaaccttctctcccacggtctctcctgtctcagtaaatgacacatccttgcttctaggttctcaggccatgaacctgggagtcaccttaactcctgtgtttgtctcttatagctctcatgatatccatgagcttacctttgaaatacaaggtggctacccagtctagataataaatgatttattgatgctacattctaatacaagatacaataacattatctatgtttctagactttatgatcaccctgtatattcaaaatccaaccacttcccaccactyacatcatcctgttttaagccacaaccatctctggtctggactatgaaagtagcctctttttttttttttttttttttgagatggagttttgctcttattgcccaggctggagtgcaatggcgcaatctcggctcactgcaacctccgcctcccgggttcaagcgattcttctgcctcagcctccctagtagctgggattacaggcatgcgccaccatgcctggctaattttgtatttttagtagaaattgggtttctccatgttgatcaggatggtctcaaactcccgacctcaggtgatccatccgcctcagtctcccaaagtgctgggattacaggcatgagccaaccatgcctggccaacagtaggctcctaactggtctctcttcttctgttcttgctcccttgctatctaatttcagcacaacagccagagctacccttttaaaacttaaaacccaagtcagatcatactactccccagttcaaaatcttccattggcttccatctcactcagagtaaaatccaaaggcctcgccatggcaacaaggccctacatgttctgctctctctctgatctccatcccaactcctctccacctcactcacagtgttaaacatgtctccacctgaagtctttgcacttgctagtccctatacctgcaaaagctatttccccagatgtccatccaggaagtactggcttcttcactttgttctagactttgctcaaatgtcctttgatttcccaacgtaaaatcgcaacccccatctcagccacactccctgtggctcttgcatcattttatttttctccctaacagtaggaccatctgatgtaccttctgtttctccctttaccagaatgtaagatccaggagggcagagattatgttttgttcactgatagttttccagcacctagaacaggactaacacagagtaggtgttcaaactttatttattgaataaatgaaacgagaatgtctgaatgcacactattaaataagaagtacatattttaccataaagttaaattgagcataattatggcaagaagttcagatattggccaggcgcagtggctcatgcctgtaatcccagcactttggggggccaaggtgggcagatcacctgaggtcaggagttcgagaccagcctgaccaacatggcgaaacctcagctgtcctaaaaatatacaaattagctgggtgtggtggcaggtgcctgcaatcccagctactcgggaggctgaggcaggagaatcatttgaacttaggaggtggaggttgcagtgagccaagattgcgtcactgtactctagcctgggcaaccgagcgagactcagtctccaaaaaacaaaataaaacaaaaaacaaaacaaaacagaagttcagatataaacaaatgacccctcaaaaggaattgattaaaaaaattttaaacaaagtatggtttaaaaaagaaacttctccactgtggctaagt

SEQ ID NO: 34 - DNA, 1001 bp, Homo sapiens
ctgcacagttgtacatattggcagggctcagcttccttaaatgccattggatcagtagggaaatggtgattttccttattgatttaatgccagttcctcttttatgaaaaatcccacgtgctgctcactggcgtatgtaccataaaaactgaacgtagggggccagaaattaagtaagtcactcatgttcttctccagccatgtgacgttaaaccatctctactttcaggctggagtgttcaatcattctccctttaaatttagcagagtgattattcctcctggtggattgcacatatgctcctttgatctatgaaatactcattctggatgaactttaagctcccaggaaatgcatgtaaaatactgtttataaatcgcgggagaaatgtttcacattcttattactcccaagtaatcataccaagcctctctctccaagattcgctttttttcctagaagagggaaaaagaacttcgggcagtagcactgtgacaatmatcaccacggtcgtactttccatgagttttacgcagtaggctcacggaagtgacaatgcatggtcgggcgcggtggctcatgcctgtaatcccaacacttcgggaggccgaagtgggtggatcaactgaggtcaggagttcaagaccaccctggccaacatagtgaaaccctatctctactaaaaatacaaaagattagccggacgtggtggtgggcgcctgcaatcctagctactcgggaggctgaggcaggataatcacttcaacccgggcggcggaggttgcagtgagccaagattataccactacactctagcctgggtgacaaaacgagactccgtctcaaaaaaaaaaagaagtgacaatgtaggatacccattcatcagcaaatatttaatgtgagcaggacaatgtgctaagtccatagactgcaaagaggagtgaggctgggttcccatcctctggggcttacaaggtagctggagaagtaaaactcaaac

SEQ ID NO: 35 - DNA, 658 bp, Homo sapiens
tgattaaacattcctgaatgcaaatgttttcaaatgtccaatgacttcccatcatccttggtatgaagtcctaagtccctggcatgctttcaatgtcctccatgatctgcccccagtccaatcactgatcccatctcctgccagtccatgattgaaccagttgggtccccaactcctatttgcacacaccattctctctgtgtgtcatatatgagctctctactctgcctagctacttgtctgcaagactcagttcaattgtcacctcatttgggaagcttccactaatccctcctgcacctgtctccgtcctaggctagattaggagcctgccctttgggttcctgaaccacttgaggtgtggttcctttatcatgctgatctcactggtttggctgacttgtttttcctacaagactgaactgtctgaggtcttaagatgggctgtctagtccacactggatcttcatgctctacacagggcttgacacagagtggggcacaggaaatgtttgttgaacgaatacacaaagcatatggatactcctgagagagagraggtgggcaagacagccttgtgaagttaagcagcagaaaatctgaaaacgaacctggatagaaatcaccaattcctggaagtacagagagaggaaggaga

SEQ ID NO: 36 - DNA, 1001 bp, Homo sapiens
tggccacccagacctccttcctgcgcttcacactcaaacaaggctgttccccatgtcttgggtctgtctttcctctacctggatcgttcttccccatggcctggtctcagcattgagttctcaaatgtccccccttccctcaccttatccgaaggacccattccccgtcctctctacattctgtcctattaccctgtctggtttattttcttcctagtattgattactactggaatcctcatattcatcagtctgctggtttaatgcctgttccctttactggaatgtaagcatgattttggtctttttctcctctgtcctgagtacccagaacaaagcgtggcctatggaggacactaaatgaacgcatgggggaaaaacgggttttattgcagagggagaccctttgtttcatacagatcgtttgtaaacttagatattttattagcaacaaattatgatagagcttacaaactccttgagaatcgctgcggtagtagrtgggggtggagcttctctaggcagcatttcagtgtgtcctagcttggatgctgtggcttcccgagctctgaatctatactgcttactctgggcttatggagtgtgtagcagggaatccttgttgaaggatccccaaacccttgatagccatggacagcccacagtggtcatggagccggagccagaatgtaattcccagtgtgaccaggagctagagtttaagtcaaggcagcaggtatactcaggtgcattttccattccctttgagggaggggtggaggtttgagccccctccacatcccaccccattggggtgcctttgtcactcttgacagctttagagtgacttagatgggagattggtggggaggagggggggaggggcactgtttgaatctaccctgctggaggcactgaatagttttataagtatgtgtacactctattgttcaagtgtttgcttaaatcactgtatcttcttagaaatttttgtaaccttt

SEQ ID NO: 37 - DNA, 1001 bp, Homo sapiens
gataataacgcctacttctcagcattcctttgagatttacataagctatacatataaaaaaacttcataaactatacctcaatgtataaaatacttgtagtttgtcccccactattttataaagtcaaaatacctcaacatagcattcaaggccctgaacaatgttttccaggtcaccttttcgatttccctctggctcccaccccattactctatattatagccagtcaaataatattccaaactcaccaacttctttcatacctcctatcattttatattggattcacctatctacatgtcagtatcaataatgtgggctattattattataattatgactgaagtagtaggagatagaaacaaatgttgcttttgtctactaagtgttttgttatcctctgtcttttcccctcatcctagtcaatattccattaaaacacaggttcgattacatttttcaatgcctactggataaaatcaccttgtagtatggataakgttcttcatgatccaacttccctctgttatttaaccttcctctgctgctccactaatagcctttgtgacagttgtagtaactacagtacatgtagtttttccaagataataggctggctcagctttcatgcctttacacatgatgtgtcctttgcctcttacgtcctcctctactttgtctatccagtgaactccctgtcatcctttaagattcaattcagatgtaaactcttctgtgaaacctgcccttaaatactcagtggcagaattagatgatctcttctctcttactatgccatacatatcttgttacaatcttctctgacggtgcctgtcacctccactagcctgtaaacgtatccagcagagggctgctttttatctccgagtccttactgtctggcacaaagtgggtgctcacggaaaatcagttgaatacatcaacaattacccgtcagtggcacctgaagccatcagtcactggagctaccccatcattg

SEQ ID NO: 38 - DNA, 1001 bp, Homo sapiens
gactttactgaagcagaggagaaggagatgatcaatctattcaatatgaagaaatatctctgttgctaatacaatatccttttgaatatctcccacatcttaggccctggtgaaaatccctttcaattgttctgtctacctcgtagggatgttgtaagaataaatgagttaacatagatatgaagtgccttaggaaaaaggctctataaaaatgcaaggcgatatcatgattagttgtttctttgactcttgatcattttcttcccacttcttatacaaaatgtctctcacttatttcctgaagccatctcttttagaactattgcttcctagaagagctgaaaatgatcctagttccaacatatttattgattcccagataataacacccactggtgttgatgactgacagggttcatgcctaagcttgagtagaacttgcccttttttcctgggtcaagaaaagtctgcaattgttcgaaaatgtgtcagtaagtgtgmttccatcacgatttcttaaataagtaacagttgctgctggataatcctgggggcagatgattcatttttgtgcccctatcaaacaaactcaaaacttgttaaagaatctttataagttgtttgaatcaaacaatagggtcgctaggtccccattttgtccatttgaggtatttgcccagcataccttggtctgtaaagaaatagcacagccttggctgggcgcggtggctcatgcttataatcctagcactttgggaggccgaggtgggcagatctccaaaaataaataataataatgataataacacagcctcatgagtcttttttttttttttttttttgagacagggtctcactctgtcactcaggctggagtacagtggcacaatcacagctcactgcagcctcaactaccctgggtttagtgatcctcccacctcagcctctcaagtagctgagactacaggtacacaccaccacacctggctaatattgtattt

SEQ ID NO: 39 - DNA, 1001 bp, Homo sapiens
gaaaccttttatatccttacaactattcaatcttcctgttcaggaaaatggaatatttaatatctttctaataatcaaatattctctatatctaggaaagtcatttttatgtatctcaatcaagttttatagttttcttgatatgggttctacacattgacttacatccatctacatttttgatttttatactgggaatgagatggagctgctgctaactctggagaaacttactgctgatcttttatctttggacatgatcctgactgttctcctaagtgatggattatcttagatttgaaaagtataggaagtaaaggacaagagggacatgtggggggatgtagtagagtctgttttatattcatagtgagaagactctgaacctcccaggagggctctaaaggttaaaaaacatgcaaccaaaagcaccgaggattagtaaaaagaaataatgtgcagtaagtgctcagagggatgactcattgcattggatcatcyttgggaaaccacctactaagcagaatttagcagctaaagcgttatttttggtgcacagtttattgctacttcctcttgggaaaaaaagattaatcctagctccctaaaacacttaagaatggtcaccctggcaaaccggcctgtcaggtaacaatgttgtttccagatcagggcagtgttaggttccctgtagggatttcttcagaacaagggagaagcactttaccacatgttatggaaaggagtatagaccaggagacagaagatccagctcttagtgctggctctgtaactgattaacaaataaatcccagagtgcaggcaggccacttaatctctgctcatctgctaaaaaacagatatcacagcttctgtcgtactccatatcatggaagaaaataacacaaaataataaaccatgtgaatgaagcagttaaaactgctgagaaataaaattaacctgctcagtaaaagtaaggctaccaatcaagaacaaatag

SEQ ID NO: 40 - DNA, 1001 bp, Homo sapiens
ggcaatccttgctttttattaccacactggattgcttctgtacacagctaagttgcctgaagcatggaaacttggacttctccatctgacacgttctggaagcctcaaggcacaagctgacagttctgcttctacagaaaaactctcacactgctctcctctcaacagtactgcctgttcccactactccacatgacacctacgagggcactacatcacgtgagggaagcttcttcatgagggcagacaagaggaggcaccacccaggcactggtctctgcctggcatctattccgagggccacctggcacagtttctaaattaaggcatatctaaaatgcttttctacctttagtttttatttttgctatatttttgcactctactatatgcatatttaataaaaacaactacaaagtcctttactttaattcctttacataatgataaaacacctagatacccaaaatactacatctatatattcaaatctactaatcrtgttacaaatgcatgcagcttatttgggggcttagtctaatttttattttcttaggtccatcaataccatgataatgaacattagatgcaaaatcctaacactttctgccttcagttgtactttcacaggactagtgtgattcagaaataaataacatacatgaataataatagaaataatttatgcaaatgtagaacaacttgaaaaaaaatcccccgcctgtcaggtgctgttcctgggggtagctgatgctataaattccatgtactaactaatatatttactacaggtaataggaaaacaaatgaataaaaagtgaggaactatgatatacatgtgtatatttttgcaaacacaggatcagaatgaaaagatatatcatgcactgtgaggtttaagaaatgtattactgctgggatttgttttattattcagactttaagatcaaactgagagttgttggtgatcacagaaatattgctagctgatacatattatt

SEQ ID NO: 41 - DNA, 1001 bp, Homo sapiens
cctttccatttaagacatgtctttgaaaatagactctagtttaaatgttagcagatagactttgaagtaattatgaggaagaacttgggactgaggatggtcaaattctaaaacacagtattggatccaaagacaggtttctccaccctttaagaataaatctgtcaggccaggtgcggtggctcaccccgtagtcccagaactttgagaggccaaggcaggtggatcacctgaggtcaggagtttgagaccagcctggccagcatggcaaaaccctgactctactaaaaatacaaaaattagccaggtgtggtggtgtgcgcctgtaatcccagccagctatttttgggaggctgaggcaggagaatcgcttgaacctgggagacagaggttgcagtgagccaagatcgtgccacactgcactccagcctgggggacagagagagaatttgtctcaaaaaaaaaaaaaatccatcagaaacgtctcacctcaatatagcrgccaatgttgtcccatgtaaaagtcagggcacatggtctattgatatgaaaaccataaatcagaatatttcccattgaaactgccttaggcacagcttgcacattgtaatatctctcaaggcaagaaaatgacctttcagaatagacgtattctagctaaatccccaggcatcccaatcaacaattctggcttccctaaatttccatctgccagagttcgggctgattctgggagtcttcttgttttgaattctcaatggggtgttagtgcggtttttaacacccctctccagcctcacccctgatgtggctgcattttggcagcgaggaaaagtctgggttagaggtttgggtttcatgagcccttccaagaacaagagcagctaagctgacacaagagcacactctccctaaacagtcttttctgccacctctcccactgattttatgtaaccgagaagaattagaaaagtgtgaaaaaagcaagactgatgtttgct

SEQ ID NO: 42 - DNA, 601 bp, Homo sapiens
gaaaatctggagatgaatcagatctgttccttctctcagtgacactgcagtctagatgggttcagtacaaatatctctataatacaaaatagctctcagaccagtctttgtagaaatagctgtatgataaggcttccaataattataataataaaaaacccagttattgtctgaaatataaacgctcaaaatgcagaaatgttttattcattgttctgtccccaggaatggtgcctggcgtatagtaggcactcaaaaaatgttagatgatggcagcaacggtacttcagggccaggggarccagcacccatggagagatgcagaggcagaaatggattactcaaattgggaacctgatgccccctcttctcactttaatggagttgtagtagttgagcttcaaagaaaggagcgtcctccagtgaggttcctgccccttcctgggcctctctaccacagcaagagccagggccagctggcagttttcaccaccctgctcatgtttttctggagacaccagcttaaccacagccaccacagatcggagggtgctggccccagcctgctgcctgctggttcttctccttcctccctcccttc

SEQ ID NO: 43 - DNA, 1001 bp, Homo sapiens
tacagtcctgcaggctgtatatgaaacacagtaccagcatctgctcctggtgaggcttcaggaagcttataaccgtggcagaaaggtgatggggagccggtgtatcacatgatgagagaaggaagcaagagatgggggaagaggcaccaggctcttttaaacaactagctctcatgtgaattaattgagaactcacttatcaccaaggggagggcacctaagccattcatgagggatccgctctcatgacccaaacacctcctgctaggccccacctataacactggagaaaacatttcaacatgagatttggaggggacaaatatccaaaccatgtcactgacctgggttcacattgtcagtctgccacttatcatcttgatattcttgggaagataactttgcttctctgagccttggttttcttctagaaaataataaaacttgcttcacaggagtgttaagaagagtaagtgagataatacttgaaaagcacttaaytttgcatatgacacacagtaagggcttaagaattgtcgccatcatcatcaatatcattattattctctgcacaataaaatgtgttggaatcacagcagataatccagttatttggatgagtttttcccacgtcatgggctgagcagatgagttgacaatgggtgactgttgagtgtctaccatatactggcactgttatggaagtgtgggcacagctcctgagagttgcctaagtggggttatgacctgtattttcctagtcatcctacttaggaaatcatccccccagttggtgtaagacagtaggctctcttatacactgttgctgggagtacaaatggatgcaatctttttggagagcaacatggcagtatttttttacgactttttaaaggcatatttggattgagtaattttcctttgcaggagaataatctggatatgctgataaaatatgcccaacgtggcatggataaatatgtttgaaacacacacacaca

SEQ ID NO: 44 - DNA, 1001 bp, Homo sapiens
ggagatattgaccactgtgaagatctgtttcctcccagctgatgcagacaggtcctgagaccaccggaatggtgcattctcaggggccccagccaggcagggtgtgcagcctgtactcagaggaccctgagcttggttttattttctcccatcagcatttgacactcttaatgatttttgaacacgaggccctgcattttcattttacgctggaccacacaaattccatagctgtttggcagccaagccaagggctgaggacagcaccttcctagagggctgtgcacaagccaagttctcagcagcaacttttctgagagaaaaccatctagctccaaatcacgtgttcattatccattttcttcccaccttttgccacttctcctttttctgtggtccctccctgtttagcaggtatggaaggtttgggggagaagccactcattttctctgcatctcttctggccctgtttctacctccaaatctgcaccatagccccrtcctcagcttccttgtatttcctgaagctgtgtcctctctcccccagcccctggccgcacccatctcagtgtaatggtaccataaaggggccaaggaagagcctgtttccttggcagcttacatctccccctgggattgccaacatgcaggagtcagcccttcctgcctcattacctgaacagcttccccttcaatccctgaaacactgcactggagtggagtctactttgaaagtgaaagtgatttagagtctactccatttcgagaatttgcatgttaaccccttgggctgggcacagccccatggagatttgtttctttcctggccagtcccctctcctgccaggtggtctttgcttctttgcagcccctcaacatgacagcatgtttgagtcctttccagcaagaagctgaactccccaggagtctgccagttttctagaaaacattggttactggctcctttctggttttgaccattctttactcagggcttagc

SEQ ID NO: 45 - DNA, 1001 bp, Homo sapiens
ttaagggggacttcaaaataaaaaactatggacacactcctggagagcagcacggaggagggatctatgatggtgtaataattgtgagtttgggctagatatgactgaacaagtaaaggttgccccaggcatctcacagcgggatgcagaaaagcatcctgatgctacccagttgaggaatccaagacatctcctcccctcctatcagggagggcacgaaggggcttcactctacagggagggtggaagcacagcagccttacattgcagctagggtgcagcaagccacagccaaggccagaattctgcagagtgtcccaggaagagaaaagtctaggtagaaatcagccaataacagagcagaagctaaagagcagacaatgcaacttccaagacaaagacttagcagaaaggactctgaagctagaagcagctgtaacaggggggatgagatggtaatggttaggaataaagaagtagaacatgaagaggggcctttcrccatgctgatagtgataaccatttctttactgaggaggaaccagacacgatgtggtaatctgctttatatactttaaatgtaatgggccatagccaggtacagtaggagaaccacacacttgtccttttataaaatccagaatgcaaaaccttctccactaggtactgttcatagaattatctgaacagaaaagacctttcttaataatttaagtcaagattctattgctctacctgggcaaatcagtaagctacactgcccttatcccttacaaaatcctgccttctgtctgggcatgataacatggttagacagggtcacatgttatatatatatatgcagagtttttcattgcagcaaaatatagaaatcaacataaatatgcaccaataaagtgctaataaaaagattatgttcatccaggcaatggaattctatgcaactattttaaaaagggtgtgaagaagtgctctaaataatatgaaagatctaagtcata

SEQ ID NO: 46 - DNA, 701 bp, Homo sapiens
cacagccactgtcttcacagggaagcttggtggccttgagctaacatgaaccggtaagtcctttcctttttaacagcactttccttggaagaatttctcgcaggccagccttacaggctcctcacatgtccactcgtgtgaggtgtaccggcagtagagttagtcccttgagaggccatatcagggcttactccacagccyctgggacgacagcccagtgtttcagcaaaggagctgcttacaatcttgtctatattaaggcccctggcctttcctttaaagaacagggatccatttaacaccaaaacattttggagccccctctctccatccctatcatcagagtcctgctttctgtgtccattcatttaaaatatccataatgggctgggcacagtggctcacgcctgtaatcccagcactttgggaggcagaggcaggtggatcacttgaggtcaggagttcgagaccagtctggccaacatggtgaaatcccgtctctactaaaaatacaaaatcagtcaggtgtggtggcacgcacttgtaaacccagctacttaggaggctgaggcaggagaatcgcttgaacctgggaggcagagattgcagttagccaagattgcaccactgcactccagcctgggtaacagagcaagattgtctcaagaaaagaaaaaagagaaaagatccataacgatcca

SEQ ID NO: 47 - DNA, 1001 bp, Homo sapiens
aactacttgtagttcctcaaatcaccatgctcactctttctcactggtcttctctcctttgtcttcttggaaaactatttcacctgtcaagattcagcccaaagcatcatgttttgtcaagtctgtctgaatgctttaggcattgctaagtatgcctttgcttctgctcacagcatccatgaataactctattatatcacttattacactgctttacaactacatctacattcttgttgttattctccactacatgatgtaaatatttttttttacttatattcaagaattaaaagaaaaaaaaaccttaccttttcatggcaaccaaaagtactgaatgtgcatggaattggggctgtagggcagtctagatcataatgattaggcatctgaaatccaaaacaaaggctgaaaaatctcttccttgcatatcattttctagtttgatgcgatcacatttaaactgtattgtcaatggctgctttgtaccacattggcagytgaataggtgcagcataaaccatcacccacaaaaattaaaagaacatctactttcaaaagttatagagaaaggaaatatcaacatctcataatatcccctccaattatccaaaattcatttcaagaaaatgaatttgttcctcttgctgggaactggcaccctctagtggcactttacagaaaaaacacctaacaatagctacaagtgcaaactggattaagactcccactatggtctaggccatttaataggaaccagtcaactgcatgcactgaagccactgactacacccatacttgcctcatgaccacctctcaaaaatcatctttgaccacctttcaacaatcttcttaacttttgttaagctgggcatattttagctacaatggggagactcagatgttagaaggtactttaaacacattaatagaagctctaaaaaaagtctcagtcctggattttgggactctaagacacattctctaaggtaagatccttt

SEQ ID NO: 48 - DNA, 1001 bp, Homo sapiens
taagtcctggtgacagttcagcttcacctctaggaccagaaggttccgaatgccctcggaaagggcttctccaggggctgccttcaggccctcaggctttcttaaaaccacaaacgtagccaacacctgaaaagagagggaagcttttattgagaactcctggcctgagaacacctcttagaggaagttggctgggactttccagcctaactaccccgaaaacaactgcgggacccagcaatagcatctattccctggcaggttcccattcacaagtttgcacagggctcttttcggttgtaacagtgtggtcaccctcaagtgggaagacagtgacaatggggccagcctaaggccagtcctgcagaaaaatgatttctaagctgtgctagactctggttccaatatgcagccatcagtttgagcactgcctgggttcctgtggcccacgatgttgtgcagtaagagatggatttttaaaaaatgtctcaaggaggacayaagagctcctcatcctggcattgatgaccatccatgatatgcccttaccaagccagtctgcatatattgctcagtttttctcaaagtatcagtgactcttcactcaagcacatctcaccttcccttacctgctgttccttcactcatttcatcaggacacactcactgagtgtttgctatttattaaccactgtgagttgcagaacatccaaagatttctaagaccaaatccctgctctcagggtactcagcctatggagaagataacagtcttttcaagtattcactcatgcaataaatatttattgagcagctactatgcatagccactcaggcactgggagatataagatggctccagaggccctggtgccctgccccgtggagctcgcaaccagcaggcactcttctatgtcatgcacagtccttcccccacacttttgctcgtaccaactactcctcttgcccagaattctcttcctttttccctctgcttattt

SEQ ID NO: 49 - DNA, 1001 bp, Homo sapiens
aaatataattaacactactgaactgtaaagtactgaaattataaagagggtatattttatattgtgtggggttttgtttaaccacaatttaaatttttttttctaaaggtcttgggttattgggtatttataaggttgaaaaaaaaatgtcatcgatgtattcaagggaagaatggctacaggttcagccaactctcaaatgtgcaaaggttaatttctaacctctattcttcccaaggcttggtaagcattaactgtttgccagaccttggaactttccagcgtcagtttctcattttccttcctactttgtctttctaggagcccctttcctggacacactcgtgtctttcccagggaatgggaagaaacaaaaggatgatgacatgacacctaataagtctggatctggaagtaagtttgatctacggttcattaggctggagcagaaaaaaaagaaagggtccggtatgttcgcctgtgtgccaggtatggtgttaygccactcatgtgccttatattccctacaacccctcaccccaatttatcacttcaaaaatgataaaagctgagacttggagaaactagtaactaaccaaaagtcacccaagaaggaggtggcaagctaagatcaagccccactttggtgggagctaagagtagcccttggtagagtcatggggttggctaattcttgcctttggaacctgtttctatctccattcagttcctttctttcctgtcagttggactttaaactctaagatcaggaaatttccctttatctatcaaatcataccctattgagtgagtgcctgcttagcctaatgtcctgcaaatggacaggactcctctcttctatgactccccagaaatattacaaaggcctgtaggaaatagctcgggacagaccagaggaaatagcatggaggattcacagtataacttataccttcaaaggtgaccaccagcctgcatcccattaaaaacaaaaacaaaaa

SEQ ID NO: 50 - DNA, 1001 bp, Homo sapiens
ccatttacattaagaaaaatccccttcaaaagcaacttaaaagttttggtgctgaaagggttaacttcagttatctggaaagcccaggccctgggtccgggaaattcggtggcagttacagggttactgggaggtatcacaggccttgctaacactcagcttatatgagtttcatcaaaaacttccaagatgtgtttctaggagaaaaagaatgtgtcatctcactttctcctcacagctgccacgccagggcatggagatggggcacagccctgcctgctggggcagtgggtagaggaagatgctgcacttagtggaaaatgcaaatgaattccactagggctccaacctttgactctgaaaagggaagtagaatcatggcccaacaacttaaaataaagaagtgggtggcttataataactctgaggcttccaggaaaaagccattctgagtgtaagtaacaaagaagtcaaagaaaacagccatgccatctgatgtghctgcctggaaaacaaggagaaactagttaccacggaaacaagagagatggcctcttttacacacaaccctcggaagcttctgcagtcagaaagcccagcgtgcaaatccttccctggaccatgaacacaggaatgacccaatgtccttccacaccaccaggatttagataatgatcggtcaaactcaactgatccattctctaattgcagtcagaatggtctttctaatgacaaccttgatgatcatgatagcaccatttactgactgccaactgtgaggcgggcacttgacatgtattatctcagcattttaaaaatgaacttagagggtcttgacttttagtgaaatggaatagaaaatatcggagtgcatcacatttggagaaaataaatttattcatgattactgggttaaaatgcctcatttatttcatacctcatatggcactcaaaactacatgaaagcacctgtttggaagcacctgtgtctgatcttacaa

SEQ ID NO: 51 - DNA, 1001 bp, Homo sapiens
tcttgccattgtttgcttcctttcaatctgtatgaaccttccctaggagtccacatcagatatagcaaggccatgggagctatttttaacttcgggaatactgtatcaaaactaaataaaccacagccgggctcgggggttcgtgccttaatctcaacactttgggaggccagggcaggtggatcgtttgaggtgaggagttccagaccagcctggccaacatggcaaaaccccgtctctactaaacacaaaaattagttgggcgtggtggcgggcgcctgtaatcccagctattggggaggctgaggcgggagaacccagaggcgggggttgcagtgagtcgagatcgtgccattgcactccagcctgagcgacagagtgagactctgtctcaaaaaaaaaaaaaaaaacttaagtaaaccacatgccaagtttctttgcagattctttggaattctgtcaatgtagtgtagtagtgctggacagaccatgtttaatagyagctgtggccagcactttagtgtaataaaataaaggcaaataaattttaaatgcagcttcatggacaaattggtcaaaacatggataaaagtagtgtattacaaagtgcaaagctccaaggtcaggtagacgtgggttctgatcccaactctgttacttattagttgggtaatcttaggtaagttacttaaccttttaagctccatagttaccactttgataagtggtgacaacaaaacttaaatactacataaagttgttgtaataattcattcttactgcctggcactgttctaagtgctttgcacatattaacacatttaatcttctcagtaactcaagtggattttattgttagaaccattttacagatgagaaaattgaagcacagaaaggttatataatttgcccagctcataaatggaagaaaagagttaaattcgtatcattcaattccagcacctgagctcatcaccacttattagcactgcgtttccagc

SEQ ID NO: 52 - DNA, 1001 bp, Homo sapiens
cataagaaaaaatggtgtcctataacagaaccagatgcagagaacattgttacatagaacatggaacatcccaaaagtagtcttacacataaaaagctacttaggaaaaaagaacaatggacagaaaattgagaaagttagattcttatcccagtttccactgttgtgtgaaaagtgacttgaatctcctcctctcttgacccttggataaataagtaaataatttgctacttttacttaaagcaattctaatgcagactggggagtgactctatgctttaaagaaaatagtattttttaaatgtaccttaaattatgatgctactagataaggataatctcaaccacacaaagaatactgactctgtaagtgatcagttattgtgattttaggcatgttaaatcttgtttattacctaaagtgtatggtcaactgtaaaattaccagtatttttaaagaaagtattaactgaaggctctaccttcataatatatccaaartccagtcccttctcacttcctccctctgctaccaccctgttgtgactcaccaccagctctctaacaggcctcctgctttctattcttgtcttccaggctgttctcaatacagcagcgggagtggacctagtaaaataagtaagatgatgtcatctctgctcagaccattgtagcagggtatctgggagtaaaagctaaaatccttataagaccctgtgtgataggcccatgattcatttcctgacctcttttctgctgcactctttgtccttctacccattcattccctctttgctatcccttgaacatgtcaggcatgctcctgccttggtgagtggtggctttagctcttctgtttgtaacactcttgccacagctaaccccttaactcttccactttggctcaaatctcaccttctcataggtcccctcaccaccgtatttataccacagcgtggttccacctttcttgccgaacaatcccaatctctccacctggc

SEQ ID NO: 53 - DNA, 1001 bp, Homo sapiens
ccaatgtggtacaaagcagccattgacaatacagtttaaatgtgatcgcatcaaactagaaaatgatatgcaaggaagagatttttcagcctttgttttggatttcagatgcctaatcattatgatctagactgccctacagccccaattccatgcacattcagtacttttggttgccatgaaaaggtaaggtttttttttcttttaattcttgaatataagtaaaaaaaaatatttacatcatgtagtggagaataacaacaagaatgtagatgtagttgtaaagcagtgtaataagtgatataatagagttattcatggatgctgtgagcagaagcaaaggcatacttagcaatgcctaaagcattcagacagacttgacaaaacatgatgctttgggctgaatcttgacaggtgaaatagttttccaagaagacaaaggagagaagaccagtgagaaagagtgagcatggtgatttgaggaactacaagtagtttgtrttgtgctagttcaacccaatagcaatgtagatgatttgaggtggaggtgggggtactagtacctgagctgttggaatacctaagtgaagacagcttgaattatggcgatgaccgtcaagatagacctaggagccagtacatatttaggagagaagatctactgcctgtgtgactaaataaatgtgatgagtgaaggagagggaggcgtctagaatgactcttggtttctggcctttgtcactgggtagatggaagggccattcggcaaaaaagagtgaacacaggaagaactgactggaggtagagtttaaaaaaaaaatctgttttaatgtattgaattacagataatgacttcacccagctagggaacaggtgggatgactgacatgcattatgtgctgtcttaagccccaaagagaaattaggactcagagtattgatttgggaaagtgatttgtggtaataatggaagttgtgattgagatcatatggcgtatgta

SEQ ID NO: 54 - DNA, 601 bp, Homo sapiens
  misc_feature (301)..(301): n is a, c, g, or t
tggaatcacagctctgccttcgagctgtgtgactttggggcagttagttggcctctctgagcctgtaaagcgggggtattagagtctagtcatgagatatcttataggtaagtaaactagcatagtgctggataatgttgtaacaattcatgtaataacaattactatgtgattttaagatgtcagctcccttttctggattggaggatggaaaggcatatttgcatattttcagttgagttctcccacccagtcctacatttactatagtaaaaccttgtagatcaaatgtaagtaatgnctctctttcctccccacacctaatgctgcacctcccattcagagtcttactagtgaagactagtaagtttagattacttattagtaagaccagagagttaggatcaatacgtgcacccttgtgagatggaatatatttctgccctgagaatctctgttggtcttagcctggaattaagatcctgtagcaccacacctctgctctctgggctttaatagctcctggctgcaagttttttagcatgtgcagcttgacattttatgtggaactgtcttctggcctctcctacaagtaatgacg

SEQ ID NO: 55 - DNA, 1001 bp, Homo sapiens
atggatggaattctctttctaggccatttttattcgatgccagattacatagtaaggtcatttcagtttgagatgcactcactcaactattagcactactgcaaataacagttatgagtatgatcactaagtgttcattttacactgaaaagaaatagaatagtcagtttccaaaccaaatagctatactccctgaacaacagtggaaagtcattcttcttgaagtttgacccagaatcaagtgcagactcagactcctaggcctacagccagtggcaacttaacacattatatggttgaccttcagggaaaaagggaaaccactgctcttaccactggtgccagaaaaaagccaactaatctttaaggcacaaaataaactattcttaaggcagaaaaagaaactgtgaggaaacaagttagaatggaggcatatagagaaaaatacagaaaatacattaccaagtaaggactagtttttccatggttctcagtgttttyatttttgggaatataattaatcagcattttctttttgggttttaactcctactacctggtagaaatgcaaagatgtacaagaaagatgcatttttaaaaaggcttggagacttaaaggcaattatctttgctaattttactttgagccagtgacattaataagttcatatagaaaagtaaatagttgctgggcatggcggctcatgcctgtaatcccagcactttgggaggctgaggcgggcagatcacttgagcccaggagttcaagaccagcctgggcaacatggcaaaaccctgcctctacaaaaaatacaaacattagctgggcatggtggcatgtgcctatagtcccagctactcggggggctgaggcgggaggactgttgaacccaggaggcggaggctgcagtgagctgagatcgtaccactgcactccagcctgggtcacagcgagaccttgtctcagaaaaaaaaaaaaaagtaaatagtgatgggatacc

SEQ ID NO: 56 - DNA, 1001 bp, Homo sapiens
atttacaactccatagtccacaaaattaagtctttaatatggcaccttccaagatcctccatagtaacaacgataatgcaaatacaataacatcaacagaaaacgtttcctgaatgcattatctcattcaatcctcaaaacaaccctttgaggtagtaattattatcatcccattttagagaaaaagaaattgaggtacacatcctcaaccacacttggcctcttgtcaatccatccttatttcagccattcccaactacttgtatcactgtgcccctctgcagacttctgtgctgtggacatccttagcctgcactgccctgccttaggccgcccctgctgtttgttgggtgaacaatggctaatctttttagacccagttcaggaaaggccaaaagctagaggaatggtatttcagcacatatgatcagatttggaagtgatcttaaagagacatctagtttcacaatctatagactatggattccaactcccattagygggtcaaagccagggtttttataaaattgaaataaaatagaataaaaaatatcagagagcagggagtgaaactatgtattgtttcaagggcaggcattgttttgtgaaggttgtgtatgccaggtcccaaagtaaaatgtgttttttactgtgggtagaggtccaaccaccaagccactctccacgccagaagccagaatgatctttctaaatctgattacgtcagactcttactttgaaattttctgtgttttcctatttccattaagattaaagacaaaacaaaacacctcacaatgcctacccagggccctgctggtctcccgttcttctgaggtcatcccaagcctttgaaggtgctgttcctgcctgtacactctacccttgccctttacaccttctaagtcccattaatccttcaagattctactcaaatatcactttccccaagaaacctctgcctaagtttcttgatctagtctaggttgctagactaggac

SEQ ID NO: 57 - DNA, 1001 bp, Homo sapiens
ctggaggaagtgggtgaatgggtcagatctcatttggtggcctcttggggaagaagggtgatatactcctgttttctctctgaaatattcttcctgaggcttgtggtgggatccagggttaaaactgagtgaagagaaaatattgccttgagaaacaataatgactctggcaacccacctattctttagtagcccatctcaattgaccttcttttaattgttcatattggacagactggagactgcagtgtggggagagtcatcctcttacttatcttggcctttggcttcccactgcagacagcccttgcaggtccatccaggttggggaagatggttttaaaaggttcattagttaagaaaggccctggggcctggaaataaagggtttgaggaggagagtagagggtggggtcttcctccccggacctcacgattgggaatgaggattttttttagctacacgggtctgactagagctgtaaacgttactcagattgytcactatgtctcttcccacgagcccctccctgtcaccacccccctgctgtcaaaccatatcttcgtggaccagccatgcgggacatccctcttaatgggagcataagagtgttgtctcagacccttattttgttagtttatgtttccatgaagctcttaatgtttattaaataaacagacaatgagtttgtgtgacatgcccacagcttctgtgtatgtgacacatgcctagcctgtgttctgggagtgtatgtcactttggcctttggctggggaactggtgatggtgggaggccactcaattactctctctgcaactgtataactattaatacttcttcagaactgtgggaaatggttctactcatcagctttatggaatgtgggttagggagaggggacagaatctcttcaaggtctggatgctaaacgtaccccttccttattccctcccaatgcagaaaaaggtctgggatgttctgacagggccatctctgcct

SEQ ID NO: 58 - DNA, 1001 bp, Homo sapiens
attttcatttgtgtttttttaaatttctagtgaggtcatctaattcacctttaaatattttatcttattcttttgttttcaaatgctctacctagcctttcaagagtattcttcacaaccaaagcagtcctaagcctaagcagaaaggagaaataaagttgatgggggaaaaatgtatatatttttttctaaaataaggcttaggagtaatttaaaacaaaatgctgatttggtattcaattgtcctctttaagggctcttaatatgctgaatataattaaaacaagcaattagcaattcactcaaatttatctatttttcaagttaaataacattctaataagctaacaagcacaaaacagatcagcagttatcataaggtcaggggtcataaatatgtaaatgcctacaaatgccaggcattaaacataaatgagtgaactgaaagcacattcactgtctcaaagggagagccacaactcagttccatcttattactgycaagtgtaaattcaagttcaattttgccctatttttcaaacttcaaaaggcataaattcagattttaatgtaaaatctcctgatttttaaatgctgaagaaaaaaatccaaaaaacaatggtgggcccttctggataagtttgttctctgccctagataaattaatagaataagaacaaaatctaatttagttattactgatgacagtaagtcaagagaaatttgccacatcacaaaaatacacatttgtatttctgaaaataaaactactgatataaatcatgacctttatgtgagggtctgaaaagatcaatatggaatcaacagtccatttctgaagatcattcacagatacactctgtcctccttgagttcaacctttagctggggttagacacacctctagagaagtacataaaactttgcaaggaccaaaatggaatacatggttttaagaaaatcaacttctaaagcttcaactttatcactctttcctataa

SEQ ID NO: 59 - DNA, 501 bp, Homo sapiens
taggggaagctttattctgagatctgcacaaaagtgggttatcctggcagcacagtgtacctcgtagttgttctctgatgtgtaaaacttggtgtaacacatctgagtgtgtgtgttggtgttttattccagtagttaaaatagacataagacaaattcatataaaatgtttgtagactgcaatgtcttctgaagaatgctgtcagaaaatcattattctaggtccccaggtttacatccctctgtgagaygctcttgtaccagttgttgggtaatttgaacagttgcctttgtggtaccattaggagtctcaacttttaaggatcacttacagttctgtgcataggtgattttcaaagcacctgggtgaagttacatggctctagaaaattgagctttagaaaacagcaataacactgaaacaatctttgggagtgagttatcagagaacgtgcattgttgccaaggatgctggcataaattctgggaacctcaaaataa

SEQ ID NO: 60 - DNA, 807 bp, Homo sapiens
aagtgtatagactgcacctccccactgtctcttcctcctactctggccaggtgaagtatttgctctccctttgccctccaccatgatcataagtttcctgaggcctccccaaaagctgatgtcaccatacctgtacggaatcatgggcctatggaaccgtgagccagttagcctcttttctttataaattacccagtctcaggtatttcctcatagcagtgtgagaacaaactagtaaacagtgtaaatgctttgtaaatagttgttagttaaactgtactgttttgggaataatgacaaagaaaagagtctgtatgtattcagtacagaggcagccatccattttttaaaaatatctttaatccacagatgcagaacccatgagtgtagagggctggactgtatacatgaatacatattgacatctttatttctatatctatatatccaaatatattttgaaaatcatgagtttacactgatacctctagtttgaatccrataacacaggttcattctagtttactcccttttcatatttatacctttcttctctgacagtgagaaatcaggcttcctttatcctcagtatattcacttactggctaatttcccctccccattgcctataaactactcatctcccattggtgctgccaccacaatccctcaatctcatatgcatatgggtgacctcctcactccacttggtctctgacatcctgtgtgagctccctgtcactgccctcccccccatatgggtgctcttctcacccctctttggcttaaaaacccaattctgggttg

SEQ ID NO: 61 - DNA, 1001 bp, Homo sapiens
ttatgcaaaccttgagttttatgcaaataagaattcagttccaagcacaaataattaaaagcagggtttttacagtcacgattgccccctggacatttgaaattcaagtgagacatggggcaattcttcattctgcagaaatttccatgcaatgccagaaacctaatatccctagccctatgtacaaaatgctagttgtgccccctttatcactgtgataactaatagggccttctgcatgagtctaaacactctgtagaggcgggtttgctatggtcctgctggtagggcagggactatgctctaatcccttgaataacttctcacttggtggagtgttgtgtacttggggggattcaatgagtagttgtgaattgatggagttacagtagcactgaacagagatgaaaggcagcaaaatcagttagtatagtacagtcttccctaagtatcctctggggattggttccagaacctccgcggataccagatacccaaatyctcggatgttcaagtcccacaattggccctgaagaacccacagatagggggtgccaagtgtatttcaaaaccagtttgatacggaatttgaaaatgtgaactgtggtaagcagaataaagatgtccacgtcttaggctgggtgcagtggctcacacttgtaatcccagcactgtgggaggccgaggcaggtgcatcacttgaggtcagagtttgaggccagcctggccagcatagtgaaaccctgtgtctactaaaaatacaaaaaataaaataaaataaaattagctgggtgtggtggtgcatgcctgtagttccagctcttcaagaggctcaggcaggagaatcgcttgaactcaggaggcagagtttgcagtgagccaagattgcgtcacagtactctagttaggtgactgagcaagattctatctcaaaaaaagaaaggaaaaaaaagatatccacatcctaatatccagaactggtgactattttatgttacatg

SEQ ID NO: 62 - DNA, 1001 bp, Homo sapiens
tctcattgcattttttttaaatttttaattattatgactacataatagttatatatattcctcatatctcaatttaattaccacaatcactgtttttacaaggtcccaggcaagaagaggtgaggcaaatggaggctctgaggaaagtggctccaaagcctacatgatggaagataactctggaagagaaagagatgacgttcctaagcttgtatagcaaaacttgagagaaggtaacgaagatgtgacatctgaactcagagaaatataacttctatagaaaagaaacaaggccttgcagctctataaggaacagtaaataaatcaagtatgcacacaagaagtaaaaaaatatatccaagtagaaaggaagcttttcatgaaatgtccacagagctcatgctctgtagtgactgtaatgcaagattcaaggctctatctagaaaactcctagccagtcttgacggaccaagccctacactgagcatgtacagagtcttyctgttccatgcagtacttgctaacaaaactaatttaaatgccttaccatgactcgatctcctttaaagtacctcattagtccttgatatccctttgctgtatctctggcttgccttgccactgctctgtgagtccccacaactcctcctccacacatactcttcccccaagagcttggcacagaataaagatccattttagatctggatttaaatagttttctttactagctcatttccttatctactaatgagggaaataccacctacgtcagagtgggaattaaatgaaataataaacctaaagaccccagctcaatggttcaaacataaataatgccaaatattcattcctctccccatgcccatatcctctcaccaagccccaatgttctatagcttatgacccaaaacgctaaaagtagaacattctaatattgagcatattaacagaagcttgaagagatatgcaagttataaatctgtttttgttcttcctca

SEQ ID NO: 63 - DNA, 1001 bp, Homo sapiens
ctacattagaaacaggttttggaggagtagtgggaacattgggtgatttctagtggggttagagaaagcagtacctggttctttggccacatctaccaaagcaaagacctagacttgtagaggagagtattgtttgcttgtttgaggattgtatttcccaggtttgttcatttgcatgagtggctgaataatgtaacagagacttcagaagtaaggaaaatggttgtcaccaaaatatcttgttttacctttatttggactaaatggaaaacacatgtttaatagctaaggctattgagtgcttatcatttgccaggaactgtttctgagcctttcacatataacacctcattttatccaccctctacccctaacaaatggtgtggtttgagttggccttggtgaggtatgaaaaggaaacaaagcagtgacctcttcctgcaggctggtcagatgtttgggataacattccttagcattcttggtggaagtggtgatttygttgaaagctgcttcccagttgctctggagtgcaggtgggaggggtggactttggcttttccaaaggatcccaggaatgggaaggaccttaaagatctagaccaggggtatccaatcttttggcttccctgggccacattgtaagaagaagaattatcttgggctacacgtaaaatacgctaacactaatgatagctaatgatcttaaaaaattgccaaaaaaatctcataatgtttaagaaagtgtatgaatttttgttgggctgcatttaaagccatcctggactgcatgtggcccatgggccatgaattggacaagctttatctagactgttctgaactactcatctgcctcccccagcccccacccccaccccacacatccagaattctccacccattggttgtctggcctctgcctgaatagctgagtacctgtcttttccaaaactaccccttgaggggagacttacagcaccctgtagcatagtatatgatat

SEQ ID NO: 64 - DNA, 1402 bp, Homo sapiens
aacttgatccttaacagaatctcatgagagctataagtcttattattatcccctttattgatgagaaaactgaggcccaaggaggttcagtaacttgaccaaggttaaacttccactagtatgtggcacatgtgtgattctaatcaagggaggctggctgcaaagcctctgcttctgttattgctagaatctaataagttatttactaagtatgtaaggatacagtctcatttaattctcacagtaacattgtagatgagtgattagaaaatagctaaaagacagacacttctcaaaagaagacatttatgcagccaaaaaacacatgaaaaaatgctcaccatcactggccatcagagaaatgcaaatcaaaaccacaatgagataccatctcacaccagttagaatggcaatcattaaaaagtcaggaaacaacaggtgctggagaggatgtggagaaataggagcacttttacactgttggtgggactgtaaactagttcaaccactgtggaagtcagtgtggtgattcctcagggatctagaactagaaataccatttgacccagccatcgcattactgggtatatacccaaaggactataaatcatgctgctataaagacaaatgcacacgtatgtttattgcggcactattcacaatagcaaagacttggaaccaacccaaatgtccaacaatgatagactggattaagaaaatgtggcacatatacaccatggaatactacgcagccataaaagtgagttcatgtcctttgtagggacatggatgaaattggaaatcatcattctcagtaaactatcacaaggacaaaaaaccaaacaccgcatgttctcactcataggtgggaattgaacaatgagaacagatggacacaggaaggggaacatcacactctggggactgttgtggggtggggggagggggggagggatagcattaggagatatacctaatgtaaatgacgagttaatgggtgcagcacaccaacatggcacatgtatacatatgtaactaacctgcacattgtgcacatgtaccctaaaacttaaagtataataataataaaataaaataataaaaaagaaaatagctaaaagatgtgaagttggctagtctaaagattcaaaagtaatgaatgggagaaagagaaattagactcaccatgtcctacttattthgactttttactgagctgaactgcttcccctacctgcatatccaggaaaatgggtaaggtctggtagatgctttcagccttatcgtgctatgatgtttgggccgcagtgttatttgctcattagtcctttcttgtttcttaaaatttaacatttagccactgttttgtaaattctgacttaggtgccaagttatggcgcta

SEQ ID NO: 65 - DNA, 2022 bp, Homo sapiens
gctgggttgaagtgaggctggaggtggaggcaggggccagtgtagtggtgcagagccactgaagagcttaagcagagaagggacataataatgtttgggttcttaaaagatcacgttcagatcctatatgagcaggtgatttgagggggcaggagtggatctgttagaaggctattgcaagtggtccaggagcaagagggtggtggcttggaatagtatcatagtagtagagatggagagaagtgaatggatgtaagaggtatttagggaggtagactgcattgaacttggagaatgactaagataggaagagaaggggacaatgcttggatttctggctttggaaaccatatggatgaccatccttgttcctgagccagacctattgtgggaagggcagattttgaaagaaagatcatggtttagttgttgacatgctgaatttaagggttggagtacatacaagtgaagttagatcaatagatctgatgatcggaggggagatctgggctgtgcataaagttgggagtcatctgggatggactgaagtcatgagagagaatgaatggtagcagggaatggggattggacatgtgactaggaataaccacagaggccagttgaaaatgtatggaaacgagaacatcaagcatgaagggccatgcccagtgctaaggagaaatctggttaggaagtgcatggatttagcagcygtgaggttggatttagcaatcaagattggcacctcaagcaggagaaatttaagtggagttgtggggacagaagccaattttgaacactagatgagtgaattggaggcaggaatatgaagacactgagtatgggtaccttttttgagaagttgggctcaaagggtagagacagttagaggggacctgcaagaggtgtgtaggatccaggcatatagctctaggtctaaacatctctatgtttggatatttagagatggaagagaaaggatatttagttgcttaaggttcctgcaaagacaggtgggatgtaacccagagcccacacgaagggacgggcatttatctccagcacttcagaaggagaggaagaggagggggtgggtacagctgcagatgcaggcaggtgtggaggtttggagtggaatggtaagtgataccattctgataatttctgttttctctgtgaagtaggagggaaagtcatcttcccagatgaagggaacggaatcaggttgctgggtaagatcagttctccagctgtgcttggcagctaccactgcaagcatggaataggcggctaggtaagttcagccaagattgaagttttactctgtgggagtaataaaaggacaaggaacacgaaggctaaggacattaacacatggaggaatgatttcagtggaggttcagttggatgaagataggttagtgctgatggagaatgacctggcagtgtcagggggcaataaacagggtagtggtagtacctgaataagggaactagctatgagtgcttctccaactgtaatgctaatgtgaatcacctggggattttagtaaaaacgcagattctgattcagcaggtctgggctgaggcctcagattctgcatttctaacaagttcctgtcacgccagcctctctggcccgtggatcacactgtgagggccaggtgtggtggtgcatgactataatccaaacactttgtgaggcccaggtgggaggatcacttgagctgaggagtttgagaccagcctgggcaacatagacgtcatctctacaaaaagtttaaaaattacctgggtgtggtggcttgtgcctgtagtagctacttgaaaagctgaggcaggaggatcacctgagcctgggaggtcaaggctgcagtgagccgagattgcaccactgcactccagcccgggtgacagtaaaagcctgtctcttaaaataaaaaaaaaaaaaaaaaaaaaagatttcgggcagagagtgggatgcctgaattagaaatcgtttgacatggtataatctcaagc

SEQ ID NO: 66 - DNA, 1001 bp, Homo sapiens
gtggcttctctttggaaacagttcactggttttctcaagggaccaatgggctatgaagaccagggactgtccaagctggccactcgggaaatgaaaaaaaatatgtgacggaacatgggaaagaaccacaagtggaagaagtttggacacacaggattctacctttttgctcattctacccaaaccatctgcacattgataaattattaggatgagctgtgcatcctactttacaatatacatgtccatgggggagaggtcaatagaaacagttaccacgacagttggtggagtcagaacatctggcggctacacagacacaccagctgcgtgacttggcaaactcagtatctctgtgcctcatattcctcatccgtaaaatggagcagtgacgaggatattgagagttcatcaaaaagcacttactatagtgccaaggacacagctaagtgctcaaagattagccatgatgatgatctgactatctatttttatccctgyttgactaatttttgtgggagaacaaggggaagaggtgaagaattgatgtaactttcatatattacctatcctacttttgtatatgtttgaaaattcttataatggtaagttaaattaaaaaaaaaaaacctaatgtgtgtgtgtgtgtggtgtttttttgtgtgtttttttgtttgtttggttggtttttttgagatagggtgacggggtcttgtcactcaggctggagtgcagtggtgtggtcacagtgtgatcacagcctaaattcctaggctcaagttatcctcccacctcagcctcccaagtagcagggactacaggtgtgcactaccacacctggccttattttgtgcaggagagaataaggtgaagaccaatccatttctaatatttttaagtttcttctatcattagattttctaaactaatagcaaacttttttgtaaagggcccaagagtaaatattttacactttgcagaccatatggccctgttgcaag

SEQ ID NO: 67 - DNA, 1001 bp, Homo sapiens
tcgtcttgaaattcttaatcatatttgaacaatgtccctacagattatgtagccagtcttgctactaccgagctgcacttgacctccccgcactcatcctggccatacttcatccctgtccctctcctttctactgcctggtgctttgtcccatttccttgcccccaaggccttaggagggtgtaaaaaaaaaaaaagataaattcctcagggaaaagatgtgatttggctcacagcatatggaatattcaaagatagacatcatctgttgcccacatttttatgagactgacatgctgcctgtagcattgagaaggcactggttgcctacacttttagaagtcatttattaatggcttcctagggcatgccaactctaaaatcaagccacaaaaatgataccaggtaaaaattgatcctgtgaataactgtgacggtggcatttgggtgaaaggtcttgaaatgggctgtgtcttttccctcaactttcctcacccgctyttatcacactctcccagccagtgtcagattacttctcttctcatctgtctcataaatagttctggcttgagttatcccctaccgtgatgacatatgattattcaaagaaagattttatagaaaatgcattgtttctatttggagttgggagactagggaaaggtataaagcacgccacaggggcacagccttgattgactttctgtgctcagcttagccgttcaagcccggggttgtgtctgggtaaagctgtttgactttgggtaagtcctttaacaacctgaggtcccagtgttcttaactttctacagttttgttctaatccagcattcttgaactagcacataagcataacttgctaaataagcaccacttgctaaatacaggcttagtgacaaggaagttatttggaaaatgaaaagagggcaattctcccatcaggacttgagaagccttggagttttctttctttattgaaaagactcatgaggcctgtccaa

SEQ ID NO: 68 - DNA, 1958 bp, Homo sapiens
accccaaggtggaagctttacatgactgagaaagcccatccactcattgtcatagaatcaactattaattcaacaaatacttatggagcctttgccatgcctatgagccttgtgctagaagccagggataagtaaaataaattctgcacctgcctcctgcaacttagtccaatttccaggtctcccttagatttttctctgttttaatttttattttgaaaatggagacagggtctcactatgttgcccaggctggtcatgaactcctgggctcaagtgatcctcccgcctaggcctcttaaagtgctgagattacaggcatgagccatcacacctagcctctctcttaaaacaactttattaaagatgtaattcaggctgggtgtggtggctcacatctgtaatcccagcacttgaaaattacttgaagttgggaggtggaggttgcaatgagctcagatcatgccactgcactccagcttgggtaacagagcaagagtccctctcaaaaaaaaaaaaaaaaaaaaaagtaattcacataccatacatttcacctgtttaaagtgtacaattcagtggctattagtatattcacagagttgtgcatctattaccagaatcaattttgagcctttttttttttttaaccccaaaaagaaacctcttccctttaacacttatccccagtccacctatccttctcagcccttggcaacagctagtctactttctgtctctatggaccggcctagtctagatattttatataaatggaattatataatatgtggccttcatgtctggcttatgtcatttagcataatattttcaaagttcttccatgttgtagcatgggttagaacttcattcttcttttattatggttgaatgatattccactgtatgaatataccacatcttttttttttttttttttttggagacagaatcttgctctgttgcccaggctagaatgcaatggcacgatctcggctcactgcaagctccgtctcctgggttcaagggattctcctgtctcagcttctcgagtagttgggattacaggtgcacgccaccgcacccggctaatttttgtatttttagtagaggtggggcttcacctccttggccaggctggtcttaaactcctgacctcatgatccacccgcctctgcctcccaaagtgctgggattacaggagtgagccaccccgccgggccacatctttttttaatctattccttcactaatagattgtgggttgtttccaccttctcactatgtgagtaatgctcttatgagcgtgcatacaagtttttgtgtgggcatatgtgctcaagtctctgatcccctagatgtcttgcctatcctacagatccaggcctaccacaaaaaagtgtagaaggatcatataccatgagaacataaaggagggacatgtagacttaattagggagtcagggaaggctgcccctgaggccaccatatccaagctgcggcttgagagatvggttgaatagaaaagtttttcaaactgcagctgatcacccattagtaggttgtgaattcagtttagtgaatcatggccagcattttttaggaggtgaactaaaatagaatagtagatgttagaggacattccatgtggtaagggtaagtattgttgcatgaaatttattttcagtagctatatgagcgcatctagcaaattgtgacgtaagaagtattctatattccgggttgcaatcagaaaaatatgaaagccactgctctagggattttttaaaaggagattatttattaatctggagctttaaatatggttccactagaagattggagagatacaggagagagaagaacctagaaagctgaagatcctttgaaagcttaaagttctgtgatttctacacttttaaaatgattcatttattcaacaaatattaaaatatttacca

SEQ ID NO: 69 - DNA, 1001 bp, Homo sapiens
tcatatactgcaacacaacacacacacacctcacttacatagacttttgatttaagctgtgttcagatttctcttagcacattcaagttttccttccttcttcccagaagcacctaaaggctgtaatgagaaacatattttttactcctttgttccctctctttgtgtaaaggcatcccaagaaaatcagtgaaggattttgtgctctatgtccctaaggctccatgtcccagttatttttctctctcaactggggcttgatttccactttattcaagtctacttcttatttccttcggtgatccgaagtactggcagatttttctaagacttcagacatgtggggagtaactttcataactccaaagaatacactaccagaaatgtaaccatctcagctgttctccgtctactctgatgttgcctgtaagaaataacaagatgccactctgttctttaaaagagatatataacatttttcataagatgtccttcattacwtggtgcagaattcgaactgatcgtttgtggattaatcataataatgacttattttgtttatgttaactaaaaggagtttatcatttttatatgatattgactgaatggtcataggaaattgagatctttttcctaaaaaggtgataacatttactggagtgttgttttagtagataacttgatccttaacagaatctcatgagagctataagtcttattattatcccctttattgatgagaaaactgaggcccaaggaggttcagtaacttgaccaaggttaaacttccactagtatgtggcacatgtgtgattctaatcaagggaggctggctgcaaagcctctgcttctgttattgctagaatctaataagttatttactaagtatgtaaggatacagtctcatttaattctcacagtaacattgtagatgagtgattagaaaatagctaaaagacagacacttctcaaaagaagacatttatgcagccaaaaaacac

SEQ ID NO: 70 - DNA, 1001 bp, Homo sapiens
cattgaattgccttattaatctcttgggtcatgcaattcagtgatataactagggttagcctgagtgtttcaaagcaagattaatggaagctcattcgccagctgtcgggttaggagattattcacaaatgttgccctgtcatttgaatctggtagggtttgctgatgaataaatgaaccccattatactgacagccacctcactaatcgatcctaactaaaccaccttatcctcttcaccttccaattgtgtagccagcaacttgccagatctcagggacgttgttgggacatgtggaaggtctgagacagagggccggaaggacagacaatgccaccaactctattaatcagtccgcatttctcagacctggctctcagcctactgaatttgacaaccaaggatttgcgtgtagttttttttttttttcattttcaattaatttccctttttatgccttcctaatttctcttcttttctgactaagctatatatttacrctgtgaaattgactgtcattaatctttttctgccttgatttcctcaactaaaaaatggttaaactaataccagccctttcattcatggtgatcttgggaggaaaaaaaaaagagataactgatgtcagagagtgctttgaacttaaagcaggaagattgttcaattataataagactcttctatctttatttttatgtgacatttagaatgttagcgttgaatacgcgtcaaggaagaaaatcccattttgaatgacagtgttagaatgacggcctgtaagatattggaattgcatgcaaaaaccaagaaaatgtgtttaaaaactgctaagaccaagccagctactgtttcttttcaaagaatatatgtagggaataggagaattaggtaactctagggcataataaaaaagaagaacatgtgctttctgattttgccaatctattttgtacttactttataattcaattttaagagtaaagtgtaatgtctgattcat

SEQ ID NO: 71 - DNA, 1001 bp, Homo sapiens
ctttgggatggttggctgtacttttaaccactactctgtcttgtctctgcatgtgtgggcatgaactttgttaggttctgaggaggaggatggggggttgggaggagctgcatatgttctctgccccagaagaatcatggcccaggggaagaggtagcaaaaggaacaactattccagtatgacttgatcagtttcttgatggacatgtgtgcaaggcactatagaaggacagaagagatttttactttaattaattgaaaattagtaatttatatttggtatatacgtaatctaataattcattaagtggagcaacttttcaaactattctaacaaaatctaacattataaaactataacatggagactgcattgctaaatacctttcatctacaaaggaaagttatagggatttattatgttttctagatttctagctctctagtgctcaaaaaaattgaaaattgaaaaattgaagaaaaactgaaattgaagtgacmctcatctttgttgaagaaaaaggaatgtgacaaaatttatttctatgtgcagtcaaaaagtgtggtttgtgaaatgtgttgttgttgttgatcttacaggagaatcatgaaaaaagtctccatggagccatctgagcgcctggctagtctccaggcgctgtgggacagccagaccgtggctgagcagggcccctgtggtgagcatgcattttaaaactgaaatgtgaatagctggatggatatccccctgccaggaagttaagtctattcctagtgtgctactgtaaaggtgcaattagtttcaaggtgtaattagcagcgcacagactttagattggtggacaaaagtcctatatttaagctgtattgcatcctgctatgtacttactatagaacagggaggagaatctttgctgttttcccccctaaaaaggaaaaggataatcagcattgtcaacatcggccatatttaagctttaaaattttaatttaaacatcat

SEQ ID NO: 72 - DNA, 1001 bp, Homo sapiens
gatttggtttctgtctctactgagttctggttgttcttttgattacaagaactactcaatttcctttaagtaaatttatttattcttaaaattctgttgcttgaaactaagaataagccctaataggcacagaggaataatttaactcttcctgatctgtttcctcatctgtaaaataaaggaaaagggcacacatatcccctgacccctcttaactctctcatctttagctagaattgggttctagtgattctcaaatggatgtgttctaaaagaggctggctggccctgtgttggggaagcagaagttttagtaattaattaggttaatatgaactttatagttatattttttctgtattccctgaataactgtgactctattacttgtgaatttatttaaaacataaatatgacagtgatgactagatgaggtctcttagcacacatgccctatgcagacctgtgagtcccctgctgtctgctcacccaatagttgarggcctgggtaggagttctgccacatgtgagttcttaacacaaaatcctcatggaccctgtgggcctggagctggatacttcactcatcttcacccttggcctcatgctaagaattaccatcctgccaccacttaaagatgcccattcatgttagtgtgtcactgctaaagtactgtcattaaagaagacctatcattactctgactttaaaatacattgttctaacagaatcactatgggagattccagacttctgtatcagcgggtgctttgaaaagaggatctgatatgtactggcccctgtgttcacctgtgggcgaacattagacatgtttgtttcttttatgctttgataacaccttacaacttgcaatagtgtgactttggaaagaatgaagtgattgtgtctggcatgctgtatgtaaacattccatttctacataatgtgaaaaggaatgaattaggtgaaaataaatggatttgcacaggtgttagagtac

SEQ ID NO: 73 - DNA, 1001 bp, Homo sapiens
taagttttgtttaacttatttaactaaaaaatgatgctaatgaatgtggaggggtgatttggatagaacctgttctgtgtggggccttcatgtaatccctagagaacgtgtaaatcaaattatgcctggaggaaattttatttccaatttcagttgctttactgatatgttaagggaattaaaaaatatttagctcggcctttcagagagctgttattactggttgaactatgactgttattttaattctcattagataactagtatcttttgagctgttgttagctaggctgtgtgctaaaaagttttatatacatcctcttatttaatcttcacgacacttataggaggtagatactacattatgtgtttttacagccaagggtgaggtgtaggggatctgataattcgctccaaatcacacagctagtaaatggtggagctggtccaggcgtgtctgtcttgagaagcgctgtaccattcaccttacaattatatctrtaggtattgtctgactcatagaatccatgcagtacatctgtgcagcttccatttctgtccttagcctcaattcctttctgtctttagttctctatctttaccttaaaatctccatgtaaatcatgctaacctagcacgatccatggtgcacccacttggcattttcagggaaaagggataaggcctataaagaaagtccacacccagcgcctggttctgcctgtgcccattctgactgctttatcttcagtgctttagatgaatgtgcatcttcctggatgcttttccttcctgcatgatttggaagaattagaatcagtcttccttccatgagtttcccagggaatcagagggactttttaagcataatgatggaatttttattgtcaccttttgttgtaaaatgctctatagatgagaaatagattatatccatccccccaccagctgtgcttcatggtaatggccaaaaaaatgttcagaattaagactgggaattt

SEQ ID NO: 74 - DNA, 1001 bp, Homo sapiens
tgtagtctggactttcttagggaagtcctttacctgaagaatgagtaggcatgagccaggtgaaggtaaagcaagagggggaagggatagctcctaaagcagaggtggggcaggagccctcctcttgggagagcaacagaaggccagtgtggctgggttgaagtgaggctggaggtggaggcaggggccagtgtagtggtgcagagccactgaagagcttaagcagagaagggacataataatgtttgggttcttaaaagatcacgttcagatcctatatgagcaggtgatttgagggggcaggagtggatctgttagaaggctattgcaagtggtccaggagcaagagggtggtggcttggaatagtatcatagtagtagagatggagagaagtgaatggatgtaagaggtatttagggaggtagactgcattgaacttggagaatgactaagataggaagagaaggggacaatgcttggatttctggctttggaaaccrtatggatgaccatccttgttcctgagccagacctattgtgggaagggcagattttgaaagaaagatcatggtttagttgttgacatgctgaatttaagggttggagtacatacaagtgaagttagatcaatagatctgatgatcggaggggagatctgggctgtgcataaagttgggagtcatctgggatggactgaagtcatgagagagaatgaatggtagcagggaatggggattggacatgtgactaggaataaccacagaggccagttgaaaatgtatggaaacgagaacatcaagcatgaagggccatgcccagtgctaaggagaaatctggttaggaagtgcatggatttagcagccgtgaggttggatttagcaatcaagattggcacctcaagcaggagaaatttaagtggagttgtggggacagaagccaattttgaacactagatgagtgaattggaggcaggaatatgaagacactgagtatgggtacc

SEQ ID NO: 75 - DNA, 1001 bp, Homo sapiens
gaactcctaggctcaagtgatcctcccacctacagcctcccaaagtgctgggattataagcataagctaccacacctggctgagaattctcatttttaactttctacctggtggccctatgtatggcagatgcacctgacagcaataatttaacttaagcatactctgtatggcagatgcacctgacagcataatttcacttatgatatgagggttgccatgtggaggttgtgtggaaggaggtggggttgggggaaggagtgttaaggaaaaatgctatataaacagcacgcttttttaaagtgatggttgttcttctgaccagcccactgccactggactgccctgtaagttcccaaataaattctatgtttcacctgctggctccatgtctcttcttcagtcttgtgaacctggtgccatccctattgaagttaataagggtcatataatccataaggcaggattctcagtcatttgtgggtaatgctctcctttgaraatctatcaccccctaacatgcatgtaacacaacattttgcttatagtttcaggagatctataggcccctgaagcccatttctggcccttctaagagaacgtgaactccagattcaacatttctgttccaaatgttcctgagcaacaaaattttctaggtctacctcatcccttggaacctgatccaactgtgttcccaaaactaccagactctctcttccatgccacattcatctgtttcttgtttttctatcatgaaattttgtattttgctactgcttttttaccaaaattcctttagataatctcacggctttgccgaaatccaattcacaatgctctgtctaacccacgaggatggactataactacttcctcccaatcctagacaatgtttctgatgtgttcctttaagctccgggagctgccagtgaatgtgtacctaaggccctagggaaagaatccctgctttaaagagcttaagaaagaccatgagggaa

SEQ ID NO: 76 - DNA, 1001 bp, Homo sapiens
cctccaggtgacaacacgggtggtgagagccgccgcatgaatccacactgcggctgaaggtcaagaattggcggtagcccatcggtagcccagagacccaaactgtgtccgatgtgagtgaaggtcaccccagatcagtgcgtcagttccgttttggcggccaaatttctgacgatcccatgtaagaaatgccacacctgtcaataggagcgactcacgcgctgggtctctttctcggatcgggtcgccaccccagtgccgggactatgctaaagactagagtctcagacttggaatttcgaggaaggtgttccaaaacgctgcgctccctccggcgagggacaagagcaggagcctggcttgcctgggtccaaggacagtagctgggaggggtgtggcagccgcttagcttgaaatctttcagataccccaccgaaatatcataaagagcacaaagaacttttacgtaggaacaaaatagtgaatctacaacaccttaarcgcctgataacttcacaatgcatgcctaggaaaccaaatagcagtcaaatggagttagtccccagagaagaggaaacgcagaggaatctgatagggagcaggcttcagaaatattgagctgcctctctcttctagaaggagagaaccaaccctgagctgaaatttctgcaaatagaactgagattataccagacaatgtcatggctgaaggagggtaggaaagtttataaagtgcttgtgttgctgggcacagtggctcacacctgtaaccccagcactttgggaggctgaggcggatggatcacctgaggtcaggagttcgagaccactctggctaacatagtgaaaccccgtttctactaaaaacacaaaaattagccggccgtggtggtacgcgcctgtagtcccaggtattgggagcccgaggcaggggaattgcttgaacccaggaggtggagattgcagtaaactgagatcatgccactgcactccagcttggg

SEQ ID NO: 77 - DNA, 1001 bp, Homo sapiens
aagcctggccaacatagtgaaaccccgtccctactaaaagtacaaaaaattagccgggctttgtggcgggtgcctgtaatcccagctactcaggaggctgaggcaggagaatgtcttgaacccgggaggtggaggttgcagtgagatgagattgtgccattgcactccagcctgggcgacagagcaagactctgtctcaaaaacaaataaataaataacaaaaaataaattcatattgtcttaaaccaccaaatttgtggtaagcaataggaagctaataaaaagccactaagatagtaccatgaatagggctaaacaggcagaaagaagtctacagggcttttttctggaacaatttttagaggccagaggagttcatggagctcacttttgttgtcattgagagccctggaggatatgttttgaactgtagagagagtcaacagaaggaatttagagtcccaccaacagttgggatttctgtatttggagtccagagtrttaaccgttataccatggtatctttgtataacaaaggttctagggaagacttgtatactattgcatctggtcagttaacctttaaaatgggcatagattcaatgtaaggaacactaatagcttctcatagggagaaaaatgcaggttctcagatgactcaatttgtggtttgcacatattcatgcccgagtccagagatagcatagagagcattcggagtgagctctgaagaagaaaaaagtcataggtggggcctctgacacatgaacctttactcatcccagcagatgattaacttacagtggtctaactgacttcaggctccagcaaagcaaagcaaagctttcaaaagaagagcttctaggatacatgagggtgatgggcagtggacaactttcagtagccagagaaaagagcaagaagcgggatgttgctccagaaaagaagtgcaaatatgtgagactatctatacatgcccaagtgtgcttctccatttgggt

SEQ ID NO: 78 - DNA, 1001 bp, Homo sapiens
atacaagggaatactgcacagtttgtaaaaggaaaaagaagcaattctctctatactaatatggaaagatctccaagatacactttacacagaaaaagcaagatgcagagggacgtgtatagaatgctatttttagtttaaacaagaggaaaaataagaatatattttaatttacttttttttagttctcaattgggttagtttacatttttaaacttcaacaagcaattttgtaacacttactgtacatcaggcactttataagtattaattcaattcttctaacctcaggaaataggtattatcattaccctcattttacattagtagattaggccactacaaacagagaggttatgtaagtagtccaacatcacactgctagtcacatgggggagccagcattgaaacccataccctctgactccacaggttatgttcctaagcatcatattaagtggactaagaagttaatacatggagggagggaggacagggtgratgagagagttgcgtgactttatgtgtatgtagttttgaacgatgtaaatgtgttacctattgaaaaaatatttagaaaaaatgtgtatgactttgctcaagttactttccatgtgagaggcagacatctcaagataagtaatagtagtagcttgtagtgagggtttaccaaagtcttatctatagtcctctgagactttagggagagaatccttatttaacctcatgagatagattccccacccccgacctgagctgagcagctaaagcttggggtgctgcaggctggggaggctgagcgcaccagcgcccatgacctacagctctccccttcgcagaccccttcttcaggagcgcccagccctggatcgcagccctggcagggaccctgcctatcttgctgctgcttctcgccggagccagttacttcttgtggagacaacagaaggaaataactgctctgtccagtgagatagaaagtgagcaagagatgaaagaaa

SEQ ID NO: 79 - DNA, 1001 bp, Homo sapiens
atgaagagtgaaggaagaaatgtaaatgagacacgtgccaggcacacggggacccagtgaccagactccaagaaagcgcaggacagggctgggcgcggtggctcacgcctgtaatcccagcactttgggaggccgaggcgggcggatcacgaggtcaggagatcgagaccatcccggctaaaacggtgaaaccccgtctctactaaaaatacaaaaaattagccgggcgtagtggcgggcgcctgtagtcccagctacttgggaggctgaggcaggagaatggcgtgaacccgggaggcggagcttgcagtgagccgagattgcgccactgcactccagcctgggcgacagagcgagactccgtctcaaaaaaaaaaaaaaaaaagaaaaagaaaaaaagaaaaaaaaaaagaaagcgcaggacagaaagagcgaggtgctaagacttagagtggacccagaggctctggccctcctgtctcccaccacgcactccatttytgtcacatttcaaacctatcgcttttacgatatatgttcaaaaattgtttaatgaactgtaaatggcttggtaagggccgcatcgtaaatggcttggtatgggccacatcgagaacagctgtcaaatataagcctaaggctaaccacggatctattttaacactgagcagttgtggctgagtgtctggagcttggcagaaagcaacgtcacaagtctggctttttcccacgtagactgaaccctcgccctcaaagctacaaacacaacaatttaaccaactgagtgatcaactaggagaagaatcaatatgatctctttcaaaagcttaaaatatgtcaaaatagtattatctcagaaagtttttttttcccaaaataatacaagacattatcgaattcttatttaacccttttctaaaatcacccacccacctcattgaatttcctttaaaaaatcttcatcctggccgggcgcgatggctcatgcctgtaatctcagc

SEQ ID NO: 80 - DNA, 601 bp, Homo sapiens
actagagataatatgcatagcttaactaaaaattccaactgctaggaaagaaagtgcacaaatgctaagggaagaatgcagagaaaaagtgctcccacacatccaggctgacatgtcactgatgtctgatgtcacctatacctctcttccttgtataagaaggggcagctccaggcacagtgcatcaaacactgctgtacaatggctctggctcccttgtggaccagaaagaagcagatgtttctggatgggagttgggaaatgatcagccaccttctccctgggccctggaatcttcctyttccacaagtgacagaagacctcagaatcttctctttcactgcctacccctgaccagctctgccctggacagtccccttccaaagccaaaggcagccccaatccacagttgtcaggtacactcacctggggagtctgtgcagcatgcctctgggtggctgttctggcagagcagcaccaaccagggcctgtttatatttccccaagtcccagtgctcatgggcaactcccactggtgtcacaatgtcaatgtcataatttctgactttgccaaaggaaaaggggtccttctgtacaatgt

SEQ ID NO: 81 - DNA, 1001 bp, Homo sapiens
agcattgtgtccctgtgagcccctctacgttattttacctctgactggaacacacctccatcatttttccctcacttcctgcaagttgctgtctaaaggtgactgttccacatttttgttatgatagagggtccttattggtaccatgtgagaaattaccttgatgccctggtaggctccaagtatagtcccatgcaagctctcccagaggacacagcacaaataggtttgcagactatgcagtgaaatgctcaaatcacagcttcattaaaaaacatagcaagcagcaaggggaaaaagaagagcaagttaatggtttagtgtgtaagtgaattggaagaaccacactatctgactcaagtgtgagcagtttccgtatatctgatctcttttacatcgctcaatcagcctgtaggatagacacagagatatatatgcctggacccaaccaattagttggttgaatagccatggattttatttttgttcctaaagtagagracttatggtgtctccaatttgtggctgactcaaggcctcatgaataatgagtcagtgcttcgatgtctcatatatctgtgaattctgaatgtgtggctccttttgtatattttgtgcatcaggaacattaggtatcttttgacccttccatcccttatatctatatttaacaacatatgctctttttactaactacttatgtctacttaaaacatcttaagcatttttgcctacattttactaactaaaagcatatttatcttttataatagaattgctcatttacaaaagtaaatatgtgttacaatccatatcatttattggtgtatccctgacatatagtaggcactcaatacatatatggaatgagagaattgtgctttctctctcccttttcgccttcccctcctcctgctttttctcctactctcacactgtctctctctctcaaacacacacacacacacacacacacacacacacacacacacattggacag

SEQ ID NO: 82 - DNA, 1001 bp, Homo sapiens
tctcagcctccaggaccatgagccaaataaacttctattctttataaattatgtagtctgtggtattctgttatagcaaaaaaaaaaagactaaaacagaaaattggtaaaggctattttaatgaggtcctagatggaaatgaggagcaaggtattggaaactagagtaaaggccatccttgtatacagttgcaaagaacttgggggattgtgtctgcgttctagggccttataaagtgcagaacttaacagtgacgaactgggatatctggtggaagaaatatctatgcagcaaagcattcagactgctgtgtggctgtttttaactgcatacaatgagatgtgagaggaaagaaataaagatggaatttataattaaaagagaatcagggtagaaatatttggaaaatgtatagcctggccatataaataatagaaaagtatgttcaggagagaaaactaagtgtgtggctaagtgactttttactaaggagataaacrtggacaaaaggaaggtgctattcattaagacaatgggagacagaccataaagcatttcaaagatcttcaagtctgcccctacaatcacaggcccagaactctaaaagggtaaaatgatttaggggaaaggcccaaggcaccctccatggactcagctcagagctgcctcaggtctgctcctggggttccagagcagcactctgtggccaccctagccatggctcattaggcccaggtatggcttgatccagaaaatgcaagctgtagagcttggcagtgtccatgtggtgctgatgcagcaggcatgcacaatgcaatagctgtgaagacctggcttcctccacctagatttcaaaggatgttgctgacagtctgggggcccaggcagagaattgtgcagggacacagccactgcagagagcccctacgacaatgacaagtggaaatgcggggtcagagctgacacagagtctccactagggctgcctagtagagcatgg

SEQ ID NO: 83 - DNA, 1001 bp, Homo sapiens
gcgggagagctgggccactggttaaacatttggaacgtttgttatgaaaagataaagcatttttcatctagagcttaggaatgacttttaggaaaaaccttacaggattcaggtgacatgtttaagtcagaatgtgaactagttatttaatgtagggcttacaagaatgttcgctgtgtttattcatctcgtgttatatgaactagaaccaataaaaaaaaatccagagccaggctcagtggctcacgcctgtaatcccagcacttttggaagctgaggcgggaagatcgctggagctcatgaattcgagatctgcctgggcatcatagcggatacaaaaattagccgaccggggtggtgcacgcctttagtcctagcacttcacagaggctgaagtgggacgatcccttgagccggggaggctgaggctgtagtgagccgagaccacgccactgcacgccagcctgggtgacagcgagaacctgacttgaggaaaaaaarataatccagtacagaatgacacggtcatatcaaattggcatgtaatagagaccccatcttgaaacttgctactatattgtcttgtgcgttgatagcatattatattaatgccgaacacattagtgacgccgaagtagctggtgcctaaatggcttaaacgcggaaaaaccacatacagatgatggaacaaaaactggccaatcagattatagagcgggctttttaaaatataagaagcttctttgtagctaggcgtctgacaaaaagcttgacaccaacttaacaaaaaccaacggctggaattcatactctaataacagactgcatgggtaaactacgtggggagtccaaccaacaccctggactcttgcttgccttgcgttactcgattagggttgagggagaactgcccgagatttttcgaatgcaaggaatcttgctgcctgatctaacatgttgtgcacagccattttttagaggtctctgggtggctctgaaaa

SEQ ID NO: 84 - DNA, 1001 bp, Homo sapiens
aagaaggcagtgacaaaggcccagaagaaggacggcaagaagcgcaagcgcagccgcaaggagagctactccgtgtacgtgtacaaggtgctgaagcaggtccaccccgacaccggtatctcgtccaaggccatgggcatcatgaactccttcgtcaatgacatcttcgagcgcatcgccggcgaggcttcccgcctggcgcattacaacaagcgctcgaccatcacctccagggagatccagacggccgtgcgcctgctgctgccaggggagctggccaagcacgcggtgtcggagggcaccaaggccgtcaccaagtacaccagttccaagtgagcccgcccaccgcggaacgttcggtcagtctcggcccacaccccaaaggctcttttcagagccactcagtcttcccaaagagaactggcactcactgttcttacagcaggtatttcttacttgctacaaagacgatttccaagattcctttagccttgttagaarctaattttggctcaagcctctaatcccggttcgggaaaccgaagcgggtggctcacctgaggttagaagttcgagacgagcctagccaacatggtgaaacccgtctctactaaaagtacaaaaaaatagctgggcgtggtggcggacgcctgtaatcccagctacccgggaagctgaggcaggagaatcgcttgaacccggcagatggaggttgcagtgagccgagatcgggccattgcaccccagcctgggcagtaagagcgaaactctgtctcaaaaaagaaagaaaaagaaaagaaattaattagcactgcagtgtactgcatgttgcagcaacgcttgagacaattttatatctgaagaaggatgaggtttatcatcagacaaacctagtaaagggaaaattcagttcctgttgaccccaaagaaaatataatacttaagtgtcactggtaaaatatccacagtgcttccggcgctctgtccctaaacttcatgtg

SEQ ID NO: 85 - DNA, 2052 bp, Homo sapiens
tgaattcagtatatgttgtaaagagggtaaggtagcataggttaattgaatacgttaatctaagggtaaatacaaattaaaaatgagaggcttaattatctgttgaaaacaaaagacttccctttcctttcccatcactttcaaaatgtctttctctgtccttttaaaatgtatgtaaatccttttaatggctaaataggccttataactcagaatattttctcaatgcctggagagccatccctttgaaatgttaatcattaaaaaagatagtggtctgtctcccagtttccagcgagaaaatgggctgaactttagctgtcacctgacttcgaattgcaaaacctatccaatgtagccatacataataagcaagatttctttctgcttttgcaacctcttcataaggtttcctgtgataagcaactctccctggtttaatgcttattcaataataaaattatttcctttgtcttctttgggagaagattttaaaattgtatttccccaacattagttaacaagtatatttctctacttgagcttctcactaatcagaagcctttttctgtatctgatttcatgagttttcgcatagcaattagtgacaaggatagcaatgaatggtaaaaggtggcagagcatgccatcccaaaatatgccattttggaataagaattattctgagatacaggcaattttaaaaagagtaggtacaagaaaggcactttgaccgttcccttttacccccttaaaagcaggaattaaaattcccmtgtggaagatgtcctccctgtaccaaaaggaaaagaacattttcatcaaggacaggaagttgaaaccaagagaattctgtccaagcagatcttaaaataattcttgttttcctttagccttcctacatagttacatttccacaatttactccattcaacctactataaaagcatttaggttttgctacttctttggggtctattattagagctcccatgtcccatgccacataaaatttatattaaatttatatggttttctcctcttaatcttatgtcagtttaattatcaggccagccataaaaactcttaagaggacagaggtaaaattttgcctcccctacaaggatatttgagtttgtcagactctttagtttctgaaattgacggtaaatttagttctgaaatagtaaacatacacgcagtataacattttaaaaaaatgttatgctaatcagtctgttttctaacaggataactgactatcaagataaacttagttcaaatagagtaactctgagttctcacattctttcacattacaaaacaaatctggcagcaaactttgtcagaggcgtttaaaccagagaaactccatcttgaataggggctgggtaaaataaggctgaggcctactgggctgcattcccagaggcttaaggcatttgtagtcacagaataggtcagcacaaagtacaggtcacaaagaccttgctaataaaagcatgcggtaaagaagccagccaaaacctaccaaaatcaagatggtgaggaaattgacctctggttatcctcactgctcattatacactacttataatgcattagcatgctaaaagacactcctaccagtgccatgaccatttacagatgccatggcaacgtcggaaagttaccctatagggtctaaaagggggaggaactctcagttggggaattgcccaccccgttcccagaaaactcatgaagaatccaccccttgtttagcatgtagtcaagaaataactataaatatccttagaatagaacaaaagaacaattttctttacttctctaataaacttgctttcactgtactctatggatttgccttgaattctttcttgagaaagacccaagaactctctcttggggtctggattgggacccctttccagtaacagttacacttgcaaagtacatcctgtgtccaaccactgtatatttaattgtgaaatttattaaatattaatttaaataagttgaaagacctttaaagacagggcaattcaaaaa

SEQ ID NO: 86 - DNA, 701 bp, Homo sapiens
ataagccagaaaatcggaagagggagaaaaatgaaaaatcagcaacaaaactgggtcgagagtgaaaatagctttagtaagaggaattaagttcaattctatcgtggccctgtagctcagcggttggagcgctggtctcgtaaacctaggggtcgtgagttcaaatctcaccagggcctaacagactgccctttgggttcyggtgtttacctacacttcttgtgtcttatttttatgtttttttgagacaaagtctcgctcacgtcacccaggctggagtgcagtggcgccatctcggctctatacaacctccgccttccgggttcaagcgattttttcccgcctcagcctcccgagtagatgggactacaggcctgcaccaccaagcccggctaatttttgtgttttagggtagagacaaggtttcgccatgttggccagactggtttggaactcctgatctcaagtgatctgcccgcctcgccctcccaaagtgctgggactacaggcgtcaaccaccgcgccctgccgaagggtgcgtttattagatgccaaaacctaaaactggaaattattcaaatcgataagcacccattttagcccaccttctcagaatacaggaatgtactggtagcaaaagtaggaaatgctagaaatacactctggttccaaaatggcagaagcaagctggcttcactgct

SEQ ID NO: 87 - DNA, 1001 bp, Homo sapiens
atttatccactcttaaaagggtatctttaaatagctgtggtatccttttgtatttcagacattttatgtaatttaaattctgattcatatccctaattttaggattaaagtgtttgttaacaactaaaaagcaaaacaaaacaaaactaggaagtccttatctgcatctttaagattatatcaaataggctactgagtgcttacctgttaacacctgctccaattgcttgcaattgtggctaatgtcttaaaggtggtagatttctctgctttccaataaaatcacattgccagcatctccagatacaattattctcattttgaatagcgaacattccattgactagcaaaacaaaacatttgaattatatgagatatctagcagatcagaaagagaccatagcaattggattaaaacagaagttaatggaagagaattttagaaagctgctgaggggatctttatagtttttatctgtgatcactttagaatgttttaaygcctagtttagaatacttacctagatgaatacacatccttacctcctttcttacctgtgtattggttgaccttatgtttgtcatcttcctcttgagttttctgattatatatatatttttaaattttttagttatttttaattttattattattatactttaagttttagggtacatgtgcacaacgtgcaggtttgttacatatgtatacatgtaccatgttggtgtgctgcacccacaccaacatggcacatgtatacatatgtaacaaacctgcgcgttgtgcacatattttttaatattaaaaaaggtgaggttcaacagagtcttcaaagcatctttttaaattgcactgtggaacaaaaatcgagacaagagaggcaacaagagttttagtcccaaatctgccatccaaagtcactgtataattgggcgagttagttaatagctttggccgtcagttttattttctgtaacattataaggttgctgttttcctc

SEQ ID NO: 88 - DNA, 1001 bp, Homo sapiens
attctcctgcctcagcctcccgggtagctgggattacagcagtatgccaccgcgctcggctaatttcttatttatttatttatttatttttggtatatttagtagagatggggtttcgccattttggccattatggtctcgaactcctgacctcaggtgatccgtccgcctcggcctcccaaagagctgggattacaggcgtgagccgccgcccaaccactttttttagtattttaaatcaagtatctttttgtttgtttgtttcttctgtgcctatgcttacccagacagtttcttcatttattttcccccgccttgggcaggcttccactcttcagaccctttcctgcacaactttgtccctgagcataggtcctggacgtaaaagaagggacatcgtctggagaaatattgaattaagaaaggcgcggctgtgaagaatagaaatcagtgtctcccttagtctctcagttcggcgatcttggtaatgccctgtcccaygcctgctaacgcgattcagcctcgatatccccgtccagtcccacgatcgcaccaagaagagcttgcgagccttcctgctacatactgacattaagaaaccggacttgaaagggatcccagacaaacgttaaacatgcaacaagagggatagggtgtaaggaagagaatccttggggcggtgtctgataaaacagatggctctcctttccaggtgtttctgaatttgatccccgacgcctggggcatcgtggaggaacttgcataggaaatcaaggtgtcgcaggaaagagaacacgcacaagcaaaagataccttaatttgtagtatactcaatatttatcgtacagaagtgtatcgacgatagacaatgtgcgatgtgatgggtgctgggaacttaacgaactctccacgcgcctagacctcattggatccactttctcttgggctgtgagccggtaaaaaaaaaaggggtggatgtggaggacggtccaaaggattcg

SEQ ID NO: 89 - DNA, 501 bp, Homo sapiens
tgtggagctccgccactcccagcccgggtgaaggaaaactgggaaacagaatgaatgtgattatctattcgaagataaatttccacaaagcatgccgtttgatagtagcttataatgtggaagtaaggcatcctgtcatccggccggttagctcagttggttagagcgtggtgctaataacgccaaggtcgcgggttcgatccccgtactggccaagtattctctgtggcttttatcaccagaatggatartaacccagacatcgatctaaacgtgtacctgtgtgtttctccaggcttaactttgccccgagaaaacggatctgtgaatttggtgcgccctcgcttactcgacagcggttaatttgaacggggacgtttctttccgctgcctccaaggcatacccacatcctacccgtaaaacaaaggggctataggcaccttacagtgacagaggtacgttacggttggaggcttttgtgatttttgtcctcctctgcc

SEQ ID NO: 90 - DNA, 501 bp, Homo sapiens
tttttgatgcggatcgaaagggactggccccggagcctacaacctgacgcaggtgggacttggggaaatgtcgagaaacctaggtctgggacttgagttggcttccagggcacacattcttgttcagaagaaacacattgcaaaaatcgggaggtgacgggcagatgaagtgtcggcgcttcgcctcgggactccagtgcaacctatggggcttttggaaatgaggaagtcgatgactctgcagggactcmtctgacccaggagcagatggcgctcgtctgggcactccccaggagaaaaggtgcatcgggaagcagcctggcttgtggatggtaataagtcactgttgatgggttgggtgcagggagggatttaagttcttgagcgacagatgctagggagtttacctgctctggataacagtatcttgtggaggatagtcacctggaaaacagaaatggcgtgactgtgttgaatacactgtttgatgattctgggcat

SEQ ID NO: 91 - DNA, 1001 bp, Homo sapiens
tggggcctaaggagattctgttgtccagaattcagaaaattctgcctccagaaatacaaatatgctcttttctaaacaagtgacaacacaatgtagccataggctcccttaagcagccacctcatgtcaactaatagtctttgctctctagcctctctcctccaaagtccatttcgtctcctgaggcttcagctattactgtcagaccctcagttacttctgatgaacagggattaggcttgagaaaatggagatgcatttagattggcagatatgggggacttcttaatgtgcttttattgctgccttatctctgaaaacaggttctgggagtttgggaataagtctgagggcatataaaggattgagactgagtgacttaggagtgtgagaggaaatatcttgatgttgagaacagggttgatgtggaggggtattctctgtgttatgcatgtaaaaagaaaaaaaggaaaaaaaaatcattactgggaaagaaaacaycccaagctgaagtccaagaaaggtacacagaggaaacacagaaacagttgtgttagcagaagatgacatgaaacccagctgacagtgaaattaggaagttgccttggaatttcaagaacttgcattctcaagtttatggttctgtgtccaacagagcagcaaaatccagcacttcttcttttgagtctccatatcgtgctaacagaaagacaaggggtcgggagatgcagagatgaggaggagctcaagagtgacagtgttgaagagattctgagcagaactccacagtgatctgtgtaactgatatccaaccctgatccctccatcgtctgcctgtccaacccttgcttagatctcaatgtaacttcacttcattgtgtccaagaagttctctgatctcttcccctgtggatttagcaaccctccattttagaggcattttcaggaatctttttgcaatgcatcatctctatgaaagctcagcttcctgctccccaggc

SEQ ID NO: 92 - DNA, 1001 bp, Homo sapiens
ttgctgtaatgaaataaacaaaaaaaaaataaaaataaaaataaataaaaaaggagcatgtccagtactacgtcataactgaagaatggtagactgcatgaaatctagaaatgagtgaaaaagaattaggctttgtcagtatgtttcttgcaatctccatggaagggagtgctctgtttccaatgaggaaaatataaatttttctagtctggccaaagaccatttattcaggtaaatagttgttttttcaagacatagctgtaaaaaaaaaaaaaaaaaaaagtcctttaggaccagattctctcatataattctatgttccaatctgttcctttttgccctacaaattgttcttcagaaaaaaaaatatatatatatatatagacatatatatatagacatatatatagacatatatatatatacatacacaaaaagttatttggggcaaaacatgaatcatgtgctttcttgaagctaccatataaaagttccagtgtraagcactaacatgacaacctggtttggattagctctaatcaattccccaaggctcattagcaatgtcataaattaatcaagattgtttcagcaacagagggtaccatgcttggctatcaggtgcaaataacttaaaagatctatctttgagtccttatttctctttatctctctgttttagaaattttaacttcttaataactgagagtaatgggcctgatatgtgaactttgtaaagaagtgttcaatttttttctgaatgcttctctccattctccacacagattttagccaccgcacacacaatattcttctagacatcttcttccctgctgacaattccaggttattcaagtagtccctgatggcccaaacttcatatagacatatagatgcagaaatatagacatctatctatattctctgtatgtttaataaggagtcacttcactattctttattctggcctggagaatgtgtttaggtatcttaatccttcc

SEQ ID NO: 93 - DNA, 1001 bp, Homo sapiens
cgcttgtaatcccagcactttgggaggccgaggccggtggatcacctgagtcaggagttcgagaccagtctggccaacatggtgaaaccgtgcctctactaaaaacacaaaaattagctgggcgtggtggcaggcacctgtaatcccaggtatttgggaggctgaggcaggagaaacgcttgaacccttgaggcggaggttgcagtgagccaagaccacaccaatgaacttccagcctggctatcaagagcgaaactccatctcaaaaaataaataaataaaattaaaaaataaaaaaagaaaaagtaaggtattctacccatgaagcttgaaagatcatgctatacaaataaaaaactctcatcttggattgacctagatgagtttgtaggccaaggcaaaaattacacttctactgcagagactgaaccctgcttcatacaaaacaaaagatacttgaaactgtactaatgctaggaagaaagacatgatgacaagctvagagtgtcaattggcaggacaggcatagttggggttctggggtttttctggggacagaattactgggaaattcactgatcttccccacatgcagaataatctgccatcagattctataaaacaagtttttctactttactttgaaactttgaagaagatagccccacaaaatattatcatattgcagaaaattttcctagatcattaaagtaaaagaaatgttaattaacagtaaataacttgttaaacttaaattttccctctgctcaaaataacttcccttcttcttcaccacaagtttactcaaattttagatatacctcaagaataatcttcccttgggaggtttcctcagaccaacgtgagttacatgtccttcctctgtttcgatttgtcacgacaaaaatattatatgtatgaatttctacatggaataaaagtaggattttattcttaaaaaatatagttcttagattttgctctgcaggcattgagttttt

SEQ ID NO: 94 - DNA, 1001 bp, Homo sapiens
ttataaaaactgatacaggaagtaatagaaaatttaaatagtgctattaaacaaatgaatcagtaatttaaaaaccttcttacagagaacactcccagcttatactgcttcaaaggtgaattcttccaaatatttatgaaacaaataacatgaatcttgcacaaactctcaagcaatagagagaaaggaacacttcctaaaatattttgtaagacaagcatactcttgggtatcagacatatcttatgtgccacctctgattctcttgccatcttaccttgcaacttgttttaccccaatagtcatggcaatcaatttcctctgagtgcagaaaacaacaggacttcactgttcacctctgttgaacttctcgtcttctgctataaggcttctctgctgctgttgaaacatgagctgctgagcgatctttgatatctgcacatgcccaacttctatatgtagggctattaatgctctatggagcaaaactttgatcagttrgatatagtagctgaccaataatttttttttttttttgagatgtgtcttgctctgtcacccaggctggaatgcagtggcatgatcttggctcactgtaagctctgcctacccagttcaagcaattctcctgcctcagcctcccaagtagctaggattacaggtgtgcaccaccatatccagctaatctttgtatttttagtagagatgggtatcactgtgttagccaggctagtcctgaactcctgagctcaactgatcctcccgctttggcctcctaaagtgctgggattacaggtatgagccaccatgtccagccgtgaccaataaatttttcccactttcttcccctaaatagccttccctgagattacactccttaatacattaataatacattataatttgattcagtggatgctgtttacatgagtgtgttcagtttgtgaaacttcatcaaggtttacacttacaggtggagttttatgtgtgtatgttatgcc

SEQ ID NO: 95 - DNA, 1001 bp, Homo sapiens
aaaccacatctctactaaacatacaagaattagctggacatggtggctcatgcctgtagccccagcttctcgggagggtaaagcatgagaactgcttgaacccaggaggcggaggttgcagtgagtggagatggcgccactgccctccagcctgggtgacagagcaagattctgtgttaaaaaaaaaaaaaaaggatggcctttttcacagcctaatgcccttgagatccatccaatttgttgtatcaacagttcctgccttttaattgttgagtagttgtttatagtatggatgtaccacagtttctttaaccatctacctattgaggtacattttagtagttttctagtgttttgctattataaataaaggattacaaataattgtgatagacttttgtgttgacatagttttcatgtcatttttattatcgttatatattattgaatatatacaatatatattgaatgctacacatgtagcattcacgtttctgtttyataaaatgtctctgtttcatcactgtgaaatgcctccttttcttttttattatgtcacgtctctatggtaatactccttgtcttaaaatctacactttatgttaatacatacgttttatgttaatttttttatggttcgcctttgtggggttttttttttttttggttgttgttgtttttaactttattttattttatttattttatttattttttgagactcactctgtcacccaggctggagtgcaatggcgtgattttgtctcactacaacctctgcctcttgggttcaaacgattgtcatgcctcagcctcctgagtagctgggactataggggtgggccaccacacctggctaatttttgtatttttagtaagagacagggtttcaccattttggccaagccagtcttgaactcctggcctcaagtgatctacctgcctcagccttgcaatgttctggaattacaggtatgagctaccacacccagcctaacctt

SEQ ID NO: 96 - DNA, 1001 bp, Homo sapiens
tgggtcaaaatgacaccggagaacggatactggactatgggcctgactgatgggaataagtatcgggctctcactgagcccagaaccaacctgaaacttcctgagcctcctaggaaagtgggggtcatcctggactatgagactggacatatctcgttctacaatgccacggatggatctcatatctacacatttctgcacgcctcttcctctgagcctctgtatcctgtattcagaattttgaccttggagcccactgccctgaccgtttgcccaataccaaaagtagagagttcccccgatcccgacctagtgcctgatcattccctggagataccactgaccccaggcttagctaatgaaagtggggagcctcaggctgaagtaacatctctgcttctccctgcccagcctggagctaagggtctcaccctccacaacagccagtcagaaccataaagctacaggcacacactgaagcactttactgatattcattcrattattccataggacagttgtttgagtttggtgccaccttattggcccctttatacagataaggaaactggggtgtagaaaagtgtattgactttacaaagcagacaggaatagtgaacaacagagctgggatctgaacaacaatgactaacattaatggagaatttaaaacgttctgagtgctgtgttatgagctttggtgggtgtcactcctttaatcctcacaacaccctgtcaggtagtctcatttggcaagtatggaagcagaggcagggcaacattaagtagcttacataactcacacggtaatttgtgcagttgggagatgttcagcttcagtccctggccaattgcccgttcttttccagcctgatttttcctgcatgggaagagcccacatgtagccctgaggttcccttcccaggacagctccaggatcgagatcactgtgagtggttgtggagttaagacccctatggactccttcccagctgattatc

SEQ ID NO: 97 - DNA, 2802 bp, Homo sapiens
tctttctacatttttgttgtttccctccccacattgattctgcccactgatgctttatactcagaggttaattttcttttcttttctttttttttttttttttttttttcttgagacagagtctcgctctgtctcccaggctggagtgcagtggcgtgatctcggctcactgcaagctctgccttccgggttcatgccattctcctgcctcagcctcccgagtagctgggactacaggtgcccgtcaccatgcccggctaattttttattttttgtatttttagtagagacggggtttcaccgtgttagccaggatggtcttgatctcctgaccttgtgatccgccctcctcagccttccaaagtgctaggattacaggcatgagctgctghgctggccctcagaggttaattttcaatcttcactcgaccactcgtgagctaaatgagttccccttttctgcagtctatttttccatacatccaatttatttaacaaggtggagcctcatctgaagcatttcctcacctgaaaaatggggataaacatatgaatctctagcgctgtagaaggcaatcatattatttactcagcccacagcaggccatgaaggaagctcctcatcttcctgatagctgcaaggccgtctctgtgctgggctctgtgtggggccttatatgccctagattcactctccagccttcagctttctccaccctcttctggaccccaggaatctgtcctctatggacagtgccactgggctcccttgtcctctggtttgctgctgtgtttggccaatgggaggccctgatagaagattagaaggagaaagaaaggagatacacaccgtttaatttcctgcttcctccctgccagcagcagctggtggtgctctaacaaggcccgaggactcttctcaggaagctccctcgttaagctacctctttctctgggttccagtaattgcctcccctttttagccctcccaggctaggggtggagacagctccccactgttgggaaccatgggggcactgcacttttccttgttgctttcccttaacccttctttctggaaaccttgtccaactacccagtttgagctcaccatctatttcttgctaggtttctgccaagcatgttcattattccttcagtcttcacctcaacccccatgaaaaacagattgcaatcatcatctaaaaatgtggaggccaaagcttggaagcattaaatcctttgaggagatacaggcagtaggtggcatgagaagcctgggaaggacaaagttctttgggcaggcatcacctcctctccttggcatttccatcctcactctccctgcagtattactcagtgtgtgtctccttcccttcacctccaccctttatgcgtcttcctacccacgaaggaagtcaagggaacttttctgctccaaatcacaagagttggagaagaaaaaaggaaaaaggaatatagtccctcaggttgttggtccagggaacatgcagtgatttactcaccaggcttgaagagggccatttttccattctgaaaggaaggagacacagataagaaaaaggtcagtatttttgtacttttcccactccattctcctctcactacatgttttctctccttttctttagagtctcttccagggtccagcttccctcctctacagctctgatggatcagaggtggcaccttctcaaaaatgtcaggcttggctccctgtgtcatggggggtgcaggatgcatggccaggctttacaagggggtgtgcaggatcaggagtttctcagaggctccagaaaagcggaggtgaacccccaccacacagaaattgagtctttagattagatctaattaatccagctgagaacatccacgggtcacagtggagaaaaagttgaaatattcagggcatgtgacccagcaaacttacagagcatcaggctgacttattggtatcggacgaagactcctctccacctacaatgaaagaaaggtagaggtgtcaccagaactctgccttttctgtgttggccccttccccttctttttgcatccatctagtctttttttttttttttttttttttttttttttttttttttaccatcccacccttccccatggtctccatcttcaggtacaattctttcttcacctcttcttaatatcaagtctgggaacatcggttgaacgctagtggcagggcaggcactgtgagagttccttcccaatggggtccagctcatctgttttgaatgtgtacctgggcataggtgtcaccatgtctatatgtgtatgcctaggagtacaagattcatccttctcaatctgtatcatttcgtaccttgctctaaaaagaatttgggaaatttaatgagcaatttcagggactagtttttgaaagcagttatgatctatctgtaccaactgagccactgtagctactcctctttattagacacacttttctccctccctctctcttttctgattttcttatttcttaaatcttccattcttgttttcctttcaacagcctctagattatgggaaacaacaagtaagtttcctgccatagaaaatgcacctcatccttctcttccctcttccttttgaagtgtacccctggatattcctcagtgctttttagagcttaagggtctgtagcccctagtacaaagagattgaagacctcttttttttttttttttttttctagagagaaaaagcactgggtggtttctccaaagagccacacttgttttctttttctgggtaaag

SEQ ID NO: 98 - DNA, 1001 bp, Homo sapiens
tgggtgaaaacaagaaaaacttttaaaaatctactctggcatcttttgctagcaggcattgacaattaggagaaggcaaggtgttaacttttactgatctcccacttttttttttgagacaaggcctggctttatcacccaggctggagtgcagtggtgcgatctcagctcactgtaaactccgcctaccaggctcaagccatcctcctacatcagccccctaagtagctgggacaacaggggcgcgccaccactcctggctaatttttgtgctttttgcagagacggggttttgctatgttgcccaggctggttgcgaactcctgggctcaagggatccgcccgcctccacctcccaaagtgctgggattacaggcatgagccaccgcgcccacccctctagtttccagtttagtcggaaagattaaaaacgccagccttgttttcctagtgctgtttttggtttttacctcgggtcttttgtcgtgccttaaaatcatrtctggttgcgcaagtgagggaaaggattgggtaaagggggcgccaccgcaagttgctgtgcaacatccagacatcaccagacccaccacctggagcctggcctggcggtgtcaaacgcattctggtctcatctttttagaaacccgtggatgctcaaggaatttccggataacgtgatcccggatgcgcttgactgacttacacggaacgagcaaagcgcaaagcagtccctgctaaggacttagtttatgccctcaagcgcaaaggtcggaccctctatggtgttggtagctatatgcacgtacctcatgtacatttcaccttaaatggctttcaaagagctagattaatttagtggatagatcaaaatgatttatgacccctcgccccccagtgataggaagagcgaaccagctcttctttagataatagtgagtggctctgaaaagagcctttgggttggacaagagcttgagaatttacttggagctggtgtactt

SEQ ID NO: 99 - DNA, 1001 bp, Homo sapiens
atttagtggatagatcaaaatgatttatgacccctcgccccccagtgataggaagagcgaaccagctcttctttagataatagtgagtggctctgaaaagagcctttgggttggacaagagcttgagaatttacttggagctggtgtacttggtgacggccttggtgccctccgacaccgcgtgcttggccagctcccccggaagcagcaggcgcacggcggtctggatctccctggaggtgatggtcgagcgcttgttgtagtgcgccaggcgggaagcctcgcttgcgatgcgctcgaagatgtcgttgacgaaggagttcatgattcccatggccttagaagagatgccggtgtcggggtggacctgcttcagcaccttgtacacgtacacggagtagctctccttgcggctgcgcttgcgcttcttgccatccttcttctgggccttggtcaccgccttcttggagcccttcttcggggcgggagcagacttggccrgctcgggcataatgaaacaatagtggcaaaaccaaaacaagaagtcggtctcctctttttatataatagtttatgcggccgaggtagtgggaaggtctctgctgattggtaattatccgtggatgacgacagatgccagttttgcccaatcaaaataggtatcctgcataatcgagtcctattggtctaaataaaaataaaacgtaagccaatcgcacagcttccttttcgcgcccagtagaggctataaaatgtacgtttttctagtttcacttcagtctttcttgaccgtatagataataggccttttgccatgtctgggcgtggcaagcagggaggcaaagctcgcgccaaggccaagacccgctcttctcgggccgggcttcagtttcccgtaggccgagtgcatcgcctgctccgcaaaggcaactatgcggagcgggtcggtgctggagcgccggtgtacctggcggcggtgctggagtacctgaccgccgaga

SEQ ID NO: 100 - DNA, 1366 bp, Homo sapiens
ggtatttcctatgatttcataatagacaaaggtttaattacacaactcctggctgaatctagagtactaaaatgtggctgttagaaaaggttgctctctgggcccgatgcagtagctcatgcctgtaatcccagcactttgggaggccaaggctggcagacagctttaggccaggagttggagaccattctggcctatgtgttgaaaccccgtctctactaggaatacaaaaaattagccgggcgtggtggcacacacctgtaatcccagttacttgagaggctgaggctgagaatcgcttaaacctgggacacagaggttccagtaagccgagatcacacctctgccctccagcctgggtgacagagtgtcgccaaacaaaacaaaacaaaacaaaaaaacaaaaaaaaagattgctcttacccagggatgatggtcagatgcaattacaggttatgaatttggcataaaagtaatgctaagtgtttcacactgcacttactgttgtcagtgttctaagtgttttttatttaccaattcatttacacttgtttgtcttttttttcaggtctccaactcctgggctcaagctgtcctcccacttctgcctccccaaaagctgagattacaggcgtgagccacccggccctactcatttaatccttacaacaacccttagagctgggaactatttttatcatcatcacataattgtttacaaaaataaathgaggcttagagagcatatgcacctcaacccaagatcccacaagtagaatattattgttacagatttggttgcaaataatctgcttcttatgattgtgctttaaatttttcaccgtgtcacatcactttggtggtgtaaaattataaaacaacatttaagtcttaactttaaaaatgtgtttttggcctggtgcgatggctcatgcccataatcctagcacttggggaggatgaggcagtcagattgcttaaggccaggactttgagaccagcctggacaacatggtgaggcaatttctctactaaaaatactcaaaaattagctgggcctggtggcctgcgtatataatctcagctacttgggaggctgaggcacgaaaacccaggaggcagaggttgcagtgagccgagatcctgccactgctctccagcctgggtgacagactaaggctctgtctcaaaaaaaaaatatatatatatatatacatatatatatatatttatatgtatagacatacatagttaaaatatatatattattttttacatcttaaagagaaacattatttatatgcaaaaaattttatttaggcccacttagcaattccagatctgacaacttttgaggatttaaaat

SEQ ID NO: 101 - DNA, 528 bp, Homo sapiens
aacataaaactctaagcatttattcaaatatattagaaatttaaatgacataaaaattgttaagtactttatttggactagtgcaaatagcataaatgtgaatttaaatatatacaaaaagttaagtaattgaatatcaataaaatattaataaacagtaaatataaattttctatatgtgactagtgagatctactaagctagtctagccatttttctcaattatctccattatttcctaaagtatcctgtggagtaactctgattgcctttactctcattaaaaagatgaggaaattaagacaaaaacagcaaaagtatctgcaaygaagccacaatttcagtctaggtttgtttgattgcagaggctgaactcactattctccaaagtaaatatttacatggaaacactaaaaaacaaagaaattacattttaaattgtgtcaagattacactttctttagagttaaaagaattccacagtgtatccatgcatgtaaaaaatattaaatatatgaaaagacgact

SEQ ID NO: 102 - DNA, 801 bp, Homo sapiens
cagccttcttggccttcttaggcgtggcccccgcgggcttcttagctttagcggcgcctgccttcttggctttgggcttggcttccccggaggccgccttcttgttgagtttaaaggagccagaagcaccagtgcccttggtctgcaccagggtgcccttgctcaccaagctcttgaggcccagcttaatgcggctgttattcttctccacgtcgtagccaccggccgctaaggccttcttaagggctgccaaagaaaggccattgcgctccttagaagcagccacagccttggtgatcagctctgagactgggggccccgtcgctttgcgcttagcagcgccggcgccggcagccttcttagttgccttcttcttagccggggatttctccaccggcgcyggggtggctgtctcggcaggagcggtttccgacatggtggcaagaaactgctagaagagaataagctcgaaatctaaagagcaggttttgcgttgctgctatgctcgggccccgggcttatataagccggcgctgccctgtgattggtggagcgtccaatccaccgccctctggccgccgccgctcgcggttggactcccaaattgtgtttgttagtcctcaaaatttgattaaatgcttaaaacaatggtacagaatttggcactttgaagctccaaaggaggaaaacagcctccaggttcacatacttgtttgtgttttcaagaatcttgtgcaattgatgaaagatattttaaaaaatcccttcagcttttcataagaatccattgggctgagggca

SEQ ID NO: 103 - DNA, 1092 bp, Homo sapiens
gatttggattcctaatgaaatcaacagtcacttatttctcattcttgaaatgctgtgcaagaaaatttaaagtagccaatgcacttcatcttctaagaactcctggagaagttggcagactatggccaaatctggacaatggcttttttctgtatggccctcaagctaagaagtgtctttatgttttaaaagtattgttaaaaaaaaaaaaaacaaaaacaaaggctgggcacggtggttcatgtctgtaatctcagcacttggggacactgggataggtgggttgcttgagctcaggagttggagaccagcttgggcaacttggtaaaaccccatctttaataaaaatacaaaacattttgctggatgtggtggcacatgcctgtagtctcagctactcgggaggctgaggtgggaggatcacttgaattcagggtgtcaaggctgcagtgagcaatgatagcagcactgcactccagccagggcaatggagcaagatcctgtctcgaaaaagcaaactaactaaaaactaaagagtgtgtgacagagactatatatggcctttaaaccctaagctatttattacctagcccttttgctgtgttataaatttctccacagagacacagatattgtataggcctcttaccgaacaatgcaaattgagaactaaagaaaaggagatcttcaygagcaaatgatctaaccaagcactttccactgttccaaacacaaaacttagaaggtccaggagaaaaaaaccccaaaactccatgtgtaatggagccagggtataacaataagagctgacactcattcagcatttactacctgacaggaagtaatcttaaatatgttctacaggtttctattaatttgctacatttacagctatacaagatgaggcccagatagagaattaataacttgtcaaaggttatacagctatgaagtggcagctctaaattttaaacctagaaacatggcctcagctctattatggagggaaaatccttgaagaggtgagaagagaactatcttcaaagcttggaagaggcagtgtcaagttgttcctacacctagcaaacagcc

SEQ ID NO: 104 - DNA, 1001 bp, Homo sapiens
gatctcaggtgatccgcccgccttggcctcccaaagtgctgcgattacaggtgtgagccactgtgtctagcctatattgccttttaattcttgttttttacaatgatggcaatccataatgttattcaattgttgtttaatcctttcataagaatgttattctagtttttctggtaattaaaaagacagctctggaaacttccgtagacttacctataaatctgttattgttttgatttcatatcacttttaaagattgtgtacattttgttttgtttttttaagtaatgtggtccagctagtcacccaggctgaaatgcagtggggccatcctagcttactgcagccttgaacttctgggctcaagctatcttcctactccagcctcccaagtagctgggactatagacatgaggcacctctcctagcttcacttttaaaggttttaaaatctaatctttctctggttttagcttgcttaatacaaaattcaattatgtyctataggaaaaatttcctctactttgggatcttggcagtgatcctcctagaaatggtgatgggcaaaacaaaaggcttttgattttgttgaaatgtgtttgataggctacattaaagccacagcacaaagaaaccttgtagagcaaaggaataaagaaattattgatgaaactctgaatcctggaaggaaactcaaagatcatcttactaaaccctacctttatttacatttgaaggaatggaaaccaagaagtatttgtgaaaaacatgctgtcacgccagaacccagatctctgggattcctgtccaatgtgtgtgtgtgtgtgtgtgtgtgtgtgtgtgtgtgtgtgtttgagagagagagacagtgtgagagtaggagaaaaagcaggaggaggggaaggcgaaaagggagagagaaagcacaattctctcattccatatatgtattgagtgcctactatatgtcagggatacaccaataaatgatatggattgta

SEQ ID NO: 105 - DNA, 1001 bp, Homo sapiens
cacagcacaaagaaaccttgtagagcaaaggaataaagaaattattgatgaaactctgaatcctggaaggaaactcaaagatcatcttactaaaccctacctttatttacatttgaaggaatggaaaccaagaagtatttgtgaaaaacatgctgtcacgccagaacccagatctctgggattcctgtccaatgtgtgtgtgtgtgtgtgtgtgtgtgtgtgtgtgtgtgtgtttgagagagagagacagtgtgagagtaggagaaaaagcaggaggaggggaaggcgaaaagggagagagaaagcacaattctctcattccatatatgtattgagtgcctactatatgtcagggatacaccaataaatgatatggattgtaacacatatttacttttgtaaatgagcaattctattataaaagataaatatgcttttagttagtaaaatgtaggcaaaaatgcttaagatgttttaagtagacataagtagttagtaaamagagcatatgttgttaaatatagatataagggatggaagggtcaaaagatacctaatgttcctgatgcacaaaatatacaaaaggagccacacattcagaattcacagatatatgagacatcgaagcactgactcattattcatgaggccttgagtcagccacaaattggagacaccataagttctctactttaggaacaaaaataaaatccatggctattcaaccaactaattggttgggtccaggcatatatatctctgtgtctatcctacaggctgattgagcgatgtaaaagagatcagatatacggaaactgctcacacttgagtcagatagtgtggttcttccaattcacttacacactaaaccattaacttgctcttctttttccccttgctgcttgctatgttttttaatgaagctgtgatttgagcatttcactgcatagtctgcaaacctatttgtgctgtgtcctctgggagagcttgcatgggactat

SEQ ID NO: 106 - DNA, 1001 bp, Homo sapiens
tattgagtgcctactatatgtcagggatacaccaataaatgatatggattgtaacacatatttacttttgtaaatgagcaattctattataaaagataaatatgcttttagttagtaaaatgtaggcaaaaatgcttaagatgttttaagtagacataagtagttagtaaaaagagcatatgttgttaaatatagatataagggatggaagggtcaaaagatacctaatgttcctgatgcacaaaatatacaaaaggagccacacattcagaattcacagatatatgagacatcgaagcactgactcattattcatgaggccttgagtcagccacaaattggagacaccataagttctctactttaggaacaaaaataaaatccatggctattcaaccaactaattggttgggtccaggcatatatatctctgtgtctatcctacaggctgattgagcgatgtaaaagagatcagatatacggaaactgctcacacttgaktcagatagtgtggttcttccaattcacttacacactaaaccattaacttgctcttctttttccccttgctgcttgctatgttttttaatgaagctgtgatttgagcatttcactgcatagtctgcaaacctatttgtgctgtgtcctctgggagagcttgcatgggactatacttggagcctaccagggcatcaaggtaatttctcacatggtaccaataaggaccctctatcataacaaaaatgtggaacagtcacctttagacagcaacttgcaggaagtgagggaaaaatgatggaggtgtgttccagtcagaggtaaaataacgtagaggggctcacagggacacaatgctcagcagtttgaggaacatcaacggggccagggtagctagagtagaggaaacaagtaagacagccctaggagatgaggccaaatacatcactggggccagagtatgcaaaacttcatagggcaaggtaagggctttggaagtttct

SEQ ID NO: 107 - DNA, 1001 bp, Homo sapiens
agacttctttagttgtcctttaggatgtatgtcctttaggacagtgaccatgttcttttgtattgactgtttctccaaggacacattcaatgataatcaatgtggaggacttccgagataatgaccctttgccatcacaggctgtctacctcttctcagcattaagaccctctgcttattcacatgcccacagctctcgagggaagaaaagaagtctagaaatacccaaccaggcgcatggacaaattggcctacgtaggccttcctccatgcctccccttcccccaaacccacatttattttcattcctttccttctagtctggcacaacatgtcagtaaaaaggacacaagactagaaagcaaattctgagatttggagcatctgtctcagaataagcagttgcaatatgccttatctttcccagaatatgttcttgctccacatctaacaataaagttccaagaaggggaattcgtcaacatctctctgactgatttracaaggtgaagacatatctgtttaagaggtattgctggtagccagacgagagaagctattgagacatctgcagtgaggtacctgttgcaaagccccaccgagaaggtggctgcggggaactcattccttctttgggatcagcatggttctgtattacatttttagaagagctgagtttccatgtgttcttaaggtctaggatgtatacaggagctccagtatcacagtggaccccacagaagtggccaactacttacatttcaatatccttctctgcttttttgtttatcagaccaaagctgaatgtgaatctgatggctgctgctttagttcaaagccaatggagtgctatacctacagaagcagaactttaataaactggcctgagcaatagcaaatggggaggacttctgaattaacgaccctttgccatcacaggctgtccacttcttctcggtaataagaccctctgcttattcacatgtccacaggtaacctct

SEQ ID NO: 108 - DNA, 1001 bp, Homo sapiens
cagtgccaggtattttaaaaactctcttaaaagttttcattatcacgcacttgtgtatacttattctgtataagcgcttctatatacacttcaacaatgtataatttggttttattttcattttatttatttatttatttatttatttatttatttatttatttatttattttaagaggtagggtctcaccatactgcccaggctggtcttgaactcctgagcttaagcaaacctcccatctcagcctcccaaagtgctaggattacaggcatgagccaccatgcccagccatggttttacttctgagtttaaaaaaaatgttattatatatgaaccttctgagacttacatttctaaaattcaaccaggtactgtgtgtacctcaataaatgcattattttgaccatgaacatgtagttgcctctagtatttttatctattaaaaatggcattttttccattctcatatgtctcctgttgcatgtgtgcaaaatattctytcatgtaaacagctaggaatcgaatggttgggtcactggagtacacttactggataaaaaatattatcaaaaaccttcagcaaatacaatttgatgtggaagagttcccacactgattcttggcaaagaccaaaatacttttaaatatgccactcctaagtgtttaaaatgaagacactcattttgatttcctgagttgggggtgggggaaaacaatggagaacagcccttctcctcctctatttttttttcttttaacatttcttccaattactagagatacagtaaacgcaagtgacacagacaagaaaacatggagcagaccctaacagaaaaagtagggaatagaaactatgttcataaataggaattccacacaagagaattatgggaatgagtaagacagcaagattcctccaaaaaacctgcactgccaagaattttcccaactagaacactcaccagagaaaacggtggccaagtttcaaactgccctcgca

SEQ ID NO: 109 - DNA, 1204 bp, Homo sapiens
tagagctgtgttcagttttatctgatagtcgagtcattttgcaatggcactggaatgctgtatggagatgaagcaaaactaaacggcttttacaccacattgttttgagatagaaagtagacattgaaatgtttacggtacatcaagaaatttaggcgcggcagctcgcgcctgcaatacagctgaaacaataagaaaagtgaggcaagagaataacaaagggagctgaaagttagagggcagaataagtaaaagcaaagggcagaagtaaggtagatgggcgggtgaacaagaagcgagataacaagcagtgaaccttttgcagccgaaacaaaagagataatgtgagcaaggacctcgtggccggcaagatctggaacaaaccagtttaagaggcagctcttcagagatgggcatgcgtattagagaggaaaagtatccttaacaaaagcccgtatgataatcagctacttaaggttcatgcatatgggctacatatcatgcatatatttaagattataagatagaggcacaagccacagaggacaaagtaagcaacaaacctatcaataaaagggcagatgctggctatagattaggcagcactgggaacagaaaacatacacacacgcacgcacacacataaaatgactcaaactacagcaagctgacgctgatctcacctcgcagaggtcagtccgctctctcccrcccccgagagtgtaatactctgtttactaaacttttgctgctttgctttgctatctgtgtgtgtgtcgtccaatttctaccgggcaccaagagcctggaactgtttggcaccatccggtaaacagaaccgctttgggaagccgaggcggaaggaccgctagagccttggagttcgaagccagcctgatctttacaaaagtaaaataactaaccgtgcctggcgtctcatagcctgtagtcctagctactcgggaggctgagaccagaaggatcacttgagcccaggagttcgaggctgcaatgagctatgattgcaccactgcagtccagcttgtgtgacagagcaagagtgtttcaaatgaacctagtgtcagatatttactttctgtattacagaggactgaaagctagctaaataatacttttcagtgtacctgggttccagagataaaattggtaaactaacctttgctccttacttgggcttttagtt

SEQ ID NO: 110 - DNA, 1538 bp, Homo sapiens
agattttaaacatgtttctcaggtatccatttatgaaactaaaccggtaagcagtgtatgccaacagtaagccttaaaagggcgaggcaattgtcatcatccaatatttgtcagtaagccaaactgtcatttctctatgtaccaggatgttaccttttaaggaggagtactccacaaatatgaaatatgcaactgggggaaaattagctgatcctaaccattttgtagtatctgaagcaagaatcaaccttattaatttacctagatttatcctgacatttatgtgttttcatctttttgcatttttctgtgctggactctccttaagatttttggaaacctgtgttctgaattcctccctttccctgggctagagtggctggaggctttggctcttgggaatggtctcgcgtccttcaccagaacttacgggaatcatgtttggctgaagagtcggagacctctccagagtcatcttttccagttaggatagaaacgagcccccctcctcacctcgcaagcccgcgccagtccagttttagccgttcttttggaagagcaagtcagttgaacgccatcgaagaggctcctgatttagatattaattgtgcttaaatgcagatgactccccactctcatgcgttcccttatttcccgttgcttctcccattggcatttacagacttgaggttgcttggactctcaattcaatactccttttctgcgggttcgtgagaattaggtgtgaacgtgatgtccgcggatatcagtggctagtgggcaagctccagcgcccaggaactttgagtcgcttgtctaggagtcctgtattgaattgcaacactaagtgcaatattctggttcttgttgtgttctgaaagagctctttcactcatgaggagagacctgcacgagactgtgaagaccaactgcttctcagcgctccacgcatccattatgagttcaccgcaggattttacctgmaaaaattttgcgtagattaagtcacgcttattgcctcctacttttgtcagtgaacattatgtcacaagcattttcccagaactattacagtcttccagcatgtcgtttctagtggcttggtaatgacctattaggcagatggagcaataataataataaacaactctcattttaatatctatttttcactatcacaattagaaataaaaataaagattcctgcatagtatatgtcttcctttggttaagcttatttcctggctgggtgcagtggctcacacctgtaatcccagaactttgggaggcggagatggaagaatggcttgagaccaggggtttgaacaaggagtttaagaccaggctggtcaacacagtgaggcgccgcatttctatttataaaatataaaacaaacaaacaaataaaaagattatttctctaggagagcggttctgaaacttcagtgggcatcagtaccagcaggatgacttgttttttgtttgtttgtttgttttttgagatggagtctcactctgtctcccaggctagagtgcag

SEQ ID NO: 111 - DNA, 1001 bp, Homo sapiens
cacctgccaccacgaggcgtaggatggcctcatcgtaggacctgccttcttggaagtaacagcggtagatcccattctcctgggctgtgacgttatgtatgaccagggccacgctgcccctgttgatgtctttgctcacaaaggtgattcttccccggtactcctccatctgctcctctgttctctctctcccacccttatacacaaacactgcgggggagaactgagaccggaaccaccgcacctccatgtcctcagcatttttctcgggtgacagatggcagcgtaatgtagtgttttctcccaccatggccaggatgggattagctggccccacgacagtaaactgggctgttcaacaagggcagaatcagacaaggatgccagttatcacaactctaaggcaaaacaaaaaacaaaaaacaaaaacaaacaaacaaaaaaaactccagggatgaaaggaagcagatattccaaggctacaggggttcttgggctgasaacccttctggggaccagtagctgtggctggtcggcagcaccaacccctgggagcagtaactattgaggctgctcctgcttcacgaaggaaacattggggagcccgccctgggcaccctgtgcccctgagattttcctccattttgcaatctagcactgtgcctgagtgtagtgtaaacttgaactgtccattagggtatctatccactagctatttaacagttccaataaaaatgaactctaagtgtaaaacacacacagattataaagatttaaaatttcaaaatgtcaaatatctcattggtaatagttctattaactaagcatttaaatattgatatgtgattatttatatgaaacaaaatacattattaaaatttatttcaagtatgtttttaccttttaaaataaaaagtagaataggcacagggtcttgcgcctgtaattgcagatatttgggaggccaaagtgggaggatccttaacagctaggagtttgag

SEQ ID NO: 112 - DNA, 1001 bp, Homo sapiens
tggatgttctcagctggattaattagatctaatctaaagactcaatttctgtgtggtgggggttcacctccgcttttctggagcctctgagaaactcctgatcctgcacacccccttgtaaagcctggccatgcatcctgcaccccccatgacacagggagccaagcctgacatttttgagaaggtgccacctctgatccatcagagctgtagaggagggaagctggaccctggaagagactctaaagaaaaggagagaaaacatgtagtgagaggagaatggagtgggaaaagtacaaaaatactgacctttttcttatctgtgtctccttcctttcagaatggaaaaatggccctcttcaagcctggtgagtaaatcactgcatgttccctggaccaacaacctgagggactatattcctttttccttttttcttctccaactcttgtgatttggagcagaaaagttcccttgacttccttcgtgggtaggaagacgcrtaaagggtggaggtgaagggaaggagacacacactgagtaatactgcagggagagtgaggatggaaatgccaaggagaggaggtgatgcctgcccaaagaactttgtccttcccaggcttctcatgccacctactgcctgtatctcctcaaaggatttaatgcttccaagctttggcctccacatttttagatgatgattgcaatctgtttttcatgggggttgaggtgaagactgaaggaataatgaacatgcttggcagaaacctagcaagaaatagatggtgagctcaaactgggtagttggacaaggtttccagaaagaagggttaagggaaagcaacaaggaaaagtgcagtgcccccatggttcccaacagtggggagctgtctccacccctagcctgggagggctaaaaaggggaggcaattactggaacccagagaaagaggtagcttaacgagggagcttcctgagaagagtcctcgggccttgttagagc

SEQ ID NO: 113 - DNA, 1001 bp, Homo sapiens
ctttaactcaaatgataattttttttttcattttctaaatacactcatcaaagggcttgaaaaattctgagtttttacccctattgttccacagacaacaaaccttttataaacccctccgttactgcaaaatggaaaagagcacaattgtgtccaggtcagagagtcttcacttctccaggattctgagctccttcctcccaagggctcaaggcctcacgatatatgaaaatgaagaatatttgagaccctgtctctaccaaaaaaaggaaagtagggtgaagtcaggacaataatgaattcataggctgctcctaagatgtctaagtcttgcattttcacatttatcatagcctgtcctcgcgcgggagaatgtacacctgttttggaaggatctaccccaccaggtaacagtaagaaagactaagatgaacagatatggaagatagctcagaggctgcaatgggataaattctgggcagaactcaaacagtggtccaygcaaccttgatcccttccctgaactctttctctcttactcaatccaacctcaatttattggctcccataagttccctgtctacccctcttgttctaggaactctccatttcaaaagtacttccaagaatataattcagggacgtccacactctaccagatctcagccttttgcttccccagggcaaacccctgctaacccctcttccacacagaagtccaccatcttcatctccacaccatcttcacttcacttcccctccaccttcacatatgcaagctgttgtgcataaattacacaaattataattataacattatacaaactctgtatgtataattttaacacgggcttggtaaatagcggaattatgtcactgtaataatgttgaagcaccattaggtcatatctgattattactaccatatcaatagtgtgtgcccccaagaaagagcagctgaccacaaagctcactagtaagccacagaagaatacagtatt

SEQ ID NO: 114 - DNA, 1093 bp, Homo sapiens
tggccttgactaagtttatggcgacagcaggtaagtctggagagaaagctttacaggacatgtgggtggcttggacatgcttctcctagcccaatgctgtccaatagaactttatcctgtatctgtgttgtccaacacagtaatcgctatgtacatgtggctattaaactcttgaggctgggcatggtggctcacgcctgtaatcccagcacttttggaggccgaggcaggcatatcccttgacctcaggagtttgagactagcctggacaaaatgatgaaaccctgtcttcacaaaaaatacaaaaaaaattatcaggcatggtggcatgcccctgtagtcccagctacttgggaggctgaggtgggaggatcgcttgagcctgggaggtcgaggcatcagtaagctgtatttgcgccactgcactccagtctgggagacagaaatagaccctgcctcaaaaaaaaaaaaaaaaaccacttgaaatgtggctagtactaatgaatttttactgaattttagtggctactktattagacaatacaactcaactctaggcagtggtttcttaataggcaggtagtataaccagattatgtcttagattatagttataatatggagaatgcattgaacagggacaagaccaaaaacagtaaaatcagtcaaaagactctcggaataatctaggtaggtgtgtgtaaactttggcccccctttagttatcagtccttaattctactctgatttttttcagttaggatgtttatttgattagtaccataaagaccaagtaacaatgattaagcaagatagaaaattttctttgtcatataaatgtgctgttgaagggcaaaccagagacttctagaagcccttctccacaaagttctccaggggtctatgttcttctagctgcttttggacctcctgaggattgccttgttcacatgggtgaaacagaatcacagcctgcaggaaggggaaagaaaatattgtgacttagaagcttccttttaagcaatgacagaatgaaagttgcatataacactttggctcacattctatgttaagctaaaacttgggagattct

SEQ ID NO: 115 - DNA, 1001 bp, Homo sapiens
acagcagcaatataaaactacttagaaataaataaaacatagccatgccaaataaagcataggaaaacttctccctcctgagacccaaaaatagactcgaataaatggaaggacagcctttgttcttgcatagaacaattcaacattatgaagatgttccctcctaagatttataaacaatgcaatctcaataaaaataacaagcttctttatgaaactagactaaggggtggcaaactatggcccacaggccaattctggcctgccacctgtttttttcaaataaaattttactgaaatagggtcatacttattcattaatgtattgaaaggcagaattgagtagtcacaatagagaccagatagccaccaaagcctaaatacaatactttctggccctttaaagaaaaatctccaatgcctaagctgtacagttgctactcaagttcactttgaaaagaccaacaaggacagccatgaagcaatgaaaagacagactaygaagggtaactaaacccatgagacattaaaataaactttaaagcttctaatattaaaacaacagagttccaaaacacaattagataaagggacaaatagaaaaggaaatccagaaataaacacatatagaaatttagtatacaataaagatgacatctcaaatcaccagggcaaaaatggactttttaataaatgatggtaaaacatcaaggtagccacatgaaaataggtacaatttggtctacacttcataccacacaccaatataaactcccaattggttagggttctaaatgtatacatggaaatgataagatactacaagaaaactaaagtaaattctacattaatcttagggtaccaaaaattttctatctgtaagactgatcatttgactaaaaataaaaactttttttaaagttttcttttatatatacatacatatgtgtgtgtgtgtgtgtgtgtgtgtgtgtgtgtgtgtgtatatatatatatatata

SEQ ID NO: 116 - DNA, 1072 bp, Homo sapiens
ccgagggcaccaaggccgtcaccaagtataccagctccaagtgagcctctcgctgcagtaacagttccgccgtgacccacaccccaaaggctcttttcagagccgtccacgtttctcaagaaagagccagttcactgttaagtttgtctcccattaggtaccctttgggactcgcttcgtacatataaatgtacttgtatrtgtgggtttttttttgttttttgttgttgtttttgaggtgtagtctcactttgttgcccaccctggagtgcaatggcacgatctcggttcactgcaatctccaccttccgggttcaagcgattcttctgcctcagcctctcgagtaggtgggaccacaggcatgtggcaccaggccctgctactttttgtatttttagtagatacggggtttcaccacgttggccagactggtatcgaactcctgaccttaggtggtccacttgcctcggcctcccagtgttgggatcacaggtgtgagccactgcgcccggcccaaaatattttaaagaggattattagcaactatgagtgaccgtggcttagggaagacacaatcccccgagaccatgagaaagtggttctgaggcagtcagaatgcaactgttttgtacattttagggaagcagaagttataggtaaagtcataaataaatatgtggagggttagtccaggcgtggtggctcacgcctgtaatcccagcactctgggagtcagaggcgggcggatcacttgagatcaggagtttgagactagcctggccaacgtggtgaaaccccgtctgtactaaaaatacaaaaaattaaacgggtgcagtggcacgtgcctgtaacaccagcttctcgggaggctgaggcaggagaatcgcttgaacccgggaggcagaggttgcagtgaaccgagtcgtgatcgcgccactgcactaacctgggcaacagagcaagactctgtctcaaaaaaaatcaggtaaatcaaagaaaatgaactggaaaaaataattgctcttaatatcactgtgaatacctagtgagtgttctgtagatgtgttacag

SEQ ID NO: 117 - DNA, 2784 bp, Homo sapiens
tgataaggtatatgacaaataagtcctaggaattattgaattatttcctctgaagaaataattcaaaatttatagtggaaaaatcatcaaagaaattaaatgctacagtataaaatatttgcttaatgcaaaaatggaatataggaggaatggaagaaccaaaaaggcatgagacatacagaaaataaaaagttaaataccagacaaatccaaatatatcagtaataataatgttatatgtaaatatattaagcaattgaatcaaaaggcagagactgtcagggtggataaagaaacagtattcagctatcttttgtctagagaagacaccatttacatttaaagatacaagtaaattgaaagtaaaaggatggaaaacatatgtcatgcaaacttcatccaaaaaaagctgtaatgactatacgagtagwcaaagtagactttaaaacaaataatgttactagggacaaataaggacagaaagggctaatccatcaggaagatatcacaattataaacatctatgcaattaataagagcaccaaaatacataacgacaaaagtgacagaaatgaagagaaaaatagacaatgcaaaaataatagttggagtcctcagtgccccactttcagtaatgaatagaacaactaagaaatagatcagtagggaaatacaagacttgaagaatgctataaaccaactagacctaacaaatatttatagaatctccattaaacagcagcagaatgtacattcttctcaagagcatatggaacattctctgagatagatcctatgctaggtcataaaacaaatccaaataaattgaaaaggatagaaataatgcaaagtatgtttgtctgatcacaatggaatgaaatcagaaatcaaacacagagagaaatttaaaaatccacaaataagtggaaattaaatttctaaatagccagtgggttaaagaagaaatattaagataaattagaaaatatttgagataaatgaaaataaagaaacgacataccaaaacttatgggattcaggtaaattagtgtttagaggaaaatttatagctataaatgcccatattaaaaaagaagaaaaatatcaaatgagtaaactaagtttttaccttaagacactggaaaaagaccaaactaaacagaagcaaaattcaggataacagtgaaattaatgaagttaataatagaaaaatgtcaagaaaatcaatgaaatgaaaaactagctcttcaaaaagatcaataaaattaacaaacctttagatagagtgaccaagaaaaaaagagaactgaaattattggaatccaaaatgaaagagtgaacattactactaaccatatagaaataaaaagactgtaaaggacagctgcgaaaaactgtatgccaaaacattagataacttagatggaatagacaaatccctgtaatgatgctaactactgaaactgactcaagaagaaatagacaatctgactagacctgtaataagtaaagagataaattagtaataaaaaaactatatacaaataaatgtccagacttagatggcttcagtgttgaattctaccaaacacttaaaagaattaataccaactcttcacaaactcttccaaaaaacagaagaggaggaaacacttctcaactcattctacaaggccagtaccagtatccttataccaaaaccaggcaaagccatcacaagaaaagaaaactacagaccaatatttcttatgaatacagacataaaaatactcaacaaaacaccagcaagatgaatccaacaacatataaaaagaactagatatcattaccaagtgggatttatcccagaagtgcaagattgttttaaattctgaaaatcagttaatatgatacaccatgtcaacagaataaaaaacaaaaaccacatgaccatctcaaaagatctctttcatgttaaaaagtctcaacaaactagaaatagaagggaatttcttcaaccctaaaaatgcacctacaattgcatggaacccttgaaaaactagaacaaagttgaaagactcacacttcctgatttcaaaatttactatagagcaacagtaattaaaacaatgttgtactgccataagcataaacatatagatgaatggaatctacagttgagaggccagaaataaacccatatgtctatggccaactgactttttccaagagtctgagactattcagtaggaaaagaatagtctttccaacaaatggtgccgggacaaattgacagacatgtgcaaatgaataaagtttgacacttacctcacaccatatacaaaaattgactcaatggattaaagagctaaatataagagctaaaactataaaacccaatatttgggaaaccactgccttatagaaagcttatacatttgtactacaaggcaaatacatgaatgtttatagcagtattatttagaatataaaaaatctggaaggtatctgaatgtgtattcacaaaaacgaacaccagagaatttaattgtgatatacctgcgcaggggaatacaataccacaacgtaaactgaatggtctccaggtacattcaataacatggatgaatatcacaaaccaaaagttgtgcaaaagaaggcaggcaaagaataaaaagacagtatatatataaagttcaaagactggaaaatacattttgtcttttgattcatacacatgaggtgtattagtatcaagtaaggaaaacagagatcacactgattattttaacaggattactagat

SEQ ID NO: 118 - DNA, 1001 bp, Homo sapiens
gcttcgaactccaaggctctagcggtccttccgcctcggcttcccaaagcggttctgtttaccggatggtgccaaacagttccaggctcttggtgcccggtagaaattggacgacacacacacagatagcaaagcaaagcagcaaaagtttagtaaacagagtattacactctcgggggtgggagagagcggactgacctctgcgaggtgagatcagcgtcagcttgctgtagtttgagtcattttatgtgtgtgcgtgcgtgtgtgtatgttttctgttcccagtgctgcctaatctatagccagcatctgcccttttattgataggtttgttgcttactttgtcctctgtggcttgtgcctctatcttataatcttaaatatatgcatgatatgtagcccatatgcatgaaccttaagtagctgattatcatacgggcttttgttaaggatacttttcctctctaatacgcatgcccatctctgaagagctgcctcttmaactggtttgttccagatcttgccggccacgaggtccttgctcacattatctcttttgtttcggctgcaaaaggttcactgcttgttatctcgcttcttgttcacccgcccatctaccttacttctgccctttgcttttacttattctgccctctaactttcagctccctttgttattctcttgcctcacttttcttattgtttcagctgtattgcaggcgcgagctgccgcgcctaaatttcttgatgtaccgtaaacatttcaatgtctactttctatctcaaaacaatgtggtgtaaaagccgtttagttttgcttcatctccatacagcattccagtgccattgcaaaatgactcgactatcagataaaactgaacacagctctacttggtgaaaaagtaggtggctctgaaaagaacctttttggtttggaccgaggtatgagtaatgaactgctccagccccgctacttgcccttggccttgtggtggctctca

SEQ ID NO: 119 - DNA, 1001 bp, Homo sapiens
aatagggctgaggactctaccctcagttttcaatctagagactgtgaaactgtagagaaacacactgtctagtagcaatccatatactttttctagtaagcatattaaaaaccgaatactatactatattccttacagcccagtgagtttcccagaatcataaataaaacccaccagtacctactatgtaactcccagtaagaggctttgacttttgtcaaagttgtgtcccagtaaaatgccttcaagataccacaaactggcctggcgcagtggctcacgcctgtaatcccagcactttgggaggcctaggcgggtggattacctgaggtcgagtcagagaccagcctggccaccaaggtaaaacccctgaaaacacgtgttagcaaacgtaccttgttagtatctacattaagaaaaaaaaaaaaaaaaaaaaccttgaaattcaggcaatgtaaacaggttaaagattaacaccgaaacatcatgagtgtactgtgkagtggtgaagcagctgaaaacggactcgtgtcatctttttatgattgttgaagtggctctgaaaagagcctttgtttttatgcgcttttcaactcggtctttacttagtcttgtggtggctctcagttttctttggcagcagcacggcctggatgttgggcaggacgccaccctgtgcgatggtgactttgcccagaagcttgttgagctcctcatcgttgcggatggccagctggaggtgacgcgggatgatgcgagtcttcttgttgtcgcgggccgcgttgccagccagctccaggatctcggcggtcaggtactccagcaccgccgccaggtacaccggcgctccagcaccgacccgctccgcatagttgcctttgcggagcaggcgatgcactcggcctacgggaaactgaagcccggcccgagaagagcgggtcttggccttggcgcgagctttgcctccctgcttaccacgcccagacatggcaaaaggtcta

SEQ ID NO: 120 - DNA, 1001 bp, Homo sapiens
tcactaccaaagtatatgactactactatagatattttattttatttattgattgatttgtagagatggggtttcattatgttgaccaggctggtcttgaattcctgggctccagggatcctcccatctcaacttcccaaattgcaaggattacaggcatgaaccactacttaaacttgtattcctttatgctttttttcatttgcaatattgactataatcaggaaaaaaaatatatcctttatgaagaagaaaaacttatgtctcattctaaggacagcagagaaattgttaactcagggaaaatgataataaaaatgataccccctctatagcaacataaagagcagtttcgaggagcaaaagatgtggtgaaatgcattgtttactctgggtgggtgcaagatccaggcaggggtgaagcatggccggctgcacagatctctgttctcttgtttcctttacatccctccccacctccctctgcagatcttgttctcrgaggccattcccagacccacagcaagagggattatggctgcaggcctcatgctcctttgttttggaagaaactgttgaggagttagtatttactgagcagctaatatgttcccgtcactattgtaactcataataattattgttaagtaatacacgaaaagttttaaatttaaagcattccaatattttaaaagtaaagggaacaaaaggccaagtgtcccttcactcactaacctctgatcttcagattagcatgcgtcttttttgagtttttcaggcatttacataaatagttatgcagaaatggatagctttgcttctgttcttcaattgaatctttagtatagttgtgcaaggtgttttttgatcacttagtgtgtctccgttatctaggttcatgacaacaaatcaactctttttacctgctgcattgaattccctccgagggatgagccgtcattcctctaagcagtctcctgatgggtggctggttcagttgg

SEQ ID NO: 121 - DNA, 1001 bp, Homo sapiens
ggggatggtgtagactgtgccaagttgaagacccatgtagggaagaggccaggagggtccctagtaagcctgacataagggtgtaccaataggtggccagaaatgcctttctgctcttaagagaacactaatactttgtgtatagcctgccgtgggagggatttcaggtgggtgggagagcacagaacccaattgcccactcccagtgagcacttttcatcttatgattcagcccctctgcccataagcaccacagaatccaagctttaccagataccatggcacatggacctttcctctttaggtgaatttcaaaattgccactgtcaacttgggacaaaatagcaaattgtcacagccagacatattaacttggggaatggaggaaatcattttaacacaatagaaaagtagactgaataagtaagaataaatacagatgggagaggtctgcagaatgcccggagtctggagcatttcttgtacctacagaagtgataygtgaagacatcagacccatgttgttgaagcaaaactggatgggaatagttactccctacatttgcccacagacccctcaggcaacaggttttcttttggggacatttattctccttcttcattttttgaagggtgcccttgttagtcatttaagtcagttgtgatctggtaaaaggaacacataggaccaatgaagagaccctttatcctccaggacagtgtgaagggaaagactcaccttagttgatccaccggggagaggaggagcaggacataaagcctttgtgctggtttaagccaagttggaaagtttctaagtaaagaaaatcccagagatcataggtcttcatttggggttttgttttgttttgttttgagatgatgtcttgctctgtcacccaggctggagtgccatggcacaatctgggctcactgcaacctctgcctcccgggttcaagcaattctcgtgcctcagcctcctgagtagctgggattacag

SEQ ID NO: 122 - DNA, 1001 bp, Homo sapiens
aaagacattcctagaagtcatccttcagtgatatcaccacttgctcagtcaccatctcaaccttatgtcacctcagccctcatctcaatgcccaaaccccttacacacaccttcagttagcttcaactgcctccgtttccacactgtgcacctttcactttccctacccagctttcctacatgctgcctctcctcagggtcccctgaatgctgcatcattgtgttcagtgcagctggactgattgcacctgtgtatttgcccctgagcactttcctttacacatgtggcttgtcttgccaatagactccaggcttataccttccatttccatcgtattctccagtttccaggatagacgttgctcatcgtctttacctaataaataagtttgtctgattgctgaaagcaacctcttaacctttcttttttaatatcaactgaaacaaaataaaacatagggcaagaaacctgcatgggaatgcagctgtctaaagctttghcattgtatgtggtctaagacccatccctaggcctgatggcagtgggctcaccagggcaggtgcacatgggggctgatgcctcatgagggaacaactgcttaccagggtcttcaagcaggaatacagaatctcaactcaggaacaattttttattagtccatcctcatatttctgtaaagaaatacctgagactgggtaatttataaagataagaagtttaggccgggcacggtggctcatgcctgtaatcccagcactttggaaggccgaggcgggtggatcacgaggtcaggagtttgaaaccagcctgacaaacatggtgaaaccccgtctctactaaaaacacaaaaattagccgggtgtggtggcaggcacccgtaatcccagctgctcagaaggctgaggcaggagaatcacttgaacccgggaggcagaggttgcagtgagctgagatcgcgccactgcactccagcctgggtgacagagcaagactccattta

SEQ ID NO: 123 - DNA, 1001 bp, Homo sapiens
cattatggtctcgaactcctgacctcaggtgatccgtccgcctcggcctcccaaagagctgggattacaggcgtgagccgccgcccaaccactttttttagtattttaaatcaagtatctttttgtttgtttgtttcttctgtgcctatgcttacccagacagtttcttcatttattttcccccgccttgggcaggcttccactcttcagaccctttcctgcacaactttgtccctgagcataggtcctggacgtaaaagaagggacatcgtctggagaaatattgaattaagaaaggcgcggctgtgaagaatagaaatcagtgtctcccttagtctctcagttcggcgatcttggtaatgccctgtcccatgcctgctaacgcgattcagcctcgatatccccgtccagtcccacgatcgcaccaagaagagcttgcgagccttcctgctacatactgacattaagaaaccggacttgaaagggatcccagacaaacgwtaaacatgcaacaagagggatagggtgtaaggaagagaatccttggggcggtgtctgataaaacagatggctctcctttccaggtgtttctgaatttgatccccgacgcctggggcatcgtggaggaacttgcataggaaatcaaggtgtcgcaggaaagagaacacgcacaagcaaaagataccttaatttgtagtatactcaatatttatcgtacagaagtgtatcgacgatagacaatgtgcgatgtgatgggtgctgggaacttaacgaactctccacgcgcctagacctcattggatccactttctcttgggctgtgagccggtaaaaaaaaaaggggtggatgtggaggacggtccaaaggattcggagctccttaaaatgctactcaaactttatttagcgcgctggagaatccctgagaaggagtattatacccagttttccgggacttacctccagtgattctacgtcgattctttgatgaggcccattaa

SEQ ID NO: 124 - DNA, 1001 bp, Homo sapiens
gaaaaatttgaacaggcgcttcacaaagacggccaaatggcaactgaacaatttgcaatcagaaaaaaaaaaagaaagaaagaaagagggaagagggtctaaacaagcaaataaacgaaaaacgagaggcgaggctaccaggtttcttccatttctggcaaacatttattgttgttgttttttccttcacagaattattttcagaaaccttccacaggagattcgtgcgtggagggggtggggtggaaagaagtagggaatggagaagattactaagaaaagtttcctgtctggaactgcggcagatctctttggatagagatgactacttaacctcactctgctttccttcgccgcggttgcggccgcgaccctgttcttaccaccagcaattcctccagggacttggtcagcagcccaacttgatctgcgtctctctgctaaggtgtttccgcaacagggtcaactccaagtctcacctttctaggaatcccgggcgcmgcgcgggggtcgggactccgacctgtatttccaggcggaggtttccctgggtcaggcggccactctctgccagagattgtcagttatccaactgtcaatagagccgccgctccagcgagtttaatttaggcacagaaaagtcctgcctgggttgaggtgggcttaggatgagtttacttgagtgtgtgatttagaaatagatctatgggacagacagacacgaaatcgggcattggggccctcgcaggcagggtatctagactggcagctgccggtgcaggatattgccaaggactcggcatccggctcagctcaaggtggggacgaagacgtcctggttgcaaggaggagccctactccccccggaatcagaactgtgcatagcgggctctggatttgccgggatgtttgaggaatttgaaatgagaaaggagaggaggaaatggtttaatggtatattgagttactggagtgtattttagtcaccgattttggtttta

SEQ ID NO: 125 - DNA, 1001 bp, Homo sapiens
tttgatcctcttaccggccacatgaggagaattagttctttaccacttttgttgatcacatctcctgtgaattctgcttccagtttctccgaaagtaagctctatatcgccactactgaactggaaacacagtctttcaaaagaagaaatgtgggcgagggcggtggctcacgcccgtaatcccagccctttgggagaccgaggtgggcggatcacttcagttcaggagttcgagaccagcctagctaacatggtaaaatctccgtctctactagaaatacaaaaattagccgggcgtggttgcgagcgcctgtaatcccagctactcgggaggctgagacaggagaatcgcttgaacccgcgggggggagtggggggggggcggcgcgcagaggttgcagaaagccaacatcgtgccactgcactccagcctagctgataagagcgaaaaaaaaaaaaaaaaaaaaaaagaagaggtaacatgtgagagctaagacggargccttcatttttgtttttaagtaaaattgagtaaggtaaggcgtgtgtgctaagggaaggggaactagcgttaaacaatttccagttttgttttagacaaaactttctgaaacatcgtttcacattaaacttgtgaaagacaaaaaaagattctatttgctgtggctggttagctcaactggttagaattcggtcatagattcccgtttgtccctgcctaagaacactttgtggtctcgcaagtcctctccaagatttaacaacgtccccaataaatctgtagaatccgatggctgttccctcacagtttaggtctttgcttttatttccatcttcatacatagaaaattggcctatgtgaattgtctccatctgagaagaaattgtaaagccatctgcacttccaatcacttccacacttgggttttcaccggatcacatgaaataggatttttaaatgacatatgtgaacaattttcattaacatcaacacactagga

SEQ ID NO: 126 - DNA, 1001 bp, Homo sapiens
ggtgcaagcatgcatgtcctgttgcttcgctgcgcgaggctgaggcacgagttgctggattttgggggtggggagtgcggtgcttggctcctggctggtgaatcagtctgtgaggatgctggggtgggcgggcggaggggatatggggagagtgggtagcgcagtgtgtctggtggttctttagttctcggattgttactatttgtgttcttatcccggctctgttcacctctctttccggacctgtttactggtttgttacatgaatacaacctgagtaaaagtctcgtcagcttttctacaaaactgaacataactctttagcattgctgcctaggtcaagaaactatttgatcaaccgcccctcttctttccaccctcaattttacattgaggctgaggacttgtgccggttttaagcagcgttcagggctggccagattaaggagtggacaattaaggaaagaattgagttagctagaggaaagggtgcgatttacrgttcccttcctcctgggcaaaaactcttcaggtgggactcccactggcagatgtgaagaacgttgcgggcagtgggaggtgcttttgagtgagtgctgcataggcgtcctggacgggtctttgtctttggcgcgcagaccggttcgtgagacgcaagaagaaggcagcagcagctgccggaggaaaaaagcggtcctacaccaaggactacaccgagggatgggtggagttccgtgacaagcgcatagccaagcgcgtggcggccagtctacacaacacgcctatgggtgcccgcaggcgcagccccttccgttatgatctttggaacctcaaggtgagaagatagatctttctgccacacctctcaccctcccttctccccaactctggcccaagtatccccatggcctctcattggccttgtccccttgtctcatctttctccctaatctgcactatcctgatcttttcttcttttctgcccacagtacttgcaccgt

SEQ ID NO: 127 - DNA, 1399 bp, Homo sapiens
tccctcatgatctgtttcctctgatttcaacaagcaggtgttctttctcctgtctcaggctaattctgcacccacatcggggagcccccaccccagcttccctcaggcttctctatttggtcaattcattaattcattcatttgacaaggatccatgaacgctaactatgtgccagtcactattctaggtggtggagtcayagaagtgaacaaaacagaaagttctcattcaaaaacaacataacttgtggtaggaggcagacaggaaatgaaataattagtaatatatatggtgtgctggatgatgataagtgctcaggagagaaataaacctggaatagcagaacttgcatttctttttgaaggggtcttgctctgttgttcaggctagagtacattggagtgatcatagctcactgcagcctaattttttttttttttgaaagacagagatcttgctatgcatactgcccaggttcttgaactcctggcctcatgcaattctcctccctcgatctttcaaggtcctgtgattacacctgtaagccctcgttcccggttggaagttacagtttaaaatagggtggttatgagcaaggggagcgaggcacagaatacttgggagaaaagcattccgagttgagagaacagcagtgccagagcacagaggcagaagcactgtggtttgtgtgaagaaaagcaatgaggctggggtgcgcagagcacacagggtgatcaggagaagaggaggtgacaaggccagagggggttgagggccagatcatgtatggccttgaaagtcatcatgctgacctgggctttacctctgagaggggagccactggaaggttagagcagaaaaaggactggactgacttatgttttaagaagttacttcacatgctagaccaagatgggctgtgggtaggggtggtggatggaggcctgaagacccagctgggagctactgcagtgatccaggggaaagatgcagatgacttgtaccagggaggagccatgaaaatgttatgatgctggatttattttcaagatagaataaaaaggctttgctgataaacttacaggtggggtgtgaaaaaggagggcatcaagggtgaccacaaggttttggtcctaagaaacggtacagatggagttgccacttactgagatggggaaaatgagggagaaaccgcttgtggaggccagaggaggagccagcacagaatccaaaggtcagttttgaatatgttgggtttgaggagcttactagagattcccgtggagatgtagagtaggcaggtcaataataagcttgcagtccaggcaacgggtcagggctggaaacacaagttattctctttgtcttctttatattcatgtttgttgccactgtgtg

SEQ ID NO: 128 - DNA, 1001 bp, Homo sapiens
tgagaaacagcttaatggtgtcttgtgataaaattgttaaattttcacgaagtcaaatttatttcaattttgtttacttatttttgtatctccctatgaaatctttgtttccccaaggtcatggaaatagcctatgctccacgacccccccccccacttacataatcatttaccttttatttatttatttttattttatttatttttttgagccatcttggctcaccacaacctccatctcccaggttcaaacaattctcctacctcagcctcccgagtagctgggattacaggctcccgccacaacaccccgctaattttgtatttttattagagaccgggttactccatgttggtcaggctggtctcgaactcccgacctcaggtgatccccctgcctcggcctcccaaaaccctgggattacaggcgtgagccactgtgcctggccacatcatttaccttttatttttaggaatatgatcaaaagacctgaacaggcrcttccaaaatagaatatgtcaatggccagtaagcacataagcagatgttgtgatatcaataaaaagtttgcttatttattttaaccagtggtgaccagacaaaagacctcaactgtctctggaaactttattttatttccagaaatcttttcaaaactcttctgtgaaggttgtgtttgtctgggggaggggtgaagttgtggtttgggatgagttgcagatgaaggagataagacaaggtttctgccttcaggatcttcaggaatatgtgtcctttaatcagactgcttaacttgatttggctgatccccctttctttttcagttccctccatccctctaatccccatcacctaaaaagacctccagagacttagttcatagctgggcttgatctatatctctttgctccagacatttctgctctgtgtcaatgccagcctgcatctatctgggatgttgggtggggtagtagagtgggatcggtctctctagccataa

SEQ ID NO: 129 - DNA, 1001 bp, Homo sapiens
aagaagctcctgaaatttttatgttagttttgtctttttattttcctccttcttcttcttcctctttttcttcttcctcttcttcttcttcacaccactatacaaaggaggaagtttagttttgtcttttactttaaattacacaagatttttttttctttctctctctgtctctttattattttaaattgtttgtagagatggagtctcgctcgaactccttagttggctcaagtgatcttcctgcattggcctcccaaagtgctgggattacaggtgtgagccaccgtacccagctgattttctctttaacctggcaatgactcttgtttctgttttattatagaatggaaactggctcgatcttgtgcaggttagtggctgggcactgctctgggtgctgagatttaacctctgaggtatccaaagacctaaaataagtggaaatgaaaaatgctgatacccttttagtgatgaacacagagattttaagttgtgggraaaaaaaaaagaaagaaagcctaatacttccttggaacacagagaggggctttggaagatggccaagagtccagcttcctgtgagattatctcacgaggcattacaagcctgggcacagtcaactcttaacatcaccctctggctgctggtgacagagggagcctgggggaatggagaccccttagcaggccaaacagccctccccctgaggagacctatcaactcctacagcagtgctctgtttcttagaagcaaaaatagtcctgtaaccataacactcaccaatggtcagactttttgtttctgtctttctctccagttgaagtgactctggacccaaacatagccctccctcacctctttctttattaggattcaaatctgtttgactggaagattcatgtcagaaactgcctgaaaaaccagagagatgtgactcctggccctgtgtgctaggcctggaagccttcacctcggagagacattaccaggaagtgga

SEQ ID NO: 130 - DNA, 1001 bp, Homo sapiens
cacccttctatgcatcctcaagcctaatctttcctggttatgtgacaagaacccggtttttagctgaactaaggagaaagtcctacaacactgccaccatgtggcaattactccaaatagaaggagaggctgaaggacacacaaccaggatgcagagaaaaagatggagacagagtctgtgcaagatgggattgatactgagactgggttagccacctctcctagacagtgaaacagatcgcaagagaggctgacccagaaagacacatgcaaaacaatgggcaatagaacacatgacctgaattagattatctgggttcaaatcctgattttgctattcattatctgtgtatcactgggcaatttactcaatctctctgtgcctgaatatcctcattcaaaatcagggatgaaaagagtacttatctcaaagggctatttgctcacttattgcacaagtaatttggcatctgatatgaaccaggtgcacctctagatgargatactgtcacattgaatgaagaccagtgaccagaagcctgcctcacagcccagctcagtgagaaaaataattccattctcacctctaatctcaaccctgtgtcaccatttatgtatagtcctttgcattagtgtctggaaaggtcattttttgagggcagaatgaataacctatagaaggatcattcttgggtataatgaattaaagaagtattatgaagctttataaggcaggattagctcataaaaatggagggttcttttgcttttccagtcccatttgttgtttcacagacaaagaataaaacaatcactgatggcaaagactgcaaactgccaacgttcatcggtagagcaaggtgacgctcgtcctgtccaggcctgtggttgggataagctcagaaagcagagtctccagggctggtcatcatctatcataaccctgcgtataaagaaagccttgagaaagaaaagaagtgacttattatgtgtcttctgac

SEQ ID NO: 131 - DNA, 1001 bp, Homo sapiens
ctgtggacactgctgaggaagcactgttaaacgcccttcttcccactgccatcatatctaagtcagcgtctcctaaagagcccgaacagctgctgaagcttttcattgtcattggagggttgaattttgtttttttcggttttgtttttgttttttttgagacgagtctctttctgtcgccaagctggaggagtgcagtggcgcaatctgggatcgctgcaacctccgcctcctgagttcaagtgattctcctgcctcagcctcccaagtagctgggactacaggcgggcaccaccacgcctggctaagtgtgtgtgtgtgtgtgtgtgtgtctgtgtgtgtgtagtacagacgtggtttcactatgttgtccaggttggcctcccagagtgctaggattacaggcatgagccactgcacctggccaggagggttgagctttgaaacaactgatgagagcctgaggagccattttgagcaatagggaacgctcacggactrtgtagtaaagaaagatccaaacaccaagcactccaggggctttgggtttgtcacatatgccggtatggaaaaggtggatacagccatgaatgcaaggccgcacaaggtggatggaagatttgtggaaccaaagacagctgtttcaagagaagattctcaaagaccaggtgcccacttaactgtgataaagatgttaaagaagaactgaagaacataaactaagagattatattgaacagtatggaaaaattgaagtgattgagatcatgactgaccgaggcagtggcaagaacaggggctttgccttgtaacttttgatgaccatgactccatggaaaggattgtcattcagaaataccacactgtgaatggccacaactgtgactttaggagtgctctgtcaaagcaaaagatgtttagtgcttcatccagccaaagagatcgaagtggttctggaaactttggtggtggcgttggaggtggttttggtgagaatgaca

SEQ ID NO: 132 - DNA, 1001 bp, Homo sapiens
ctaccttgacagctataaaaagtcgctctaaagaaaaagaaccagctctggccaggcgcagtggctcacacctgtaattccagcactttgggacaccaaggcaggtggatcacttgaggtcaggagtttgagaccaagcctggccaacatggtgaaaccctgtctctactaaaaatacaaaaattagtggagtgtggtggtgctcgcctatagtcccagctctcaggaggctgaggcagaattgcttgaatcagggaggcggaggttgtggtgagtcaagattgcaccactgcactccagcctgggtgacagagtgagaaagaaaagaaaagaaggaaagaaaagacaggaaaaccagttatttccactgttttcacagaacaaatcaacagactgaagtttactcgtgtcaacagtgtgtgaggttacaatgtgatacttactattcttgagatggaaatgttcagaaaagaagccacataaagcacatggtggaagagmaaaaatgcaaaacaggcttaaagaactgtgagagtttagaaaaaagcaatagatcaaagggatcaagaatgggcattagaagatgaaactgaagacagaatagggagtagggggttccaggcatggaaataggatattctgtatgaggaaaagagaagaacctctttagttgggcatgaaacatacattctaagtagaaataattttttttttcttgagatgacatctagctctgtcacccaggctggagtgcaatggcacaatcttggttcactgcaacctccgcctcccaggttcaagcgattctcctgcctcagcctccaagtagctgggattacaggtgcccgccaccacgccctgctaatttttgtatttttagtagagacggggtttcactgtgttggccaggctggtctctaactcctgacctcgtgatccgcctgccttggcctcccaaagtgctgggattaccggcatgagccaccgtgcctggcccggta

SEQ ID NO: 133 - DNA, 2091 bp, Homo sapiens
gtaagtaccattaacagcttctcttgaactggtttctctaaaaattcctcctttacctttcttctaaagtgtcggatcctttacctttcaaaaacgaggaataggtctcgtggctcatgcctagcgagacctcatctccacaaaaaataataataaaaaaattagccaggtgtggtggtgtgggcctgtagtcctagttactggggaggctgaggtaggaggatcacttaagcccaggaggtcaaggttatagtgagttatgatcgtgccactgcactgcagcctaggtgacagagcaagaccctgttccccaccctctgcaaaaacaaacaaacaaaaaagcatcctgataaacatagacatgaaattgaaacatacaggtgaagggtcacagatttatgcctcagtcttctcatctgtaagacaaagacagcctcatcacttttaatgaggtgagygaatgagggaggagaccacccctcatattgtcttatgcccgatttctgcctccaaagaaagaagaagtaaaaactaaaaagcagaaatgaaatccacaggcagacagcccggcgccacgccctgggcctggtagttaaagattaacccctgacctaacactggttatgttatctatagtttccagacattgtatggaaaagcattgtaaaaatccctgtcctgttctgttccgttctgattactggtgcatgcagcccccaaacatgcaccccctgcttgctcagttgatcacgaccctctcatgtggacccccttagagttgtgagcccttaaaagggacaggaattgctcactcagggagctcggttcttgagacagaagtcttgccgatgctccaggccaaataaaccccttccttctttaactcggtgtctgaggggttttgtctgcggctcttcctgctgcacattaagtgaggtacaccactgcatattacatggcaggtgctcagtctcctccttccacttcctcactggttttctagtgaagagagaatgaaggggtgggttgcccctccacacctgtgggtgtttctcgtaaggtggaacgagagacttggaaaagaaaaagacacagagacaaagtatagagaaagaaataaggggacccgggggaccagcgttcagcatatggaggatcccaccagcctctgagttcccttagtatttattgatcattcgtgggtgtttctccgagagggggatgtgtcagggtcacaagacaattgtggggagagggtcagcagacaaacacgtgaacaaaggtctttgcatcatagacaaggtaaaggattaagtgctgtgcttttagatatgcatacacataaacatctcaatgctttacaaagcagtattgctgcccgcatgtcccacctccagccctaacgcggtttttccctatctcagtagatggaacgtacaatcgggttttataccgagacattccattgcccagggacggacaggagacagatgccttgctcttgtctcaactgcaagaggcatgccttcctcttatactaatcctcctcagcacagaccctttacaggtgtcgggctgggggacggtcaggtctttcccttcccaagaggccatatttcagactatcacatggggagaaaccttggacaatacctggctttcctaggcagaggtccctgcggccttctgcagtgtttgtgtccctgggtacttgagattagggagtggtgatgacgcttaacgagcatgctgccttcaagcatctgtttaacaaagcacatcttgcaccgcccttaatccatttaaccctgagtttgacacagcacatgtttcagagagcacggggttgggagtaagttcatagattaacagaatctcaaggcagaagaatttgtcttagtacagaacaaaatggagtctcctatgtctacttctttctacacagacacagtaacaatctgatctctcttgcttttccccacagagaaggcccatgcaacacagacctaaacccctttgagaggaaaatagggcatttggtggaggggaggggaggagtcctggcttgcggctataaaaatgtttttccac

SEQ ID NO: 134 - DNA, 1001 bp, Homo sapiens
cctctttccctgttttattattatttttctccaatcgcttatcactattattttgtttatttaatgctttattatccgcttccgccactgccatgtaatcttgagggcaagggtctctcatgttttcttcaccgttatctgcagtgccttgaacactaatactggttgaatgaacgaacgcattaatggagcggtgatattggggcagagaggatgcagggcttgcttttcaccgccatttttcagccggcagagacagaccgagaaaggaatgaaggccacggggcgtgtgcagaagtagctaccagagagtccatgcgctgcgagcctggaccagcgggcaaacgcggcttacaggcgttcacccagatattacgggtacaacctagtttcttatgaaatacctcgcccctaaggtacgcgcagggccagtggcgcaatggataacgcgtctgactacggatcagaagattccaggttcgactcctggctggctcggtrtaagcagggtcgttttacaactttctgactccgcaggagtaaggaaattcctgcaagataaatttgcctggaagactcagaagcaagaggggcagctcccgacaacatatggggttatcatttctttgcggagcattctgccactgaccacgtggtaacgccaactacgccagagaaacgctcgccctacccaagttgtgcccagccttgcctggccattttggccgaagaacgaaggaccgttcagagattaaattaaagtctctattgtgttcttccctattcagtcatttgtagaataaattctatggcttcagtttgaacactggaggggctgggtctgagcttttcattggtttttctggtttgagaggtcggtacagagacgcacgcgcacatcagcaaaacacgcacttggaacgaagaaacacggaactaggcaggaagaactatttactctgaaaaataagcccttagtgggtttccgtagtgtagtggtt

SEQ ID NO: 135 - DNA, 1001 bp, Homo sapiens
cgcggggagaccccaatggatttcaagtccatcgccttaaccactcggccacgactacgtacctccttcaacaacctggatatattcccatgaggaatatatgtttcttttcacagacatctttaaatttgtttattttgacaaggtaacaactctggaatgtctctcatcctggttaaaaaacaaaatcaaaattttaaagatttagatattggctaaaagagatattgcaaattgcaagacttgtctgatgtaggaagtacgaaagactttacgagggggccacacgccaacccctaaatggtctccaaacctacgaaactggctgaaagctctccacacctaattagtaggattacagatattgaagcctacaaatgcgcatttccaccaggataccttgtggattcttacacgggtcaggtccgctgacgtttagcacgcctactttaaaacctcttttctgtagggtcctagtcttcaagtaaaatatatgcggcyatatagcagaggatggtttcgatccatcgacctctgggttatgggcccagcacgcttccgctgcgccactctgctgtctcgacagtccgctccgccactctgctgtttcaacattactcttgtcaagtatgtattagaggctacaattttcggcatcttcctaattttaaatgatttgttgtcgtttgccaaattatcctggagaatgagaagtgcacactggccatccatatggggctgcacgccacttccaaacaccagcggtttagaattcttcctcgataaattcgaatcagctgaggttgaagttctctaaaacggaagcatgtttcgagttatgggaaaacaaagtgcaggctaattggcataatttataaaggtgaaattataaatgcttgggcaaatttcagccattcctggataccggagggagtcgttattacttccaaacattttttacttgagattttcatcgaaaatgttcacaggaaaaaaaaaat

SEQ ID NO: 136 - DNA, 1256 bp, Homo sapiens
ctgttaggctttctccaacagcagaaggctctgtgatctccatctcttgggaggcagaaaattaccacaagaaaatagccgggaggcagcggattgaaccctggaaacggcccgctctttgtgctgggcggtgctcgaagggaagaaactgagggcccgggagtcgagtgtgtccagttgtctgccaggcaggataaggactgggaaaaatgaaaaaaaaattcctagacatacacaacctaccaagcctgaatcatgaagacacagaaaatatgaacataccaatagtagataaggaaattgaatcagcaataaaaacatctcccatcaaagaaaagcccaggacctgtagcgtctctagtgaattctaccaactatttaaagaactaataacatttattatggaaaacagtattgtggttcctcaaaaaattaaaaatagagataccatatgatccagcaaactctctagtgggtatatagctaaaggaagtgaaatcagtatgtccaagagattatctgcataccaccaagatatggaattcttcttyttttttttttttggtggcacagaatctctctctgtcgcccagggtgcgattttgactcactgcaacctctgtctcccgggctcaaacgattcttgtgcctcagtctcccgagtagctgggattacaagcctatgccaatataccccgctgatttttttttttttttgtatttttagtaggggcgcgttttcaccatgttgcccaggctggtcttgaacttctgggctctcctcggcctcccaaagtgctgggattgcaggcgtgagcaacggcgcccagccaagatatggaattcttgtgttcaccaatggatgaatggatagagaaatgcgtttagcttccctgtgccttggaagtatcatttccaatttatcatgggtgtgtacatttttattggtgtacttgtgagctcatcactaatttttgcagtctgttaatctaccatagtttcagtttcattgtattttcttatatatttatattgtgtactgatgtgtgcatggattagtaatgagtactctattatttttaatgtcataattattcattatttatttattatttattaaaaataatatttaatattaaatattatttattacttatattatttattattataataatttataatatgtcacattataaaatattatttaattaaaatttaatgtcactctattattttaatatcataaaatacat

SEQ ID NO: 137 - DNA, 7021 bp, Homo sapiens
ctaatagagtcctccctctgatcagtggcaaagagtagccattatcattttttaatggtaataatatttattactttttaaacttattttttaatggtaataacatttatattatactgggtgtctgtatattgagttgccattccaaaggactatataaaaaatatatatctaaatgcttgacaaaaaaaaaatgcaatttttttggaaaggaatatatttggtggctgcctcatgcagcttaagtgtccaaaatctgatagattggtgtatcccagtggtagttttctgttgccacaaactccaatcagcaggaatgggggttgtaactcctgtacaatagttctaccttatccacagttctgttttctgcagtttgagttgctcctggtcaaccttggtctgaaaatattaaatgaaaaacttcagaaataaacatttcatatgttttaagttgcaactgactctgggtaggataatgaaataccaccctgtccaggatatgaatcatccctttgtcctgcttatccaagctgtgtatgctaactgcccattagtcattgacatcatctgcccctgacatccaaccacagacgttatcatggctcagtgatccaggatcacccaggcagatgatcctccttctgatgtatcatgaggtcaacagtagcctaacgttccatcacagtgcctacttcactcatctcgcttcatctcaccacttaggcattttatcacctcatcatcataagaagaagggggagtacagcacaagacgatattttgagagagagaccccattcacataacttttattacagtgtattgttataattgttctattttaagctagtgttgttaatctcttactatgcttaatttataaattcaactttaccataggtatgtctgtgataaacattgtatatatagtgtttgacacatccatagtttcaggcatccactgagggtcttggaacatgtcccccaaggataagtggggactactctagtgccatcaggctagcaggctgtaaaggttttaatggcagtccctggaccatggcttatttaattgcttccaaggcccactgctacaaagggcctcattcaaagctggtggctttgttggtcaccctgacttaggggaccaaaagaacactcaggtggggtacatgttgcctccaatgcccaagtacccaaagaggccttccagctgttgggcctcctttttattagtggatgtctccaaaattaaatttttttgcttggttgtatctagaatacttttctggcttactgcccatgtggccttcgcatttagcccagggacagtccactgttagtctccacatccgaaagcctttttgactagccaaactgagctgttacattatgacagggtagtttgtagcatttccatttgtaacaataattaacacaataatgtcctgttcttcagttagtatgcagtactgtttttttgaataacccactgggacttgggtggcttaggtggcagacaggcatggatatgccccgccgtaacggctggaattcttagctgtgagcgggcgcacccctcaggcagtgatgatgtgctgagccccaagcagccaaaatgtcaatgactataagacattcagccacaggaaccaaagtcaccggcacctcaaatggccagaggcaccccacagcagataagcaccataggtcactgcttttgtccccaagcctcttaatgtcaccagtttaatttttcccttaaggagacctggaaatattgtcacatgggttccaatatctaagaacaccagaaaaatatgaattcctttttccccctttttatcttttaaaggaatattattaattttaaaagcagggaccatgctaatcatctctatatcattccaatttcagtatatgtgctgctgaagcaagcatgtctttttttttttaatttttaaattttaaattttatgagcacatagtaagtggatatatttaataggtacgtgagacattttggtacaggacgcaatctgtaataatcacatcatggaaaatggggtatccatcctttcaagcatttatcctttgtgttaaaaacaatccaattatactcttagttattttaaaatgtacaattaagatattattgactatagtcttcctgttgtgctgtcaaacattaggtctttttcattcttctgtttttttttgtttttttttttgtttttttcttttttcagatggagttttgctcttgttgccctggctggagtgcaatggcatggtctcggctcactgcaacctgcgcctcccgggttcaagtgattctcctgtctcagcctcctgagtagctgggattataggcacacaccaccatgcctggctaacttttgtatttttagaagagacagggtttcaccatgttggccaggctgatcttcaactactgacctcaggtgatccacccgcctcagcctctcaaagtattgggattacaggcacgagccaccacatccggccctttttcattaaccatccccacctcctctcccgcttcctcccacttccactacccttccaagcctctggtaaccatccttatattctcttatctccatgagttcaattgttttgatttttagatcctgcaaataactgagaacatccaaagtttgtctttctgttcctggcttattataagaactcctgttttatcttgacaggaatatagagtgactgacctccagtggggaggaaaccagagaccgtggccccattcccaactgggccattcagcctgagacatttggatttgatagaacctctttgatagaaccatggcttattgatgaagtggaaggagtgatacccgaagtacccagcccacggtgtagacatcaacctacaggggtgcggaagctggacacaccacccagcctgcacaagatttagctggctattctccatttttattctttggataatgagtttctgctctgtaaatgcccttatgaactgtgtttggttccctctcagatgcctcagggaccaccagaggacctcttcctcttccctctcagggttctcagggatcaactgagtatccatttcctgagttctctagctctcgggaatgaacaaccatacaagtgtccaacaatcagagggtggcttgccactgtcctattctatatttctttctctctgccccagtcagtgcagccagctcactcatatccgcagggttgggggtgacctatgtcctgtttacaaaaagagtcaaactgtaaaacatttgaagagatttattctcagccaaatatgagtgaccaatggcctgtgacacagccctcaggagatcctgaaaacatgtgcccaaggtgatcggggcacagccaggttttatagagtttagggaggcatgagacatcaatcaaacacatgtaaaaaattcattggttgggtctggaaaggcaggacaactcgaagctgagaaagggtggtggggtgagggtgtggcttcctggttataggtagatttaaaattttgtgattggcaactggttgaaagagttattatcaataggaaggaatgtctgggttataatgataaggggttgtggagaacaaagctttattatgcagatgaagccttcaggtagcaggcttcagagagaatagattgtaaatatttcttgtcagacttgaggtatgtgttgatgttaatgctggtcagcttttcctgaaagccaaacttgagtggggtataattggcccttctttcctgtcatgacctgaaccagataatcaggtaaactttggaatgccctggccaagaggaaaggtccattcagatggtgagaaggccttcaaattttattgttggcttataatctcacctctcattcttccttttataaatcatctggctgcttgtccagctcctgcacmcctctaggttgatgtctacaccctgggctgggtacttcggggtatcattccttccacttcatcaataagccatggttctatcaaagagggccctgctcacttcaccaattttgtgaaccagattcaccatgcactggtgaattttgtgaacctgcctgagcctggtgagacagaagacactcacatgcaacaagttacatgaagcaaatgtattacttacagataggaagcaagagacaacagaagactagaattcattatgtgccagtttcccaaggcttatgaaagctgccttgggtggatggagcttcaattgcacatggcctactgttgttgcagctgaggggccccaaaagcagcttaccccaggctcagtacctcaggggccacaggaatcactgggtaaatctcatcctactttcagggagagaggaacaaggctctggttgtcctagcagttcctccttaattcaatatgttacattctttaggagagccaggagccaggcccaggctgtttcaggcagttcctccctgcctcaggatatgggcattcccacacactctacagttgttcttcagactacaagcaagaaatggaggagaactgggtcagtgcctggccacttggagaacagttctgcagaaagaagtcacacctgtgaaaactgcctgccaagaggaaacaactacattgacatgtatgtgagcaagaaatcaattgctatttggttaagccattgaaactttctatttttctttctttttttttttcttttttttgagaaagggtatcactgtagctcaggttgtagtacagtggcatgttaatggcttactgcagccttgacctcccagatccaagcaatccttttgagtatctagaaccacaggtgcacactaccatgcccagctaaattttaaactctctaaagagacagggtctccctatgtggcccaggcttgtctcaaacttttaggctcaggtgatccttccacctctcgacatcccatagtgctgggattacaggagtgagccgtcttccctggcctgaaacttttacatatatttgttacagcagttgacactactctaagcaggatatataccttgcatgttcaataaagaatatatagaaatagcaacagttttcaggggaacattgtctttgaggatgaaactctgactttttttcttatcttggccaaactcctccctaagggaccttgggagtcacccctacaaaccataaagtttcatcagaggggttttatttaaccctatgtgacgtggtttgctttccaacctggctctggcatgacctcacataataaataaggaaagaaatgaaaatattttagccccaaatatatttccttgtcttgaaatgaccctgcaaagttgtctctctcttgtgggaataaaatctacatctttttttttttttttttttttttttttgaggcgaagtttcgctgttgttgcccgggctggagtgcaatggcgtgatctcggctcactgcaacctctgcctcccaggttcaagcgattctcctatctcagcctcccgagtagctgggattacaggcacatgccaccacacctggctaatttttttggtatttttagtagagacggagtttcatcatattgttcaggcaggtcttgaactcctgacctcaggtgatccacccacctcagcctcttaaagtgatgggattacaggcgtgagccaacgtgcccagcccgttcttttcctttttttttttttttttttttttttgagatagagtcttgctttttttcccaggctgcactgcagtagcgtgatcttggctcactacaacttctgtctccaggttcaagtgatcctcctgcctcagcttccagagtagctggcgtgcacctccacacgcagctaatttttctatctttatttatttatttattctgagacgaagtttggttcttgttgcccaggctgcagtgcagtagtgtggtctcagctcactgcaaactctacctcctgagttcatgtgattctcctgccttagcctcctgagtagttggggttacaggcatgagccaccatacctagctaatttttgtgtatttttagtagagatggggtttcaccatgttggccaggctggtctcgaactcctgacctcaggttatccactcgccttgacctcccaaagcacttggattacaggaatgagcaaccgcagctggccaacttttgtatttttagtagaaatggggtttcaccatgttggccaggctggtcttgaactcctgacctcaaataatcagtctgtcttggcctcccaaagtgctgggattacagacatgagccatctcgcccggccaaaactttttttttttttttttttgagacaaagtctcactctgtcacccaggctagagtgtaatggtatgattatggctcactgcagccttgaactcccaggctccgcttcccaagtagctgggactacaggtgcatgccaccacgcctggctaatttttgtatttttgtagagattgggttttgccatgttgcctaggctggtgttgaaatcctgggctcaagtgatccactgtgcttggctttttttttcttttttttttttgagaccgagtctcgctctgtcacccagattggagtgcagtgactcgatcttggctcactgcaacctccgctcggctgggtgcggtggctcacgcctgtaatctcagcacttcaggaggccgaggcgggcggatcaccagaggtcaggagctcaagaccagcctgggcaacatggtgaaaccccgtctctacaggaaatacaaaaattagccaagagtggtggcgggcgcctgtaatcccagctactcaggaggctgaggcaggagaatcattggaacttgggaggcggaggttgcagtgaactgagattgcacccatgcactccatcctgggcgacagagatagactccctttcaaagaaaataataataataataataatgttttcatgatgctttgttgatatctccttcatcttaaca

SEQ ID NO: 138 - DNA, 2457 bp, Homo sapiens
ttcacattatcctctaagccatttccagattgactgtagatctgaatataaaagtaagcaaacaaagcttgtagaatacaacatcggggaatatctttatgactttgacccaaggaaatattttctagacttgatgctaaaagcgttagtcataaagggcaatccttcccgtctagatcttcaagtccttcagttctgagaatttttcttatatttcttggtaaaattatcctccatttttcctttgtcttgctggaactcccagtaatgagatgatattgaatctctggaatgggttgttcaattttctttccactactattttccatctttgatgttttcctactgtttttgaagtagttctaaactgtaacttccaaatttttcattaaatgtttttcttttcccctgctactttattctttatttctaggagatcttgtttcattatcataaaaagatagtaccccaagttactatttccaggtgagatgaagtgtgttttacattttttctcctatcaaacacaactataagttatgggcagaatgcatgaaataactatttgaagactctgataataaaagagtaaacaaaagagtgtaaggatggaaaaagaacaccagaattatcctatatgttctccccaaattgagtatagatgtaatgcaattgctatcaaaattccagtagaattttttggagatagagaaaagctgattctaaactttatatggatagatgaaagaattagaatagctaaatcaattttgaaaaaatgcagtgaataatcacattacctgattttcagatttaataccaacttcagtaatcaagatagtaargtattggcagaaatataaacatgtagatcaattgatcagaacagagattccagaaataaatttacacaaatatggcgaattgatttttgacaaaggtgcaaataaaataaatgaagaaattaaaattgttcaacaaataatattgggacaatgggctatccatatgcaaaggaaagaaagaaaggagagaaaaggagagaaagaaaggaaggaaaaaaagtaaggaaggcgtggaagaaagaagtgaaggaaaagtggaaggaagaaagaaaagatatcctaacataaatctaacaatttatacaaaaattaactaaaaaattgatcatatatgcaaatgtaaacataaaactataaaactgttaaaagaaaacataacagaatatccacatgaccttgagttgggtgatgagttcttagatatggcactttccaaaaaagaaaaaaaaatacattggacttaatcaacttttaacacatttgctctgcaaaagaaactgttaagacattgaaaaaaataaagactggcagaaaatatttgtaagtcatgtatctgatagagaaattttatctagaatatataaagaatccttaaaactcagcaataagaaaacaacccaataaaaattgggtaaaggcataaacactttaccaaacagagtataaggatggcaaataagcacacaaaaaatgtttgacatcattagccattatgaaatgcaactttttttttcacaattgccccaaactggaaacaaatgtcacacaacacaaatgtccttcaatgagtggataaactgtggtacatccgtgcaatggaattctattcaagagcaaaaaggaatgaaattttgatatttgtaacaacttgggaaaatcttcatttatttcttttttttgagacggtgtcttgctctgtagcccaggttggagtgcagcagcgcgatttaggctcactgcaagctccgcctcccgggttcgcgccattttcctggctcagccttccgagtagctgggactacaggcgcccgccaccacgcccggctaattttttgtatttttagtagagacagggtttcatcgtgttagccaggatggtctcgatctcctgacctcgtgatccgtcctcctcggcctcccaaggtgctgggattacaggcgtgagccaccgctcccagccaacttgggtaaatcttaaggcattatgctaagcaaaagaagctgatctcaaaaagttacatactgtatgattccatttctacattttccaaaaggccaaaatatacaaatggaaagagtatttatgattgtcagctgctatgtgtgggattaggatgagactataaaggaacagtgctagggaggcttatggactgatagaactggtgtgtatcctgatatggtaatgggtatgtgtatatacatgtaagtgctttttaaaagtcaattttacttaatactttttaaaaatacagatagctcccatttgtggcatagactgtaccttctccatggtttctgtgagaaacactttcaccgagctcttgaaagagtttattttgagcagggtttggaggagagaaaacccggtgagaccctggagcactgcacg

SEQ ID NO: 139 - DNA, 3772 bp, Homo sapiens
aatcgtacatgaatatgtattaatttagcaaatatttactgatttctccactctttagaatgcaataattagttgttattctatgtctggtagttgctgatgagatattgttatgtggaaaaaacagaatccaaaacagttttgcaagattatgatttttagtttaaaaaaaactgtattatgggatgatttatatatgatarcgtgtacaatttgatgttttggcatatttatacatacatgtaacaactaccacaatcaaagtagagaacatttccatgatcctaaaaagttcccttgtggcctgtgatagtgaaacctgtgaatatgttatctttcacagcaaaaggaactttgcagctgtgattaaattaaggattatgaaatgaggtgattatccacaattacctggattgggcgttgtaatcacaaggatccttttaagagggatcattgtcagagaaggagatgtgacagtggaagcaaaagttggaatgatgaggccgggcgcggtggctcatgcctataatcccagcactttgggaggctgaggtgggcagattgcctgagctcaggagtttgagaccagcaccaccaacatggtgaaacctcatctctactaaaaatacaaaaattagccagtaatcctgactaaatgctcctgtaatcctcgctactcaggaggctgagtcaggagaattgcttgaacccgggaggcggaggtcgcaatgagcagagattgtgccactgcactccagcttgggcgacagagtgagacgccgtcttaaaaaaagaaaaaaagttggagtgctgcagggcgatgagccaagtaatgccagcagcctcttctagctggcgaaggcaaggaaacagattctcctctagagcttacagaaggaagatagccctgctgactcactctagacccctgacatccagagctgtgagataataaatttgtgttgttttaagctattaagtttgtggtaatttttcacagcagtaataggaaactaatgcatgccctttcccagtcagtcacactccgaccacacaatttccagtcaactataggccctttccatcatgatggttttgccttttctggaatttaatctaaatggattaaattatatgctatgtactctagttcctggtttttgctcagaacatttttgagattcattcatgttgttgcacatatcagtaatttattccatttattagcactttattggtaaaatgtattctatttgtacagacatgccacaatttgtttttccattcatgtgtgggtgaacatttttattattttcacattctagctattataaatagggctgctgtgcaaatttgtgtaacaagtctttgtgtagacatatataagccagagttcttcagaaacagaaaaccaatagtgtgtgtgtgtgtgtgtgtgtgtgtgtgcgtgtgtgtgtgtagacagtgattttaaggaatggacttacatgattgtagagtctggccagttcagattctgcacggtatgccagcaggctggaaacccaggaaaaagttaatgtggcagctaaaactcaaaggctgtctgctggcaaaagtccctcttcctagggagagaagttagtcttttttctcttaagtatttttcaactgataggaagcaatctgctttactcaaagtgtactgaattaaatgttaatctcatccagaagtaccttcacatcaacgtctaaactagtgttcgatcaaatatctgaatactatgagctagccatgttgacacgaaaaattaaccattgcatatgttttcacttcttttccaggaaatacctaggaatggaattgctggtcatttagtaagtgggtgtttaactttataagaagctaccagtgttttccaaagtggtggttcactttacattccaaaaagcattatatgagagttccagttgtacaacctcctcagcatttgttattgtcagacttaatgtttatgcaaagatatcctatgacatctttgcctatttcataatcatgattttctcctatatttccttctcagagatttataaattagcacttttgtttaggcctatgatctattttcagttaatttttttatgtattctaaaataaggatcaaagttaatttttttccatatggctatctccttgtttctgcaccatttttgaaaagactatcctttcctcataaagtacataggcacttttgttgaaagtaaatttattatacatgtacatctatttttggagtccctattttattccattaatctatatgactttcctaattatactttaatttgcaggccagttaggatggctattatcaaaaaccagaaaataaattggtaaggatttattggtaaggaactttatgtattgctggtggaaatgaaaagcagagcagccactgtggaaaacagtaagattcctcaaaattttcttttctttttttttttttgacagagtcttgctctgtcccccaggctggagtgcaaggcgcgatctcagctcactgcaacctccgcctcctgagttgaagcaattctcctgcctcagcctcctgagtagctgggactacaggcgcacgccgccatacctggctaatttttttcgtattttagtagagaccaggtttcattgtgttgcccaggctggtcgcaaactcctgagctcaggcaatctgcccaccttggcctcccaaagtgctgggattacaggcatgagccactgcaccctgccaatcctcaaactattaaatgtagaattaccatatgatccagcaattccatttttgcatatatatccaaaataaattaaaacacgggctcagattcatagcagtgttattcacaatagccaaatatccatcaacagattaatggataaacaaaatgtggtatacacacaatggaatattattcagccttgaaaggaaattctggctgggcacagtggctcatgcctataatcccagcattgtgggaggcccaggtgggtggatcacctgaggtcaggagttcaagaccagcctcaccaacatggcgaaaccccgtctctactaaaaatacaaaattagcggggtgtggtggctcatgcctgtaatcccagccggaggctgaagcaggagaatcgcttggacccaggaggcggaggttgcagtgagccaagataacaccattgcattgcactccagcctgggcaacaagagcaaaactcagtctcaagaaaaaaaaaaaaaggaaattctgacacatgctaaaacatgaatgaaccttgaagacattatgctaagtgaaataaaccaatcacaaaaagatgaatattttatattccatttatataacgtaccaaagtagtacaatttatagagagataaagtggaatggtggtttccaggggactagaaagaggcaaggatgtggagttagtgtttaataagtacagtttcacttggaaaagatggaaaagttctggagacaaatggtgataatggttgtacaacaatgtaaatgtacttaatgccacagaactgagcacttaaaaatggctaagatggtaaattttatattatggttgcttacataataaaataattacacaccagagacctatgacatatgtattagccacatttttaaaaatgataaaagtgtaacaccttattagagactgactcaggtacctacagcaagtaataggtggagttgtcagtagcctctcaaactcaggtgtttgatggtccct

SEQ ID NO: 140 - DNA, 1001 bp, Homo sapiens
ttttggaaggtgacgagtgtattttgtgagagagactggggtcataggtggacagaggtcctatctggtaggcagcctctaagatgacccccaataatctctacctcctggtattcttgccctggtgtagttccctatgtaccaggggtggtctttgtgtctaatgtaagtgatagataagctctagagggaagccagttactatgtcaccagcagtcctgtttagtagcctatttggggagggagtgagccttcctgccaacacccactagggagattggaagaagatcctccagacacagtcaagccttacgatgactagagccctagcctggcatcttgattgcaaccccaggaggaaccctaagctggaactacccaaatacaacactttgattttcaagttacagacacagtaagataataaatgtgttgttttaaaccactacatttggagttatttgttacagcaattgataagcaatacaaatctcaaataarttaagtttataacttaaggctccctggactattcaggaaatgcacttccaggatgccgatctactgtaggtcacctttgtggctttgatttatcaagatgaagatattttctacttcttttctttacttggtgcattcctaagtgacaagactacttttcgggcagttcactagggatgatagttgagttttctctctagattattattaatctgcatgtatgacactgaggacgtgtagagtggttctccattttcagcaggtcctagtgacttcggttttcctcaatttagaagctgccaaagcataagcccaaatttgcctccatgagcaagagctctaaaagcataagcaactggttgttgtggtgctctgcttatctgtgttctcatttccttttacatttgttttacatgtctcttaggtttctttaatgttttatcacttcattgtctaaaacaaacctttaaagaattgatttagaacatattttaataaaa

SEQ ID NO: 141 - DNA, 1001 bp, Homo sapiens
caggtacttgggaggctgaggtgggaggatcacttgagcctgggaggcagagatttcagtgagccaagaatgcatcattgcactccagcctgagcaacagagccagaccctgcctcaaaaagaaaatatatatgtatattagtttgataaactccaatataacttttttacataaaattgattttttaagtttataaatataaatatttaaatatgatatttaaatccaattttgctggaaagcctaaacacaatgtggaagctattgacttgtcccattatcaatcttacatactattataaaataaatgatataccattatagcttctcccaactatccaaatgcttatgggttaggtgtgaaacctacaagatgaagcaaatgaggctttatctaggggtgacagttttatggaaagaaatgagtatcagggaaggctacacaatgcaaaaacaaaattctgtgaggacttgaacccaaggcattttgcttaccagayaagtaagttgaatgacaaagcaacaattccctgtcataaaagttaatttatttgctattacagtatagacattttaaaacacaccagaagaattttagagtttgaaaatgacaagttgcattttgttttgagcaggaaacatatcaagacaaacttccttcatactagacagtattgtaatcccagcgactcaggaggcccaagcaggaggaccacttcaggccaggaatttgagattagcctaggaaacatagcgagacctcgtctctaagaaaataaattagtcattgtagtagcacacacctgtagttctagctacttggaaggctgaggtaggaggatgacttgagcccaggagtttgaggctgcagtgaaccatgatcacgccactgcactccagcctgggtgatagatcgagaccccatttctgggagggtgggaaaaccagacattgacaaggcctgagcagaggaggctgccaactgtagaaattgcaagtt

SEQ ID NO: 142 - DNA, 1001 bp, Homo sapiens
tatgtaatactatacatatttttaaaagaatgaagaaaacttgtctattctgatatggaaagtttgcaaaagtacattgtaagtaaaaatttaaaaaggcaagggacttaaaaagtgtataaaatgccactattcatgaagagaaaaaagaaaacacttgtgtaactttgtctatgtattcaaaatctctggaacgataaacaagacattaaaaacaatggtaaagcttttgggaaacaatggctgagtagacaacgattgggtttaacggcccctggaatggtgactagaaccacatttctagcatttttcaataccaaggtcttcgaagcgacctttgatttgaggtcactttaggaatctgaaggaacacataggaagactcccaaattgaggatctagacataagaaacctgggacgatctcgatcatgggaccatcgagaatcagactcgttgggaatatccttcaagtaccaatttgtatgttgtattagtgagyggcttttacgaagcaaagactcattaatatttcaccgaatctgattcattgtctgcatgtattgactagacattcagaaggcagcaaatatttccataaattgctgggccattagccacagtttgaaatgtttaagcgtcctctttcaagtctacgaatacagccattttgctttgtttttgcgttaagaggaaatttctcgttatttctattaagactctaaagcaactaagaaattgttcctccctgtaagacaaacaggaattacgttgaagaatttaatactttcacggagaaggggcgaggatgcgggtgagatgaataacaaaagcacagatttgcggtcggccggttagctcagttggttagagcgtgctgctactaatgccagggtcgaggtttcgatccccgtacgggcctttggctttttcccccctcgagaaatttggttttcatgctctaagatgattcaaattaaccgtccccatttcttaacgaac

SEQ ID NO: 143 - DNA, 1001 bp, Homo sapiens
cgagaccgggtagatatactcccttgggttggtgtgagcctagagacttagggacctcatcagagcaagaaagtgcaagtaggcttttctgcatcattttctggccctccagttcagacacaaatcaaaagttagtcccttcttgaaagccattagcattcatcaaggagcctcaatgagaggaagtttcaaacaaaaactaaatgtgtcaggcccagatttacggtgagggtctgattccacttccttgcggggtcagtttgggtccaggtgagagaggtacagtggtctctagttttctggaaacggtactgctgatagggcaaggactccttgcggctgccccagagaggttggcttgtcttatccaacttgcacttcacgttagagtttctaatgaactcgcagactccagtttcttgcccaggaaaccatttttaccgtattttgttcttttgaccgtttcttgtcagttagctggtgtaaattctgtttaaagahgtgaagggagccttctccattcgtgtagtcgtggccgagtggttaaggcgatggactagaaatccattggggtctccccgcgcaggttcgaatcctgccgactacgggatgttttactgagaacagttcagcgaggaaataggatctcacatttgctttcagtttgggagtaaagaaactcgtgatagagcctctgcgtgtcacctaacatagcctgaacttttgccgacttcgggatgttttactgagaacagttcagagaggaaatacgatgtcatatttgctttcagtttgggagtaaaggaactcgtaatagagcttctgcgtgccacttaacgcagcctgaacttttgccgacttcgggatgttttactgagaacagagaggaatcgtatttacttcagagaggaaatacgatgtcatatttgctttcagtttgggggcgagggaactcgtgataaagcttctgcgtgccacttgacgcatcctgaactttaaaa

SEQ ID NO: 144 - DNA, 1001 bp, Homo sapiens
cgaatccgagtcacggcagtaccttgatgtcgcctcaatttctcaacgtactgagcagtaccttgacgtcgcctcaatttttcaacatactggagtggagacagtctcggaaaaacccttgcaaaattgaattgacttacgatctaatctgtacacaaaaaacactagtattcatcatggtgccccaaccagtcagccaagcagagagtgtctacgcttgttgccttgtcttttttttcccctctccaaagattctcttcccaaccctacccaagccctacagtcttgttggcattggctgtatgtgaagaaactgaggtaatttttttttaatggaaaacttttactttcaaacactggtaggcatgaggaaaggactgttcaaaaggggatccaggtttgttgtggagatctttcttaaaacacaaaagacaaattattaatcacgcgtttctaagtatcctagctggaccaatgctgaaaaactgtaacctttgatcrtctggagaaaattaaagaaatttgagtaattgaaggaatttgggtgggggggaataatggcccagaagaacagcccccatttctagcccgttcagtttctagaatgagttctaaagagccaagtagactgggtgaggcgggagtggaggagagctgatctgagatacggaggtggctggaaagaagtagttggtgctacctaggaccagtaggaggtggctggagacaggcagatccccagaggcgcttccatgagcccagttctagttagtagcacagcactctgagaacacattaatggcacttcgtccctcctggccctggtggaaggttagtattcaaacaggtgtggtggctcatgcctataatcccagcactttgggaggccgaggcgggcagatcacctgaggtcgggagttcgagaccagcatggccaacatggtgaaaccccgtctctactaaaaatacaaaaattagcttggcatagtggcataggcctg

SEQ ID NO: 145 - DNA, 2290 bp, Homo sapiens
gagggagagaaataacgtgatttctctcacatgaactcaggggccaactttggatagaactgaaagctgtacctgagaaacaaagagaaatattccttcctccttcattttatactatttccagcaccaaaaccttttcttctctctgcctgcccccttccacacaaactgtccaactccattctcatttccccactgaggtggatgctgtggtgccctgccctggtcactccgtgttggactgagacacacaatcaaccagctgcagagagtgttggtggctcagggccctcagctgactccataccatgaattgttaaagagccaaagagagccctgtkgcccaaggttattccacctctcagtgagtggaccacatccaatgactggaaaacataggtgtaaaggtcctggaccccttgcacaaggtacacaactctgaagggtcaccccagttccagagttcattgtgagactgcattatatttcaacttttccttctgtctatcctctttccttaacttcctcaaggtattgatgctgcggggctctccagtggatgtcctatagtctatttctctggaaccaccaaagacagggattcttaaaagtgtggtctgaccctaagattctttcaggggatccatgaggtgaagacttttttttttttttttttttgagatggagtctcactctgtcacccaggctggagtgcagtggtacgatctcagctcactgcaacctctgcctcctgggttcaagctattctcctgtctcagcttcccgagtagccaccactcctgcctaatttttatatttttagtagagatggagtttcaccatattggtcaagctggtctcaaactcctgacctcaggtgatccacccatctctgcctcccaaagtgctgagattacaggtgtgagccaccgcacctggccaagacaatgtttataatgatactaaaatgttatttgtggctgggcatggtggctcatgcctgtaatcccaacgctttgggagaccaaggcaggcagatcacttgatgccagaagtttgagacctgcctgggcaacatggtgaaaccctgatctctacaaaaaatacataaaattatctgggcatggtggtgagttcctgtagtcccagctactcaggaggctgatgtgggaggatcacctgagcctcggaagtcgaggatgcagtgagccatgatcacgcctctacactccagcttgggtgacagagtgagaactctgtttcaaaaaaaaaagaagcgagaggatcacttgagcccaggaattcaagaccagcctggacaacatagtgagacccccatctctatttttaaaaataaataaataaattttttttaagttatttgcctcttttactcacatactctcacatgtgtgcattggagttttccagatgttgaagacatgatgacatcatccctctgacacctattggaatgtatgtcacaatgtgtattattgtgtttaaaatgctgtgttttaagggccgggcatggtggctcacacctgtaatcccagcactcagggaggccgaggcaagccgatcacttgagcccaggagtcagacctggccaacatggtgaaaccttgtctctatgaaaaataaaaaaattagccagacatggtggtgcatgcctgtaatcccagctactaggaaactgaggcaggagaatcacttgaatttgggaggcggaggttgcagtgagccgagattgtaccactacactccagccagggcaacagagcgagactctcatttaaaaaaaaaaaaaaaacctgttttatttatttatttgagacagggtctcaatcattcgcctaggctggagagtagtggtgccatctagactcactgcaaccttcacctcccaggctcaagtgatgttcctgcctcagcctcccacgtagctgaaattacaggtgcatgccaccacacatagctaatttttgtatttttttgtagagacaaggtctcactatgttgcccaggcttgtctcgaactcctgagctcaagcgatccacccaccttggcctcccaacgtgctggagttacagatgtgcaccaccacacccagcccagttttaatttttaaatgctaagtgttgatagatataactcacataaataaaaactctctgggattctcaattattttcaagagtataagaaggtcatgagaccaaaacatctgagaattgctgctctaagataaccaaatctaccctgggaggaaaaggctgaggttttaaa

SEQ ID NO: 146 - DNA, 1001 bp, Homo sapiens
gaaacaaatacacatgaaaatacagtatggcacaaataaggagcaagaggtgaagaaagcttcagtcacacccaaaataattttgtgaaaaatataaaatatgcagttatagacagcactaactctggataccagaaaattctataattcggtaatggatctgagacctgaattttggaggtactaaaatagatgcaatagatctagttttcattatgttcatactttcatttggctctgtggtaaaagatgataatatccaaaacaaaagatgataatatcctccatgtaacaattacatgcaaggggatgtctgcaaactgccacagtatcattttaattaatacctatcttctcttcttaaaatcttttcatttttccactcagttctcctgatatttctgttatgatataaaagacagctgaatgtgaagaaacactgattgtacacgtaacacacacattaatgattcaaatatgtaaacacagagagctgcaaayactttgagaggtagggctgaaacttttcgtcaatgtgtacaattcaatatcgtttcagttttcattctaaccgtccccagtggcttctgcccagcaactgatgagaaatggtacctctgagccaatcaaaacacgaattcctacaaagaggattctcttagtgtttctcggaccgagtgtacagcacatgctttcttttcctttattctggatcagagaatcttaactaaagcagaaataattgtgttaaattaaactaaatttggtatgagatatgtatacatttagcctgagggatggctcttgagcccttaaataatgaactgcaacctaacttagtatgtaaactaactgaaagcttaaggcatgggagtatacttttgtaacaaatagctgagtctcagccaatcccagtagccgaacttcagtcggcggcagtcaaccctgcagccaagtgatcagactatgttcaaataaggccaactctgagctgtaaccaa

SEQ ID NO: 147 - DNA, 1001 bp, Homo sapiens
gagtttctcttggtctgtgtgggagaagatggagatcacagctggagggggaagacaaggggttagatggaaaatgggtgcctcttgggaataggcagcttgctagcttgcttagctacttaatctgtgaggttatttcccggctttcaaaagatgggttattttggtgtcctgggacatggacaactgcaatctcttccggcagctgaagattttctagcacttgcataattaattccttgtgggccaaatcttggcccttactattgatgaggcctcgttcagtccagatcttttccgaaggcatacttggagtaagtgtaaatagttccttcctgattctgcagggattttaaggcttggtttaatgcaaagagttcacatatttgggcagaccacttatttggcagtctttctgactctaccactgtgagggtttccctatcaactatggagtacccgttgtgcctttttccttcaatgacctgggaggagccgtcyataaagaggtgatgccctgtttggaagggggtttcatgcctggatgcggtctgactctagtttgaaaactgattagatctaagcagttatgctcacattcctcctggtttggatttcctgttaggaaagcagcggggttgagtgaattgtcagtggttagtgttaggttatctccctctaataagatagcttcatattttaaaatccttgagtcagtgagccatctccctgccttctgattaagaatggttctgacttgatgaggggcacttacgaagaggtttcccccaaaggttattttcctgctttcttctgttagcaaggcagttgctgctatggattgaacacattcgggccatccacgggttactgggtcaaggatttttgacagaaagactacaggctgccggtggcctccatgtttttgggtgagtacccctaaggccactcctttgcttacattaatgaaaagatggaatggctgttctaaggagggcaaa

SEQ ID NO: 148 - DNA, 501 bp, Homo sapiens
ctccagtgcaacctatggggcttttggaaatgaggaagtcgatgactctgcagggactcctctgacccaggagcagatggcgctcgtctgggcactccccaggagaaaaggtgcatcgggaagcagcctggcttgtggatggtaataagtcactgttgatgggttgggtgcagggagggatttaagttcttgagcgacagatgctagggagtttacctgctctggataacagtatcttgtggaggatagtyacctggaaaacagaaatggcgtgactgtgttgaatacactgtttgatgattctgggcatcaggtgaataggaaatgtgtaacgttatggatgagtgtgtgctcatcggacagtagcagtgcatcttaacagtcggcctctcagtcctcctcttccttagaatcacctatagagctttaaaatttcctggataatgttaatgtgcagccagcgatgatgaccattgggctacagtcaaatccaagaggcgc

SEQ ID NO: 149 - DNA, 1001 bp, Homo sapiens
cccacctcggcctcccaaagtactgggattacgggcatgagccaccatgcctgtcctacatatatcttattcattgtcttattcaatcatacaacttcctgataaaatgaggctgattttcacccctattttgctgttaaggaaactggtataatgagtgtcactgacttgtttgtgatcacacagtggacaaaatggcatttgtttctttgtggtgatctcacaaaggtcaagatgaccttagatcctcagttttggctgttttttttttgttgtttttttgtttgtttgtttgttttacaccaaggaaccaggttctagctcctatgtttgttcattgcatggaaaggaacaggaagatctgggggccactgaatggaaggttagatccattttcttggttaagcttgtaggttttctcgtctcttttccttcctgcagcacaattcttatgaatggcaatatcttctattaaaattctcagtctgtagtcttcttgtycatacagaaaatagatttcaggtcaacacatttgatagtctggactgtgctaactgctccaatatttgagtacatcttttggggatgtgggaatttagtgttgtaggcctcaagtggggttcgttcccagaatttggagaggctatagaaatataacctggttggccaggcacggtgactcatgcctgtaaccccatcaatgtgggaggccgaggcaggtggatcacctgaggtcaggagttcgggaccagcctggccaacatggagaaaccctgtctctactaaaaacttttaaaaaattaggcgggcgtggtggtacgtgcctgtaatcccagctacttgggaggctgaagtaggagaatcccttgaacccgggaggtggaggttgcagtgagctgagatcacaccattgcactccagggcaacagagtgagactccatctcaaaaaaaaaaaaaaaagaaaaagaaatataacctggccataatataagcataaata

SEQ ID NO: 150 - DNA, 1181 bp, Homo sapiens
gaggtcctggctgagccaaggagtaatggaccagatctacctcagtattcaagttcagtggggacaccagtggcttcaaacttcctggtttcatgatatcttgagacgccttacaaatgatggaggattccaaagagtttttgtttatttgggttaatatttgttggtatttatggcatttgagattgaaactaagaaatgttttaatttattacctttacaacatttatttacattacatacatacatttacaacatttattaatttatattaaaatagcatgaataagccaattataggttaatataagtagaatgtttgtgaaaaataagtatggtatccaaagcaaaataaattttattgtgaagtgtggcattgattvactttttccagatctaatgtgtggcttgaaagaatatgactggattctcatatctgcctttatactcactctgttgagatatcatagactatataggctcaagaaaactttatcctagtgacagaatgagattaaaaacaacaaactgtgttttattattaatatgaaaatacgattattaaccttgcaggccccttaaaacagttctggttaactgagaccttgtctctaccaaaaacaaacaaaaaaaattaggtgtggtagcgcacgcctgtagtccctgcttcaggagactaaaaagactaactccaactccttgcttgagccaggagttggagtttgcaatgagctgtgatcctgccattgcactccagcctaggcaacagagtgagactctgcctcaaaaaaccaaaacacaggtcgggcacggtggctcacgcctgtaatcccagcactttaggaagccgaggtgggtggatcacctgaggtcaggagttcaagaccagcctggtcaacatggcaaaaccccatctcactaaaaatacaaaaattagccaggcatggtggcgggcacctataatcccagctactcaggaggctgagacagggaatccttgaaccccagtggggtggaggttgcagtgagccaagatcgtgctgcttcactccagcctgggtgaaagagtgaaactcccgtctcaaacaaagagggggagggaacttatgtcagagaccccccccaccccaccccaggaatcctgaaaccatatttgagagttgggatagaggattcgggaa

SEQ ID NO: 151 - DNA, 1205 bp, Homo sapiens
ttatgggaagaatcaggaacatatatttaaatacctgatttgttaaggcagaaaacagggttgtttatgtgcatgttttagtctgcccagacagctatgacaaatataccaagactgagtcgtttataaacaaccaaaattttttttcttgcactctgggggctgggaaatgtaagaccaaggcaccagcagtttggtaactggtaagagcctgcatccttgttcacagccttttaaatgtgtcctcatatggcaaaggagaaaagtagatctttggtttttgtcccaagaaactggaaagatgggccgggcacggtggctcacgcccgtcatcccagcactttgggaggccaaggcaggtggatcacttaaggtgaggagttcgtgaacagcctggccaacatggtaaaaccctgtctgtactaaaacccagaaggtggaggttgcagtgcaccactgcactctagcctgagtggcagagtgagactctcaaaaaagaaaagagagagaaggaaggaaggaaaggaaggaaggaaggaaggaaggaaaagtaactggaaagatgaagttgttaatttctgagatggggaaacggagagacaaggagcaagacgggagtggtacagaaccaaaggttcagttgtggatacattaaggttgaggagtctatattagagatgcacatggagatgcagagtagtccattgaataaccaagagtccaggtgagacctcaaggctggagrtagagattccatactcaactttcctatatgtttgaagagtttcatgatacactgtagtgggtagagggaagaattgtattttgttattaataacagtcctgaatatcattggctttgacaaaatgaggacttcttttcatgtcaataaatatggatggtggccatcaagggctgatctgagagcttgaaatgtcatacatgccccagcttagttctgtctttattttcttctgtcttagcatgtggcttgcatcttcaatgttgcctcatggtcacaaaagggctgcccagctccaaagtccatattctagataagaggaagtagaaagtaaggggagtgtaagggtctaccagctgttttagcctccccttaaataatctgtctgataaacttccaccctcaagcaattggctcaaacttagtcccttggcttcccctgtctacaaatgagatggacac

SEQ ID NO: 152 - DNA, 1001 bp, Homo sapiens
cttgtcagatcccagccccctggttgagattttcctggactatgaagcaggaggcatctccttctacaacatgagtgacagaaccccttatctatgctttccccaaaggctctttctctggctcccttcagcctttattcttcttgtggtcatgcgataaaaagcccctgaccacctgcccaattgttgatggactttcaggaggtcacagtcttgtgaagcctggggcctaaggagattctgttgtccagaattcagaaaattctgcctccagaaatacaaatatgctcttttctaaacaagtgacaacacaatgtagccataggctcccttaagcagccacctcatgtcaactaatagtctttgctctctagcctctctcctccaaagtccatttcgtctcctgaggcttcagctattactgtcagaccctcagttacttctgatgaacagggattaggcttgagaaaatggagatgcatttagattggcagatatggrggacttcttaatgtgcttttattgctgccttatctctgaaaacaggttctgggagtttgggaataagtctgagggcatataaaggattgagactgagtgacttaggagtgtgagaggaaatatcttgatgttgagaacagggttgatgtggaggggtattctctgtgttatgcatgtaaaaagaaaaaaaggaaaaaaaaatcattactgggaaagaaaacaccccaagctgaagtccaagaaaggtacacagaggaaacacagaaacagttgtgttagcagaagatgacatgaaacccagctgacagtgaaattaggaagttgccttggaatttcaagaacttgcattctcaagtttatggttctgtgtccaacagagcagcaaaatccagcacttcttcttttgagtctccatatcgtgctaacagaaagacaaggggtcgggagatgcagagatgaggaggagctcaagagtgacagtgttgaagagattctgagca

SEQ ID NO: 153 - DNA, 4000 bp, Homo sapiens
atatagtgtttgacacatccatagtttcaggcatccactgagggtcttggaacatgtcccccaaggataagtggggactactctagtgccatcaggctagcaggctgtaaaggttttaatggcagtccctggaccatggcttatttaattgcttccaaggcccactgctacaaagggcctcattcaaagctggtggctttgttggtcaccctgacttaggggaccaaaagaacactcaggtggggtacatgttgcctccaatgcccaagtacccaaagaggccttccagctgttgggcctcctttttattagtggatgtctccaaaattaaatttttttgcttggttgtatctagaatacttttctggcttactgcccatgtggccttcgcatttagcccagggacagtccactgttagtctccacatccgaaagcctttttgactagccaaactgagctgttacattatgacagggtagtttgtagcatttccatttgtaacaataattaacacaataatgtcctgttcttcagttagtatgcagtactgtttttttgaataacccactgggacttgggtggcttaggtggcagacaggcatggatatgccccgccgtaacggctggaattcttagctgtgagcgggcgcacccctcaggcagtgatgatgtgctgagccccaagcagccaaaatgtcaatgactataagacattcagccacaggaaccaaagtcaccggcacctcaaatggccagaggcaccccacagcagataagcaccataggtcactgcttttgtccccaagcctcttaatgtcaccagtttaatttttcccttaaggagacctggaaatattgtcacatgggttccaatatctaagaacaccagaaaaatatgaattcctttttccccctttttatcttttaaaggaatattattaattttaaaagcagggaccatgctaatcatctctatatcattccaatttcagtatatgtgctgctgaagcaagcatgtctttttttttttaatttttaaattttaaattttatgagcacatagtaagtggatatatttaataggtacgtgagacattttggtacaggacgcaatctgtaataatcacatcatggaaaatggggtatccatcctttcaagcatttatcctttgtgttaaaaacaatccaattatactcttagttattttaaaatgtacaattaagatattattgactatagtcttcctgttgtgctgtcaaacattaggtctttttcattcttctgtttttttttgtttttttttttgtttttttcttttttcagatggagttttgctcttgttgccctggctggagtgcaatggcatggtctcggctcactgcaacctgcgcctcccgggttcaagtgattctcctgtctcagcctcctgagtagctgggattataggcacacaccaccatgcctggctaacttttgtatttttagaagagacagggtttcaccatgttggccaggctgatcttcaactactgacctcaggtgatccacccgcctcagcctctcaaagtattgggattacaggcacgagccaccacatccggccctttttcattaaccatccccacctcctctcccgcttcctcccacttccactacccttccaagcctctggtaaccatccttatattctcttatctccatgagttcaattgttttgatttttagatcctgcaaataactgagaacatccaaagtttgtctttctgttcctggcttattataagaactcctgttttatcttgacaggaatatagagtgactgacctccagtggggaggaaaccagagaccgtggccccattcccaactgggccattcagcctgagacatttggatttgatagaacctctttgatagaaccatggcttattgatgaagtggaaggagtgatacccgaagtacccagcccacggtgtagacatcaacctacaggggtgcrgaagctggacacaccacccagcctgcacaagatttagctggctattctccatttttattctttggataatgagtttctgctctgtaaatgcccttatgaactgtgtttggttccctctcagatgcctcagggaccaccagaggacctcttcctcttccctctcagggttctcagggatcaactgagtatccatttcctgagttctctagctctcgggaatgaacaaccatacaagtgtccaacaatcagagggtggcttgccactgtcctattctatatttctttctctctgccccagtcagtgcagccagctcactcatatccgcagggttgggggtgacctatgtcctgtttacaaaaagagtcaaactgtaaaacatttgaagagatttattctcagccaaatatgagtgaccaatggcctgtgacacagccctcaggagatcctgaaaacatgtgcccaaggtgatcggggcacagccaggttttatagagtttagggaggcatgagacatcaatcaaacacatgtaaaaaattcattggttgggtctggaaaggcaggacaactcgaagctgagaaagggtggtggggtgagggtgtggcttcctggttataggtagatttaaaattttgtgattggcaactggttgaaagagttattatcaataggaaggaatgtctgggttataatgataaggggttgtggagaacaaagctttattatgcagatgaagccttcaggtagcaggcttcagagagaatagattgtaaatatttcttgtcagacttgaggtatgtgttgatgttaatgctggtcagcttttcctgaaagccaaacttgagtggggtataattggcccttctttcctgtcatgacctgaaccagataatcaggtaaactttggaatgccctggccaagaggaaaggtccattcagatggtgagaaggccttcaaattttattgttggcttataatctcacctctcattcttccttttataaatcatctggctgcttgtccagctcctgcacacctctaggttgatgtctacaccctgggctgggtacttcggggtatcattccttccacttcatcaataagccatggttctatcaaagagggccctgctcacttcaccaattttgtgaaccagattcaccatgcactggtgaattttgtgaacctgcctgagcctggtgagacagaagacactcacatgcaacaagttacatgaagcaaatgtattacttacagataggaagcaagagacaacagaagactagaattcattatgtgccagtttcccaaggcttatgaaagctgccttgggtggatggagcttcaattgcacatggcctactgttgttgcagctgaggggccccaaaagcagcttaccccaggctcagtacctcaggggccacaggaatcactgggtaaatctcatcctactttcagggagagaggaacaaggctctggttgtcctagcagttcctccttaattcaatatgttacattctttaggagagccaggagccaggcccaggctgtttcaggcagttcctccctgcctcaggatatgggcattcccacacactctacagttgttcttcagactacaagcaagaaatggaggagaactgggtcagtgcctggccacttggagaacagttctgcagaaagaagtcacacctgtgaaaactgcctgccaagaggaaacaactacattgacatgtatgtgagcaagaaatcaattgctatttggttaagccattgaaactttctatttttctttctttttttttttcttttttttgagaaagggtatcactgtagctcaggttgtagtacagtggcatgttaatggcttactgcagccttgacctcccagatccaagcaatccttttgagtatctagaaccacaggtgcacactaccatgcccagctaaattttaaactctctaaagagacagggtctccctatgtggcccaggct

SEQ ID NO: 154 - DNA, 1181 bp, Homo sapiens
gaggtcctggctgagccaaggagtaatggaccagatctacctcagtattcaagttcagtggggacaccagtggcttcaaacttcctggtttcatgatatcttgagacgccttacaaatgatggaggattccaaagagtttttgtttatttgggttaatatttgttggtatttatggcatttgagattgaaactaagaaatgttttaatttattacctttacaacatttatttacattacatacatacatttacaacatttattaatttatattaaaatagcatgaataagccaattataggttaatataagtagaatgtttgtgaaaaataagtatggtatccaaagcaaaataaattttattgtgaagtgtgrcattgattaactttttccagatctaatgtgtggcttgaaagaatatgactggattctcatatctgcctttatactcactctgttgagatatcatagactatataggctcaagaaaactttatcctagtgacagaatgagattaaaaacaacaaactgtgttttattattaatatgaaaatacgattattaaccttgcaggccccttaaaacagttctggttaactgagaccttgtctctaccaaaaacaaacaaaaaaaattaggtgtggtagcgcacgcctgtagtccctgcttcaggagactaaaaagactaactccaactccttgcttgagccaggagttggagtttgcaatgagctgtgatcctgccattgcactccagcctaggcaacagagtgagactctgcctcaaaaaaccaaaacacaggtcgggcacggtggctcacgcctgtaatcccagcactttaggaagccgaggtgggtggatcacctgaggtcaggagttcaagaccagcctggtcaacatggcaaaaccccatctcactaaaaatacaaaaattagccaggcatggtggcgggcacctataatcccagctactcaggaggctgagacagggaatccttgaaccccagtggggtggaggttgcagtgagccaagatcgtgctgcttcactccagcctgggtgaaagagtgaaactcccgtctcaaacaaagagggggagggaacttatgtcagagaccccccccaccccaccccaggaatcctgaaaccatatttgagagttgggatagaggattcgggaa

SEQ ID NO: 155 - DNA, 4000 bp, Homo sapiens
agacgtttacctggagttggtcctttttagccgccagaaagatacagggattaaaaacacaaattgtaaattgagtgataatatttcttacaaaggtaacattaaaactgtgttgagtcctattactattattggatagtgtcctgacccagatgctgccattcataaatgggagtgctaacttccatatcgactgctgaattgggcccctctttccttgatgacgccgctgaggcaaaggcggactaaagcctgttccgtgccaagccagttgcgtggcagattaggattgaatcccaatgcgatatagcgaagaaatgttaaatgttcaccaccagtggcagcgaagtttgttccatgaggtctgattctcatctctcccaaatgaccacagggaccccagtcaataatgtctcccattaacatagacttgtctagctaaggggtcaagacactggatccaaggaggggggtgagaattattgaagggagcccattctgtataatcaatacaatttggacgatggggctgggagagattagtaaatccaccagtaatattattagagctaaggcctaataggtacataatgtttccatggtgactcaaccatgcctgggattggactgcaaggcaactgccattgagcgatgtatccttggtgatgcataaagggagtccctccaatggggcagtgtaattgatactattgttctgacagtctaatagttctgtgtcagggggagttaggggtcctggggtccatgctccctgatcacgatatacctcaggaggagtgtcactccagagtacaggtcgcactactcaggggttaggaacatatgcccgacatgtttttgcttctacacaggggaaacataccacacaggacactacagctagtatggccaagaacattgattcaggggtttttgcctgaccctggcactccagcattttctcagcttcctgcatggttttcttgatctgtccccatgttatgagggtggatgtcaatgtgactccagtcggcccttgttccatctttgcattcagattcaactggcctatggcttgtactgggggaaccgggcccatggttgcgatccacggatccctccagtctcccgttccatggttgcacgtacctggagggcacctacacagtttgtccatctcctgtaaaaacacaagcataccctcatccccacatcagcaaatccactgggcctttcctttgtccttcttctggggatttccataacacctttggataaacttgcctctttccctctaacacttgccaatgttgttctgctagagtcttaccatccataccaggcatcaaaaaatttaaagtaaacaagactaaatgtaattttgtttaaggtggtagctggtctcctattccccctttttttctcaacatacgctgtagtgtttgatgtgcccgctctataatgccttgtccttggggattgtaaggaattcctgttttatgaatgattgcccataactgtaaaaaattttgaaaagcatgactaacataagcaggtccattgtcagtttttaattgtttagagacccccatatgggcaaatgacgacaaacaatgccattggacatggccagcagtttcccctgtttgacatgtggcatgtaacatattggagtaggtgtctatagtcacatgaacatagctaagtttgccaaaggctgctgtatgtgcaacatccatctgccagatttcatttggagccaagcctcgtgggtcgcatccttccacgggtgcaacaccagggacatgctgacaagtggagcaggcttgcacaatagcttgagcttgactgcaaggcagatgaaacatatgagtaagggcagaggtgttttgatgcagtaatgcatgggaagcttgggcttgttggaatacagaaccaattaatttatctgctttatcattaccttgagatagtggtccaggaagttgcgtatgagagcraataggagcagcacaagagagaatagcttgctgaagtcttagaaacaaattaagcagctctggttctagggtgcccttaatagtggcagtctcaatgcaactagctgcatttacaacataggctgaatcacaaacaatattaataggagataaagccgtgagctctaaaacctgaataactgcgattaactctgagcattgagctgaaactccagagatctttattgtttgagtatgtttagttgcataaatagctgtgcggcctttgtaagagccattggtaaaatatgtctttccacctggaatgggcttgtgatgggtaattacagggaggataaaagggtgaactttataaaattgcaaaatcttgtctgatggataatggttatctattattcccacaaaatctgcaaaagcaatttgccatgcagtcgacatttcccatgctgcggcctgttgttgggaatccaagggaacaataattttatcaggatcatatcccgtaagcattttttacctgtgcctacctattgttataagttgagtaattaaagaaagataaacttgcaaagatttcactgtcagattgaataaaaaaaaaaaaagcctttatattaccattacagatttgtctatgaattggcctaaaaatcctgatggagaatggggggtaggaagaataaacaaaagcaaaggcttttgtggctgtagccgggaggcatgttgttgctgaaggatctgttctacacgctgtcactcagcttctgcctcgttagtaagttgccgaggagaatctaatgaagaatctctttggagggtttgataaaggtgtgtgagttggtagatggcaatacctagcatcaggcacagccaattgatatcccctaataattgttggaagtcattcagagtttgtaccctctccctacagagagttactttctgaggccgaacacttcttccagtaacaatagtacctaagtactggtatggggaggttgtttgcaccttttcaggagctattttgagattccatgcagtcaagactcattttatttccctgaataactgatgtaacatttgatctgtaggagcggccaaaagaatatcatccatataatgaatgatgtaggcattgggaaatatattgcgaggctcctttaaagcttttcctacaaaatgctgacataacataggactgttgagcatgccttgggctaaaactttccactgagagcgagagacaggctctctttgattaatagaaggcacagagaaggcaaattgaggcttatcctttttgtgtaatggtatattaaaaaaaaaactctttaagacctattactacaagagtccaatctcttggaatggctgctgaggatgacagaccttgctgtaatgcacccactggtttaatctgtgcatttaatagctctcaaatcatgtagcagttgccattttcctgacatttttggatcacaaatacaggtgaattccaggggctgactattctgtatgttctgcttccagttgctctctcactagctgatggagttgcatcagtttctcctgtgataggggccattgatccacccacacaggtttgtcagtcagccactctagcggcaaagcagtgggtggaggagaaataccaatgacccccaccaaaaatcctgatgacctagcccttttctgttttgtccagttattgatattggatcagggtttccctgcaggggctttcctaagccttttccactctgaatcccattttctttaacattttaaatcctggattatcaatagtttcctttttaagtctcatgtcccatgctgtcagtaaatctcggccccatagattaacagctatatttgcaacataaggttgaaaagtacatgactgtccatgtggtctgagacaggataaaatctcagcactccactgaacactttgagctttcctagtcccactaaggatgtagaagttaattgcaggggtc

SEQ ID NO: 156 - DNA, 3639 bp, Homo sapiens
agttagtatgcagtactgtttttttgaataacccactgggacttgggtggcttaggtggcagacaggcatggatatgccccgccgtaacggctggaattcttagctgtgagcgggcgcacccctcaggcagtgatgatgtgctgagccccaagcagccaaaatgtcaatgactataagacattcagccacaggaaccaaagtcaccggcacctcaaatggccagaggcaccccacagcagataagcaccataggtcactgcttttgtccccaagcctcttaatgtcaccagtttaatttttcccttaaggagacctggaaatattgtcacatgggttccaatatctaagaacaccagaaaaatatgaattcctttttccccctttttatcttttaaaggaatattattaattttaaaagcagggaccatgctaatcatctctatatcattccaatttcagtatatgtgctgctgaagcaagcatgtctttttttttttaatttttaaattttaaattttatgagcacatagtaagtggatatatttaataggtacgtgagacattttggtacaggacgcaatctgtaataatcacatcatggaaaatggggtatccatcctttcaagcatttatcctttgtgttaaaaacaatccaattatactcttagttattttaaaatgtacaattaagatattattgactatagtcttcctgttgtgctgtcaaacattaggtctttttcattcttctgtttttttttgtttttttttttgtttttttcttttttcagatggagttttgctcttgttgccctggctggagtgcaatggcatggtctcggctcactgcaacctgcgcctcccgggttcaagtgattctcctgtctcagcctcctgagtagctgggattataggcacacaccaccatgcctggctaacttttgtatttttagaagagacagggtttcaccatgttggccaggctgatcttcaactactgacctcaggtgatccacccgcctcagcctctcaaagtattgggattacaggcacgagccaccacatccggccctttttcattaaccatccccacctcctctcccgcttcctcccacttccactacccttccaagcctctggtaaccatccttatattctcttatctccatgagttcaattgttttgatttttagatcctgcaaataactgagaacatccaaagtttgtctttctgttcctggcttattataagaactcctgttttatcttgacaggaatatagagtgactgacctccagtggggaggaaaccagagaccgtggccccattcccaactgggccattcagcctgagacatttggatttgatagaacctctttgatagaaccatggcttattgatgaagtggaaggagtgatacccgaagtacccagcccacggtgtagacatcaacctacaggggtgcggaagctggacacaccacccagcctgcacaagatttagctggctattctccatttttattctttggataatgagtttctgctctgtaaatgcccttatgaactgtgtttggttccctctcagatgcctcagggaccaccagaggacctcttcctcttccctctcagggttctcagggatcaactgagtatccatttcctgagttctctagctctcgggaatgaacaaccatacaagtgtccaacaatcagagggtggcttgccactgtcctattctatatttctttctctctgccccagtcagtgcagccagctcactcatatccgcagggttgggggtgacctatgtcctgtttacaaaaagagtcaaactgtaaaacatttgaagagatttattctcagccaaatatgagtgaccaatggcctgtgacacagccctcaggagatcctgaaaacatgtgcccaaggtgatcggggcacagccaggttttatagagtttagggaggcatgagacatcaatcaaacacatgtaamaaattcattggttgggtctggaaaggcaggacaactcgaagctgagaaagggtggtggggtgagggtgtggcttcctggttataggtagatttaaaattttgtgattggcaactggttgaaagagttattatcaataggaaggaatgtctgggttataatgataaggggttgtggagaacaaagctttattatgcagatgaagccttcaggtagcaggcttcagagagaatagattgtaaatatttcttgtcagacttgaggtatgtgttgatgttaatgctggtcagcttttcctgaaagccaaacttgagtggggtataattggcccttctttcctgtcatgacctgaaccagataatcaggtaaactttggaatgccctggccaagaggaaaggtccattcagatggtgagaaggccttcaaattttattgttggcttataatctcacctctcattcttccttttataaatcatctggctgcttgtccagctcctgcacacctctaggttgatgtctacaccctgggctgggtacttcggggtatcattccttccacttcatcaataagccatggttctatcaaagagggccctgctcacttcaccaattttgtgaaccagattcaccatgcactggtgaattttgtgaacctgcctgagcctggtgagacagaagacactcacatgcaacaagttacatgaagcaaatgtattacttacagataggaagcaagagacaacagaagactagaattcattatgtgccagtttcccaaggcttatgaaagctgccttgggtggatggagcttcaattgcacatggcctactgttgttgcagctgaggggccccaaaagcagcttaccccaggctcagtacctcaggggccacaggaatcactgggtaaatctcatcctactttcagggagagaggaacaaggctctggttgtcctagcagttcctccttaattcaatatgttacattctttaggagagccaggagccaggcccaggctgtttcaggcagttcctccctgcctcaggatatgggcattcccacacactctacagttgttcttcagactacaagcaagaaatggaggagaactgggtcagtgcctggccacttggagaacagttctgcagaaagaagtcacacctgtgaaaactgcctgccaagaggaaacaactacattgacatgtatgtgagcaagaaatcaattgctatttggttaagccattgaaactttctatttttctttctttttttttttcttttttttgagaaagggtatcactgtagctcaggttgtagtacagtggcatgttaatggcttactgcagccttgacctcccagatccaagcaatccttttgagtatctagaaccacaggtgcacactaccatgcccagctaaattttaaactctctaaagagacagggtctccctatgtggcccaggcttgtctcaaacttttaggctcaggtgatccttccacctctcgacatcccatagtgctgggattacaggagtgagccgtcttccctggcctgaaacttttacatatatttgttacagcagttgacactactctaagcaggatatataccttgcatgttcaataaagaatatata

SEQ ID NO: 157 - DNA, 1001 bp, Homo sapiens
tatataattattgggagtctctgtgagcctactctgactcagaaagccgctcctaaagaagaaaaaagaacaaacaaacaaataaaaaacccgaattatttttaaaactctttattttggatttttcagtttctacattttgttactgtagattttactagattgaacagccttatccataaatatttgcatcaatctctaaatttttttcttcaacactaacttttatagttggaattttgggggcaaataatacaacattttaaaggcacttgccatgtgtacatggccaaatgcttccagaaacatttccacttccattagcaaagtatataactacagagtatttaaggttttattcctttatatttttttctttggcaaaattgtctatagtagaaagaatgaataataaataacctaaaaaataaaagttctccctctgaggacagcagagaaatttttagcttagcttaataatacctccttctccttaggagmataaagagcagtttcgaggagcagaagatgtggtgaaatataatgtttagtctgatggtggatgcaagatccaggcaggggtggagcatgaccagctgcacagacctctgttcccttgcttcctctacatctctccccacctccatctgcagaccttgttctcagaggccattcccagacccacagcagctggtatgatggctgcaggcctcatgctcctttgttttgggagaaactgttgaggagttagtatttactgagcagctaatatgttccagtcactattattcctcataataattagttattaactaatacatgaaaattttaaacttaaagcattccaataattttaaaagtaaaggaagcaaaaggccaaagcgtcctttcactcacttaacctccaattttcagtttagcatccatcattttagactttttcaggcatttacatatatagttatgcagaaatgtatagctttgcttttgtttttcaattg

SEQ ID NO: 158 - DNA, 1001 bp, Homo sapiens
ttaaaagtaaaggaagcaaaaggccaaagcgtcctttcactcacttaacctccaattttcagtttagcatccatcattttagactttttcaggcatttacatatatagttatgcagaaatgtatagctttgcttttgtttttcaattgaatcattagtatagttctgcaaggtgctttttaatcacttagtatatctccattatccaggctagtgacattaaatcactctttttaactgctgcattgaatttcctcctagggatgagccatcattcctctaaccagtctcttgtgagtggctggttcagttggtaaccacttttatactttaaaaatagtgctgcagtgtcattcccacagaggcttctctctgcacccatgcgagtacttcgctgaagtaaccatcaggaagtggaattgctgggccaattgtgaacattctaagtctcatactcgatatttttgagtaactaaagttgaaatggttttgtcccatgacygagatcatcaagcttgtgacttgtagagcctttacctattgtctaccctctttgtgttcctaactctaccatagtgggtccagcccattgtgggtgctcagtaaatatttgttgaataactttatgaagggaagaaagaaaagatgagtaaagcctggtcttattcaaagctctcctaatcaatatctttgtgattaaacgtggtgggttcagcccctgactgacttcagagcctctgccaggcagtctgcctggatcccaccaggagccaccaggccataagttgactgtagtaatggccaagagtttgacgcttgaggagtccatagtgttggacacccacagagctgaacaagggtgggaccagggaatccagtgaagagggtccttcatgaatcagagggggatgatggaagcttggacctggcaagggaagtgtggggaagtgataggattatgaatattttaatattttaatgcagtagagtcagagatgtcct

SEQ ID NO: 159 - DNA, 1263 bp, Homo sapiens
agaactcctttcctctggccaccagagatataagcgaagtgaaggacgagggataggaagcataagaaaccatctcttcagtgactggtacacagtcattttggtttagttgtgtaacagatggcttctgttgtgtctccaagtgcacactaccatgggtcctgggaggtggaatagtgactgtatctgctgccagtgttytccaactagccatccccaggaatactcctgtagtagaactagctgtatttcttacgtgttgcagtgaggaagaacacacatcatggggagctgtggcggggtctcagtaagaaggtgttagagcagacttggtatacaatttgggcttgtgttaggggattggggccgggggagttcatagacttagccctctgctctggatgagattccatcaggaaggtgtgggcaggttaattctgagtgagagccttaatcaatcttatgtaggaagaaggagaccagggtgagacaaaagctgtaattgatgaaggggcagcaatccctcattgctgaggggggatgtttggtcactgctgtggtttggacaatgttcatgtttttctctatgctcacatatgatgtggggtggtattgtttttcccatgatccatcatagtcacaaagtgccattgtctgtgttctgtgaaattgcttatgttcaacaggatgacacagagacccggtgtcagtttccatatgttgggacagcttttctctttctcagtgcaatcccttgccctgtggctgctggttaggtttggtttaaggggatctctagcagacaatcataggaggaagagaaaaggaagaagtctgggtgcttattcactggcttccttactgcaagttaccctcaggctggctgcattgccttgctgaaggtaacagctcctctaaaggaagtcctcaatgcatgaatctcttcttttttgtgttcaaaacagcttcctctcctcctccctctggtaattggggtgggtgggaatagccccactgtttctgaccctgggatactgcactagcaaatttagttttcccctcatcatgaccacacttttgtaaacagctcctgaatgaaatatctcttgaattatcaaatctgagcctgacattgattcccattgagaccctccctaatacaggagctatccagaatttaggccaaattatccttccacagcactgggttctaatcttcacgtcgaagtgaagggttatgaggatggagggatccatctggag

SEQ ID NO: 160 - DNA, 1001 bp, Homo sapiens
tacacttcaaaaggaagagggaagagaaggatgaggtgcattttctatggcaggaaacttacttgttgtttcccataatctagaggctgttgaaaggaaaacaagaatggaagatttaagaaataagaaaatcagaaaagagagagggagggagaaaagtgtgtctaataaagaggagtagctacagtggctcagttggtacagatagatcataactgctttcaaaaactagtccctgaaattgctcattaaatttcccaaattctttttagagcaaggtacgaaatgatacagattgagaaggatgaatcttgtactcctaggcatacacatatagacatggtgacacctatgcccaggtacacattcaaaacagatgagctggaccccattgggaaggaactctcacagtgcctgccctgccactagcgttcaaccgatgttcccagacttgatattaagaagaggtgaagaaagaattgtacctgaagatggagaccrtggggaagggtgggatggtaaaaaaaaaaaaaaaaaaaaaaaaaaaaaaaaaaaaaaagactagatggatgcaaaaagaaggggaaggggccaacacagaaaaggcagagttctggtgacacctctacctttctttcattgtaggtggagaggagtcttcgtccgataccaataagtcagcctgatgctctgtaagtttgctgggtcacatgccctgaatatttcaactttttctccactgtgacccgtggatgttctcagctggattaattagatctaatctaaagactcaatttctgtgtggtgggggttcacctccgcttttctggagcctctgagaaactcctgatcctgcacacccccttgtaaagcctggccatgcatcctgcaccccccatgacacagggagccaagcctgacatttttgagaaggtgccacctctgatccatcagagctgtagaggagggaagctggaccctggaagagactctaaagaaaa

SEQ ID NO: 161 - DNA, 1001 bp, Homo sapiens
agtgtgcatatggtgaatgcttattacaggaaattcatgagaaatgcacatgttatagactagagaatgaagtgtacctgccaatatgagtggatttattttatctagcaccaagagtagcaaactgagtaataattctcagtcatgatcctgtggttgtagtgtatactctgattcaacttagtttcactcctgactgagaagctgggactctgcatttgatggcaatggagtgggctgatttctttccaaataagttgaggtgggactcctggtagagtaagagggctttaatagggtatgtctgggtgcctaaaagctttctctctctttttttttttcagagacagggtctctctatgttgctcaggctggccttgagctcctgggctcaagcgatcctcccgcctcagcctcccaaagtactgggattacaggcatgagccaccacgccctgccctaaaaatgttcaaaagtcgtatttacagctactctcaaatycctttttttttgtgattccttataaaacctttctccctgcatttatcttgttatattacagtagaattatgaggggaaaatcctttggtggaagtctagggacatgctcagttcccaggaggcttaatgtgaattttagtgaattgcttaagatccagtattagatctgctggtccctgcccaccccccttttattttttgagacagggtctcactttgtcacccaggctggagtgtagtggcatgatcctgtctcactgtagcctccatcttctgggctcaagcaatcctcccacctcagtttcctgagtagctgggaccgcaggcatgcaccatcacgcccagctaatttttaaaatattttttgtagagatgaggtctcactgtgttgcccaggctgctctcgaactcccgttctcaagcgatccacccaccttggcctcccaaagtgctgagattacagccacggtgctcggctcccatcttgaaatcaatacctg

SEQ ID NO: 162 - DNA, 1001 bp, Homo sapiens
taaacgttactgaacttgcttcttcccgactacattaaagcacttacttgagatattaaacattttctcattagtcctgtttgcctagtcagtcacttgtatagacagggcaacagcacggcctgaatattgggcaggacaccgccctgcgcgatagtaactttgcccaacagcttgttgagcttctcgtcgtggatggcgagctgcaggcgtcggggggtgacgcgggtcttcttgtctcgggccgcgttgcccgccaactccaggatcttggcggtcaggtactccagcaccgcctccaggtacaccggcgcaccggcccggacccgcttggcgtagttgcccttgcggaggaggcggtgcactcggcccacagaaaactggagaccagccctggaagagtgcgttttagccttggcgcgagctttgctgccctgcattccacatccagacgcagtgaagtatttaaatacttgtttagaagaaggaaagtgattgatyctagtaaaacgcaagagctaaactcttataatctatattcggcaaagtagactgtgctatctcctgaacacagatttcagccaatcgaaaagcaggtgtttaaaaaaatttaaaaaaaaaaaaaaaaaaaaaaccacttctgacttacatacttatagttgaaaggtcaaattatgcaaggttgagcttctgggagagccgatgagatttaggagttcagaaatggcctatcatatattcagacactaaaagaaccaatgagaaaccgaaactcagccagcctcatttgcatatacacgaggtaaataatgagggcgtttgggctcaccagcattttcctgtggtcatttgacggtatcacttcggctgcgaacatgcctgaaccagctaagtcagctcccgccccgaagaagggctccaagaaggcggtgaccaaggcacagaagaaggatggcaagaagcgcaagcgcagccgcaaggagagctattccgtgtacgtg

SEQ ID NO: 163 - DNA, 1001 bp, Homo sapiens
gacctcagctcactgcaacctctccctcctgggttcaagcaattctcctgcctcagcctcccgagtagctggagctacaggcacccaccaccacacctggctaatttttgtatttttagtagagacggggtttcaccatattggccaggctggtctcgaactcctgaccttgtgatccgcccaccttggcctcccaaagtgctcggattgcaggcgtgggccaccgcgcccggcctccttggactttttatctgcattgcaggcactcagtggtccaggccacctacttctgctctacctttggacatcctggcaatgtgctgctcctcagcctgaccacaacacctgcagtgtcccaaacatatcatgcagtttcatgcctctgcacccatttcctctccctggtcaacacacctgggtgacccctattctactcactcagacaaaccaggacaggatccttgacctttctgcaactctatttttctcacctagaaataraattaatgacatctacttctttagcagatgtttaggaatgagatacggtgtggagagcacctggtgcgaacacagcgcgtatctgtgatagtgaccgttagccgttatcctcatcaccacatcctttccccacatctcagatggtgccacagtctaccacctcagagagaaaatagaaaagggaggtcccaaacttcctgctccaccacctatacctgtccctcatgatctgtttcctctgatttcaacaagcaggtgttctttctcctgtctcaggctaattctgcacccacatcggggagcccccaccccagcttccctcaggcttctctatttggtcaattcattaattcattcatttgacaaggatccatgaacgctaactatgtgccagtcactattctaggtggtggagtcacagaagtgaacaaaacagaaagttctcattcaaaaacaacataacttgtggtaggaggcagacaggaaatgaaataattagt

SEQ ID NO: 164 - DNA, 1637 bp, Homo sapiens
catttctttttgaaggggtcttgctctgttgttcaggctagagtacattggagtgatcatagctcactgcagcctaattttttttttttttgaaagacagagatcttgctatgcatactgcccaggttcttgaactcctggcctcatgcaattctcctccctcgatctttcaaggtcctgtgattacacctgtaagccctcgttcccggttggaagttacagtttaaaatagggtggttatgagcaaggggagcgaggcacagaatacttgggagaaaagcattccgagttgagagaacagcagtgccagagcacagaggcagaagcactgtggtttgtgtgaagaaaagcaatgaggctggggtgcgcagagcacacagggtgatcaggagaagaggaggtgacaaggccagagggggttgagggccagatcatgtatggccttgaaagtcatcatgctgacctgggctttacctctgagaggggagccactggaaggttagagcagaaaaaggactggactgacttatgttttaagaagttacttcacatgctagaccaagatgggctgtgggtaggggtggtggatggaggcctgaagacccagctgggagctactgcagtgatccaggggaaagatgcagatgacttgtaccagggaggagccatgaaaatgttatgatgctggatttattttcaagatagaataaaaaggctttgctgataaacttacaggtggggtgtgaaaaaggagggcatcaagggtgaccacaaggttttggtcctaagaaacggtacagatggagttgccacttactgagatggggaaaatgagggagaaaccgcttgtggaggccagaggaggagccagcacagaatccaaaggtcagttttgaatatgttgggtttgaggagcttactagagattcccgtggagatgtagagtaggcaggtcaataataagcttgcagtccaggcaacgggtcagggctggaaacacaagttattctctttgtcttctttatattcatgtttgttgccactgtgtgtttcacttacctaaygcattcgtgatttattgctgcataacaaattaccacaaacttagtggtttaaaacagtacacttttccagcctgggcaacatgatgaaaccccatctctactgaaaacgcaaaaaataaaagataaaaaattagcccagcgtggtggcacacacctataatccccgctacttggtaggctgaggcacaagaattgctagaacccaggaagtggaggttgcagtgagccaagattgtgccactgcactccagcctgggcaacacagcgagactctgcctcaaaaataaataaataaataacagtacacttttatcacttcagtttctgtgggtcagaagtccaggcagagcttagtgggcttctctgctcagaacttcacaaagcaaaagtattattcatgcatgtaaacctctaagcacaataccaacatcacggtaggttctatgtgagtataagctattattaagaataataatcaatcctcttccctctcctccatccctaaggcctcatcatttcttgcctggagtgtcacagtagctttcttcctggtctccttgtcttctaccatct

SEQ ID NO: 165 - DNA, 1001 bp, Homo sapiens
cctatcttgctgctgcttctcgccggagccagttacttcttgtggagacaacagaaggaaataactgctctgtccagtgagatagaaagtgagcaagagatgaaagaaatgggatatgctgcaacagagcgggaaataagcctaagaggtatccaacgcaagcagagaatctaagctcttggcttgcatgccccagcctgaaaacctcacctctctcccctaccctggcactgcatcatgtttaaggtttatttcccgaaacaccaacctcacccataacagttcatctttttttttttttttttttttttttggttattttccagagagcctccaggaggaactcagtaagttaccattcccccagagatccagacatgtcttcctatcctcgctttgagcaccttgatgactcttccctgttcattccattgcagagaggaaaaaaatccagtacttgactcgtgagtggctttgacattttctctgaattcaaatctrttactctctctctgcttcattattttccagcccataagtcatagcccagggttgaaaagtggtcttggatccctttacccagaaaaagaaaacaagtgtggctctttggagaaaccacccagtgctttttctctctagaaaaaaaaaaaaaaaaaaaagaggtcttcaatctctttgtactaggggctacagacccttaagctctaaaaagcactgaggaatatccaggggtacacttcaaaaggaagagggaagagaaggatgaggtgcattttctatggcaggaaacttacttgttgtttcccataatctagaggctgttgaaaggaaaacaagaatggaagatttaagaaataagaaaatcagaaaagagagagggagggagaaaagtgtgtctaataaagaggagtagctacagtggctcagttggtacagatagatcataactgctttcaaaaactagtccctgaaattgctcattaaatttcccaaattctttt

SEQ ID NO: 166 - DNA, 1001 bp, Homo sapiens
aactgctctgtccagtgagatagaaagtgagcaagagatgaaagaaatgggatatgctgcaacagagcgggaaataagcctaagaggtatccaacgcaagcagagaatctaagctcttggcttgcatgccccagcctgaaaacctcacctctctcccctaccctggcactgcatcatgtttaaggtttatttcccgaaacaccaacctcacccataacagttcatctttttttttttttttttttttttttggttattttccagagagcctccaggaggaactcagtaagttaccattcccccagagatccagacatgtcttcctatcctcgctttgagcaccttgatgactcttccctgttcattccattgcagagaggaaaaaaatccagtacttgactcgtgagtggctttgacattttctctgaattcaaatctgttactctctctctgcttcattattttccagcccataagtcatagcccagggttgaaaagtgktcttggatccctttacccagaaaaagaaaacaagtgtggctctttggagaaaccacccagtgctttttctctctagaaaaaaaaaaaaaaaaaaaagaggtcttcaatctctttgtactaggggctacagacccttaagctctaaaaagcactgaggaatatccaggggtacacttcaaaaggaagagggaagagaaggatgaggtgcattttctatggcaggaaacttacttgttgtttcccataatctagaggctgttgaaaggaaaacaagaatggaagatttaagaaataagaaaatcagaaaagagagagggagggagaaaagtgtgtctaataaagaggagtagctacagtggctcagttggtacagatagatcataactgctttcaaaaactagtccctgaaattgctcattaaatttcccaaattctttttagagcaaggtacgaaatgatacagattgagaaggatgaatcttgtactcctaggcatacac

SEQ ID NO: 167 - DNA, 1001 bp, Homo sapiens
gaaccacctagtcttcaggtttgcctggtgctcaccagctgaagaaatcctttaacgacctttattcagtcaagtaaattgttttcttttggcaacttgcatgttattttttaggttttcatttatttatttttttatatttaaagtcatattttcttccttttattcactttgctggtctttctcactttgatttttttttgccttgttttgcatttgtttactttaacattttttgtaacttatctcttttattttggaaattattcacattatcagttttcttttgctaggcaattttgatattctaataaacattattaacataaaatataaagtttactaacaccaagcccaaacaatacaaagtcttagggctctttaattgcaattatttaaaaatatttgctacaaattgttcattattttatatttacgttgtttttcttattcccacaaatcacatattgttggtgtgtttgttaaataaaaatctttaaytgcaattgtttaaaaatatttgctacaaattgtttgttattttatatttacgttgtttttcttattcccacaaatcacatattgttggtgtgcttgttaaataaaattgtgattgcttatatatattttttcacatcctttcttcttgtaatattttggaatttacatccagttaattatcctttattctatagtatatactgtaaaagttactagtcttgctagtaaaccctcagtttttggattgtctgaagatgtctctattttgatctgctcttgaattctaaatctaattgacataaaattctagatttgccattatcatttattagcctttcaaagatattccacaattttctgactttcaatatttttgttggtaaaaatggggattgttaatcggcttgcatattctgttttggatattccattgtttccttataatttgtttatttataaggaaacttataaacaaattataaggaaacaatagaatatcc

SEQ ID NO: 168 - DNA, 1001 bp, Homo sapiens
agccggggggtgcggagattgcagtgagccaagatcgcgccactgtactgcagcctgggtgatagagcgagaatccgtctcaaaaaaaaaaaaaaaaaaaaaaaaaaaagtgggaagcaaccagtggaaagcaatggtaagagcctgacaaatctcataaaatctcccattatttttttcttggtgcaagaaaaaagcaagtcattaaaaaggaagagaatgtcgtggtgactgtgatgggcctactttgtacttttcactgctctggggtgttcttgcctgtctaaaagaattttgacaaacgtgatacctaccacaattttttcagtggacatctaacgtttttcattaagtttaaatttttctgaaggatatagtgacttgtatcataggaatctaaaaaccacagtaatttaatacttaccagcaaccttttaaaagagagaggtgaacattgctacctctttaattgtggaagattttacattgatcctttatttytctgcattcatagtgccattgcctgtctcttatagaatttttatcccagtacaatgtcattttgtagttttttcttgatctttctatgatacttctttggaccaaatataggtataaatattgaagtccattgttatttcctgttacccaaaatgtgtgttaaaaatagtttttctggattgtgttatatttgcatctactgctagtacataatcaaaacataataggtaaataacaattttaaagcccctttactgaaaggtgtaatggaagtcaatgtggaatttgtcatcccctttcctccaagaaattgtacacaatatgcaagtccacctcgatggatggaggctctaacttagtattcccaattgtttccatgttgggagctcgagaggagagaatttttaggcctggagcaatgtgtcataggcaaacaactaccagaaatttatcaagtgatatctttccatggagtgccatcactgatttgattatcagac

SEQ ID NO: 169 - DNA, 1001 bp, Homo sapiens
agataagcaaaggaagagtcaggaagcaaagagggcagggcatgagcatggaaaaagcgccaatgtttaggggtttatgtgtaggaaaagttatctaatgccaaaagagagcgtttaatctccctttaaagaggtggccaaagatagactgtccacgaggggaattcttcattttagagtcataacagcaagccaagggcaaaagagacagatctcacttatctgtgaatgcagaaaacaaaacacgtcctttaatgtcaacgtcttgagttctttttcccaggttgactgactaaatatctcagtacagatacttttgcccccttccaaaacgcaaccacccatgaccccgacgtgatttgaacacgcaaccttctgatctggagtcagacgcgctaccgttgcgccacgaggtcacggagaccctccattttccttttaagataagtatctaatcttatcctcctcccaaacaatttctttattatttgatttgatctyttttcacagttttgctaaggcttttttgagaaaaataagggagtggctggattaaatattaaccccaaacccaaataaatgctccatatatgaaaaacagtggtttctcaagttcaatctttctatttctcgaatttctctgtttcgagaaaaagtgtctatgtgttgggtttagattagcagtgaaacagtaataagaacggttatgaagtttgtactactactttctgtaaatgcgctagactactccctcttcaggaagagaattccagcattgcactgccccgcaagacctggcctagctagcacttacttcactcaaacccatccgcacacccgccccatcctcaacctaatgggattcgaaagcctaacataaataatatctctagcctaaacgttcacttctcagtccaaattcgcgggccctctggtctctattgtgtacacaagccattcagttcacaacaataaccccaaagaatccgttaacatttact

SEQ ID NO: 170 - DNA, 1001 bp, Homo sapiens
gctgttggatgccaaatgtaatagtctaatcatgactctgaataaatgtgtctctttgaaaaatgtgctatgtaaagttagtctactctgaagccatcttggtaaatttccccaacattgtgaagggaattccttcagggtgatgccacattctatttggaatttgtatatgacctgcttgggtggagaagccattatcttcagtaaccttggtgtagttgaactgatagttactgttgtgacttgaagttcaccattaaaagagttcaccgggccaggcgcggcggctcacatttgtaattccagcactttagaaggctgaggcaggagaattgcttgaacccagaaggcagaggttacagtgaggagagatcttgtcattgcgctccagcctgggcgacagagtgagactccaactcaaaaaaaaaaaaaaaattaggctcaaggattccagaaataacatggaagtagatatctggctatttgactttcattctgggmtgggggtagggggttctttacagcctggggcaatgaaagtctcagctccctgttctgctttcttcgagaagtgtgtgtgtgtgtgtgtgtgtgtgtgtgtgtgtgtgtgtgtgtgtgtgttggaggtagagggaatgcaccttgttacagcttgatggaagtctagattccccactttgcctttgctgttgtgtgtgaaggtttggacgacagttgttttttttttttttttcctcttccagcttcccaagagcagaagtccgtagaaatggagtttgtaactccactgaacacacaaaattagctaaaaaaaaataacaagtcacaaaacaaaaattttaaaaatgtaaaacttttagaagtagagtcaggcttcggccgggcgcggtggctcacgcctgtaatcccagcactttgggaggccgaggtgggcggatcacgaggtcaggaaatagagaccatcctggctaactcggctaactcggtgaaaccccgtctct

SEQ ID NO: 171 - DNA, 1001 bp, Homo sapiens
cacttggtttaattttctgaacaatgcaatggttgatcaaaccaatttaaccaataaagcacatgtccagttctcctttttacgtttgtaactcgccagttcctttagcagaatgtccagatgctctatagaaatgaaatgaaatgaaaaaaacaaaaacaaaaaaccaaaaaacaaagaactctaaatgtggatgccagatcccaagatgcatagatgtacagatcccactttatggtcagaaaaatgttaatcgacaaaatgaatttgatgcatcttgagaaagctaattgtttggttttaatatattatatttaaccggaagtaacaaagtgccttttacatagcattctatttaattcatatatcacggagaaagtttttttccagaaaactgaatctttttcaaaatcaaataatttccttttatctgtacctagagaaagttaattatgtcatgactgataaacagaataaatgtggtcatggaaagtaagaatrcatcacacttactttctatatatagatgtttatatcgaacaagagcattactaatgtgttttttattggccatctttggaaaacgtgcagtcatttgctttaaaagattgtataatgtattttaaatctttattttcagctgggcgcggtggctcacacctgtaatcccagcactttgggaggccgaggcggatagatcacctgaggttaggagttccagaccagcctgaccaatatgatgaaaccctgtctctactaaaaatacaaaaattagctgggcgtggtggcatatgcctgtaatcccagctactccggaggctgagacaggaggattacttgaactcgggaggcggagattgcagtgagccgagactgagccattgcactccagccacttcagcctgggcaactagagtaaaattccttctcaaaaataaatacataaataaatatttatttattttctgcctgtccctttaggactatttttggagcaggcc

SEQ ID NO: 172 - DNA, 626 bp, Homo sapiens
agactacttgtgattcatgtcaaaacaaagtttaatcaagccatatttaaagagaccctacaaatcataagagaaagacctaacaactaagtagaaaaattagcacagaatactatgcatgtaacagaaaaggaaatacaaatggcttttaaacatataaaaaggtgctcaaggacaatataaccagttaaatgcaaaataaaactccctgagggatcattttcacatttcaaactggaaaaaacaagataaactctgttgagaaggactcaaccatgctcttcagagtgtgtgagagacagccctagctaagggttgggcttttcttgtacaatcatttggaaactatgaaaatcctggggagtggctcttatttcctgggaggtacctagaactagagtttcttacctgtggccttccggtcaratagcctcagaggttcagttcctggtggaattgaaaatcctggagtaggccatggatgtgagcggtggatatgagggatttttccttctattggcaatctgataggttgtggtagagaatcattcacacactactgcctgttgaggcgatttctttagatttgaagacaaaaaaacgtcagtgttaacgcaaaggggtag

SEQ ID NO: 173 - DNA, 656 bp, Homo sapiens
ggctgtatctcacttttagatatgtcttcagcatgttccttctcctttctccaaatgtttgcgtaactcctttcttactcatatcttatttggaaaggcatatcttacttgggaagaggaggtgacaattctcatgtttacttccaacaaattacctatcttccagtgaatagaaaatacactgaggttgaatataattttatattttcttgcactcgaaggcaaaacactgttactgacttttgcctgagaccattggttattgtaaatcgttattgtctttttgcttctacgggagcctcctgcttcttttgctcttttgttcatctctatgcatgatttattaaattcatttcgtgtactgtgaattcttctctaaagctatctgttacgatggccaaaagacatcatttataccctcctccttccatacttacagaaactagacacatggartgttatgagaaagagaagcaacaatgaagttaagtgtaaaatggttgattctacttggatagatttttttaaaaaatgtaaatggtagaaaacataggggtacatttaaagcattttgtgaatcagaattccatgggcaaactcagaagaccaataatctttattttgtctgcttaccttctagaagcattttaactaac

SEQ ID NO: 174 - DNA, 101 bp, Homo sapiens
actgcctggcttggaaaagttaagaagcccctcaggaagagaatcgaggcyaagttcctctgcgccgagggccccgagcatatccgccaaggctcagctgc

SEQ ID NO: 175 - DNA, 51 bp, Homo sapiens
  misc_feature (26)..(26): n is a, c, g, or t
ggtttttttttgttttttttttgttntgtttttttcctccttgcttggcaa

SEQ ID NO: 176 - DNA, 1168 bp, Homo sapiens
cactttccagaaggaaggtccctctggtgcaggctcactactaggtggcactgtgcactactgggctagttctggtaaaatacccctgccccagctaaagtctctccttccctccctccctccttccctccttctctcgctccctccctccttccttccctccttctctccctccctccctccttccttcccctcctcttcttccttccttcctcccttcctttctctctctctctttctctctccctttcttcccttctttctttttttttgagacggagtttccctcttgttccccaggctggagtgcaatagcgcaatcttggctcactgtaaccttcacctcccgcgttcaagcaattctccttcctcagcctcctgagtagctggaattacaggtgcccaccaccatgcccagctaatttttgtatttttagtagagacggagtttcaccatgttggccaggctggtctcgaactcctgacctcaggtgatctgcctgcttctgcctcccaaagtgctgggattacaggcatgagccaccacgcctggcctctttcttttcctttcatttcctttcctttctctttctctctctttccttccttccttccttctttcttttctcttttccwctttattttcttttaaattttaatttaatttaatttaatttacagagatggagactctctatgttgcccaggctggtttcaaactcctgggctcaagtgatcctcccacctcagcctcccaaagtgctaggataacagccatgagccacggtgcctggccagagcttcagtttctatggacaggtgttttcgggcttgctaaatcaaaattctccagaattcctaagatcagccaattttaagagcagtaattttttttttaacagtcttgctctgtcacccagcttggagtgcagtgatgtgatctcagctcactgcaacctctgcctcccgggttcaagcaattctcgtgcctcagcttcccaagtagctgggattacagccacgcaccaccacgcccagctaatttttgtatttttggtagagatgggtctcaccatattggccaggctggtctcaaattcaagctgtctgcccatcttggcccccagagtgctgggattacaggcgtgagccaccatgcccggcctga

SEQ ID NO: 177 - DNA, 701 bp, Homo sapiens
atgtggaagaaaggtggtcgaaaatgaaatttacaggtgagttcctaaaaggcctacccttccccatgttgagttaagtgtcaaaacatttctagggagatgactgtggtaaacccgcggggcggtcagaggcatgcctgagagggggccgtgagaactcagcagaaagctgggggagtgctgtctgtttcaggttgagcrccatgtgttagcttggtgggagaagagggggcatgagcattggttttaatgtgtaaaacctccggataaattttttttttttttttgagatggactcttgctctgtcgccaggccagagtgcagaggcgcaatctcggctcactgcaacctctgcctcccaggttcaagtgattctcctgcctcagcctcctgagtagctgggactataggcacgtgccagcacgcccggctaatttttgtagttttagtagagagggggtttcaccatattggccagaatggtttccatctcttgacctcatgatctgcctgccttggcctcccaaagtgctgggattacaggcatgagccaccacgtcctgccctcttaggatgaatttttacaaattaagtttttattttaccaaattgatttttaaacattcccctttattcattttatttttatttcatttttttcattttatttttatttattttttgtttgtttgtttgaggt

SEQ ID NO: 178 - DNA, 1001 bp, Homo sapiens
ataaagaatcaacaaggtttgtccagctgtcttgagcaatcccactgatctgctcaggaaataccacatttcactcattagatgtggctcaatcgatcaagccactcaggcctgatttgaggctccagttcacagtgaaatggtccctgcactcttccatcacccttcaataggtcaactcacctccttccctgtcagtcaacacaagagagtgagctcggccgcaggagacctgcagcacccgtgtctcctgaggtctgtccagaggcagggagacgggtgagggctccaacacatactcgtagcccctcgctggaaaagacacaggacactgattgaggcatgcatttctaccactggaaatcatactgtccaactccacgctactacactggaaaaaagagagtcggaggtaggaaagactcatcaagacaggtaagttaggcgcagagcaaggaccagaagcccaactcccagcccatggcatgggctgtctctatyacataatgcgggttccagaaaagcatacttggtcttctggctgggcgcagtggctcatgcctgtaatcccagcactttgggaggccgaagcgggcagatcacctgaggtcaggagttcgagactagcctggccaaaatggtgaaccccatctctatttaaaatacaaaaattagccgggcatggtggcgggcgcctctaatcccagctactcgggaggctgaggcagaagaactgcttgaacccggaaggcggaggttgcagtgagctgagattgcgccattgcacttcagcctgggggacaagagcgagacttcatctggaaaaaaaaaaaaaatgcatacttcgtcttcttattaaagaaatcttggccgggcagtggctcatgcctgtaatcccagcgctttgggaggccaaggcaggcggatcacttgaggtcaggagtttgatacccacctggccaacaaggtgaaacccccgtctctactaaaaatacaaaatt

SEQ ID NO: 179 - DNA, 1449 bp, Homo sapiens
aaccccatctctactaaaaataccaaaaaaattagccaggtgtggtggcaggcgcctgtgaacccagctacttggaaggctgaagcaggagaatcacttgaacctggaaggcggaggttgcagtgagccgaggttgagccactgcactctagtccgggcaacagagtgagactccatctcaaaaaaaaaaaaaaattaagaaaaaagacaagaggccaggtgcagtggctcatgcctgtggtcccagcactttgggaggtcaaggtgggcggatcacctgggatcaggagttcaagaccagcctcaacatggagaaaccccgtctctactgaaaatacaaaaaaaaaaaaaattagctaggcgtggtggtgcatacctgtggtcccagctactcgggaggctgaggcaggagaattgcttcaatctgggaggtggaggttgcagtgggccaagatcgtgccattgcactccagcctggacaacaagagcaaaactcagtctcaaaaaaaaaaaaaaaagacaagagaaaatatttagacaggtaacgaagggttttatgcaaatatatcaagtactcctacaaagtaataagagacaaacaatccagtatgggtgcggtggtggctcacgcctgtaatcccagcactttgggaggctgagacgggcggatcacctgaggtcaggagttcgagaccagcctggccaacatggtgaaaccccgtctctgctaaaaatactaaaattagccaggcatggtggtgcacgcctgcagtctcaggtacttgggagactgggacatgagaatcacttgaacccatcaggcagaggttgtggtgagccgagatcggaccactgcacttcagcctgggcgctgggccacagagtgagactctgtctcaaaaaaaaaaaaaaagagacaacccaatagaaacgtcaccaaggatatgagtagatttgcaattctcagtagaggagacgtgaaactgtaagatgttcaactyttccagagattacagaaatataaagtaaataaaaaatgagatatgtttcaagtagcagattggcaaacatttaaaaaacgtgggcggggcacagtggcttatgcctataatcccagcacttggggaagctgaggcaggaggattgcttgagcccaggagctggagtccagcctgagcaacatagagagacccccgtctctgcaaaaaattttagaaatgtccaggtgtggtgaggtgtgcctgtagtcctagctacttgggaggctgaggtaggagtatcacgagagctggcaagattgaatctgcagaggctgcagtgagctacgatggcaccactgtactccagcctggttgatagagtgagaccttgtctgggaaaaaaaaaaccaagtcgtgtagcagggggatatgtaaaagcaaatcccactcataatattgaagcacaact

SEQ ID NO: 180 - DNA, 501 bp, Homo sapiens
ggcctctcaaagtgctgggattacaagcgtgagccactgcgcctggccaaataatttttaaaatttgccgggtgaggtgatgtgcgcctgtgatcccacctactcgggaggctgacgtgggaggcttgcttgagtgcaggaggttgaggctgcagtgagctatgactgtaccactgcactccaacctgggtgacagagcaagtccatctcccctcaacacacatagcaaaaaaaaaaaaaagagagagagwgaaagtggtagaatctgggcaaagttagagctgccggaggaatctgaaggaatggtgtggagcgtgggaggaataagatgcttccaaggcttctggcttgagtaagtggaggaatggagtttcattcattgagctggagaagactgcaggagaagtgtggggagcgtgagacatgttcttcttgggatgcctattcattctccaagataaaaattttttttcttaagtcgctgtacaagtggagatttca

SEQ ID NO: 181 - DNA, 601 bp, Homo sapiens
ttattattcactgaaccccttctgtaatccactctgatgtctattttagactgagcttgggtgtatgattgtcatttgtattagggcctttactaaattcctataactgtatcaatcattcttctcaactactcccccctcaaaaaaaatataggctagggtatttttatttaatgattttattctactattgtttgacctacactatggagacacagacacactgaaacacatgcatccatgcatacacacatttgttttaaattctcttccagtttatgtatcagtgaccttgaacaawgtcacctagattctgtgtttcagttttctcttctccaaataaaagaagttactttacataaatttgttgggattcaatgaaatattatttagaaatgtgctgtgtgtggcatatatgtctaaaggacagaattaatggatatatatatatatatatatatatatatatatatatataggaatgtattaaatactcacatgatcacaaggtcccacaataggccatctgcaggctgaggagcaaggagaaccagtccgaaaaactgaaggatttggaatccaatgttcaagggcaggaagc

SEQ ID NO: 182 - DNA, 549 bp, Homo sapiens
ggatcaagaagttgcagtctgtgtcctaatttccactccctgccatgggtgcggaaccttgagcagtagattgggccctattggggacatctggatggtaacacagactccaaaatgcaagggctaatgacccatcccctagtccgtgggagactgcaagtctctggggcattttgggctccccgaattgtctctatgtgcccagaccacttacagcatgatgtctggacacaggattcaggcatcactatttggaaaaaaagccatctcagtggattccaatatggcgccaaagtcaagaaccactgctcagcggattccaatatggcrccaaagtcaagaaccactgctctttgagaagtcagctcaaggtcacatccaaggtggcacaggagagagagggacagagcacagcattggaggaggcaggtggctagaaaggtgggctctgaggcagtactctggccctttccagaacgtgtgtgtagaatgcagaaatcttgaggaccacatgttccaggaggagagtggtgaggaagtggaagaata

SEQ ID NO: 183 - DNA, 601 bp, Homo sapiens
gtgccaaaagaagaactcaaaatccctgtctctcacctgaaaatgatacagaagactggacctaggggtgaggcctctgcaagcggggattggagaagcctgacctcaaatctagaagatcctataatttatattgcataatcacaggtcatagactcagccacactgttgggctgtaggaaagcattggtttacttccaagcaaagagggatgcctgtgaagagccagcagtccttccattcctgattttcctccttctaccaacccacaggaacattcctaggctgccccactctgaayccagtgttccttctgtaagaaaggccagatatgactgtttattttcaggatgcatgctaacagggccgccaggaaggtatctcagctttcatgccagaaccaatagagtattccccagctggaatttagagtgatccaggcctgaaatctcactttcagcaataattaaaattttattagtgcttcagaatttaagatatgtgtttctcattcaccatttcatttaattatcatgacattatattgttatcccacttacacagaagataaaactggggttaagagaagttatgtatccaa

SEQ ID NO: 184 - DNA, 401 bp, Homo sapiens
cccctatccacaacccacagggataaacagggtaaagaaaggaggaccagagcagaggtgggtgtggcttcagtagaactcagcttatccagaaaccaagctgaaatttcagccacactctgtgggtttccccagaatttgtcttctgaacactctataaatcccagaagactgaagggcttcctattgaatttcagttgycccattggactcaatatttttattgagaatttaatatttttattgggtccaatgggacaactgaaaatcagtatttttgggatattttgggaaactcatcagccaaggtcctaaggcctggccaggtcatgagtcccttctgattagatgatcgttactcacatcttagagaccattcccactttagagaggagtaacta

SEQ ID NO: 185 - DNA, 1001 bp, Homo sapiens
agtcacccaaatgctttgtgaagatccatgtttcttcctcgtgggctgttcacagttaatttgtgatcccatcttcatctcactcatccgcccattcactcattcaatgtgtgtgaatgccctccataaatttgtactgtgctagtcactgaagtacagagctgaataaaacaagactgcttctctcaaggagaggagaggataaaggatataaacaaataattattttggaaaggatcttagtctacctctccagcttttactaacaccatgatgaactctgccccccactacagtttcacgctgcgtttcacactatgttctgcaagcacctgatgacttgaagcctcacaaaggcatcatcctttgccttcaagatgtggcctctgtttctcctttcactactggtgtgctaccctgccctctcttcccagttaattcttactcatccttctaggctcagctcaggtgtcagtttatccaaaaggtaacaatgatgtmtcctccccataggttatgtgtccctcccatcagctcccaaagaatgtctcagattttcccaacacacccttcacacacttaacattgtaattatctggatatttttctttctcgtttactatattgagaaggctaagagggaatggagtcacgttacaattgttttggagcctagctcaatgcacaacgtacaagtgctcaagaaatgtggaaagaagaaattaactgtttttgtataaaggagggagaggtcaattctggagtagggaatcagagagggcttcacagaaactattgaattgaatcttgaagaattaacgtaaattcaccagatggacaagtttcagaaaaaaactttccaggaaaaacaaacagtacatacaaaaccaaaaagaaagaaaacaaacattcaaagaaatgtaagtatttaacatgtctggggtataaattgcgatgattaaaatttggctatgattaagaagttcaccctcaccaatgtg

SEQ ID NO: 186 - DNA, 1001 bp, Homo sapiens
tcacccaaatgctttgtgaagatccatgtttcttcctcgtgggctgttcacagttaatttgtgatcccatcttcatctcactcatccgcccattcactcattcaatgtgtgtgaatgccctccataaatttgtactgtgctagtcactgaagtacagagctgaataaaacaagactgcttctctcaaggagaggagaggataaaggatataaacaaataattattttggaaaggatcttagtctacctctccagcttttactaacaccatgatgaactctgccccccactacagtttcacgctgcgtttcacactatgttctgcaagcacctgatgacttgaagcctcacaaaggcatcatcctttgccttcaagatgtggcctctgtttctcctttcactactggtgtgctaccctgccctctcttcccagttaattcttactcatccttctaggctcagctcaggtgtcagtttatccaaaaggtaacaatgatgtctyctccccataggttatgtgtccctcccatcagctcccaaagaatgtctcagattttcccaacacacccttcacacacttaacattgtaattatctggatatttttctttctcgtttactatattgagaaggctaagagggaatggagtcacgttacaattgttttggagcctagctcaatgcacaacgtacaagtgctcaagaaatgtggaaagaagaaattaactgtttttgtataaaggagggagaggtcaattctggagtagggaatcagagagggcttcacagaaactattgaattgaatcttgaagaattaacgtaaattcaccagatggacaagtttcagaaaaaaactttccaggaaaaacaaacagtacatacaaaaccaaaaagaaagaaaacaaacattcaaagaaatgtaagtatttaacatgtctggggtataaattgcgatgattaaaatttggctatgattaagaagttcaccctcaccaatgtgaa

SEQ ID NO: 187 - DNA, 1001 bp, Homo sapiens
gtatatgtggaggtggggagacagaaacagagacagagagagagagagagagagaaatactgagacctagaaagcttgaataactcatttcaagtcaagagcaacttaatggtaaacttggatcaaaacacaaaacactattctttttagtcctgtattgtttccactatatcacaatacagtgttcaatagttctctttaaatcacataccaggagctaaatttactgaagtattacaaaaccaccaaatgagctttcacaggagacctaaaagaggaaattaaagatgcaaatagtttaagaaaaatctgtgtttgattcagaaacttaaaaccagtttcttcaaaaacttgttaaaagagaaagaaacaggcatttttacccaaagaaagaaataccatattctagagattcactaaataatttttatgattctctatgctactttcaagaaactctgacttcagttatgtagactaaggtgacaagaaccatttatrtaatcaactgtaattacatgaaattctctctttagcacatggtacccactgaatgtggcacaaaagaggatatgatcagttgattcaggatgatgtcatttccatgattctaaaccaagaatcttcaagaaagcctgggctgcaagttccagggtcaaattgcagactgcttgcagagagtggctctgctattccaagaacctcagatggctcactggagtgatctgctttagatagtgtgatcatatgtcttgaaatttccatgacagtcttgtttatacatgttgctccagaatatttattatagtgctctctttcacaatcagaggtgttccgctttgaatggtgagttataaaatagttaccctagccatgtggagtgtgctcgctcacttaacattcaacatgcagtaagccactttcacacatggccctgtgctcacgacttaatagaggttattaggcaaacccagcttcactctgctaaaggtattttattt

SEQ ID NO: 188 - DNA, 1001 bp, Homo sapiens
caatcagaggtgttccgctttgaatggtgagttataaaatagttaccctagccatgtggagtgtgctcgctcacttaacattcaacatgcagtaagccactttcacacatggccctgtgctcacgacttaatagaggttattaggcaaacccagcttcactctgctaaaggtattttattttaaaattactcaaagcctgtctgaattccaccctaactccataacagacattgggtgccttcaggaaattacttagcttccctctggtttattcatgtttactatgaaatgggaataattgcatcagtcttaccacaccaggtaataaataatggtcgaggaagtaattaggcttagaagctggatagaaactaagatgcctaagtactaattaggaatacagctgagtagattgtggttgatggccgtccaaatgaatatgtcacctctaatttctgccttgtttcttgtcttattttaattgtatctatcttctaagygtcttatctttacaaagtaccaatcctgaaccaacgaggttagatgcttaatttttctcgtgttttgctgggcatttgctggctctaacagcaaaggggcattaacctaaccaaaaataaaatggtttcatatcattataaaaattattctgtcagtgtgaaatgccataacaaaaaagcttgtatatgttgatgtcatatatatatatttatatttatgtattcatttattcttattttacatatatagttatttgtggataagcagttttggtgaagaatagctagtatgtttttgagtagtgtcaaggcctatacttttgagctattttctaactccaaacagatctagaatcaattaacctttaccaagggcctgctatatttcagggtctggactgaacagacgattatgtcattgaatcttcattgaattcctgcataatggatattctgattctcattttgcaggtgagttacctaaaatttagaaagaaaaa

SEQ ID NO: 189 - DNA, 401 bp, Homo sapiens
agtcctggattctgagtgcaaagtatagccttctctgttcttgatgctaccagactgtattcaggaacacttaagagaaatgatggaagtcagagctgaaagctgtgtcctcgccagatcagtggaagggcacgacaatcattcagctaacgaaggaaactccttggctagccatgagttcattataaccaaaagtgggartgggcaggatggggtgttgagggatacatgaattgttgagcaactgctttggaagggcaccaaacttcatgtttgttcccttgcacacttgtcctttccataattcatagaataattctatctaaaggttaatatagaccttgaagttctcctagcccagcccccacttcacgtttgaatgttttctatcacatctcacc

SEQ ID NO: 190 - DNA, 401 bp, Homo sapiens
ctatcacatctcaccaaacatcatgcctgggtaagtccaggaataaataactcattgcttcctgagccatcccagctcattttgaggcaactctaactatttgaaaaaccatcattcatttattcaataaatatttattaaatgccaactaagtgcccaagcctggttttagatgatagaaaaaaaaagtaaacaaacaarcaccccgcacgcccccaccaaaaaaatccctactttcatgaagtttgcttttcttacactaagccaagctaaaagttgatcttacctaaccttcttcctcactgagctacttacaaccctctaggtcctctcattaggcatgggaaaagtgcttagttcttctcccatgtaaatatttaaagacactggtagtaccccgt

SEQ ID NO: 191 - DNA, 1001 bp, Homo sapiens
cacatctcaccaaacatcatgcctgggtaagtccaggaataaataactcattgcttcctgagccatcccagctcattttgaggcaactctaactatttgaaaaaccatcattcatttattcaataaatatttattaaatgccaactaagtgcccaagcctggttttagatgatagaaaaaaaaagtaaacaaacaagcaccccgcacgcccccaccaaaaaaatccctactttcatgaagtttgcttttcttacactaagccaagctaaaagttgatcttacctaaccttcttcctcactgagctacttacaaccctctaggtcctctcattaggcatgggaaaagtgcttagttcttctcccatgtaaatatttaaagacactggtagtaccccgtttggccttgtctttttagttcctacatttatccatagttacatgttttcaaggctcttcactacaccggctccaaatttctgggcttgttctgcttcgttgttsttccttttcaagtgcaatcctcagaagttaatcagctactccagatgagttctgaccagcacagaatatagcagcggcatcattaccttgttctagttctcggatgtccattaatacaatctgagtttaagttgccatttttgatttcacaaatcactgctgatgcacatgaaactcagctaattttttcaaccctgttattatgtaagatacttacttagattggaaataggtccacagcaaccagcaacaaccacactgctcatgagattctcctgaaaaacaagctcagcctccctcaaagagagctacgggacattttcagccagcctgaagaccacaagtgtgcctggtgccagccagaattgtcttccattgagagaatttgcagattctagtaaatctcaagtctaaacctcagctaaattatttagaaacaatgagcaagggcagctctaacttggcccaatatctgcaataataaaagttaatacattttg

SEQ ID NO: 192 - DNA, 1001 bp, Homo sapiens
aatcccttgcccaaacttagacagattttaagggcaagtaggactcaaatatagatgagtggactccaaagcccatgtacctaaccactctaatcaccagacttctcattttcattgctaacctgtcaagcaatgttgcttgagagggaaggagatgcattcccccaacacattattctttctaaattttttaagaaatgttaataatcaagcttagaaacaagcaaaaaaaaatgactccacagacatattagcttgggagggatcaagttggtttctcccacaggttctgagaagcagggaggctatctgggatcctctcataaaaaatccttctgattctgattctgatgtccacctcacaagtcaaatggggaactgagcttgacaacaaatagccgctttcttatttctactcctttcccataattttcaacaggagatgactatgttttatctaatgatctgactctgtggagtggtctctaggttgcacccccvccccccccgagtgtgagctaatggaaatgttttggagaccactgatccaacttgctctagagttagggctggccccctccatccaaaacactcaagggccctgatatcttagtctgctcagtacaaagccacacaatctgactctaccctgcccaggcaatagtgcagtcctaaacactgtcctctgacttcaggtagctcatgtaccagggagagacctttcaaagaccggtgagaatacccaactgaccagtgattaagaaagggaaatttcagattcttgcacagtgaatacacagttgagccaagtacagaattttgattttctcctctctgcttatggataattcattcttttatttcttcatctatatgtgaaaatttgttttccttatattttctgtgttgcttctattcctatcaggctttcctgtacacactgtgtaactccaacagaaacaacctgaactcctaaggatacaattgaaactattagtttg

SEQ ID NO: 193 - DNA, 1001 bp, Homo sapiens
tcccttgcccaaacttagacagattttaagggcaagtaggactcaaatatagatgagtggactccaaagcccatgtacctaaccactctaatcaccagacttctcattttcattgctaacctgtcaagcaatgttgcttgagagggaaggagatgcattcccccaacacattattctttctaaattttttaagaaatgttaataatcaagcttagaaacaagcaaaaaaaaatgactccacagacatattagcttgggagggatcaagttggtttctcccacaggttctgagaagcagggaggctatctgggatcctctcataaaaaatccttctgattctgattctgatgtccacctcacaagtcaaatggggaactgagcttgacaacaaatagccgctttcttatttctactcctttcccataattttcaacaggagatgactatgttttatctaatgatctgactctgtggagtggtctctaggttgcacccccccbccccccgagtgtgagctaatggaaatgttttggagaccactgatccaacttgctctagagttagggctggccccctccatccaaaacactcaagggccctgatatcttagtctgctcagtacaaagccacacaatctgactctaccctgcccaggcaatagtgcagtcctaaacactgtcctctgacttcaggtagctcatgtaccagggagagacctttcaaagaccggtgagaatacccaactgaccagtgattaagaaagggaaatttcagattcttgcacagtgaatacacagttgagccaagtacagaattttgattttctcctctctgcttatggataattcattcttttatttcttcatctatatgtgaaaatttgttttccttatattttctgtgttgcttctattcctatcaggctttcctgtacacactgtgtaactccaacagaaacaacctgaactcctaaggatacaattgaaactattagtttgct

SEQ ID NO: 194 - DNA, 501 bp, Homo sapiens
acagaaacaacctgaactcctaaggatacaattgaaactattagtttgctataacttttctatttgatttaccaagatactctccctatagccaaaataattatatagcaatctatgttgtagcaaaaggaaataaacaacggtgtttcttaaacacttacatagagagtttagatgtattttttaaccttcttttctctttttcatctaatttaaggtgagattccaggatctttctcatgaaagatccycagagaatgtgcctgctaaacttgatagagtcacaaagctaggttacaaaagagagcaaattaaatttagacccaaaagtgttgataccacatatactgacgcatttcttcaacagttttcctttgtttatttattcagggcactagagaaggtgctctaatcttttaataacagactcaatctgccattgtcaaaattatcaacaaaaataataaaatgggttaaatacaaccacaaaaattcactgtg

SEQ ID NO: 195 - DNA, 401 bp, Homo sapiens
agtcagtaaaatccagcaagcacaggtaccaacattataaagatgattcatacatggttccaggcttcccaactagtggaagaggcagagctagaaacagatgagttcaatgtcatcttttaaaatgatggttattcataggatgcttggaaatgcagaggggcactaaatatttatgctcaataaatagttgtggcctcvctgtgtgggagtgtttggagatctaaaggtagcatgagatgtacaaatgtggagtttagttttaaagagaccaccaagaattgcttcatttatgagtggccctggccctgccactgattagctccatgaacttgagcaagtaatccttctcagaatgtttcttttgttgataaagttaggagttgcatgataatgatgtc

SEQ ID NO: 196 - DNA, 501 bp, Homo sapiens
ttttatgccagatggctttattatttccctggttccagatccctttccctcttgcctttcacgccctgtgccctagggctgtatggtgtgtacccctataattctcccagcctgcagggcaaaatgtaaaaacttcaagcctctttttcagcagacagaagggagggtcagggcaggatctcggtaggttttgtccaagcagtcggctcactcttaagctggcctgaggcagcagcacctccttacgctcvtgtgcagagatccagccctcccagtgccccgctttgagtcccagggcttttctcagcccttgcagccagctgagccacttctaccactcccaccagcttataagagaaagagacttcttctgtgctatgtctaatattatcaggtccattttgaaaatgagactaacatagccacagctcctccctccaagggagactctcatagcactattcaaattgcatgatgaatcaagccctgctgaactgcatt

SEQ ID NO: 197 - DNA, 1001 bp, Homo sapiens
aggtgttcctcagggcccagtccatgacacatgcttttccatattaatgtatggaaaatactcctgtagatttgagcagctaccattgctttccctagccctttgctcagaagtaggcaccagtccactggctgttgggcaaaagcctgctgagaaatccaatgccttggccaaagatgctttgaagaaatagtaagtgaggcagctctgacctcttcttatagaactccctgattcataaaatcaaacagcaaagactcctagagaccactgagtccaagcctcttcattttatagaagagaaactgaggtccatagaagcccatttttttatagaatgagaaggaaagtgacttgcccagggctcctgcttacagtagagttgggactggcatttacatctccttatcctttacttagtcctcttcgtaataaacagcgaaacactcaggggtccttccttcctctttccaaaccctggaggagctgagggggagacaygggggctttactcctcgtgttgtttcagactcagacttctcagcttccacattgagagactatttgcaattgcttctccttgttgcccaaattcctggctggcattccagactgacaccagagacttccttcccagggacatccatcctgggcaggtcagcagtttgcatcttccctggggcagaagtggcagagtctcagaactcttgcttcttaagactcagctcaatctccacctgactcagcagaggtttctggaatctcagatgggtcctaaccagaagcagctaggttgcttctctgtttctataatgagaaaacaaaaaaaaaagctgactatgaccattgagaaagaaaatgcacccatgtaaacacagcaatctttaccctataaataaccctaattaaaatgaaaacacccgagtgctcccatcttttttgattttttctttctgctggacaccatgggaggtccttgcagcagagctctggtgcttgcc

SEQ ID NO: 198 - DNA, 1001 bp, Homo sapiens
ctatatctccaatctcctcttctatccgtctccctctcttaatcagtttttgataatggtggcctgatgttctttcctaccacagtccccagcaatcttcacacacacactgtttcttcagcctgggattctcttcaccatctctaaaatgtaagcagctcctacacatccttcacttacagagacaccgtatcttccacacagacactcctcggtcatctccagactaactcgctgctagtgagcaactgcaacttatgttcccatgtatccattcaatcttctcttaataagcatattccctcatttctgggggactctctgtccctcgctcttgaaccacatctcattttggtgaggctccacatggcacaggcttatgccaaatggtggttggtatgaagatgggttcattacacaatcatactttttctgaggatgttggaatcaacatctcactttttcctactgtcttggagctgggatgtgagctgtaatgchgctgtagctggaaccctctcaaaatggcattaacacagtagacgcagagctttgaaatggagaaagagaaaccagatataaatggctatggaattactgttgccagggaagcctgaaggcttcaacttataaaattcctcttcttcttcttcttctttgtttttattttcgattaaagcagcttgacttgagttttctctcatttttaaaagaaaaattctccgttgcacactttgagcaccctgagtcttctcacattttggcattcacgacaagggtaagcatttgttcaatttctatctctttcatactagattggaaattccatggaagttggaatcctatgagtcttatatatcactatttctctcgtttctagtacaatgtggagcacataatgaaatatcaataaaatatttctgaatttaatgaatgaatgaatgggagattctgagatcccaacccctatcaggccttttgttccatgatcctgatctgaa

SEQ ID NO: 199 - DNA, 601 bp, Homo sapiens
tactttttctgaggatgttggaatcaacatctcactttttcctactgtcttggagctgggatgtgagctgtaatgccgctgtagctggaaccctctcaaaatggcattaacacagtagacgcagagctttgaaatggagaaagagaaaccagatataaatggctatggaattactgttgccagggaagcctgaaggcttcaacttataaaattcctcttcttcttcttcttctttgtttttattttcgattaaagcagcttgacttgagttttctctcatttttaaaagaaaaattctccrttgcacactttgagcaccctgagtcttctcacattttggcattcacgacaagggtaagcatttgttcaatttctatctctttcatactagattggaaattccatggaagttggaatcctatgagtcttatatatcactatttctctcgtttctagtacaatgtggagcacataatgaaatatcaataaaatatttctgaatttaatgaatgaatgaatgggagattctgagatcccaacccctatcaggccttttgttccatgatcctgatctgaaaaaagtgaatctagttcccagtgc

SEQ ID NO: 200 - DNA, 601 bp, Homo sapiens
tcttggagctgggatgtgagctgtaatgccgctgtagctggaaccctctcaaaatggcattaacacagtagacgcagagctttgaaatggagaaagagaaaccagatataaatggctatggaattactgttgccagggaagcctgaaggcttcaacttataaaattcctcttcttcttcttcttctttgtttttattttcgattaaagcagcttgacttgagttttctctcatttttaaaagaaaaattctccgttgcacactttgagcaccctgagtcttctcacattttggcattcacracaagggtaagcatttgttcaatttctatctctttcatactagattggaaattccatggaagttggaatcctatgagtcttatatatcactatttctctcgtttctagtacaatgtggagcacataatgaaatatcaataaaatatttctgaatttaatgaatgaatgaatgggagattctgagatcccaacccctatcaggccttttgttccatgatcctgatctgaaaaaagtgaatctagttcccagtgcctagacttgctgttctgttatggaaagatctctattagggagcattc

SEQ ID NO: 201 - DNA, 601 bp, Homo sapiens
ggcaataaaggcaatagtttaatcttcaacctgtggaatccattggctatcccttagctggttataaacaaaggtaggaaaaaaatgggatactacttattttccttgtgaagcccaacatatggttggaaacatttagaaatagaaaaggattggaatttggtaaattaaatggcatttttacctcaaggcttcctgtggggccttgattataggcatgaggctatagattttagcaactaggtattgtgggattttgaccctatgtcacggggttggttcctatatctgtgtggctggyttttaactagtgcacttgtaaaggccttagcctttagaagtaaatcatatggcattttgacttttataagtcactagagttaacggcaactttgtttgcaaatgataactttttgtaacattcagaaatctaagcaaatgccaactaaatggggtgaggggcttagtaaacctgtgcaagccatgttatttctggcaaggatctgatcaaaggaaaagagtcttcctgttacacacatttaggcactgtggcagaacagggaggagccgagggatatccaggaaggggtgccgcagaaga

SEQ ID NO: 202 - DNA, 601 bp, Homo sapiens
gtggctggtttttaactagtgcacttgtaaaggccttagcctttagaagtaaatcatatggcattttgacttttataagtcactagagttaacggcaactttgtttgcaaatgataactttttgtaacattcagaaatctaagcaaatgccaactaaatggggtgaggggcttagtaaacctgtgcaagccatgttatttctggcaaggatctgatcaaaggaaaagagtcttcctgttacacacatttaggcactgtggcagaacagggaggagccgagggatatccaggaaggggtgcmgcagaagagtcgtttgctgtttgaactgtgtttctcagtcaagaaaggagttctctattttaaacttcaaaggtagctactttgcgtttgtgctacagagcactgttatatgtgagatgctagctttacacttttaaaccaagaatagttagtccttgattaagtacccataattttgttcattgttgatattattttgaacctcttttagagcctggagaggaggtagggaagaaataactttgaattcaagtggtttatccacagatccaagagtcaccacagagtaaattgctttag

SEQ ID NO: 203 - DNA, 1001 bp, Homo sapiens
ctggagtgattcccaagtggcacctacaacttcacctgtcttgactttttctggtctttttctcctgattttgtattttcacttttgtttctttacttgaccaagtttggctctgggtatgatttatctgtggctgatgtggtattccccatagacggcaacaatgattgagaatctggttttgtcatctgtccatttggtgatctcttggataacaagaatctagtctctctaaggtgagaaacagtagataatgtggttaattaatttttgtttgtctttttgtctacccatgagctcaaataaatattgtatgtcttccaaaaaggataacaaatctttgagatccagcccggtgagtgtgtttttgtgtttactttgactcatgtctgaagttatagaactgaagccatgggctctctgtatatctgtaagtgaagaaagcctttacctctcagtacataaatgtgaaatattcttctacctctggagtgtattaakaaattatgtcacaaagtattttaaattatgttctatgttgtaattagcttagagagaatacgtgcttaaatgaatctattattttcccagaattcagaatattttcctagaaaataaactaaaattttaatattttaaatatattttaaagactatactttaagtattttttaaaagtataaaaagccctttttataaaaataattagcccaaaagcatttttatgtaaaaatccaagtttactgaatcaaggtgaaatttttgttaggtcaaactggtttgtttggccattttgtttcaaaatagccatatatatagttcccctgatcttattagtgtattaagcgtaagtatatattttagttttataagatttgaggtgtttcctgataaagtgactagttattctgaacttcctaaatttcttatattgacttactgatcaaattagctaatatgacttctacataatcatgattgtgaaaattgtaaaattatgt

SEQ ID NO: 204 - DNA, 601 bp, Homo sapiens
tataaaaagccctttttataaaaataattagcccaaaagcatttttatgtaaaaatccaagtttactgaatcaaggtgaaatttttgttaggtcaaactggtttgtttggccattttgtttcaaaatagccatatatatagttcccctgatcttattagtgtattaagcgtaagtatatattttagttttataagatttgaggtgtttcctgataaagtgactagttattctgaacttcctaaatttcttatattgacttactgatcaaattagctaatatgacttctacataatcatgaytgtgaaaattgtaaaattatgttttcaaccaaattgaaatacaattttaacaaagttttaacacattctataatgtttctgcttaaaaataacttccaagatccttagttaattttaagatggactaacattacacctagttaattaatggctaattgttggatgcctagataatttccaagtaagatagaatactccaaaattgatcaccatatacatagtatatatatatatatatatagagagagagagagagagagagagagagagagaaagagagagagagagaaagagagagag

SEQ ID NO: 205 - DNA, 601 bp, Homo sapiens
atatagttcccctgatcttattagtgtattaagcgtaagtatatattttagttttataagatttgaggtgtttcctgataaagtgactagttattctgaacttcctaaatttcttatattgacttactgatcaaattagctaatatgacttctacataatcatgattgtgaaaattgtaaaattatgttttcaaccaaattgaaatacaattttaacaaagttttaacacattctataatgtttctgcttaaaaataacttccaagatccttagttaattttaagatggactaacattacrcctagttaattaatggctaattgttggatgcctagataatttccaagtaagatagaatactccaaaattgatcaccatatacatagtatatatatatatatatatagagagagagagagagagagagagagagagagaaagagagagagagagaaagagagagagagagagagagagattgagagagagtaagaaactatatgtacatagttttttacttttatatgtcatggagtggctacacctttcagtcatgttaatgaatatgctcttttttgccactttagaaaggatttgtgt

SEQ ID NO: 206 - DNA, 601 bp, Homo sapiens
tgatgggcctgatttgacccagtgggccacagtttgtcaacatgtgatctaaagcatcctaaaatttttctatttgctaccctgggaccttgattatttcagggccaacctaatttccaagtccaaggtatatgaagcataagctttctttggaggactttttaatgggcctttggattggtgaaaccattttcttttacctctgtctaattggatattttatcttctatgtggtagaggctaacaggcaccagtcatcttctacccaagttggaattaagagagaaacacctaagttagrcaagtagggattaaaatgtcagttttattatagataaaatccatttcagagaatccagctgaggtttacagctagtgactatgcaagtaatttattctgaattaaacagacctgctcacccaatcacaagcacatctggacacaggcctctccacatggacctatgtcggtaaaagctagagtgcaaagcaacaaggatgtgttcgctctgcagcaatatctcaggagatgaggaaggaaggtgctgaattatgcatccccaagtttatctcccaaattctcaattggaaaatattattc

SEQ ID NO: 207 - DNA, 714 bp, Homo sapiens
ataacttcttactcttttactcccttgattaaaatgttaaatgacccctctttcctcaaaagaaaaaaaaaatcagttctgatatcttatcctggtattaaacatgcttcactctctggcactagactactactacctagtatgactctcctctctggccaggtaagtctgtttataacctctgtaagatgacacttaaattttgcctccttgyctttgccaaggccattgcttccacctggaatgcactctttaattgttttacttgattcatatctatctttcagcgcccagctctagcctctgtgaagccttcctggatcactctagttctcaaagccctctctgcccttgaactactaaagtccttactgtctgtatcttaggcatttgcagttggtgttgttaattttgcataattatatcctatctccaaattgagatgttcagttctttgaggatcagaaacatttgttaggcatctttataccctcaaagcaactagcacagtgatttcacataatgtaagggttcatatgtttgctcatgtgttatataccctttaaaataatttattaaataattatttaattacttatgttatgttataaatatataacaacaacgacttctcactaatccagactagctccattagtaaaagttaatgaggatgtgctctattcagaatacgtttcatgtgtttttgtgctg

SEQ ID NO: 208 - DNA, 701 bp, Homo sapiens
cattgcttccacctggaatgcactctttaattgttttacttgattcatatctatctttcagcgcccagctctagcctctgtgaagccttcctggatcactctagttctcaaagccctctctgcccttgaactactaaagtccttactgtctgtatcttaggcatttgcagttggtgttgttaattttgcataattatatcctatctccaaattgagatgttcagttctttgaggatcagaaacatttgttaggcatctttataccctcaaagcaactagcacagtgatttcacataatgtaagggttcatatgtttgctcatgtgttatataccctttaaaataatttattaaataattatttaattacttatgttatgttataaatatataacaacaacgacttctcactaatccagactagctccattagtaaaagttaatgaggatgtgctctattcagaatacgtttcatgtgtttttgtgctgctgttgcctagawccatgaaacagatttgtagttggttgtttccagtcctgaggaaatgtgggcttgctgagcttctgaactacatccttcttgtgagcagcttagatttcaaggttacgtgcttccagaaatagaaagggagtatttagattctttccttccctgtcaagaaactctgttgaatcatcttttggcaataatgccaaagtaat

SEQ ID NO: 209 - DNA, 701 bp, Homo sapiens
cttctgaactacatccttcttgtgagcagcttagatttcaaggttacgtgcttccagaaatagaaagggagtatttagattctttccttccctgtcaagaaactctgttgaatcatcttttggcaataatgccaaagtaatttgtaagcgttagaacatttgtgcagacagcataagttccttcaaataatgcagttgcayaaagcagtaatgttaattagtcaaagcaacttttttaaaatcagtagttctatgcacatgtgacaccaccttggtaaaaagagctttagaaatttgaagaaaattttgagttgtcccaatatcgagaggggatgccactgtcacttattgtgaaatagctagggatgctagatgtcctgcaacgtgtaaggcattctcatgcagtgaaaaattgccccacattctaactggtcttcaaatgtccctccatacatttatgtggatgaaaactatttaaacttatctgagcctaacacttaatgccatttacatataaacacctaggatctagtttttgtacagtttaaatacatgattttgtacagtttgaatttttgcaactgttatgtaaatcaaagaaagattacgttttgtctcatatggaaatttaacaagcttcatttatcattgtgaaaaatcatgttaccagtggaagtaccacttttggtatttgaataccc

SEQ ID NO: 210 - DNA, 1001 bp, Homo sapiens
cctcaaagtggcttaaaataacaacgatttaattatcatttacaagtctgtggatcaattaagaggttctgctgatccaaccccagctctaatctcagctgtgcttccttatgagtttatggtcagctgggagttggctggtctgggacagcctcagtcaggatcctccagcagactagcctgggctttctgggtaatggtggggttcaaagagagtaagcccaggcctgcaaagccttctgagactcagaattggcacagtcaccactctgcagcatttcattgaccaaggcaagtcacaaggccagcccagattcacagggtaggaaaagagacttcacccctcggccatggaaggagctgcaaagtcacattttaaagagggtaagagtgtagacacaggaaggggtggccattgttgtaatcagcagcaccaagttaaggcgtaaagaagggataggagtcaaccaaacagttagctgaagagaactgtggtcagcrtgtcaaggccctgaggcaagaaatagcatgcagtcgtccagaaggctaagaaagccagagcggcagcatgctgagagtgaggggtgagttgtacaaaatgaggctggtaagaaggaaagggtcagatgttgcagagccatgtagtgtgggccttgttgcgattttcatcctttatctgaagaaatgttttaagcaggagagggagatgattagttatttaaattttctccagtgataccaatgtgcaaccaaggttgaaactctctgtgtaaaagaaaggcacaacttaggaagttgttattacttgttatccaggtgaaagacgacagtagcttgaatgagtgtagttacttagtgaatgaatgaataaataaaattaaactccaagggagagatttaggatccacaggaagactgccttgtttcaaatcacagctccagcacccactagctgtacttgctggggaaacctcagtacattctttcatccctttgtgcca

SEQ ID NO: 211 - DNA, 701 bp, Homo sapiens
tgtaaaagaaaggcacaacttaggaagttgttattacttgttatccaggtgaaagacgacagtagcttgaatgagtgtagttacttagtgaatgaatgaataaataaaattaaactccaagggagagatttaggatccacaggaagactgccttgtttcaaatcacagctccagcacccactagctgtacttgctggggaaacctcagtacattctttcatccctttgtgccacagagccttctttcccaaaacggagatagcaataatacctaccttagcagtgcattataaaaactaatgcattaatgctcatagagcagttatcatcatgccaggcaaatgataggcactccataaacgttaactactgtgattgttgttaaaaggatgatgtctgaggcagtacagtatctcatgcagaaaagctctcatcccaaaatgaatctctattctaatcccaactataccctgtagctctgactgtgctcatgtggttgcrattaagccaaagcccaaggtgggaccagatactgtccatttcatctcggcttgtcatccatcctcctcaggtctgcctggtgctctgacatctggcttccactcatctgggggaggacagggagaagccagacagccatgaatcctgctgtctgctcacaaattcgcagtctagggagggctagggggagttgctgtcag

SEQ ID NO: 212 - DNA, 401 bp, Homo sapiens
gtcacctaggtgctattggtagatacaaagtgttttatgagcgatgctggtaagagctcttttccaagttatctccccaggcacctctgcctgaaattggtggtggttacaagcagagttttgaagaaagacctgggtctggaccctctctcccctgcttacagttgtgggattccaaaaaagctactgtctctgtttctyatctggcgctggggcaatgactcctgccttacacagccattgtgtgaatactaatccatgatgtcataccgcacatgcccaagagcaggcaggaggccctctccctcacttcttccaggctctgatggaatggcagcttagtaacagccttgctgtagtcaccccgtattcagcagaggctctcctccagcccaacacat

SEQ ID NO: 213 - DNA, 701 bp, Homo sapiens
aaaggctctccccagcctcctgccctgcttcaccattccccagtgtctttatctccacctgaagtttcacatgtacttgtctgtctctccgaagaatttaagtgccacgagggcacggtggtttattcacctctttaatagtagctggcatgcagtaggcactctgtaggcatttggaattaatgaataagtaaatacctggattaattaactagtatttcaagggagagtgggatccttgggaaagaaggatagattacaccacagtttgctatagaaggatgcctaagattggtctttgtcagttaattactcactgatataacattggctagtcagttgctcttgagcctcagttttccatatctaaaaaagagacaatgtcacttaccatacttacctcaaacagctagatggaggataaatctcaaacatgggaataagtctgctttgaacactgtaactcaccatgtaaaaatgagaatttggatttttttaagwaacttagcagttaatttcctgggtaatatcctaatagagaaatgtcccacgtggtatgggacaaaggagaatgcctcatttggatccacatctgattttaaaccttgctgcatcaacctgacccacccaacacaacttcactcccttggtcccagattggcaggcacacaagccctgaggacagtatggcttcaggtctc

SEQ ID NO: 214 - DNA, 1001 bp, Homo sapiens
gccctgtcaagcaagacgcgcagcttggcacagccagccctgtagccagcccaggcctcgtaatgggatacagagctcgtcgctaggtgcagcagagtttgcatcaggcgttgtcactgtctggtggttgcctggtgaccctaatggaaaatgagtggaggcagcccctaccacagaaaccactccctcagctggcaggcttgtcggaaagcccagtgccatgggagggggaggggctgccacagaggagctgtcacccaggcgccctgtgtaggtggtggcagggacggggagagaagggcgcagagccacaggagggctcagcagtggtgtctgctctcccttctgcatgaattgttgctcataaaagatgggtgagcccagcacagtaactaatgcttatccccaggcccaaatttaggtaaaagcacacaaaaagtctcatcagtggtcaatgctccacagctccaaacacaggaaggtgcattctcaagctgttaygagaagctcactcaagctgatggtattgacagccacagcccccatgcagggaaggctggacccgacacctgcccacgagaagcagcatacctgggactggagggacttcctggcctataagaagaacactaagaggggaggaggactcgggctgattgggaaaacagatggtgagctccatccgtgggaaaataaatgacagcgtgcatttaagaggttgagccccagagccaagcctgctgaaatgccagcttatcaaaagcacaggagcactgtgtgctagacgctctatcatactctcttccatcctggtttctcttaatcccaagataatgtctgtaggcattggaaagtcttgcttgagagacgaagaaatgtaggctcagagaggttgaacagtttgtctgaggtcacacagctactcaatcacaggatttaacacaggcttttctgctttcaagtctaacattccttctcctaacatcgtgggagaaagtgat

SEQ ID NO: 215 - DNA, 1001 bp, Homo sapiens
gttaattgtggctcaccaaggcttggagagagctggatgagaggggagcagagtccagcgtgggtggggctggactggcagtggcagaggagaggcagctgctgttcacatcagggtctggatggccttgtcgccgcaggaggctgcgctgctccaccctcccaagcgtttcccagctccgtcacagggtctccgttcccaccacagtgtgtcccagcagttccatttgtatttgtacccagagagctccactgaggcctgtggtcacagagtgactcccttccatgttctgccacaggttgcaagccatagggtgaaggtcacacagttttgtttggccataacagctgcctccatggcaacagcgtgtgatatcactggaaaagccatttgtgggactccaagctggaaggaaaaggcagagttggagagagctgtagcgggagacagagaaagggcagggtctctccggatgctccaaggtgctggacgcacaggtcsctttctgtagtccttgtcatgtaagatcttttcatttaggctaagcaaatccagatgttcttcaaataattcaggcatatttggcccaagcataaacttgtcttcatttttcatccaatctgacaaacgtttgcaatcgcctcactctgtgagttccaggacaccttcgggctggaaggggttaatgagaacaagccctccctggtggcttcccttccccctggtgctgcccctcggcccctcccaggccagcaggatttgctgtccaaaggccctcaaaagacatccaagcagtcttttcttagaaacaggaaactgtcttcggccaagtacaaatgaagtgaagcacccagaaacctgaggaccgctccaaactgaggcctggaggcagacagggagggcccaactcctggcagggcctccaggactcaggctctcatgaatgagactgagctcagctgcagcctcagccattcttcgttgcactcaacccattatgt

SEQ ID NO: 216 - DNA, 1001 bp, Homo sapiens
agggatagctgactatgagcggccccactgggctctcaaggtaccatgaaggatccagttcccctctggctgagctgtttgatcctaagacatccctgttggttggcagggaccattttgtcactgttttctgtcatgccttgttttctcattctttctgtcacatatttctaagtgagagggaaagttaaagccacggaatcgcttatcatctcctccctctgcctttgggtttactcagagaaagtcatatcttgacattcccaggagtattactatgcctttacccattttcagtagtaataataaccaagttccctttcccatttccacctacatccagccactgaaatggaattaacaagagtaccagaactacatatattgccagcagttattcctgggaagatggaagaagaaaagtcctaaacatccaactcctgggtacctgcttgcttgaaactctaaacatcagtcttattcgctagttatggaagtaahgatatgttaggtgatactctgagaaagctgtgagctaaaagttgccttacattgcagaactctcagtttccagagaagcagcagacaacacagattatagactctgcagtcaaccaaccagtcctgttaagaacaaactcagccacttagttacgtgaatttggacacgttgtttaatcactccccatacttgcctcagttttctcataagcaaaataggcatattgagagtacattgctcttaacattgttgtgacaatgaaatgatataatttatgcagagtgaacaacactatgcctgacacatagcaagggctctacaaatgttagatgttgttgttgttactattattcggtatactggataatactgccagattcaacatgtttgtgcatttctctcaaattcgcggttgaaagtatacaaaaaacaaaatcaaaaaaatgtctatttctcttagccctgtggtgtctctggcacaactcgttctaagaaaagt

SEQ ID NO: 217 - DNA, 501 bp, Homo sapiens
tttctcataagcaaaataggcatattgagagtacattgctcttaacattgttgtgacaatgaaatgatataatttatgcagagtgaacaacactatgcctgacacatagcaagggctctacaaatgttagatgttgttgttgttactattattcggtatactggataatactgccagattcaacatgtttgtgcatttctctcaaattcgcggttgaaagtatacaaaaaacaaaatcaaaaaaatgtctmtttctcttagccctgtggtgtctctggcacaactcgttctaagaaaagttagagctaggtatggtgaattgtcccaacaacaaagctttcatcaaacaaagcagcagggagattctcaagtctccttttattattattattgtactttaagttttagggtacatgtgcacaacgtgcaggttggttacatatgtatacatgtgccatgttggtgtgctgcacccattaactcatcatttacattaggtat

SEQ ID NO: 218 - DNA, 1001 bp, Homo sapiens
ccccggtgtgtgatgttccccactctgtacccaagcattctcattgttcaattctcatgtgagtgagaacatgcggtgttttttaatgggctttccacctttgtctgtagcgggggcaatgttatctattcagttcagttcagacacacaagtgggctcccaacttccctcaggctccaatattagccattttcctcttagtgtgaattccaccagaatattatcattcccccactgtagtagtgtggaaacacttatactcagtgtcaaatggaaatttgggagcagatgtgcaagcacgaagttcttccagggaattctaaaagacaaacagggaaggcacttgtatatgggaacctcaagtgctcggttgtcaagtagagcctcaattcaaatcatctcatttgttattttcataaaccctcaatgttttctggaaactatattttccaggatgtttctcacacttggatgtagcaaggaaatcattttttatatcaygtgagtctcaaatttagtccatgaaattgagcaaattcattaatggaaagacccttggactgagaatttattctactgtcactagaggactttaatgggctaagaaagagaagaaattacagataatatccaaagcccagcacgataccataaaggcccctcccagatgagtccaagacctccagaaagaactaccaatgcctgaagttccagtaaaaacctccctcaagaatgatcacattcataacagaaagttattactaccatcatccctggagaatctcaaagcaaaatctattatcctaatacagcatcacttgaattataaagtctgatgaaaccagacttggaggctaaatgatgtacacagagttgcggcatctatcagggagctcatcctagaacttgattgtcataacaggttcattgcaattttcgctgcctgtggaactttgtgccataacctgactctccaaccaaatgtgaatgtagcttaatta

SEQ ID NO: 219 - DNA, 401 bp, Homo sapiens
tatattttccaggatgtttctcacacttggatgtagcaaggaaatcattttttatatcatgtgagtctcaaatttagtccatgaaattgagcaaattcattaatggaaagacccttggactgagaatttattctactgtcactagaggactttaatgggctaagaaagagaagaaattacagataatatccaaagcccagyacgataccataaaggcccctcccagatgagtccaagacctccagaaagaactaccaatgcctgaagttccagtaaaaacctccctcaagaatgatcacattcataacagaaagttattactaccatcatccctggagaatctcaaagcaaaatctattatcctaatacagcatcacttgaattataaagtctgatgaaac

SEQ ID NO: 220 - DNA, 1001 bp, Homo sapiens
gcagagccccgaggcagatatggcatttacggagactttatcatggaagcacaacagcttgtcctcagtggaatacagcaggagatccctcgaagatctgtcaggcttggccatttagaggcttggacccctgactcctgccaagagcagtaaggaagcgtgggggccaacacctgtgcacatactctcatgccctcactctccactcattgtgcagagcagaaaccagactcagaagtgctccaggccaggctttcttcaccaaccttcaccagcctctgctggatttggccgtttgcagtgaaaaatgagcctgaaagccctggaggcttcctggtgatttaccgagaattttacttccacatgggctttccagctgcagccaaccccaagaggcagaggtaggaagaggaagaaaatcataaatggatagtaagatgagaaacagatgtttggaggcttcactggaagggaattctccacctctactccctttcttcrtgagatgagaaggctcgggccctaatgagcagtttctcactatacctgcaattcatctccttcccccaccaccagctctctcaagtgtcacttttcaagggtcttcctggtcctgccacatgggcatcaactttgttgggtgatttgtttctggttttagccaaaataaatgaatgctaggtgctctgaccatagacacatgttagacaatctcctgccctcagggtgctcaccagccggaatgaataagcaggtgcaagcgtctgccccctgacagaggcaaggactggaccctgaaaacccacaggaggggcagcaaacccagccttggctcaaggaggcactggagggtcaaaggaaagctcagctgagttgtaaagatgttaatcaattgaaaatggatagaagtcactttggaggtattaacctagcaggcttcaagagagttgtatatttattcagtgtaacacaagggttgagagcaacatccccaaagctag

SEQ ID NO: 221 - DNA, 601 bp, Homo sapiens
ccacatggactggtgcacaacccatctctagcccccagctctctctcacccccgctgagtcaggttctcactgctgttcacatcatatttttgacgcccaaattttctcatagcattcctcaatttaagattcttttgtggtcccccattggctattgaaaagtaacggaattccttaatgtgacagatccctttgtgaatcgattcttattttcctatccagtcccagctctggacaccctcagtgcctccacccagtggatgtattcttccgtgaaaccactgtgctcctgctgtggayacgttgtctcccataacaggaacagtgtctctgtcctgtccaccaaacactccgactttttccctaagaattttcacattgcttcgtctgtgacaacgtctgtgattcctttgggtccccctttctcaagttccttgtgctctgcacctgtctacatgaatgatggggagggttggaaggagcagaacatattaatagcactctccttttctacccaagctctgcaaaaattaagaaataaaaataaaaacaaaaaacagcatatgagacaggataccaaaatatgacccttattactga

SEQ ID NO: 222 - DNA, 401 bp, Homo sapiens
gggagcttcctaatgatatttccagattaggctaacttacactcccaaatgcaggctcagatgaacaggtcacctttccccactcgggggcctataccagtatgagaattatggcatggcctaacaaaaacaaatataaatccctcacgggcaggactaatttcttctttcaaaacccacccattaaacatagtattcctrggaggggagcaagcaaggagcagagaaaagctgggagtgtcacactaatggagctccttccacattaaaggaaacaccaggagtaaagaagaaaagtgccaacatgttatatagtattttcatttttgtgtctcttgatgaaactaaaagctatttgtaggcgagaataatgctttttcatctaatattttcatcctata

SEQ ID NO: 223 - DNA, 701 bp, Homo sapiens
aaccccgtctctactaaaaatacaaaaaaaaaaattaactggatgtggtggtgggcgcctgtaatcccagctactccagaggctgaagcaggagaatcacttgaacccaggaggtggaggttgcagtgagccgagatcatgccactgcactccagcctgggcaacagagggagagtctgtctcaaaaaaaaaaaaaagaagaaagaaagaagaaagaaagaaagaaagaaagaaagaaagaaagaaagaaagaaagaaagaaagaaagaaagagaaagaaagaagaaagaaagaaagaaagaaagaaagaaagaaagaaagaaagaaagaaaagaaaaaagaaaagaaaagaaaagaaaaaaaaagtattatgtgcatggactttgacccagtagagtggaaacagagttgcttgccaggcactctgttctggaccctgtctgcccaccctcaagagaagcccccagtgatgggtgtctttccccacagccacagctacayaggcaggagtaagcactgagccccgtcctctggatttttaaattgtaacagagaaagagagagatttggcctcttgttatgtagctggaccgatgatgcataaattctggaattgctgcaaggtcatgcttcctatcatgtggaacaagaaaaacagtggaaacttgcctaccaagagagagaagaatgccacagatgca

SEQ ID NO: 224 - DNA, 1202 bp, Homo sapiens
tttagaaacagctgctcacatataccattagtagaaatataaagataaatcattttggagagaaatctgggaatatacattaaaagtgtggctcatgcctgtaatcccagtactttgggaggccgaggtgagtggatcataaagtcaggagttcaagaccagcttggccaagatggtgaaaccccgtctctactaaaaatacaaaaaaaaaaattaactggatgtggtggtgggcgcctgtaatcccagctactccagaggctgaagcaggagaatcacttgaacccaggaggtggaggttgcagtgagccgagatcatgccactgcactccagcctgggcaacagagggagagtctgtctcaaaaaaaaaaaaaagaagaaagaaagaagaaagaaagaaagaaagaaagaaagaaagaaagaaagaaagaaagaaagaaagaaagaaagagaaagaaagaagaaagaaagaaagaaagaaagaaagaaagaaagaaagaaagaaagaaaagaaaaaagaaaagaaaagaaaagaaaaaaaaagtattatgtgcatggactttgacccagtagagtggaaacagagttgcttgccaggcactctgttctggaccctgtctgcccaccctcaagagaagcccccagtgatgggtgtctttccccacagccacagctacataggcaggagtaagcactgagccccgtcctctggatttttaaattgtaacagagaaagagagagatttggcctcttgttatgtagctggachgatgatgcataaattctggaattgctgcaaggtcatgcttcctatcatgtggaacaagaaaaacagtggaaacttgcctaccaagagagagaagaatgccacagatgcacagacaggagaaacaagagatggagaggaagttctgacagtttttcagttcctggctctggaacctgcacagttccagctgccttcctgacaatcacagaggcccatcactcacctctgaatctagaaattttttttttttcccaaggagagctcaagatgcttcctattacttgcaactaaatgagtctcaacagtaattccattcctaagagttttagccttaagaaacagtttcagacacacagttgcatatgtaaagataaataccatagtattgcatgtaattttgataaaatgatcgatttggatattaatgtgac

SEQ ID NO: 225 - DNA, 1001 bp, Homo sapiens
gatgcacagacaggagaaacaagagatggagaggaagttctgacagtttttcagttcctggctctggaacctgcacagttccagctgccttcctgacaatcacagaggcccatcactcacctctgaatctagaaattttttttttttcccaaggagagctcaagatgcttcctattacttgcaactaaatgagtctcaacagtaattccattcctaagagttttagccttaagaaacagtttcagacacacagttgcatatgtaaagataaataccatagtattgcatgtaattttgataaaatgatcgatttggatattaatgtgactcttgtcaaacaaaccatcttaatagtagaaacatattaatatcattaattaatgcttaagccttacttcatattcattttgtctcaggggttggattttgtgcttcacatacatctattttaatcctcacagcagccctagaagatgggtactattaccttaagataaacaygtaaagtgtttagcatattgttttgcatatagcaggacttgcaaaatagctaactactattattccaatttctacagatgagaaaattagaacttttttagctttatagccagaaattccaaaggtgctcagataaatgtagtgggaaaatgtaatgatgtgtgggaaagtgagacaggcagagcacctaaaaggtaccccctcctacctattgatcttgacagcaagtatcagatggctgtacttagattgagtgttagaggctaatacagtaattcaagatgtgtaaaagtcaacaaaaagaattagttatcaaacaagttacattcaaggtatggaatgaactatacacaaacggtcaacagacatgcaaacacacatgcacttttctaccaataacagcagatatagccacacgttgggcagttaataccaagttttgcttgttggctaagggaactttcagtatcctaattctgattccattttttttttcactg

SEQ ID NO: 226 - DNA, 3766 bp, Homo sapiens
ctaactgggctatgaatgacttgagcttgtggtcttggcctcattaacactggacaacaaccaactgagctaatcagccactgctgacattacagagaaactttattgaggtataattaaagtacattaaaccatacatgtataaaatgtacaatttgatcagcttttgaatacgtatatactcatgaaaccatcaccacaatcaaaataacaaacatttaatcaactccagaagtttctttgtgtccctttataatccattattcctgcacctccatcctcagcaactgctgatctgttttctctcaggacagaataatttgcttttttctagaattttatataactgcaataatacagtttgtactatttggcttgttatattttaatatctttagaaactagatatgccccctctctcatttttgatattggtagtttgtcttttctctttttgtgctaataagtctagctagaagattattgatctttatgagttttgcaaggaaccatctcctgatttcattgattttttttcaattgtttttctgttttccagtgcatttattttggctctgatcatttcatgtcttttcctttctttgggttttatttgcttttattcttctagtttcttaaggcagaagctgagttcattgatttgaagatgtttttcttttttaatatgaaacctttttgttctataaatgttcccctaagtgctgcctgagctacatctcacatattttttgtattttgttttcattttcatcgagttccaaatactttccagtttctcttttgattttgtcaatgatccatgagttattttaaatattatcttgagactacttgggatatcccagatatctttctgatacactcatttctgatttaattcaattgtggttactgtaggacagattttctattacttgactccttttaaatttactgggatttgttttctcattcaacatatggtctctcttgggaaatgtttcattaatacttaaataaaaagtatattcggtggttgttgttgttgggtgcaatgttccgtaattgtcagttaggtcaatttagttaatagtgttattcaaatcttctaaatacttatggactttctgtctatatgttctatcaattactgaaatctctgactataactgtgaatatgtttgtttttccttaagttttgctccatgtattttgatgctcagttattatatgtgtaaatatttaggattgttatatcatcttgatgaggcgactactttatcattattaaatggccctctttatccctggtaatctttgctttaaaacctactttttaatatgaatatagcctcattagctttattttgatgagtattaacattgtatataacttttcatctttttattttaatatgtttgtatatttaaagtgcattccttataggtaacatatagttgagtctttctttttatccaatatgacacctctgacttgactttgaagtgtttaaactttttgtatttaatgtgaatatgtatatgatcggttttaaatttaccagctggctagttttttctgtttattccatctattattctttgttccctttttcctctatgctttcttttgggttaattatacttttaaaaatatttcgtatatcctttgttgtattattttagtggttgatatagtgtcattgattacgtctttaacttatcacagttatctttcaagtaacattataccactttgtacatgygtattagaaaaccttgcaacaatgtacttccattctctgtctcctgaattttatactactgttgtcgtcatacatattatttttatttctacatatgtaataagacctatattacattgtttctgtgtttgctttaaaaaaccaagttttcaatgaaatgtttaaaatgagaaaatatatttgtctacataattttttttcaaggctcttaattctatccagtatatcagacttctatctggtatcatttttcttctgcttgaaagatgtcttttatcagggatgccctctcttaccactcctattcaacatagtgttggaagttctggccagggcaatcaggcaagagaaagaaataatgggtattcaattaagaaaagaggaagtcagattggccctgtttgcagatggcatgattgtatatttagaaaaccccatcatctcagcccaaaatctccataagctaatcagtaacttcagcaaagtctcaggatacaaaatcaatgtgcaaaaatcacaagcattcctatacaccaataacagaaaaacagagatccaaatcatgagtgaactcccatttacaattgctacaaagagattaaaatacctaggaatccaacttacaagggatgtgaaggacatcttcaaggagaactacaaaccactgcgcaacgaaataaaaaaggacataaacaaatggaagaacaatccatgctcatggataggaagaatcaatatcgtgaaaatggccatactgcccaaggtaaatttatagattcaatgccaccccaccaagctaccaatgactttcttcacagaattggaaaaaactactttaaatttcatatggaacaaagaaaaacctgcattgccaagtcaatcctaagcaaaaaaaaaaaaaaagctggaggcatcacgctacctgacttcaaactatactacaaggctacagtaaccagaacagcatggtactggtacaaaaacagagatatagaccaatggaacagaacataggtctcaggtataacaccacacatctacaaccatctgatctttgacaaacctgacaaaaacaagaaatggggaaaggattccctttttaataaatagttctgggaaaactggctagccatatgtagaaagatgaaactggatcccttccttacaccttatacaaaaattaattcaagatggattaaaggcttaaatgttagacctaaaaccataaaaaccctagaagaaaacctaggcaataccattcaggacataggcacgggcaaggacttcatgactaaaacaccaaaagcaatggcaacaaaagccaaaatagacaaatgggatctaattaaactaaagcacttctgcacagcaaaagaaactaccatcagagtgaacaggcaacctaccgaatgggaggaaaatgtggcaatctacccacctgacaaagggctaatatccagaatctacaaagaacttaaacaaatttacaagaaaaaacaaccccatcaaaaagtgggcaaaggaaatgaacaaacacttctcaaaagaagacatttatgcagccaacagacacatgaaaaaatgctcatcatcaccggtcatcagagaaatgcaaatcaaaaccacaatgagataccatctcacgccagttagaatggtgatcattaaaaagtcaggaaacaacagatgctggagaggatgtagagaaatagaaacacttttacactgttggtgggagtttaaactagttcaaccattgtggaagacagtgtggcaattcctcaaggatctagaactagaaataccatttgacccagtgatcccattactgggtatatacccaaagatcataaatcatgctactataaagacacatgcacacgtatgtttattgcaacactgttcacaatagcaaagacttgcatccaacccaaatgtccatcaatgatagactgaattaagaaaatgtggcacatacacaccatggaatactatgcagc

SEQ ID NO: 227 - DNA, 938 bp, Homo sapiens
ctggcactctgctcatttttctttgcaccctttattttatatgtgctttattatgggtcgtttctatgctgggacttcacagtgttgaatctgccattaatcccacccaatgtatctttcatgtcatatgttatatagctctcaactgcagaattttgacttaggtcttttgtatcgcatttggcatgtttggtcttttctctagcttcttcaacatgtgaaattgttactctcttttaatgtccttgggtactaattctatcgtctgtgtcatttcttggaaattttcaactggctgatttttttcttcattatgggtcatattttcctgcttcttagtatgcctggtaattctttattggatgccagacattgtggactgggtggatatttttgtattcctaaaaatactcttgagttaagttacttggaaatagtttgaccctttcgagtcttgcctttaagctttatttggcaggaacagaacagcatttactctcrggctaattttgctttactattgaggcaaaacctttcagtactatacccaatgcccataaattataaagttcaagaacaggcaaaactatgccaatagaaatcagaatagtgattgacggtagggtgtggatattggaattttctggggtattgcttacacaaatgtacctattaaaattcatcaaactgctcaaaatctgtgcatatcactgtatatcaattttacctctataaaaatcatgtttggtatcaaatatatgtgtacataattaaatgctgaaaagatttatactaaaatttcaatagtgaagaatatcaggtagttttctaattggcttctgaatattttcatgttatctaaattttcaatatatataaccttttaaaaatacataaaactaatatttaatgaaacaatttaagggggactctctacc

SEQ ID NO: 228 - DNA, 401 bp, Homo sapiens
acaatataacaactctatcaagtaggtattatcccatttgcaaaagagaaaacagtgattcagacttatggttatgtgtccaaggaccctcaacttgatcttaggtctgcctgcttctgaagtcggtattttgattctaagagaattaagccctcaagacggatttctgaaattcagagagtaaagaatgcttggtaggayagaagaatcccagaaatacattactgtctacgagcataggaattggcacattggactctgggagttaactattaaaatgggaaagtgaattatccaaatgtcagagtcacaaatcaagcacagttaatctgaaacccaagaaagtctgacctgagacaaggaaagaggtgggtggctcagaggaaaaaaaaaaaaaaaaa

SEQ ID NO: 229 - DNA, 1001 bp, Homo sapiens
gggctgtgggagagcacacccatgaggttgctcagggagcaatgggccacagcagttttccctgtgaattgtgttcaggtaagaccctgcagtcagaccagctcactcctcctttgctatttctttatatatagtctctttccattccgaaaatgtactctgagccctggcctttaacagcttcatttgttttccttcatctcccagtttacaactgtgaaggaaacattcattgatcaagttctttcagcttggaatggagtctctgactcccaaaaatctctcccaggaccaactgcaagggggtagtggatctaggattaaggctggagcctgaagcactgctgagaatggggagtctgacacgtaatgacctccatatatacaagctggtcagtgctctctcagagcctgcatgtggctttgtccagagaatatgaatcccagtttgagcagcaatatggatcagagttggtagagaggaagattgaggctctcacvctaggatgtcttcagcatccttcttgtatccttgtgtgcaaaatgggagcctgggaaaggaactagaagaactgaaccccatccctctgatacatacacattgcttttttccttctttatagcatagcttggctgtccaaatgttctggcagagaccaagctccaggctcagtggggggttctaattttccatggctcattcacttctgagaactttggctcagttgcataatggggggctacttcctgccagttgtggccctgttgtgtgataccttctgacacatacgtttttttgaaaaaagattgtctgctgggaactggactgaaaccaacatataaccgtttgtttcatactggttaggaagccaccaggaaggcctacccaaagtggttttaaatacatacacacacagtcctctcctcttagagccaagaacaggccattagtgatgtgttagaaaatccaggctgaccttctcagtcatgagggaagctcc

SEQ ID NO: 230 - DNA, 501 bp, Homo sapiens
cacacagtcctctcctcttagagccaagaacaggccattagtgatgtgttagaaaatccaggctgaccttctcagtcatgagggaagctccctgggcccaccagcaggcttttgccaagaatgggctccatcttgagcccacagctcttccctagcttcccagcagaagcaaggggagagtggagaagtcaaacacttcttgagcattgcttactatatgtcaagttctaccctggaccctcaatagaaastatttcactgatcctcacaatagatctgtggggtaagtgtcactattgttattttgaggaaactgaggctcagaaaagttacatgtattcccaaagtcacatagtaaactgagtgtgtaaacttgagtggtagagtcagaatttaaacactgatttttatctgttgcaaatgttgggcttttcccaccaccagcagaaatcttgctggccctcagcaaatattcctttacagcagtcatttcaaaacttt

SEQ ID NO: 231 - DNA, 1001 bp, Homo sapiens
cttagagccaagaacaggccattagtgatgtgttagaaaatccaggctgaccttctcagtcatgagggaagctccctgggcccaccagcaggcttttgccaagaatgggctccatcttgagcccacagctcttccctagcttcccagcagaagcaaggggagagtggagaagtcaaacacttcttgagcattgcttactatatgtcaagttctaccctggaccctcaatagaaagtatttcactgatcctcacaatagatctgtggggtaagtgtcactattgttattttgaggaaactgaggctcagaaaagttacatgtattcccaaagtcacatagtaaactgagtgtgtaaacttgagtggtagagtcagaatttaaacactgatttttatctgttgcaaatgttgggcttttcccaccaccagcagaaatcttgctggccctcagcaaatattcctttacagcagtcatttcaaaacttttctgaccctatactcycatcagtaaacatttttaagaaccaccttcaatacagacatatttatttatttataaactccacgcactagctaatatctgttagcattgcctggtaatataataccccagagcactaatcatcattaatgacaataaatatatatccatgtttaatgtagtcttcatgacttggaaaactttttggccagatcttgtgaaatctaattaaattgcttttgttttagcttcaatacatggctggcaaataatttgttccaggagtagaagaaatgatatggcattcttcttaccttcttgggcatgagttgctcctgctgtcaacaatctccagtttccttacagaagaatttttaagacacttttccattttttaaaagtgattcggttaaaatgggataatatggtttgtaaatcgactcactgtgtttatgcaagaccatggaatactatgcacccatataaagggatgagttcatgtcctttgcagggacatggat

SEQ ID NO: 232 - DNA, 1001 bp, Homo sapiens
atttttatctgttgcaaatgttgggcttttcccaccaccagcagaaatcttgctggccctcagcaaatattcctttacagcagtcatttcaaaacttttctgaccctatactcccatcagtaaacatttttaagaaccaccttcaatacagacatatttatttatttataaactccacgcactagctaatatctgttagcattgcctggtaatataataccccagagcactaatcatcattaatgacaataaatatatatccatgtttaatgtagtcttcatgacttggaaaactttttggccagatcttgtgaaatctaattaaattgcttttgttttagcttcaatacatggctggcaaataatttgttccaggagtagaagaaatgatatggcattcttcttaccttcttgggcatgagttgctcctgctgtcaacaatctccagtttccttacagaagaatttttaagacacttttccattttttaaaagtgattcrgttaaaatgggataatatggtttgtaaatcgactcactgtgtttatgcaagaccatggaatactatgcacccatataaagggatgagttcatgtcctttgcagggacatggatgaagctggaaaccatcattctcagcaaactaacacaagaacagaaaaccaaacaccacatgttctcactcataggtgggagttgaacaatgagaacacatggacacaggaggggaacgttacacaccggggcctaccagggggtggtgggctaggggagggctagcattaggagaaacatctaatgtagatgatgggctgatgggtgcagcaaaccaccatggcacctgtatacctatgtaacaaacctgcacgttctgcacatgtatcacagaacttgaagtatatatatatatatatatataaaacaccataatatgctaaaagagaaatcagggcaccagtaggacctcccccacccaccttgcagaatttcactttcctcaca

SEQ ID NO: 233 - DNA, 1001 bp, Homo sapiens
tgagttgctcctgctgtcaacaatctccagtttccttacagaagaatttttaagacacttttccattttttaaaagtgattcggttaaaatgggataatatggtttgtaaatcgactcactgtgtttatgcaagaccatggaatactatgcacccatataaagggatgagttcatgtcctttgcagggacatggatgaagctggaaaccatcattctcagcaaactaacacaagaacagaaaaccaaacaccacatgttctcactcataggtgggagttgaacaatgagaacacatggacacaggaggggaacgttacacaccggggcctaccagggggtggtgggctaggggagggctagcattaggagaaacatctaatgtagatgatgggctgatgggtgcagcaaaccaccatggcacctgtatacctatgtaacaaacctgcacgttctgcacatgtatcacagaacttgaagtatatatatatatatatatatawaacaccataatatgctaaaagagaaatcagggcaccagtaggacctcccccacccaccttgcagaatttcactttcctcacagtgcttcgcacggatgcaaatgactcgtgggagtctgagggtaccggggtccatatatacattcaatattagtacatagaaaagtagttcccatttttagattgaaagtacctatgaatagaagctctaatggtttcttcccttatctcgtgttctattctgcgcaattcctggagcgggcagtccccgccttggagactcctgccttacaggaaggggtcacatattcctgaattggaccccactcagatgcagaaggctaagagtttggatgagaaaagcgggccagtgaacaggagagccggtgggtggggtggatggaaggaggtgcccactctggagggcaagagaaaggcacgaaagcatggggccacatgagcgcggcgttctgggccatccccggtggactcctgcctag

SEQ ID NO: 234 - DNA, 1274 bp, Homo sapiens
cagagcactaatcatcattaatgacaataaatatatatccatgtttaatgtagtcttcatgacttggaaaactttttggccagatcttgtgaaatctaattaaattgcttttgttttagcttcaatacatggctggcaaataatttgttccaggagtagaagaaatgatatggcattcttcttaccttcttgggcatgagttgctcctgctgtcaacaatctccagtttccttacagaagaatttttaagacacttttccattttttaaaagtgattcggttaaaatgggataatatggtttgtaaatcgactcactgtgtttatgcaagaccatggaatactatgcacccatataaagggatgagttcatgtcctttgcagggacatggatgaagctggaaaccatcattctcagcaaactaacacaagaacagaaaaccaaacaccacatgttctcactcataggtgggagttgaacaatgagaacacatggacacaggaggggaacgttacacaccggggcctaccagggggtggtgggctaggggagggctagcattaggagaaacatctaatgtagatgatgggctgatgggtgcagcaaaccaccatggcacctgtatacctatgtaacaaacctgcacgttctgcacatgtatcacagaacttgaagtatatatatatatatatatataaaacaccataatatgctaaaagagaaatcagggcaccagtaggacctcccccacccaccttgcagaatttcactttcctcacagtgcttcgcacggatgcaaatgactcgtgggagtctgagggtaccggggtccatatatacattcaatattagtacatagaaaagtagttcccatttttagattgaaagtacctatgaatagaagctctaatggtttcttcccttatctcgtgttctattctgcgcaattcctggagcgggcagtccccgccttggagactcctgccttacaggaaggggtcacatattcctgaattggaccccactcagatgcagaaggctaagagtttggatgagaaaagcgggccagtgaacrggagagccggtgggtggggtggatggaaggaggtgcccactctggagggcaagagaaaggcacgaaagcatggggccacatgagcgcggcgttctgggccatccccggtggactcctgcctaggggaggggtgcgtcggcggcggcagcccagttttctggatttctttatttctgagtccaggtctttcagaagcctct

SEQ ID NO: 235 - DNA, 1001 bp, Homo sapiens
tgggagctccagagtgggcgaggacttcgggcagacccggcgttgctgttggacatcattcagaagtccccgctcagcgggggcagcccgaagagcaaaacaaacagagcgaggagtagtggaaaatgctgagtcctggagctggccggaacggccttcgcctttccacgcccaaagccagccgctctgcccacctgcagctgcaatagcaagcagggccgcagcaggcagggaggccttggcaccagagcccgtccagggctgggaaggcggggaacagacactcctctctcttcagacaggccctccagagtcctcaccctgaaggctgaggtctttttcttgttccaggagtccagtgaaaaaatagttctcaaaaacggagaaaaagactttcttgaactgcagtttcagatttactaatagagtccatttacatagcacttactaaatgtcaagcaccaacacagatgaattggcaatcaccatgtcagtcctgcraggttggtacttttatccccatttcacagatgaaaaaagccaggcacagagaagtcaaataacttaacccaagttcacaatgctcaacaatggcagggccaggatttaccacctggtttaaaatttaaaacgtaggatttaaaacctactttacagtcttaaaggtgactgccttttctcttcagcttattagatttcctctctaggaatacaagatgtgcaacacaaagagaggaaactcaagatggagagtaaagggaatgaatgagagacaggagaatcaccaaggactagaataatacaaaagatttatttaaaaagcaggtggccatcggcccaggagaaggagtgtgagaccaaggtacagaagtggcaagaaatgctgagctggggctggaaggtatgacagtactagtcagacaggcacctgttctgtccaaaacaggattccagaagtaatgtgaagaggtcacttggcaaagggggctcacacagctcta

SEQ ID NO: 236 - DNA, 501 bp, Homo sapiens
ccattcctctaagccaagagctcttgtccccagaggaaagaggagaaggaagaaaggaacaaacaaatgaacagaggaaggaatgaagagagagagagagaaggagggaggaagggctggaaggaagaaaggaaggggctgttttttttcttgtgtttggaagaacaagctgccaaccctcattaaatgcataggattggctttagagttactacacctaaattctaattctgtctctgtcaccggttagyaatgtgatctcatggaaatcactgaaactcccttaacctgaaaccccatgtctatacaatgaggacactggaattcacctctaaggttctctctggatctaaaatctacactctgatgatactgagaccaaggacagggactttgattgttgccttttcatgccacccaaggtctacatcctagcacagtgcccaccacccatccacaccgaccagacacccagggctagtgattctgtgttctcaacac

SEQ ID NO: 237 - DNA, 401 bp, Homo sapiens
ctggcctttgttgattccctaggttgctgtgggcagatgatcatcgccatcattactttggatgtcaggacattgagatacaccaggcaatctgatgcaactggctttcccagggcagaagcatttgccaggaaagtggaaacagggaaagggactggaacattgagtaaatcaggaaatagcactgaccaagggacagaraggccagagccactttaccccctcatttggggttctaaattcttatcaaattttttttcctcaagttcaaaccttgtggcattttcaccaattgatcaacaactgcctttatcagactccttgaatctctgcctcactgcaaaaagtgccaggggaatgcttttctcttctattatttaggtgaggattctcacggcatg

SEQ ID NO: 238 - DNA, 1001 bp, Homo sapiens
ggcagatgatcatcgccatcattactttggatgtcaggacattgagatacaccaggcaatctgatgcaactggctttcccagggcagaagcatttgccaggaaagtggaaacagggaaagggactggaacattgagtaaatcaggaaatagcactgaccaagggacagagaggccagagccactttaccccctcatttggggttctaaattcttatcaaattttttttcctcaagttcaaaccttgtggcattttcaccaattgatcaacaactgcctttatcagactccttgaatctctgcctcactgcaaaaagtgccaggggaatgcttttctcttctattatttaggtgaggattctcacggcatggagggatctcacagagtagtgagatgccagcagcatgccgagccaatatgcccataaatgcaagggccaggtccttaatccagccatgaggatggtcaaggatccctgtatacaagccagagaagggactytgtacaactagaactgagtcgcaaaccatcttccagagcagcccctggggaaaagcagaggccaaacagcagtatggaagtgaaaaggctcacgtactgaaagaagactttgtccttgtcccatatttgatgtgtgaaacgtaccccttagtaaccaggcctgtggctcccagagctggtgagccatcagccagcatcatcaaaagagacttttcagcgttctatgccagcaatacggcatcatggaaagaacagggcttagaagtcagatggttctctgatgaacctgatgacctcttgtactctcttccaccgtaggctctagaataaaatgagcttcatgccaagtaaacatggaatgtggatagatatctacacaggggtcacaaaattaaattctacagggacaaggcaggaatgtcaatgtgtgggcctgacctatgagagttaaaataggggactgatatgcacctaaaggaggcagcttcagttcagtgccc

SEQ ID NO: 239 - DNA, 1001 bp, Homo sapiens
gatgcaactggctttcccagggcagaagcatttgccaggaaagtggaaacagggaaagggactggaacattgagtaaatcaggaaatagcactgaccaagggacagagaggccagagccactttaccccctcatttggggttctaaattcttatcaaattttttttcctcaagttcaaaccttgtggcattttcaccaattgatcaacaactgcctttatcagactccttgaatctctgcctcactgcaaaaagtgccaggggaatgcttttctcttctattatttaggtgaggattctcacggcatggagggatctcacagagtagtgagatgccagcagcatgccgagccaatatgcccataaatgcaagggccaggtccttaatccagccatgaggatggtcaaggatccctgtatacaagccagagaagggactttgtacaactagaactgagtcgcaaaccatcttccagagcagcccctggggaaaagcagaggycaaacagcagtatggaagtgaaaaggctcacgtactgaaagaagactttgtccttgtcccatatttgatgtgtgaaacgtaccccttagtaaccaggcctgtggctcccagagctggtgagccatcagccagcatcatcaaaagagacttttcagcgttctatgccagcaatacggcatcatggaaagaacagggcttagaagtcagatggttctctgatgaacctgatgacctcttgtactctcttccaccgtaggctctagaataaaatgagcttcatgccaagtaaacatggaatgtggatagatatctacacaggggtcacaaaattaaattctacagggacaaggcaggaatgtcaatgtgtgggcctgacctatgagagttaaaataggggactgatatgcacctaaaggaggcagcttcagttcagtgcccatggtggttgctatgaaggaatatgctagaatccaaagacatcccattaacctactacggta

SEQ ID NO: 240 - DNA, 1001 bp, Homo sapiens
ggtctgacaaggccagggacattccacaaaggatgacacaatatattcaaagattgggatgttcgatgacttccctatattcctgttatatttctcaccttattaggaaatctttatctccaatggtcctgagctagtgagatcagaaagactaaactgcatccctctgtgcttgcctctggttggttgatttgtcctgctttaatacatgatccagacaagaaagaatcaagccaaagccacagcattatgaatgaaattctttgtttttaatttcacacagtttaaaatacaatatgaaatcaggctacagtatataaaaaactctccagcaaaatgatgtgccagcatcagctactaaaataaacaaacaaaaaactccgccataagaatttttttgcatttttttttaaaaaaacatcgacacttacatcgctacatctctaagctacctcagttctgatttttaaaaagcacctgcttttcctttttttcatcttrcttctaaattttcagcttttaaaaaatataaattatatgaaaatacaagttggaaaatagtcaaacacaatataacatctttttcatccctatacttctcagcttaaaaaaaaagtattcttaaaaaaaaaagttcaataactgaggcagtattcctgataattttattttaatatatatattttatatatgtatatgtatacatatatttatggttccttgaaacttctttggaatgtaggtaagagttcaacaaatttatatagaccccaacagagtaagcggcatgcacagcatgactagaagagagatggtgtatttctcaccatgaaggttaggcaggttaatgctgtaaaacccagagtgttcatctccaaagtgaggaaaagcacatctgatctttgaatgctacctccaatccccacagccacaaaaatcagggctctatgtaggggaagtccctctccagaatggagaagggaacaaaagtgactctgaac

SEQ ID NO: 241 - DNA, 401 bp, Homo sapiens
aattttattttaatatatatattttatatatgtatatgtatacatatatttatggttccttgaaacttctttggaatgtaggtaagagttcaacaaatttatatagaccccaacagagtaagcggcatgcacagcatgactagaagagagatggtgtatttctcaccatgaaggttaggcaggttaatgctgtaaaacccrgagtgttcatctccaaagtgaggaaaagcacatctgatctttgaatgctacctccaatccccacagccacaaaaatcagggctctatgtaggggaagtccctctccagaatggagaagggaacaaaagtgactctgaaccctaaagccaaaaccaacaaaggttaaggcatctctgggaaaataagggtttcacccagct

SEQ ID NO: 242 - DNA, 601 bp, Homo sapiens
acattagtctctttctctgttaagccagagccttcaagcttctgagaaggcccttctccctctcctgaaaatttgctcaagaatttctggtcccacccaccccacaagtcctggctttcctttcccaactgcgcacaattgattacagctgcaactgacttagctcccacccctgaaggtaaaaaatgagttctggaaaataaaaaatagaataacaattcaaaattcagagtccaaccaacacggctgtccttggaaggtctcagcagggtttccccagccccttcagtgccatcactcrtcggcatctggcttgacgtccagcatggcgtgcagctcctcaggggtgtaccccagcaggctctgcaggtcacacacaaagcggtacacgtagcgtttccccgctgtcttgtggatgatgtttttgtcgtaatagtagcgtaggccacggctcagtttctcataattcatcttaggtttgtttttcctctttccccatctcctggccacctgaaatttaaaaagaaaaataaaggaggagtaggcaaaaatctacaagacaggccaaatatatatgtttctatgcctatgctatacccat

SEQ ID NO: 243 - DNA, 1001 bp, Homo sapiens
atacccattcatggtgacccatgatgctcaagtaagatgatttgagattcatgtagatatagaaaatatttttcgggcctatctcctgaattccatttttcatgggttgggcaaggatgggagtcacaatgattctttaagttgatgaaaacacagtgaccctgaactaggattaaatatgtgactttaaaaaacaaacaaaaagccacactatacattctcctctttccgcatattattagtaaaatctccttgctttgcaagcatgaaatctaacagggaagtgtgaagcggaggagctgagctgcaatcatacctgcctttcatcaacaggaagtgttttttttccataccagggcacaaatattttctcatgtctgccagaacaaagatgttgtctctcctgttcattgttttttatcctcagaattgggcatggcacggaaccactactccataaacatgtgtgtaatgaaataagaaactaatgagccaatctcycaaggcctcttgaactgtctggcccctttcacactcacagagccaccgggctaggaagaggctaagtcacaggaggcagctctatgggtgataactgacctactgccaggcacgttaatgccttctatcagctaatcctgtaagacaaatggggtaacatagatcttttctctattttccaaataatgaacctggagctcagacaggctacctagcttgctccgggtggcaagtggcagagctgggaatcccaatcctggaacacgtcattcaggcccacgccaccccttccaggagttttctctcatccttcctcaacacagtactcgcaagcccctccttccttacctcatctgggtcagaaagtttgaattcccagccatctcctgtccagctgataaaagactgacaggatttatcagtgagtaattccagaagaaactgccatagctggattggtccactgcctagaaacacaagccattgtgaatcattacacc

SEQ ID NO: 244 - DNA, 1001 bp, Homo sapiens
cacaaatcaggggccacaggctccctactacagagcagtgcttatgagccataacttgtgtttggaactggcaaagacattcattccttcgttaatatgtttcttacttctgaaggcaaaaataatgacttagtttttgcaggtgtaaaagattatgctgccttagaatatcccagaggataggcacagtgttctctttctagaatttgtttagcaataaaaatgaaccgatccttaagttaatcaaaataaagcacttgacacattttcttccatgcttttgttttatagggaggcctttgtcttttctatctgttcgagctcataacacttcctccgacatgtgcactgtctgttgccttcattttctcctggctggatgggctgagagaagagggatgtgggagtgccgtgtgtggggattagctgcgtagagtgctgaatatctggtgtaatgattcacaatggcttgtgtttctaggcagtggaccaatccagctrtggcagtttcttctggaattactcactgataaatcctgtcagtcttttatcagctggacaggagatggctgggaattcaaactttctgacccagatgaggtaaggaaggaggggcttgcgagtactgtgttgaggaaggatgagagaaaactcctggaaggggtggcgtgggcctgaatgacgtgttccaggattgggattcccagctctgccacttgccacccggagcaagctaggtagcctgtctgagctccaggttcattatttggaaaatagagaaaagatctatgttaccccatttgtcttacaggattagctgatagaaggcattaacgtgcctggcagtaggtcagttatcacccatagagctgcctcctgtgacttagcctcttcctagcccggtggctctgtgagtgtgaaaggggccagacagttcaagaggccttgggagattggctcattagtttcttatttcattacacacatgtttatggagtagt

SEQ ID NO: 245 - DNA, 401 bp, Homo sapiens
tcaacactctgacagtcaatttattctatgctaaaaggtttatatcacaccgatttcctttgaggatacttttctcatctgaaatgacaatgccaccagtgattcttaatttataggtgtcggtggagagacaaataggggttcaaaagtccatgcttcttgttacactgccccttataacataaacaaactgggcagagygggactgggaaagacccagtccatgtctctggatacagcccaggaagcaccagctcctacaggaaagctttgctcactaaggctctaatttttcaccggagttgcaaatttgtctgatccaaagtaaactgagatttaacaggaaacaaactttaagttccctctcaatctaaaaaagaaattgccttcataatccataa

SEQ ID NO: 246 - DNA, 601 bp, Homo sapiens
ggcaacctccaatgaagtaaagaaacagctactgacacgagctatcatcccacagccaaaggaagtcctcctccagtaacaacttcctaatggtggtttccaaggctcctctcagcacttgccacgctaaatatgaaaacatgaaatagctctacctcctctttctgagaatggaccattagctctttaaaactatcttgcaagaaataccttacatgtattccacaataaaatggctcagtgaatgcctataaaataaagtaacattcgaacaacagcccagagggccgcactggtaaadccgtagcttcctctgtttctactttcattcaataaaaaccgtttcgtattcaactcagggacatttgcaggtttcttgggagttgcctaaagtcatgagctacttgttttctgcctgggctcacaaaactaaccgtgacattctcagaggaatccactgagaagccatcctaacaggcacaaagaagtaaaacagcaaatcgctctcaagaaatgcagctgccagagccctggtcacagaataggtttcttggagaaactcacgataactatagagactgaagagagacatgaagaaaac

SEQ ID NO: 247 - DNA, 1001 bp, Homo sapiens
accttacatgtattccacaataaaatggctcagtgaatgcctataaaataaagtaacattcgaacaacagcccagagggccgcactggtaaagccgtagcttcctctgtttctactttcattcaataaaaaccgtttcgtattcaactcagggacatttgcaggtttcttgggagttgcctaaagtcatgagctacttgttttctgcctgggctcacaaaactaaccgtgacattctcagaggaatccactgagaagccatcctaacaggcacaaagaagtaaaacagcaaatcgctctcaagaaatgcagctgccagagccctggtcacagaataggtttcttggagaaactcacgataactatagagactgaagagagacatgaagaaaaccattctatcccaaagctatgtaaaagaagcctcggaggagagggggttgccttagaccctgacagagaaaaactaatgagtgctatgcttgacggtgcacctactacrccgcagacactgtgagtgacgctctacactcgtttccttcattcctcccaataattctgtggggtggatgcaactgttgtgctatttgtttctaccacttcacagcagagaaaactgacacactgcaaggccatttagatcagcagtggagtagccgggactggaacccatgcagcccatccccaggttcttcatctcaatgctacgttgcccctggacaggaccaggccaaaggcctggcatctaaactgcctgactgagtgcaatgttccaagggataaggggacctgacttgaaaaactctctcccctacttctcacagcagttgcaggacacgggatagccagtggttctcccagtcatccgaccaccagtggccgtgccaggccccgccatggcatccacctccacaggagatatttccagcatcctcttgtggtagccattatgttacattacttcattgtttctccttcccaatgttcacctttgaacctctc

SEQ ID NO: 248 - DNA, 1001 bp, Homo sapiens
cagtcatccgaccaccagtggccgtgccaggccccgccatggcatccacctccacaggagatatttccagcatcctcttgtggtagccattatgttacattacttcattgtttctccttcccaatgttcacctttgaacctctctcccactatctgaaaatctctttggggcacggggtctcatgacaccaagccgaggaaagggatgggaagatcgagatccttcccccggatgagtctttggcagggagctgtcagcacatctgctggtgctggagaacagggcccaggagcacactgcagtctcctgcccttgggacttggcagccacaatgcagagaagggaccttcaattcccgtggtttgcaccagctcccagaggacgaaccctctgacggaatggttagttttccttttctaccagtgcattttccaaactgaaatgtcaagcagtcataggctgtagatgccctgccctgccctttctctgtgatgtcagcrtacgggacccggtgagtctgggacagggtgagtactcgtcagaggacttttgtcctcattgtgacttttcctttgttcaaaaggaatgaaagaaaaaaaaattaaattcaggccctagaagcccaagtcctaggtgcagagctctctaactcttttttttttctgtttacacccaaggaaagagggaggatagataggaaaagcagatacctaaagaaataatgggaatatgaatgggaagaaatctctcccgttggcttcataataggacagtcaacataacagagatgtcagttcctggctccctcccccgattcctgtagagaaaccccacaggcgcactccagcctaactggtgcacacagggctcacccttcagaaagcccacatttttgtaccaagtgagaggagttcatgatggccgctgaagcgtcccctctagcacctttttgctgactcctaaactgcctttttgttgtggggagcaagagaactaggaa

SEQ ID NO: 249 - DNA, 1001 bp, Homo sapiens
tctctcccactatctgaaaatctctttggggcacggggtctcatgacaccaagccgaggaaagggatgggaagatcgagatccttcccccggatgagtctttggcagggagctgtcagcacatctgctggtgctggagaacagggcccaggagcacactgcagtctcctgcccttgggacttggcagccacaatgcagagaagggaccttcaattcccgtggtttgcaccagctcccagaggacgaaccctctgacggaatggttagttttccttttctaccagtgcattttccaaactgaaatgtcaagcagtcataggctgtagatgccctgccctgccctttctctgtgatgtcagcatacgggacccggtgagtctgggacagggtgagtactcgtcagaggacttttgtcctcattgtgacttttcctttgttcaaaaggaatgaaagaaaaaaaaattaaattcaggccctagaagcccaagtcctaggtgcagrgctctctaactcttttttttttctgtttacacccaaggaaagagggaggatagataggaaaagcagatacctaaagaaataatgggaatatgaatgggaagaaatctctcccgttggcttcataataggacagtcaacataacagagatgtcagttcctggctccctcccccgattcctgtagagaaaccccacaggcgcactccagcctaactggtgcacacagggctcacccttcagaaagcccacatttttgtaccaagtgagaggagttcatgatggccgctgaagcgtcccctctagcacctttttgctgactcctaaactgcctttttgttgtggggagcaagagaactaggaaagacatggaaatgttcttccagccagaaacactgggccagggtgggcgcagttcctggctgggcccgtggatggtctaatacaggagcctgtctccacagcaatgcatcaccctcacttcaggtctgggaggggacttca

SEQ ID NO: 250 - DNA, 1001 bp, Homo sapiens
tcagtgacctttgtcccctagagcagaaaacggtactaataatagcgccagtcatgggaaggggagctcacatgttcaatgtgactcataatggtgtccctgtctgggatctccaaggcagtcaacagcacccttcacgatgctgcccgggagtgtcacacatcaggaatccagtggcatcactgggaaagtatgcttctcaagtcgaagctctgagccacaacaacagaggggtccctgttagaaggaggtctctttccagagccatgcgggcgggagagcaccacacacacactccacacacccatctcccatggcacggagcctccacaccccctgctgtctgctccctctccaccctccctctcaggcggctgcaggggaatttccttctactgctttgttcttctcagcctctggagaagaggacagttcttactacacactgacaggtctgatttgaagaacgtgctacaagctctgaagaagaaataccaggtrggaacttggagagctcccaagcctacaaagcaaatcacaccaaggatgttcaccccctaaggggacccccaaggctcctcaaatctaaggcaacaatctcactttttaaaaaaagtaaagcttcaagtaaattactgctcatttgggtcatatttccttgtctgggagctgcaaggcccactatctgtctcaatgaggagctggttattaaaaatcccctgctattctggtcccttgccctgaggctgagaactgagcagcataaatacatatatagcaatgggctaggacaaggtgttagtaacatgctcttgatggaaatcccttccatttcccgatttgtcagtatcattcttctcattttccagatctgggagttgcctgcctgtgacaaggacatcctcacagcaagtgaacagggtcaggttgaacttcactttttccttctactccttcctcatttccatttcaaccacaagttctcactcttgtcacctgtg

SEQ ID NO: 251 - DNA, 1001 bp, Homo sapiens
tcacgatgctgcccgggagtgtcacacatcaggaatccagtggcatcactgggaaagtatgcttctcaagtcgaagctctgagccacaacaacagaggggtccctgttagaaggaggtctctttccagagccatgcgggcgggagagcaccacacacacactccacacacccatctcccatggcacggagcctccacaccccctgctgtctgctccctctccaccctccctctcaggcggctgcaggggaatttccttctactgctttgttcttctcagcctctggagaagaggacagttcttactacacactgacaggtctgatttgaagaacgtgctacaagctctgaagaagaaataccaggtaggaacttggagagctcccaagcctacaaagcaaatcacaccaaggatgttcaccccctaaggggacccccaaggctcctcaaatctaaggcaacaatctcactttttaaaaaaagtaaagcttcaagtaaattmctgctcatttgggtcatatttccttgtctgggagctgcaaggcccactatctgtctcaatgaggagctggttattaaaaatcccctgctattctggtcccttgccctgaggctgagaactgagcagcataaatacatatatagcaatgggctaggacaaggtgttagtaacatgctcttgatggaaatcccttccatttcccgatttgtcagtatcattcttctcattttccagatctgggagttgcctgcctgtgacaaggacatcctcacagcaagtgaacagggtcaggttgaacttcactttttccttctactccttcctcatttccatttcaaccacaagttctcactcttgtcacctgtgctctgctgagaggagaacacaggagttttcttccaaacagaaggaggtcaacgctgggcaggcaccttcccaggcagtctcctcatatttccatagtacatggcttacaccaagaccaccccattggtttggtc

SEQ ID NO: 252 - DNA, 501 bp, Homo sapiens
ggattagaaagtccgctcaaatggcttctctctattaaacaatatttggggccaaacaatatgggtgaccctcaggctgcatttcatcaacgtgttcccaaaaatgaaaatgactacctgtcctttgggagttaatttgctactttaagaagctaatccctttagctctattctaaaagtcaaatcaaatacctcggtgtgggcaggacaccacatttattttaacctatgaaactctcatggttggtcamccttgcaatagggctgactctgccctgatagcacacatctggcaggtggccctaaaacagaggaacaggcctgctggcccctcccttccagccaggtgtctctacccacagccaaacgatgatggcaaaaacagaacattcgaatccagaaatgacccatctgttcacaagtgtatcaatctgcctttcatgctaccacaggaggacgcacctctgagggtggggtgggtgactccccagtccaagcatc

SEQ ID NO: 253 - DNA, 401 bp, Homo sapiens
atccagaaatgacccatctgttcacaagtgtatcaatctgcctttcatgctaccacaggaggacgcacctctgagggtggggtgggtgactccccagtccaagcatcacccctttctgtcaaccctcttctaaatcaccattcacaaaggcccctaaatctcctgatttccattaagtttaaggacaaaacagaaaacatyctgacagtttcttggcctctggaccaagctcaacctgaagctgcacaaagtcttgttgcctgaggatgaataactcaagaaactgtattgctggactgactggcaatcaagaccctgagaaaattattttaagaagattaagggccaggagtgcttgatattttggctgagttctatgtctctcatttcttctgagttgt

SEQ ID NO: 254 - DNA, 1001 bp, Homo sapiens
gtgttcctgtatcagtggctaataactcaagggcagtgattgggaatataacttccaataattcaactcaaacaacaaagaacattctgacaggtgtttggaaagcatacttgctgaacacgatgatgaacaaacaacaactttataaacttgtatttgttgctgagatagccagtatctaaccatgaaaaagagtgagaaaacagctctcaaatcagttaaaaccagtctttgactgccgagttcatgtctcttgcatgttagatcaaaaacgaaaggaggaggagtgtcaaaaaatttaaaaataaaagccattttacatgtcaggcagtggagtactgagtgatgacggcatcctataaaattaaaatatatgatgcctgtgggaaagccccgggtagggagttgagggtacgaggctttgatatcagttcttacctgaatcaccatatgcaatcttatgcaactcatttaatctctctgggctttactttttccttycctaaaatggaaatagtaatctctgcttctctttagtttataaaaatgtaaattaagtccttattacaaaaatctgcatatatacatatatatagacagagagagagaaagacacttaaagaggtgaacaatttaggagcaactgaatatacaataatggaattacaaagaagaatgaaacaacagaaaatatatttttaaaaacaattttcagtaaaaaacaagaaaaaagatgcatttaaaaaaaattgtaaaagcactagaaaaaatctaattagacttccaaggattaaattggccttcgtatggcaactttgaaaaagtagaaagttggaggttaaggaaaaaaaagttacagtatacgaatgtaaaaatttttaatattttcaatgagaataagcatttaggacttttttaagttagggaagactctgaaatccttgttcccatgttaaaagtgcacacgcaccaaaagagacagcagatgcaaactgctttgc

SEQ ID NO: 255 - DNA, 601 bp, Homo sapiens
ttatttggccagtctgacttgggtctgagaacaagacagttacacatttttagggtatgagggaaagacctttgtttttgctctggctctgcacacctgcaagtgctcaagtacacatgtgtgggggcggcagcaggagaaaggggactgttcctctcttaaaggggcagtctctattcaaatgcaaccacctctttcttctaaacccatcagtaactctgtctaacacattcaagctaacactcagacacaaacttggacagtgagccagtgaagctcaagtcaggaagtgggtttcttyatagctctttcctcctgatgtcttctaggtaaccggttcttttaagaagtcaccagagatgggttaggtttggatttgggggaaggggataagaattttgttataaaccaaagaaaaggtttttccagccactataaatgtacaaagaaaaatcttcctaagtgtgtaggtaatgagaagaaagaaagatatgttcactgatcagggttagaaaacaggactttagaagtctgaagattatagtcttttctcagtaggattctcaacttgctctctggaatttattttatcctaggggtt

SEQ ID NO: 256 - DNA, 501 bp, Homo sapiens
atggtctgaaggttccgctgccttctcttcgctgcctttttttccttcatagatgctccttccgtaaacatcttgcacatctaatcatgtcttggcacctgctttccggcacactcaaactaacacagtattttgaatattttctgacatgtgaaaaccctgaaagtcatcttatttgttgtttgctgtgtaacattgggctagacctcctcctctaaaaagaaaaaaaaaagtctcgattccctcatttrtacaatgggcataacagaaacttcctcatgtgatatttggtgaaggatttaaaaagtcagtgtatatgaaggagtctaagcacacagtaggaacttaatacatctgggattgagctaaataattgaaaagacctaattattattaaatgcctgctacgccccatgacactgccagcaattactgcaattctataagtaaaatgcgttgttccctggcctcaaggaacttagaattatactggaaaaataa

SEQ ID NO: 257 - DNA, 714 bp, Homo sapiens
tgaatattttctgacatgtgaaaaccctgaaagtcatcttatttgttgtttgctgtgtaacattgggctagacctcctcctctaaaaagaaaaaaaaaagtctcgattccctcatttatacaatgggcataacagaaacttcctcatgtgatatttggtgaaggatttaaaaagtcagtgtatatgaaggagtctaagcacacagtaggaacttaatacatctgggattgagctaaataattgaaaagacctaattattattaaatgcctgctacgccccatgacactgccagcaattactgcaattctataagtaaaatgcdttgttccctggcctcaaggaacttagaattatactggaaaaataaaaggtttggagaatactatggaatgtaggtgacagctagcacttagagcctagcttcctgtatacccagcactgctccaagtgctctccataaactaattcattagttctcacaacaagcctatggtatagaaactattattactgccatttgcagatgagaaaacagatacagagatgttagcttgccaaaggttacacagctgctcactggcagggcctgactccatgctctcaattctacagggatggcccctgaatgttgcccttggtaaaactgcatgggatgaccactctttcttgtgtttaacttggacttctctacctgcaggcatccccaagtgact

SEQ ID NO: 258 - DNA, 501 bp, Homo sapiens
ctccactgagatccccaggtccacgccaggcacccctttaggatccactgctaaacccagcaccgtgaatggaatccctgccagcatctcagctgctggctgacaggaaggctctatttaagctgagggggctgccagcttcctgcaactagttaatcacaacagcctctgagcaagaaagggaagacactctgtttctgcccttctcattcccaagctcttttcctcttatccaatcaggtactgcccarggatggtctacattgagactgtgatggcttcagcaagcctggaagccagccccagctttgcctggcctgcagacctcagtgaaatgccctaacttctctgggcctgactttagccaattcacactgtcttacacaacagcatttacatggagagactttagattccagagcttcgctcctgttatctccccaaattaaaaggctctacgctgttcctaatcacatgcccacagcacaaattcacactgca

SEQ ID NO: 259 - DNA, 601 bp, Homo sapiens
tctgtggctatgtctgacaatctggaatgaagttcaataaaggtgatttataggtcaataattctggacggaagccaaggccagctctcttccctcccacatacccctaacccacatgcatatagtgttcattagtgacaagagggagataaggtcctaatcagtctaggcaggcaactgcaataaccaaggagtactctcattatctaatatgaagaaaagattttctattcaggtgagacatttggtgcttaagattcaattcagaagctacctctgtgcagaatgcaattacatacayggccttgaataagtcatttttttgtgcctcagtttcatcatctatgaaatgggactagaggggttgagaggaagagagactactatgtgacaacccattatattattctatacctactgaaatggagaagcaagaggaagaagagatgcctatgtttttcaaggacttggaaagcgttttgcttaggtctataaaatgtatatagaaagcattgggctacttctctaggactgtgttgtaattagaaggggttcataatgtatcttcgaacaaaagaaaatggagctttctgatggtatc

SEQ ID NO: 260 - DNA, 1001 bp, Homo sapiens
tatgtttttcaaggacttggaaagcgttttgcttaggtctataaaatgtatatagaaagcattgggctacttctctaggactgtgttgtaattagaaggggttcataatgtatcttcgaacaaaagaaaatggagctttctgatggtatcagtttgataaccgtaaacagttcacagtaaggtaagaaggtacattttggcggaagccaacattgcatttgatgtattcttaactcagctaacaggcaggctttcaagccacgttatctgcccccgcatcttgacctcatttaacaagttgctatgggagcccagtgaaggttgatgcaattttcttatctttggaggaagaatgtaactgtgcaggagaatgtgaaaattcagtttctaactggcttccgcacttacagtgcagtaagaaagacatcctatcaagaagtaaaatgtattcctttggacgtgatagggacaaagacccagactcctggtgaaatggcaggdagatggattctcttcccagcttggagaatctaagcatgcaccctttagttcaggccaagtaatagtgacatagagctatgtgtacccctactgtgtggccaaacatactctggagcaatcaaattttaagggaacagacagaaaagttgagcagaacctgagaaggtgagtgtgacttttacaagcaataaaatgtattgccaacaagtctatacaatgatttctgctttccaaagtacttttgcaaatttcagctcatcttaacatgtctgcataaagctagacagccatttataggcactctagtgactgcctcaggtggtgggtgaggctgtatgggcacatttcatccgcttccctattccctaggacgcatcttaaatgaggttggcgggggcaccatgagggtgtgagatcaccctcagagggtgagtctgcagtacaggcaggaggtgttcaccaggtatcaattacagggaaaaaataaatactaaaatgtg

SEQ ID NO: 261 - DNA, 1001 bp, Homo sapiens
ggagaaagaattaaatggtaagaggcttcaaaaatgttttttcattaaaatgattacttcagactttgagacttttaagagataatcaccaccccttctcttctactcactaaatgttttactcccttatcccatttctgaagaaagagagagagaaaagaaggaaaggagggaggaagggaggaaggagggagggagagagggagggaaggagggaaggaaagaaggaaggaaggaaggaggaaggaaggaggaaggaaggaggaaggaagggagggagggaggaagggagggagggaggaagggagggaggggaaggaaagaaggaaaggaggtagggagggagagagggagggaggaaggaaggaaggaaggaaggaaggaagggcagaagagagggtgggcaggcaactatcaatctatccaaacataactcagacctagagcatagttttctctgcaccacaaaaacagaagcaagcactgccaattagagataaygtctacctcccaaggccacaaagtcattttagagctacctctgcctttcctttctcttcccaattaagcagcacatctcccttcctttatcactatattcaactgcagtctagttctttaacccctaacaggtataactgcatgagctggcactcttgtacttcctgagagtgacttaatacacttttcctcatcccagacgtttttaatggaaatggatatacttcctaataatctcctttcaaagatgggaaaggactcccttgaaaagtactaagttcctacatgctagccatgttcaagcaaagaccaccagggtattgtagaaagaataaagtaaggacctttaagttccattcctggccttgaccttgttgctactccaacatgtagacataattcctgagcactactcatgcaatgaactgcactaggagctacatggaatgcaatataagagagatactcctgatctttgaaggaggagtaagttttcaagc

SEQ ID NO: 262 - DNA, 501 bp, Homo sapiens
gaaaaacacccaaaatgtaagtttcctaccattcttggaaatgatccctttgaagagaatgatactatttgcttccaaaaatcaatggctattcacaagcagagtggctggagagagactaaagaattcttagagagacttctcccccgtgccctgcaaaagggagtctctcgtcgtctctggtcagaggtgcagagtgccttccaggaccccacccacagaaacgtgcagatggagttggcctaagcagygggagggcgcctacctgtgtagccagctagggcagcagcaggaatgacaggcttgtccttattgaggtcagcacggtcccgcacatagtccttgaaggtgcccttgggcttgtggttgggcagggcagccggatagtcctctgagtcgaagctgtcataggagggaacacgctgcaggctgttgaaagatgactggctgctccaggactgggtgaggcgatcacaactatcgtagctctctatgctttca

SEQ ID NO: 263 - DNA, 1001 bp, Homo sapiens
caggctgttgaaagatgactggctgctccaggactgggtgaggcgatcacaactatcgtagctctctatgctttcaaaagagtcctggcccccgagtttacctggaggtaaaggaggaggtaggaagaggacagggggaggagggagtgggaaaaaaaaaaaactgtaaaaaccctcttatggaggacagattgctaatcagatctgcaggaaggacggaagaagggagaggcgagtgggaacagaagcttcaggggtcatgggtttactctgaggaaaggggctgcactaggccaccatccgagggtccacggccactctgctgcctggtttgagaactccaagtacagagattcagagtcaaacgttgctcacatctgtcggagtagcgtttgggtcctcaagagttctaaagccagaaatctagaagctgaggatcacacatgttatgatatgatttctggctgatgtcgtaggcccaatgaataaatgaagaaatcrgagcaatgtcaggctgaattccccactccagctcaagccaatgagatgacttcaaaaggcccagtttggaaaacattttggtcataagaaaaaagaatcccattagactaagagcagattagcctgttttgaccttggaactaagtgctattttttagcatttttcccaaatactattttaatatgaaatacatgtactgaccctatgccttttcaaatagagtaagatggtgtaagatgcttttcccaagagattttttaaaatcacacacactatcactcttctaaacagaaaaccatattctttatcctctccaagtaaaattatgtacttgaaatttaaacttcattggaaaagtgtaggcaatatttaaaaggtttattaaagagttaaggtccacagcagtgtcagaaatcctttactgtgtgagttgcttaaggcattcttaactgaccacaagatcatgcaagttcattaatttcccaaaccaggttataaa

SEQ ID NO: 264 - DNA, 1001 bp, Homo sapiens
agcaaaaaaaaaaaaaaaatagttttggaggaaaacaaatgaatctaagagcgaaaaaggctcgcaggaatggtttttatatgcaactttcagatacttttcaagtaacctaagttaaatcataggagactagatggtcacctcaattcagcacaggccaaaaggcaaagggatgtgacaaatgtttacggagaaatatccgtaagtcaactcttaattgttcaggggtggttgatctataaatttcaaatcccagaataaggctgacttatacaacttcatattagtgtgcctccagtgtatttttccctccatgacagcggagattggttaaaacaataaacatcaaacatgaacagatgcccaaacctaaattaaatatataggaaaatatgttgctcccaacattgtttaaagatccggataaaatgtattcggttgagtgtgtactttttgtaaaatccactgctgtgggttttctctacatcctgaccccctctrgaactgctttaaacagaaaggtggtgtcatccgtttcatctcattccttcctccactcatccattcagaggagggtaatctctggaaagcaaactgaagagcttcatggagttatcagccctgcccacccagtccactagcaaaagggcacctcttcattcttactaaaaatgaatatatatttctttataattcttaaaaattctttcccatttacccaccagaaaagtcatctttttcacctttttagagatcatttaattttctttcaagaaattcacactaaatgatttaagaaaacagcctacaaccagaatgtcaaagccttgttttagcagaacaggaaattctgtggcgtctcataaaaaggtatttgttcataccagctactgatcttcatggtcacttattttctctttgagacaaacataccaaaagcctaagaaggagaatttatattttcatcaacaccgcaccaagtcgatagtatttatgctaaa

SEQ ID NO: 265 - DNA, 1002 bp, Homo sapiens
caggcttactgcagggtcgttcagagctttctgtccgcaggtgcacttcgtctcccttcctctccttttcctaggggagttggcatctgggcaggagcttgactgggttgctcttctctcccttgacacaagcgcagtcgcatttcaccaaatggagtcaccttaccagtgtcctgcttcttgtctgggcctgaacttgaaacctgagggcaatgggaaaaatacaaaacaaaaaccagacatctgttagaggaaatggagaacgtaaaatctatggcctaaagactgcaatatatttttgagaaattttgaaattgattagtttgggggttggggattgatcctgctaacctgggatgtactcaagcctttggctatagtgtggtcgacatacacgcagcacgaatgcattgagaatgaatgctgaatgccttctgagcccttagagattactcatggattctctttccaagatactaaatcccattttgcagctactgaaataataaccttagtcatatttttttgatctcatctttagacaaggccacagtcaggacagactcagataccaacccagttaatgagtatgcagatttcttagaaaaggggttgagatcattgtggtctttgcatccaagatccttttaggccaagcatgacttgaatattgacctctttgttccttccctatctgttcattacagaggatgtgaaaccatatcaagttaatggagtcaacccagcctatccagaatcccgctatacctcggattacttcattagtaagttcatttctacccctcttctctcatgataatagcaaactaggaaaagacccctatctcagtgaatctcaggctccttcatggtaattctatcaaaaatartatcttcttagatgtagactcttctttgttactttattttattattttccacaaagcacaaagtttcaacctatatatatgtttcattaacctaccaagttcctacacacta

SEQ ID NO: 266 - DNA, 1001 bp, Homo sapiens
actgcactccagcctgggtgacagagcaagactctgtctcaaaaaataaataaaataaaataaaataaaaatatactgaaagttgaaataaaatgaagaaaaggagatgagtgatactgaagaaatcgcctaccctgagcttcattttacagacaaggacaataataggacttgtccttactatctcacagttattttgataatccaaagagaaaatgtatttgaaagcactttggaaacagggagacatgatagagatattaattgtaactacaatcagagatgggcttagatagcccaaaacacctagcagctccattttgataaatggaggaaaacagcctcttagtagaatatactgggttacacagtctgattgaatctgctattgtgtttagaagtcaacagtcaaatcagatctgttaggagcctgccgtatcgtttccctctataaacaggtcgctcatgtcaacacctatgagtgggtgtctgtgcatggadaacatgccggtgctttgcaactgcctgccatcctcggtaaaagcagccacagaaagactcacctagttctttcctgtattcctttatgtcttatttttcaacagaaagtgaaaagaaggaataaagataacatttttgagcacagagaaatctagtttgggtctctcttgagcactgcagaatggaatatattcttaaccaaaggaaggtataatgcggggtaaaagtgctaatcctgagttttgctcccctcccccagcgtctgtgccaagggttagagctgatgaccacagggaaaggatgggcctgggttagagagggcaatgggcttctaggcttacagtcagctgaagggcactgctgactgctggtaactgcaatttattttaagaaaaaattcaaaaaaataagcacaaaaacacccaagtttgccgcctgctgctgtttctatactcagccaggactgtggtacatgagtcacttggtccaaaaaggttgga

SEQ ID NO: 267 - DNA, 1001 bp, Homo sapiens
ataaaatgaagaaaaggagatgagtgatactgaagaaatcgcctaccctgagcttcattttacagacaaggacaataataggacttgtccttactatctcacagttattttgataatccaaagagaaaatgtatttgaaagcactttggaaacagggagacatgatagagatattaattgtaactacaatcagagatgggcttagatagcccaaaacacctagcagctccattttgataaatggaggaaaacagcctcttagtagaatatactgggttacacagtctgattgaatctgctattgtgtttagaagtcaacagtcaaatcagatctgttaggagcctgccgtatcgtttccctctataaacaggtcgctcatgtcaacacctatgagtgggtgtctgtgcatggagaacatgccggtgctttgcaactgcctgccatcctcggtaaaagcagccacagaaagactcacctagttctttcctgtattcctttaygtcttatttttcaacagaaagtgaaaagaaggaataaagataacatttttgagcacagagaaatctagtttgggtctctcttgagcactgcagaatggaatatattcttaaccaaaggaaggtataatgcggggtaaaagtgctaatcctgagttttgctcccctcccccagcgtctgtgccaagggttagagctgatgaccacagggaaaggatgggcctgggttagagagggcaatgggcttctaggcttacagtcagctgaagggcactgctgactgctggtaactgcaatttattttaagaaaaaattcaaaaaaataagcacaaaaacacccaagtttgccgcctgctgctgtttctatactcagccaggactgtggtacatgagtcacttggtccaaaaaggttggaagaggctgttaggggaggccatgtcattataaggttgcaacatagcgtcctgatataaccccagttcctgctccagatgtaaaaggt

SEQ ID NO: 268 - DNA, 1001 bp, Homo sapiens
agtggcgtgatctcagctcactacaacctctgcctcctgggttcaagcgattctcctgcctcagcctcctgagtagctaggattataggcatgtgccaccatgcccagctagttttttttatttttaggagagacagggtttcaccatgttggccaggctggtctcgagctcctgacctcaagtgatccacctgcctcggcctcccaaagtgctgggatcataggcatgagccactgtgccagcatgagcaggcaacatttaaggggctttccacattgtgctaggtctaaaatgtcctgcatccctgacaaacaaatatgtttactcttcctgaacacctctactagtttatacacagtccctgcttatctttcacatttaccgagaatattaatgttactacatactttcagttacctatgaaaatgaaataacaatattcattcattcaacaaatgattatctagcacttgctttgtgcaaggaattaaagaaacaamagtgagcaacacagaaatagtctccacaggagctagctatctgattcttgcagtagattcagccactaaaaatctatctacacagttaaatgttcaaatgcaatgtcaataagggcttcaaaggagaagtacatgatgcaacgttaatgtgcaacaggaattcctggaagtctgaaggaaacaggaaaggcctcccttagaagatgagagatgtttgacctgaattgtgaaggatgcatgagaatttaggaagaaaagaatactccagatcagtggttctcaaagtgtagtcctcagagcagggacatcagcatcaactacaaaaagatcattttgttttaagatcaccttatccgttctgtaaagagtgatttaggggtgagtatgaatggatgagcaagacattttagaaagttattgcatcagtcctggtgagagaggatggtggctttgactacaaaagtggcaaggcagataacataagtgaacatgacttcaag

SEQ ID NO: 269 - DNA, 401 bp, Homo sapiens
ggaactgaagaatgagactgactaggaggcccccagaatcttctcaacatgaaagctgggacagtgggatgccagtgtgaggtgacagccaaggacgacagcagaaagcctgaaaaagaagttccttgagtctgcctcccataactacacaagccctggcagtgtggtctggacaggactgctgagctgacaattctccaygtaggtttctgcttcctgtcagggggcaggcacttctgggttctcacttgttctctcccaggaaagcagctagaattacttttgcctttccacctcaatgccatctccacaagcccagtccacgtgctgttggggccccatcagaggtgcctggctctgcccctctggctgtgagactcaagtgctagatctctttaaaa

SEQ ID NO: 270 - DNA, 1001 bp, Homo sapiens
gctgagctgacaattctccacgtaggtttctgcttcctgtcagggggcaggcacttctgggttctcacttgttctctcccaggaaagcagctagaattacttttgcctttccacctcaatgccatctccacaagcccagtccacgtgctgttggggccccatcagaggtgcctggctctgcccctctggctgtgagactcaagtgctagatctctttaaaaaaagggttcacatcccagctgggggaaaccatccctgtccacttaggacacttgcatttggacttgatcagctccagagaaggcacagcattgtctttggagccaaaggattcagatgtaaaagtcagaactttatcctataaagtgtggaattgtagtttaaaaagaaaaaaaaagtcaaactcccttctataactaagtgaacagttggcaaagattgtctttttcggttgtgtgagcattgctcttaagtgatgactaatcatgctcaaaaatgtayattaaatagaaaataaactcaccatataaaatactaattcaaaaattctcttcatgttgtttgcagattgtagcagttctgttcaatatactcatcaaaaacaatgacaaaatcattacacgggtgaaaaatctgacatgacttagcctaagcagatatcgctttactcttaaaatactttacttcatcacctattataatatttttacattaggtacaaaatatttctaattttagaatcagtgtctgaaagttaatcactacctccatagacattaactaattatattttatggaaaaatactgaaatctcctttgtgctaataattacaatatcttaaattcaaataacgtatttgtttcaaaatgctgagaatccggcctggagaaacactacgccaacacagtggagattctaaacacaacgcactggaaaatgaggacataaatatattgcaattatattagatttcctgcccactgattattccttgggaccc

SEQ ID NO: 271 - DNA, 1001 bp, Homo sapiens
catccctgtccacttaggacacttgcatttggacttgatcagctccagagaaggcacagcattgtctttggagccaaaggattcagatgtaaaagtcagaactttatcctataaagtgtggaattgtagtttaaaaagaaaaaaaaagtcaaactcccttctataactaagtgaacagttggcaaagattgtctttttcggttgtgtgagcattgctcttaagtgatgactaatcatgctcaaaaatgtatattaaatagaaaataaactcaccatataaaatactaattcaaaaattctcttcatgttgtttgcagattgtagcagttctgttcaatatactcatcaaaaacaatgacaaaatcattacacgggtgaaaaatctgacatgacttagcctaagcagatatcgctttactcttaaaatactttacttcatcacctattataatatttttacattaggtacaaaatatttctaattttagaatcagtgtctgraagttaatcactacctccatagacattaactaattatattttatggaaaaatactgaaatctcctttgtgctaataattacaatatcttaaattcaaataacgtatttgtttcaaaatgctgagaatccggcctggagaaacactacgccaacacagtggagattctaaacacaacgcactggaaaatgaggacataaatatattgcaattatattagatttcctgcccactgattattccttgggaccccaaatttcagttaatatttataggaattcccctagacctctgaaaggacagttgtgcagaagctggtgattaaataaccattgcaggagattgcacagtatttagacagaagtgagcaggtagctttctctgaatctacagaagaataagctagtggcattttgaatgcagggaaacatctgctcatttttcattgtggcctaaccctgaaccacctcatagatgtttcaagtgaaatgtaaaacaaggg

SEQ ID NO: 272 - DNA, 1001 bp, Homo sapiens
caatcaatgatcatgtgaagactggagcgtctgggatcctagggttaggagatgagggatacagccaaggacaagaaatccaaggtgcatgtcccagttttgcatgaccattgaactgggcccaaccccatcagattatgataccagtcatgtgtgttgggtatggtcacactcaatagcagcatgaaagaaatactaagagtgagtaatatgccttatacctgagaaatgctttacagtttgccaagactcttcacatacactattccaaaatatcctctaaacataaaactggaggggcctggaaaggtatcacaaggtccccatttcacagatgaggaaatcaaggccctgggagatcaagagcttgacctaaagtcacaaggccaagagggaccagctggggctagaagccagtcttctaactcttaaagttcagggtctttctctctattccactgcaaacagaaatggatcagatatccaggaaaactaacattkttcagagctgagaaaaaaaaaatgggacttttcctttcttattttgaaagattttaggagtgattaaaaacttaaaactattccaagaaacccagggtttcatacagctagccccgtaagaacataattaagagccatttacagaatcaactataatcttttcttttcctggcactcaggcaactgaggcttccttccatatgaagcaaatgagttaagtgaaaacctggcttccttctctgtccaaccctgactcaacctaatgggtaactttgcatataacagaagtttaatttgttacataaaggcttactgaaatatattttttaaagtaaaagtaaaccaagaataaaccttctggtccacatggagaggataaaagaacagttctccaaactgaaagataggattctaaagacaaagaaaaaagagagagaggggcgtgcattgttgataacttgttgatcaaaatccataggttctgatttcacatacgccat

SEQ ID NO: 273 - DNA, 1001 bp, Homo sapiens
ctaacatttttcagagctgagaaaaaaaaaatgggacttttcctttcttattttgaaagattttaggagtgattaaaaacttaaaactattccaagaaacccagggtttcatacagctagccccgtaagaacataattaagagccatttacagaatcaactataatcttttcttttcctggcactcaggcaactgaggcttccttccatatgaagcaaatgagttaagtgaaaacctggcttccttctctgtccaaccctgactcaacctaatgggtaactttgcatataacagaagtttaatttgttacataaaggcttactgaaatatattttttaaagtaaaagtaaaccaagaataaaccttctggtccacatggagaggataaaagaacagttctccaaactgaaagataggattctaaagacaaagaaaaaagagagagaggggcgtgcattgttgataacttgttgatcaaaatccataggttctgatttcacwtacgccattagtgtagacacactggataagtcacttactcaattcactttgaaaagaggtctgttcataggtggtgtctatatccctcatagagttttacattttttatttggcaattttcaaacatacataaaagtagagagaaactctactcaaaatttatcaatactacccgtttttatttcatcttccacacacatgcacacccatacacacacgcagaagaattatacacctaatcccagaaaacaagtcatttcacccacaaatatttcattgtcacaaggatattttttagataaagggagatcatagagttaaagttcaataagaggcaaataaactcaaggaaaaagaaaaaaagccttcaagttactttctctcatgcttaaatctaggtctatatttcatgcattggcccacttgaaccacagaacttctttcaaagcaacactgtcatgatctggaaagtgccaatgttggatcacagagatgatttc

SEQ ID NO: 274 - DNA, 1001 bp, Homo sapiens
tactcaattcactttgaaaagaggtctgttcataggtggtgtctatatccctcatagagttttacattttttatttggcaattttcaaacatacataaaagtagagagaaactctactcaaaatttatcaatactacccgtttttatttcatcttccacacacatgcacacccatacacacacgcagaagaattatacacctaatcccagaaaacaagtcatttcacccacaaatatttcattgtcacaaggatattttttagataaagggagatcatagagttaaagttcaataagaggcaaataaactcaaggaaaaagaaaaaaagccttcaagttactttctctcatgcttaaatctaggtctatatttcatgcattggcccacttgaaccacagaacttctttcaaagcaacactgtcatgatctggaaagtgccaatgttggatcacagagatgatttcaaatcaagatggtaagccagttccagggacttccayttcctacaagcagaaggctgcagtgatatttcctcttaatggtcaacatcctcatgaacttacaactgtaactaaagtgtacaaaacaaataaaaaggctcggagttctggccagcacagaagggcagtgtgaaaggtaatatcattgccaaactgccgacaacaagtcccagtttaggagataaggtgcctttaccccttcagaccaacacaaatagagaaatggctgcagccacactgacggctctgcttctgaagttgatgacccctggagggtggtcactggtctacaagaggattctcctgataaaaaagctaatgatctcagaagaatgtgcaaaggaatctcaaagaaagacagtctctattgccctctctcattcatataaaggcagggttgaagtagagtagaagggagtggtaagtgattcctgtgataggcactagaaaccgggcaggcaggacttccagcttagggaggtactataatccacaaagct

SEQ ID NO: 275 - DNA, 1001 bp, Homo sapiens
ctgatttttgcgtttgtttttcttattttctcagtcgcttatttgtacctggagaaattgccagattccttcttgatgtttctgtaagcattgggaaataaaatctttttttttaagtctttatattttataagatgcttttcagtataatcaagtagccaatgatttgttgagcacctactatgtcttaagctttggcattgtcacacatagtccacttaatcctcacagcatggtgggtagagcatcctagagaatgaaagcgagcttcatctgaggggctttgagacctggtttatgtaccttcacttgccaggctgctagagaaaaacacatatttaaaagcctttccagcaggacacattcattcatgtatttcctattttaggccatttgcccaatgtttagggtgggagatttgaactagtctaaggaatgagcgagaaaatttagctacaggaccaagggggcagttctgctttctggctgggatcctggaayggaagagcctctctgggtttccctgaacacctggaattgatttgggttttgctctgacttcgaaacatttgctgaggtggaggatggtggaggaggtaggaaagaaataaatccagtgattaaaaatagcttgtgcatgtcaggtgcctgaacgaatttgggaacatgcctgcaatcccttttgtctggcaggtctgaactccggcgctgccgaattacaactgctttcatttgtttttcctgcttccctaccatgtaatggtcaagggctcattggaaccatgtgtgagcctggtgagtcaccaaatcctcaggacttcagtggtaataatgtgttaaaactccttttgggggatggggcaggaggtggatgaagggaagagggagaagtctgaggtcacttcctacagatgttcagtgtgctgagccctctctacaggcttctttctcaggcctggctgcaggacctgaaaccagcttctccatgcaatttggagctg

SEQ ID NO: 276 - DNA, 1001 bp, Homo sapiens
tacacctgactcccaccacatgacatactttatagttcctaaatgtcccagaacagtgtgacttctttatctgaaaaacacagagccatggtctctacattactcaggaggaaagaatgagttgggctctttcgtctccatggctttgcagagaaccacattgcatcctattggttcttcccacatcttacacttctgaatgaggaaaactcctgccctgccttcactaaaattctcatgacaggatcatacggcttttggtaccaacatgacataggataaccccatccaggaagacaatggagaatatctgacaactacatcttgctataatcccagcttccactaattctggtttacataatagcctttgaggcctcatcctctgagatcttgcagatgctgatgaattgggctaaccaatttattttaatttcacttaactcccacctataattatcattcctgctatttgactagaactgtatcttttagaaagcrttttcttgaatattctcatatgatttttcaaaacaagcacttgtagttattatctttatcatgtaggtgaggaaactgaggctcacaaatgtttcttaagtgacttaactaagattatcaaaccagtaaagtgatataacaaggattcaatcccacatcttcagacacgcaagccacgtgttttctccctgcacctattcacagaattaaaagcaaatgaggcaaaaatgatggggcatgataacatttcttttttcattttctccaacattttcattctagaaaaagctctttctgtagcagggaagaacctcaatccccgagactctctaccgacagcaggctccattgcacgtcctacccagaactggcctggtcaaacctcggctcggggcccacttggcacttggtcggggggtaaaacaggcatcgggagagtggtgctgagaatcaccaagaaggccaggctgggcaaggtgtacgatgaggagttttctcca

SEQ ID NO: 277 - DNA, 1001 bp, Homo sapiens
atcttgctataatcccagcttccactaattctggtttacataatagcctttgaggcctcatcctctgagatcttgcagatgctgatgaattgggctaaccaatttattttaatttcacttaactcccacctataattatcattcctgctatttgactagaactgtatcttttagaaagcattttcttgaatattctcatatgatttttcaaaacaagcacttgtagttattatctttatcatgtaggtgaggaaactgaggctcacaaatgtttcttaagtgacttaactaagattatcaaaccagtaaagtgatataacaaggattcaatcccacatcttcagacacgcaagccacgtgttttctccctgcacctattcacagaattaaaagcaaatgaggcaaaaatgatggggcatgataacatttcttttttcattttctccaacattttcattctagaaaaagctctttctgtagcagggaagaacctcaatcccygagactctctaccgacagcaggctccattgcacgtcctacccagaactggcctggtcaaacctcggctcggggcccacttggcacttggtcggggggtaaaacaggcatcgggagagtggtgctgagaatcaccaagaaggccaggctgggcaaggtgtacgatgaggagttttctccatgggcaaatgaaaaatctgggcaaacaaatggagtagagcccgtttatttaggctggaagaggtaaagtttttctgcacttttgaactgttttctcaaggcctgcctctccctcccacgcaggaaacaaacacagagacaggcctcttccagtgagggcttcagttgttcaaagttagcccgggaagggcagaaggaagaaaggcttagagaaaggaaggaggaacgggggctaggaaggtggtgcagtggccatgggggtagccgccaagggagaaggctggagctgggatcagacagaggaggagagctggccaagaag

SEQ ID NO: 278 - DNA, 1001 bp, Homo sapiens
cacatatctttgtcttgaccacaaatatatcatggaaagactcagacaaaagcattactggaatcaaaatatgaggttacaatattcagttggtctcccacttgtggagccagttctcccctcgagtttctaagcatctggcaagtgaaaggtggctgatagtacaaatggttgagctggaattcagacccctgtacagtgaaataaagaaagacagagaaagggggtggggtggagagagagagagagagagaaagagagctgcagccacagcattgctttgcttctagaaacaatgggcagttagagaacaatggctacagacaaagtcttggtctatttatatctgccactgttagtcccagacaggaggaactggaagtctgccctgtatgcacagctccaactggacccaagttgggaggaagatgaggtcaccaagaaggctgcctgcttagaaatgggcttcttttttcttcgtatagttgcttcttagcctaraggttctcttaagcttgcttgccttctgctaaaatacagccactgctgagaagggagagatgagaaaagtaactgctgctctgcccagcccaaagcaattaaggcctctctgtacagaggttgcaggaaggtgggaacgccaaggaaaaaataaccaatcgatggaggtcaactctatggtttctgaaacaacagtcttattaggtctgttaattatacatgtttaggagcactataaaggagcttttccctgggaaagttccctcctcatttctttggagacaaataaagaggccaagagctgaaattcacagatatgtatgcattacatctcagggacaatctcttcttccctttatttcagcccctttttgatggtatctctattttctggaatttcatcttttgctctaacatggctttggagagatactcaattttaatccttcccaaactgtgttacttgtatccttaatcctcctacagccttactaaaaaga

SEQ ID NO: 279 - DNA, 1001 bp, Homo sapiens
atttccctgcctctgtccctctatcccgccctcactatagctataggatgcataaagccttatccaggaccaaaaagcagaaaagaggaatttacagaatttgctataaaactttaacaactccttggagggatgttctctttccttgcaaccagacatagttataaaatggatgaaaagtggagagaaggaggagccaagctctgccactggtcaggggtcttacactattcctggaatacagaattagaagacgctttcgatgtcatctagttcaaaccttttcttttactggtgggtaaaatgaagctcaaggtgacatcaacttgccttaagtcactggttactaattctagaactctggctccctctcaggatttttttttcctctacatcattgctgtttacttacaacagtggactgggagggagaggctttctcctatatcttcactactatcaagtcctggttcatcattctggataaacactactcctccycaagttattaagaatcacagaggaatgagccatccaaagatctaataaatatgatgggattttacagattcatgatgctatccactcctatttcaggttataagtctggaataccaatggtcagactctaaggtggaaaagcttcctcctagcaaagatccttgttgcataccagggatattaagcaactttcaacagtcaactccgatagcatgataccatggtgtctgatggctctgaaatttgagggtgctattcctgtcaatccagaaagagtgaagactgcagttaacttcagtgatctatgaacctttatctaaaaagcactgaaaggcagagtgcctcatatcatttaaaggttttacaccactacccttctagtcctgctggtattccaaatagggtcactgagccatggtgatagggttgagggaatacaacaaaccccactgacaaagccagaacttaatatcaggggcactggccagtaagttgaatct

SEQ ID NO: 280 - DNA, 1001 bp, Homo sapiens
tacgagcccttctcctcacatcccagctggacagcattctttttttcagaaagagctactgactgctcatgagcatggggcttcttttgggagtgatgaaaacattctggaattagacgttgatgatgatggcacaactctgtgaatgtactggaatgcactgacatgtacactttaagatggtaaattttatgttatatcaattatatctcaatttaaaaaaaagtaaatgttagagagagaaagagctactggcccactgctatgagcccaacaatgaataccttggtgatagatccctcaggcagagtttccctctagtgggagaagcaaacaccgcctaagtacagaagcaatagctatatgctcacaacagacgatgagtgctgggatcacggctgaagcggaaggttttgcaatgcagagtgagtgaactagcggggtccagaagcactaggggagggggtaggaaggagtgcacgtaagatgtcctgggtgtasggcgtgagggacagaaggcgggcaaggtgtccaggatggcgcccctggcagttggtggcattactgaaagggaagacgagaggatgagatctcccacagccacctccgccacctggaaatccttgtgagatggaagccccgcgatgctcactgggagaccgaccgtgggagaggctgggcacgggccatttccagaggcagacacctggtaactgcaatttctgggaccacttatgtgaggactaaagaggaagggccacaggttctaggagacgaacaaaatccctcaagttccctaccctaaagatgctcccagaaaaggctgccgagtgctcttttaaagtgatatgtgcatctttatacttacatacaaaagattctcaaggggaagaagtctccatcagacagggctctttcgccctccagtccctggtgggggagacagaggaaaagctgatagggcggtggggtgtgggggcggtgaaggctcactgcacagg

SEQ ID NO: 281 - DNA, 1001 bp, Homo sapiens
tgaggaaggtgcagtcacaacactgtgatgccagggatctttttgggaaattcttttccaaaagggatcatgaattttggcccctggaatgccccagagcacctctgattggttccctggccctgactcagatcgagccgggctccaccctccatgagtaaataaaggcagggacggagggagggagagggaaggagagggagcggagtgggcagacaggaaccagaaggccagcgctggttcagggaacacaccagatgagatttcagcgacgggtggtgtggcagaattcaagacataattctctgagccttacacaccactccagttgggattcagccctgccttggcagccggctcagtgctgctttataatatactgaattagtcactggattagcaagcacatttacacacagtggcgcacagctgtttaaagacgcaggatccccttttctaggtgccagattctggctataaatcaaccattgcaatcagcarccagcaaaccccagaggtgcatggttcctgcagacatcttccttaggggaagcctgctagaactgcgatggccattttctggggacaggagggacatctgtggcaaagaaggaaaggtcggtgggctttttctgtcttgaatcttattatcttcagggggctgccaggtcttcactgacctggaccttcccggcagcagcctagctcaggaaatgacgcctgggagaacaggagttctaatcctgcctggctgtattatcaagtacagagtttttctcctaaaccttgaatggctgggtcacctcccagaaaagaaaagactccagggcaaagaggacagtacttcagcaattaaaataattttaaatcctgataacatcaattccaaaaaactgccttgttgaagtggcaagggcaatgtctaaaaataatgctttagagttggaatcataactcaagccctaactcacgttcggtaagaatgcgtgagaggcatttga

SEQ ID NO: 282 - DNA, 654 bp, Homo sapiens
cttgtgcctctgaacatcccctccctggagaactctcaagctggggtggagctctcacttcattcctcaattgtctaatctggagagtgggggccaaagcaccaattctgtacacaagtttagtaaatttggctagccacctttcatgtgtctactttggatttgaaaatgcaccatggaaatcaggtgaaaattttttttttttttttttttttttttactttccyactactaacacatcccaatggtagatatgtataagtgaaatgagtgcgttcttcctgcccctataatgacaagcctgacagagaacacatcacacagaagaatgtgccaagaatcaagacctcttagaagaatgttagaaagttttctctccaaatggattctgtctaagtaggaaggccttggcaactagaaaggtctaagatcaaatttatgacttgaaaactctatggctttgggcaaattatctgaacttaattctggactcaatttcttatctacaaaatgggaattaaggcatcaacctcaaagggttgtttaaagaatgtgattatgtatttctgtaaagcacattgcaaagtatctgacacatagtaggtactctctgtaaatattagcttcacttctctcactcctccaactgaactg

SEQ ID NO: 283 - DNA, 1001 bp, Homo sapiens
agacatgtgtccatatctggtggcttaaggtaaagccagacttgggtatcctgattctcacatcaggcaacagaaggtaataagatgaccacctatgccaccctgcccagttaacagcagagaaaatattcaaaccgggcaaagctaagaccaaggaccccttaggcctgacccaaaactattggtacatggagggcaccaagccatagtgctgaaccccaattggaggaggagacacacttcgtgacctcactaggatttgctttacaagataagattttcctggcaagcattgaagttagtgcccagattcaaaacagcaaacttaaaactattatcttcatgcttgctataatcaggtgtaccgcccaacttcccatccctacctccccttccctagtaatccagaggtactcaaggtcactactggctacttaaggtttacatccactcccaaggaaacaccagcaaccaaaagaatacttcccagatggaaaaccmgtcatttgaccttggaatgctctgcctcccataatgaccaaaataaggtccggccagaggggcttacgttttttggtaaggaacaacacattgttttagagagataatctgacataactctgctaagctctgagtgtctatgcatggtaccacagcaaacaccctatgtcccaaatggaaactagcagggtgaaaaaattgttcatctaagatgacattaatctctgtatgcctccttggtacagttcttttccacaacatgcagcttaagattcaacaattttttcattgtgttttgtgtttcctgaagcattcctccagctacctgaagctctcactgattaaaatagacctcctttactaaaaggggtaaactgaggcacagaagaacaaagcaatgtgccttatagttcagaataggtaaacaaaaattggacatctattattttcaaatctctttagattaaaagaaaaaaaaatgtatttctcaaagtccaaag

SEQ ID NO: 284 - DNA, 1001 bp, Homo sapiens
agacacacttcgtgacctcactaggatttgctttacaagataagattttcctggcaagcattgaagttagtgcccagattcaaaacagcaaacttaaaactattatcttcatgcttgctataatcaggtgtaccgcccaacttcccatccctacctccccttccctagtaatccagaggtactcaaggtcactactggctacttaaggtttacatccactcccaaggaaacaccagcaaccaaaagaatacttcccagatggaaaacccgtcatttgaccttggaatgctctgcctcccataatgaccaaaataaggtccggccagaggggcttacgttttttggtaaggaacaacacattgttttagagagataatctgacataactctgctaagctctgagtgtctatgcatggtaccacagcaaacaccctatgtcccaaatggaaactagcagggtgaaaaaattgttcatctaagatgacattaatctctgtatgyctccttggtacagttcttttccacaacatgcagcttaagattcaacaattttttcattgtgttttgtgtttcctgaagcattcctccagctacctgaagctctcactgattaaaatagacctcctttactaaaaggggtaaactgaggcacagaagaacaaagcaatgtgccttatagttcagaataggtaaacaaaaattggacatctattattttcaaatctctttagattaaaagaaaaaaaaatgtatttctcaaagtccaaagtcaaccttctccaaagggaaactgcatgtctgtctagtaacctataggatcattcacacttttttttccttgagaaggaactaacttgccagcctaccaacaattttgccagtgccttggcatcaggcatatctgcacaacctttccagagcctatatcatagtgatctgttcaagctgctcaaagctcagtaatcatactaatctgtgcatagtgaccagtgctacctgct

SEQ ID NO: 285 - DNA, 1001 bp, Homo sapiens
aggcatatctgcacaacctttccagagcctatatcatagtgatctgttcaagctgctcaaagctcagtaatcatactaatctgtgcatagtgaccagtgctacctgctcaaagctcagtaatcagccagctatgtgggacttgttatagatgcataaaatatgtgggtgaaatctacctccaccaaaagagaaaagaatgccttgttgacactttgatctcaagctaacgtttattaataacatcattattatatttaagtgaatgtactagatactcatcgaatcaaagaaatgtttaaaatccatgtggctgaactcaaatgtcaggggatttggagaaactgactggagcttcatgttctaactctccgcttatttgccctggaaccttgggagggtaacttggcatcggtgcactgcactttccttatttgtaaaatattggtaactctaaggattaccatgagctcaaatgtggtgaagtcacatggcaaactgtmaaatgctaccagatatagccaagtattaagatgaactagcaaacaatatgcacaaacggaccttagtatttcccccaaattccacaaacacccaaatatttctgagaattctgaaaacaacagacatggaattttcaagttagctacagctgggtttgaatctgaactcctccactcagcagctttgcaaccttgggcaagtcgtttaatctcagtttcttcatctatgaaatggcaataataatgcttcactattggggcgaaataatgaggatactggcacaaagtttgcgcccaataactatcagaaaataaacagaacatgaggaaaaaagaaaagatggatggagatgagaagtgcttacacaagcaccagtagataaactctacactgtcatcaatgatcgttttccttgtttttcccccaaaaactggcatgctgaacttaggtccctgctttggaaagagaagggtaactgcgacagacctttctcaaaatg

SEQ ID NO: 286 - DNA, 1001 bp, Homo sapiens
aatacggtaaggtcttccttatcatctgtgattcttcattgcattctgtgcatttatttcgtgtcttaatgatgtgagacaactgatgcataaggtatggaattaacttaaatttttggcaaaagatatcaaataggagaaatgtgtaggtactagaagtacaaaagtcggttacatggaaactctttcactgaaaatttcctgtgataaatttcttaaagggtatttcaaaatcagacttgggcaggggcagtggctcatgcccgtaatcccaacattttaggaggccaaggtggaaagattgtttgaagccaagagtttaagaccagcctgggcaacatagcgagacctcatttctacaaaaaagaaaaagaaaatcagactcaacaacacatttttattctgaacatgaatgatactaatgcatcacacaactctaaacgcatcacacaactctaattgcacacaaaaaaagtaattaattgagaacaggtataacasctggcacatagtgggagaccctagatacttcaaaaaacccgtatctacaaacactcaccaggcttagcagattcctgtgcctgaccgaggttattttccatttgtaccttgaaaatatgtacctgattgattttgtcatcttctctgaggtttaacgcttattctgataaactgatacagaggttttaacaacagtatgagtaggaggaaaagtaaccaaaaaaaaaaagttacctatctcataagcttactcaataactctgctctacccttaaatattcctactttcaaaggcaaaattcatcctgaggttcaaaacgctctttgggtcctggcctcctacttccttccttcatccctttctacaagtaagttttttttccttcatgtttatctaagcatctctttcattccaaacttgcagcattcttcccacgctgctctctatatggaaaataatcctttccctgttcttacacctccttcaaatgcttcagaag

SEQ ID NO: 287 - DNA, 1001 bp, Homo sapiens
tagcttacttagatggtctaaaccctgaaattggcaattgagagaagatattctagaaagtacgattgaccaaatttagtgtctaactcgggtggccctcatctgtggggagagccccagttaatgtctgtcattctgatgcaattattaatagtgcccctttacactctcaaaggtatcccagtttgggtggtaaattatacgattttctatctctacaccattatgatctgaagtccaacagccttaaaatttctaatattactttgggtctaaaagcactatctgggtcaatattccacaactcttagagacagtactaaatgctacaagaaagaacaattgagaaaagtggaaggggcagtaataagccacatttgaagtgtcaagtgacaggcttgcacccaagcagtagacactggaaagcacctgggaaatatgacagcgttggccaagtgatcaataaaatatttacggcttgaatagcaatattttgagcgygtctgttaagcatggctctctgccaatgaaaccagacctaccacaatccaccctgcagacctatgtctttctgtatctgcatggagattatacattatacaatcagaaggaaaagggggtgcagataggcgaaggcttcagaaaagcagccaagtagaaatagcctgtttatgcaatttggaaaacatccactgaagttttgaaaaagatatcatcaacccgacagaaaaaataaagcagaaagtagctagagacacatgacaagtaaaaatgatagatttgggaatagccttgacattcctaaccctgagttaagaacagcttaacagctgtgagcgaagggtagacctagaatactgcaaacatagaggcaaatgctatcagaggttccttgtgagcaggaaaatggagccaaggttttcattaaggagcagctaaataaaaacacggagatgatgttgttcatatacaaattcctctctgcggtgacagtgtgggcc

SEQ ID NO: 288 - DNA, 1001 bp, Homo sapiens
acaagaatcctggttctctgcctttcattctgaggtaagcattgctggaactttcaaacatctttctaaagcaacacatctggactgccaggcctggggacaacccacaggatggaccctttccccaagccgtatgaagcactgagctaacaatgaggccacctgattcagctcagggggctcttgcagagatagcagggagccactgtacctcctgaacccccaaagcaccgaccagcattgccttctcacctgcctgtgttctaatttccagagtttttgagaataactcaaaattttaggtataaaatgcctacaacatctcatcagtttctaaatttctagagtgtggccttaggccaagtatgcatctctcagaaactcattttcctcatctgaaaaatggagaaaataatacttccaccacacctcagagtaagtgtgaagcataaaagtgctcttttatctggctgtgcccagcacacaatgcaggctcgatgygtgcttcagaaatatcccaacaacttttgaatgacaagaacctaccaccttcaatgcaagctcatggaattccaccacagccatggattattcattacacaaaccagagagacatctgtaattacactgtcactgtaaccattgcagagttatctgctgtattctgaaacagggagactctcctgaaaaatcctgacctacactaaccagctctcagtttgcagagatttgatggagcccagagagacctgggctccgggaggttgaccacgagctggtttgtctcctggagggaggcgatgctcctacagggtggtctggcctctttaagagaaaaaaaaagttacacagacaaaaaaacagcaacacaaaccaaccaaaaatgccaggaatgcaagctctgccaaccaaataaataaataaaataggagatgctttataataactggacatgatgcatttctcagccctgcataattgaaaacttgacttttccatca

SEQ ID NO: 289 - DNA, 1001 bp, Homo sapiens
tggctttggcacctggccccttcacagcaggctccaccaggagagaaccaggagtgaacccaatggctatatttgtttttaagctatttaagatccttgcaatcacactgttgcaatcaaatagcatatcccaccttactcttacacttgcaaggaaaagtcaattctactgttatttcagagtatatgttaatttagcacttaacgctgtcaaactcctgtgaagtctcaaaatagaataaaagtgcataaaggttcttggtcaggtcctagccaggaaaacaaataatccaggtcttgcggctcctgtttggacaccccactttcttactgcctctctttggcactcatgaatttgggagggggtggggagaaaattctggtttaatcatttaagccagataagatcccacactagctgtctccacacataagaaactaagcaacccaaagaaatcattctgacaaatatttaagtcacagctgtggataaaaagctaygctgtgagaagttaaactttaaacacatgtcctatatggtctgatgggcaaggcaaatccgcacttagccaatgtcttgtccttccactaacaaaagcagacagccctggccagaaacaccgtttctcccatccttgctttgcacctgcaagttaagtctcagctgaggtttctttgctgagcttttggaaggtatcttgcaacattactcaaagcaatatacattgcgaagttagaaacaggaattgattgtacttcagccactggctcactacatatttttatgtcaattatttacctttcctgtgactctattttcctctctgaggtatgggcataatgttcgcatataagcaactaaaggtccagaaaaaaaaaagttgattatagtctatatattttttcaagtttttgtctttattttttccaagataataaataatggtgctagaaatcaaacctctttacaatgaatggcagaagactgcccaatttctttg

SEQ ID NO: 290 - DNA, 401 bp, Homo sapiens
tctttggcactcatgaatttgggagggggtggggagaaaattctggtttaatcatttaagccagataagatcccacactagctgtctccacacataagaaactaagcaacccaaagaaatcattctgacaaatatttaagtcacagctgtggataaaaagctacgctgtgagaagttaaactttaaacacatgtcctatayggtctgatgggcaaggcaaatccgcacttagccaatgtcttgtccttccactaacaaaagcagacagccctggccagaaacaccgtttctcccatccttgctttgcacctgcaagttaagtctcagctgaggtttctttgctgagcttttggaaggtatcttgcaacattactcaaagcaatatacattgcgaagttaga

SEQ ID NO: 291 - DNA, 1001 bp, Homo sapiens
ctgagcttttggaaggtatcttgcaacattactcaaagcaatatacattgcgaagttagaaacaggaattgattgtacttcagccactggctcactacatatttttatgtcaattatttacctttcctgtgactctattttcctctctgaggtatgggcataatgttcgcatataagcaactaaaggtccagaaaaaaaaaagttgattatagtctatatattttttcaagtttttgtctttattttttccaagataataaataatggtgctagaaatcaaacctctttacaatgaatggcagaagactgcccaatttctttggccagttgaaattttgttgtatcgaagttcacatacaaaagatgaccaatggcttggaaatcttttttgaaaaagaaagccattgcaaatatgcttattataatggacgctgactgtagcgttaggccttattgttcccattttacagaatagaaagctaaagaaagttacttgcccwgagcttatttttaatcagtaactgaaatgacggcaccatatacattgtctctaatatttaatattaaattaccaaaaaaattgcctcagctgttcactgtgatctgaaacatgtgttgccagggctctttttcattcccaggatgaaagatcccttgtaggtatgtggactgacatatcgacacgatatttcccagatgaccaaatctgtctcttcccccataaacacccataacaacacatataaacaagctgttcttaaggaaaggacctattagttgagtttatatctttgatgtgaactatcttttcacttctatatatggtttcaatcaactgacaaacagaactcattctagcttcctcgaacccccaaacacaaccatcatagaaacagcatttctgaattgtaggcctaagtgccttaaatgtctccatggttccagctgcgctctcagcattgctcccaccaccatcatccttgcgaggagacaaaatctc

SEQ ID NO: 292 - DNA, 1001 bp, Homo sapiens
tcctctgaggcagcgtccatctccccttaacattaaggaataaggccagagggttctcgctcatttgggaaaataaaaaaagcaggaatggggcgctggaaattctataagcttttccccaccactcacaaaaacacagctgtgaaaataaataccaccccccaaaccaagggtctagggccaccaacagtcctcctcctcctcctcctcctccttctcctcctcgtcctccagatccagctgccaacagcatcccccgctcctgaagaaatgcaccgcccagaagggaacggcgaaagggggaagaagtccaggggacccccggcctctggccgagagcttgggtgggggcctcggccgtcgccactcacccggggaggggaaaagctccagatcgactttttccgtcttgatgatggtgagagtcggcttgagatcgacggccgccttcatggtgccaggagtgggggacgtacgggatggtagcaagtttgcagttabtgttgtttttctttttaatgaggattagtaacagggggaaggggacgggggaaatccgactttcttcccaaaaatctcaaattcccgctgcctttctttcccccgcgcccggacggtgcgcgcccggcactccaggggaagttggcactttgcggcgaagtgagcgcgctcgggtcccagcctcgcccgcgccgcgcccgctcctcctgcccggccctcgcccgctccctcctctccgccggcggctgcctcgttcgctctcgatctcccggccgctctccctccctctcgccctcccgcgctctcccctcctctttagggcgtttctcgcggcgccgcgtctcggccgctgggtccgcgcgccctgggccgggcgatgtccgcttgggggagcgaggggcggggcgtcggggcagggcggggagccgggggcggggccgagcaccgcggccaatctccgcccgcggcccaaagcgaaaggaagggctggcgagcgcggg

SEQ ID NO: 293 - DNA, 401 bp, Homo sapiens
agcatttgactgtaactgtaacctctgcctctggtaagttttgacacacaggcttaccttcatctaatcccagttttgtgcccttgaagccttagtaatttgcagatttcccacagcaaatcggggaggaagccaggaacagaaaaatctgtggctcctggtctaaactccagattaaatccctccttagtgaccagaggraaatatttgtatgtgatagtcctaatttttgaaagaacaaagactgttgcaatccagctgtgtttccacaaggtatgagaaaacaatgctggcctccagatgacaagaacagacccttctggtcctgggaaaagcctagagaaacagctgatgaatgaattgtacatttacacgtccaaatgaaccacaaaaaaaaaaag

SEQ ID NO: 294 - DNA, 1001 bp, Homo sapiens
taacggctgatccagaaccagtttatgactcacagatgttgatttactggtataaatgtaagatttagaaaaaaaaaaaaaaaaaaaaaagccctcaattaacaacaacctgtctgagctgcatttgtggtctcatttttctctgagaaaaggcaacagtctctgtcatacacagaaacaagctttgaaagcttacttctaaggcaagtggtttctatgtgagaagtttagtcattaaaagtcacactagggaagaaaaatgcctggcacttcaatatctacattatcaagcagcaataaaatggaaaattagagataggaaggaaaattaaaataactctcttaattaaacttggatgccaaaaagccttagggtcagttaagggacccaagccaggggactcagatggtactgttgctgactgcaggctggctctgtgacctcaccaaagccacttaacctttttgtgtcacaacctcatctctgtttcagggaataaratcagccctagctctccctagaatggaacacagactcattggctattgtttagaaggcacaataaacaatgagggtaggaggagctgcagtcaggagggaagaagggagggtggggtggggttgggggagaggggaggacttgggagcctgtttgccctggaaagctcaatataagaaaacaaagaggatagtagtgtgggctttggaataagactcaggttcaaattcttactctaccaactagccagctgaattgccacaggtaagtcatttaaacaatcccgaacctcagttcctccatgtttcaactagggataatagcagcacacaccttttaaggctatttgaatgattaaatgagataatgtatgcaaagaatttagcacagtgtctaggtgagaattagtatttgattattgttattaagatctagtatacggtagaatatgtgggaaatcacattaaatgtctgtctacagccatctctttgcagaatagc

SEQ ID NO: 295 - DNA, 1001 bp, Homo sapiens
cagttcctccatgtttcaactagggataatagcagcacacaccttttaaggctatttgaatgattaaatgagataatgtatgcaaagaatttagcacagtgtctaggtgagaattagtatttgattattgttattaagatctagtatacggtagaatatgtgggaaatcacattaaatgtctgtctacagccatctctttgcagaatagcttggatgctcaattttcctgaacgatctccagcgagagatagaacaactatcaccacatttcatttaaaaatctcttcaagacccttcctcagttcttaaactggcaacctgcccagcatcagcctcacttgagaaattcgagaactacctgattggagaagagaactagatttatatttgttttgagtcacagaaaagtgacagtttaaattctgaaagaagatcacatttgtagtgcctctttggagacaaaaccttaggtcttggatttgtcacatgttagagctcartgggagtttatcagtgctctccaagtccagcactcctatttaccagaggtgaaaaatgagtgtgagtgaggaaattattatttccagggccacacaatctaaaaaagtcagtgtcagtactagaaccagatgccctgatagcagttctctccctggcatctccttgcatttactttgcatttcactttggcaggagaagtaccagacacccttgagacacaagacaggatacaatggacatgggagtagatagatgagcagactcaatttctagaaatccaacttctctacactggatgtattgtctttgggcaaatacattgcaggataaccacactatggttccctgtgggagacagcttggcatgggctgtcaggagagaaagggcctgggttggctctattgctgtctgcagtttctttagactataattatgaaccattcaactgcatctgcagccccaacaatgtggggtggattggcctaatccacagaccaa

SEQ ID NO: 296 - DNA, 601 bp, Homo sapiens
tgtgaaacactttcaagagtccagggctggcagtgagaggtaatgacaggtaacgtgcagaatgaagaaagcagaaagcatatagaagttgcttcttaatggaaacgtgtttcatcagaatgatcagaaacatgtgttctccccagattgggaaaccatcttgaaagacttcatcacaaaaaggccttgggtgggaagtaccacaagggacccatccaggaggggtgggaggaggtgcagctgggtgggaagctggcaatggactgtgagaggaaaaaacaaagggcagtcagcgctctcrtggcagattcccaagagagaaccctttccaggaatttaaaattctgaataattgttgagaatttctaaaaatcaagaagattataaacttttctttcaggggattccacagcattgagagagaccagatggctggcaacaaaattccagatccaggaaaggtccagcatctacatatccatccacttttagtgagctaatgctttctcctacagagtgtatttgtctaattgaattgaattgaattgaactgaggtgtggaggtaaaaaggctattgcaaataagtgttcctgtttccaa

SEQ ID NO: 297 - DNA, 1001 bp, Homo sapiens
taattgaattgaattgaattgaactgaggtgtggaggtaaaaaggctattgcaaataagtgttcctgtttccaaatagtccatacaaaaacctgcagtttcttgccaagcagaaactaccaggctttggtttcctcactatagaataaatttaaactctaaaataaccagggaggcaacatagtagagtgggttaagagcacaagcttggcagtaaatagacgagagtttgaattttagcttggctgctctccagatgtcagtctttgacctcagaaagcctcagtttcttcatctacagaatggagatgcggaaagtgcctagttcacagagttgaactgagatgagatgagatgaatgggtgccaagtgctttgcactgtgcatgatgcagaatgaagactcagtaacccttcactgctattattgattttaaaaatcagaattgtgacttcggatttagtgagcataaaattttcatgaatgttaatccaaactgtartatatagtattcttatgaagaaatgaggacacagtgtcctatcttcatgtgcgctgttaaaatcatgacatagtgacaaagataagttttggtctaggtatgcaaatcatgcaaatccttgacaccatccctcttggatgaaaggggattaattcccactatatagatgtgagatacaattatgaaagttctaatcatatactcacagctacattacaaattagcagcaaagagaatatgtaccctcttgaatttcttccagtattgggttctccactctctggattgcacgtttgatagccaatgatttttgcaacctaaacaaaataagaccttcttaagcaactggcctcagcatttgactttcaatctgggaagaatcccacatgctattcaatatgcccccatagcactctgcctaggtacttcccaaactagcacccattaggcagcaccttactgcactcacttcacagaagtctttttctatgttattgcat

SEQ ID NO: 298 - DNA, 1001 bp, Homo sapiens
tgatggggacatactccaaaatgtacatggctgagtcctcttgctctcctttttttttttccccagtgactttggggaggtttgggcagtgatcctgcatacacaatactgttcttgttcttcttttctcttacagagcagccttgaatagctctgtctaaaattattagcaggggcagccctaggctccaagagatcacagccctcatgctgggcctgaacaaagaccctgctttttcccaacaattagccctgcaaaaaaggacatctatctccctctattaaaaccaccacgtgccttcaagtcagcccattgtaaagctaattaaataacacgcctctctccccatgcaggtctcctgattagctttcctctgtcagaaacctctgcaaagagcctagtgatagacaagccaatgttccacttctccttagccccgctcccatcgccaattagccgtcgcctttgaaaagccatccttatcaatgttggtgagtttrttcacgctccatatccatccaaagcccagacgctagtcacctccaccttaaaggaatggataaggttcatactgcttttaaaataaattatttggaaaggcaaaagttttcatcacagtgtaaaatctttggccagcattccccacatcgcaatacacaagggctgccgccgccattgcaggagagtgtcagagaaggacttttctgaaagtcagagagcctgggcaagatgcagccaaggtggccatttctaccagatttctaaaaacaggatgcagaagaccaccctttaggttaaactcccttagatactcctcaccgccaaacagataaaatccaagcacagtccaaaaggccaaaattggtcctctttaccttttgaccacacctcaccttctcccccacatagggaccctgctctctgacaatcctggacttgtggcaatcccttgaacacactctagttcttcactcttttatgcatttttacaggctttttt

SEQ ID NO: 299 - DNA, 1001 bp, Homo sapiens
ggcagtaagttctttattactctcccttaccacagtgtgcctccattctcagatgtttccttaaagaagagtaatctaagacctctaaatacataaaaaataggataataagtaaagacaaagagaccctcatttttatatagatttgtctcctccagatgcagcttggcatgtatacatgtatacaaagcagccattgagaattaagcatgtgaaaatcacacctgttaatttgtcaaggacagaccaagtaaactataaggcagaaataaaactgtttcaacaaagataaatggaaaacatggttgaaaaagaagaatgatttggaatgaatgtcatagtattaatcaaataaaaatataagatgcatatagtcaatataatttattcaaatagtaagaagagaagaaatatgtatcataaatgaacattatcatgagatattgggtacaagaattcaatacattgggtaaacagactgtagagatcttaagagcttargatttcagagaatagcatacattctgtggtctagaaaaagctgttttctgatccaattgagactgtgagcaatgttaagaggcataacagccaaatcaagacacacaagaagcctctcattaggaggagaaagagcttggaattggttgaagggagcagccgtgttgacagttcatgtcaatacattccagttagcaggttatttaagcaatgacttcaggctaagctggccttgtaattctgcaaatcagatcccatagaagagcaattagcagacattcatttcatactctcttcataaagtttgggtcattttaaattttttatgtgtcaaacttcagaagtaaatatgaatacacatcacctctttcctttgattaaaacaatagggatgctttaccttatttagcatgaaagatcacaaaataattccaacatcacctcacagcacctctgagaaatgcctaagaggtgggaaaggatcccagcctcactgtatg

SEQ ID NO: 300 - DNA, 1001 bp, Homo sapiens
atagtattaatcaaataaaaatataagatgcatatagtcaatataatttattcaaatagtaagaagagaagaaatatgtatcataaatgaacattatcatgagatattgggtacaagaattcaatacattgggtaaacagactgtagagatcttaagagcttaagatttcagagaatagcatacattctgtggtctagaaaaagctgttttctgatccaattgagactgtgagcaatgttaagaggcataacagccaaatcaagacacacaagaagcctctcattaggaggagaaagagcttggaattggttgaagggagcagccgtgttgacagttcatgtcaatacattccagttagcaggttatttaagcaatgacttcaggctaagctggccttgtaattctgcaaatcagatcccatagaagagcaattagcagacattcatttcatactctcttcataaagtttgggtcattttaaattttttatgtgtcaaacytcagaagtaaatatgaatacacatcacctctttcctttgattaaaacaatagggatgctttaccttatttagcatgaaagatcacaaaataattccaacatcacctcacagcacctctgagaaatgcctaagaggtgggaaaggatcccagcctcactgtatgcagtatctgtccagggtacagagactctctccaatgttttgcacaactttgatccaagtcagctgtgcaaaatactgaagatgcatattagctcaactctttcaaatcattcatgtgtccaaaatcactttcacctaccaaagtccttaaaatgtgattttctcctgccaagtctttagtcgtcatttgttggtttttttaattagaccttttatcactatgtaccataatttacctgagacattattttcccactaacacagagtgtgtagggggagagggagggaaagcatggcatggtgaataaagagactattaatccactaattcctacttg

SEQ ID NO: 301 - DNA, 1718 bp, Homo sapiens
gaggaaccacttaatacaaataattattttgccatagattaaggaggtagttcgtaggtgacatatgtatttaaaaatctctatccacgacagtggacagacaatggagaaagaatactcttttaacaaataataggggagaaccagatacacatacgaaaaagaaagaaactagacctttgtgcataaaagttaactctaagtggatcagagacataaatgtaagagctaaagctataaagctcatataagaaaaaacaggattaaatcttcataaccttgtgttgggcaataatttcttaggtacaatgctaaaagcactagaaaaacaaagaaaavatagataaattgggctatatcaaatctaaaacctatggtgctgcaaattctaaacatccagaaagtaaaaagacaactcactttatgggagaaatatttgtaaattatatgcccgataagggcttgtattcagaatatgtaaagaactcttacaactcaacaataaaaagacaacccaatttaaaaacgggccaaggattttaatagacatttctccaaagaaggtataagaatgactggtaaacacgtgagaaaagctcaatatcattaattattaaagaaatgcaaatcaaaacgacaatgaaatactactgctcattcaccatgaggataaattggaaccctcttacattgctagtaggaatgtaaaatgaagcagccactttcaaaaacagttgggcagttccacaaatagagttaccatacgacccagaaattctacccctggagaaatgaaaacatattcacacaaaaaacttgtacattaatgttaatagcagccttatttataataaccacaaagtgaaaagcacctaaatggccatcaaattatggataaataaaatgtgccatggccatataatggaatattattttgatgataaaaggatatactgatgcctgctacaacatgggtgaaacttgaaaacattatgcttagtggccagtcacaaaggtcacatattatataactctacttatgagaattccagaataggcaaatttataaagatagaaattagaccagtagctgttgaggtgtggagacaggaagaatgagaaagaatgaagatcgactgctaatggatataagatttctgttaagaagaataaaaatgttgctgggcgcagtggatcatgcctgtaatcccagcactttgggaggccaaggcgggcggatcacctgaggtcaggagttggagaccagtctgaccaacatggtgaaaccttgtctctattaaaaacacaaaacattagccaggtgtggtggcaggcgcctgttatcccagctactcaggagtctgagactggagaatcacttcaacccaggaggcggacggaggatgcagtgagcggagattgtgccattgtactactccagcctgggcaacaagagagaaattccatctcaaaaaaaaaaaaaaaaaagaagaagaagaaaaatgttctaaaattaaattgcaatgatagctgcacaatactgtaaatacactaaacagaactgtacactttaaataggtgaattgtatagtatgtgaattatatctcaataaagctcacctcaataaaccgtttaaaaaaaaaagttggttttctggaggtgaaggcaagacaaaaaaagagggagaatttcctatcatccaggaaagcctgcccag

SEQ ID NO: 302 - DNA, 1719 bp, Homo sapiens
gaggaaccacttaatacaaataattattttgccatagattaaggaggtagttcgtaggtgacatatgtatttaaaaatctctatccacgacagtggacagacaatggagaaagaatactcttttaacaaataataggggagaaccagatacacatacgaaaaagaaagaaactagacctttgtgcataaaagttaactctaagtggatcagagacataaatgtaagagctaaagctataaagctcatataagaaaaaacaggattaaatcttcataaccttgtgttgggcaataatttcttaggtacaatgctaaaagcactagaaaaacaaagaaaaaatagataaattgggctatatcaaatctaaaacctatggtgctgcaaattctaaacatccagaaagtaaaaagacaactcactttatgggagaaatatttgtaaattatatgcccgataagggcttgtattcagaatatgtaaagaactcttacaactcaacaataaaaagacaacccaatttaaaaacgggccaaggattttaatagacatttctccaaagaaggtataagaatgactggtaaacacgtgagaaaagctcaatatcattaattattaaagaaatgcaaatcaaaacgacaatgaaatactactgctcattcaccatgaggataaattggaaccctcttacattgctagtaggaatgtaaaatgaagcagccactttcaaaaacagttgggcagttccacaaatagagttaccatacgacccagaaattctacccctggagaaatgaaaacatattcacacaaaaaacttgtacattaatgttaatagcagccttatttataataaccacaaagtgaaaagcacctaaatggccatcaaattatggataaataaaatgtgccatggccatataatggaatattattttgatgataaaaggatatactgatgcctgctacaacatgggtgaaacttgaaaacattatgcttagtggccagtcacaaaggtcacatattatataactctacttatgagaattccagaataggcaaatttataaagatagaaattagaccagtagctgttgaggtgtggagacaggaagaatgagaaagaatgaagatcgactgctaatggatataagatttctgttaagaagaataaaaatgttgctgggcgcagtggatcatgcctgtaatcccagcactttgggaggccaaggcgggcggatcacctgaggtcaggagttggagaccagtctgaccaacatggtgaaaccttgtctctattaaaaacacaaaacattagccaggtgtggtggcaggcgcctgttatcccagctactcaggagtctgagactggagaatcacttcaacccaggaggcggacggaggatgcagtgagcggagattgtgccattgtactactccagcctgggcaacaagagagaaattccatctcaaaaaaaaaaaaaaaaaagaagaagaagaaaaatgttctaaaattaaaytgcaatgatagctgcacaatactgtaaatacactaaacagaactgtacactttaaataggtgaattgtatagtatgtgaattatatctcaataaagctcacctcaataaaccgtttaaaaaaaaaagttggttttctggaggtgaaggcaagacaaaaaaagagggagaatttcctatcatccaggaaagcctgcccagt

SEQ ID NO: 303 - DNA, 1799 bp, Homo sapiens
gaggaaccacttaatacaaataattattttgccatagattaaggaggtagttcgtaggtgacatatgtatttaaaaatctctatccacgacagtggacagacaatggagaaagaatactcttttaacaaataataggggagaaccagatacacatacgaaaaagaaagaaactagacctttgtgcataaaagttaactctaagtggatcagagacataaatgtaagagctaaagctataaagctcatataagaaaaaacaggattaaatcttcataaccttgtgttgggcaataatttcttaggtacaatgctaaaagcactagaaaaacaaagaaaaaatagataaattgggctatatcaaatctaaaacctatggtgctgcaaattctaaacatccagaaagtaaaaagacaactcactttatgggagaaatatttgtaaattatatgcccgataagggcttgtattcagaatatgtaaagaactcttacaactcaacaataaaaagacaacccaatttaaaaacgggccaaggattttaatagacatttctccaaagaaggtataagaatgactggtaaacacgtgagaaaagctcaatatcattaattattaaagaaatgcaaatcaaaacgacaatgaaatactactgctcattcaccatgaggataaattggaaccctcttacattgctagtaggaatgtaaaatgaagcagccactttcaaaaacagttgggcagttccacaaatagagttaccatacgacccagaaattctacccctggagaaatgaaaacatattcacacaaaaaacttgtacattaatgttaatagcagccttatttataataaccacaaagtgaaaagcacctaaatggccatcaaattatggataaataaaatgtgccatggccatataatggaatattattttgatgataaaaggatatactgatgcctgctacaacatgggtgaaacttgaaaacattatgcttagtggccagtcacaaaggtcacatattatataactctacttatgagaattccagaataggcaaatttataaagatagaaattagaccagtagctgttgaggtgtggagacaggaagaatgagaaagaatgaagatcgactgctaatggatataagatttctgttaagaagaataaaaatgttgctgggcgcagtggatcatgcctgtaatcccagcactttgggaggccaaggcgggcggatcacctgaggtcaggagttggagaccagtctgaccaacatggtgaaaccttgtctctattaaaaacacaaaacattagccaggtgtggtggcaggcgcctgttatcccagctactcaggagtctgagactggagaatcacttcaacccaggaggcggacggaggatgcagtgagcggagattgtgccattgtactactccagcctgggcaacaagagagaaattccatctcaaaaaaaaaaaaaaaaaagaagaagaagaaaaatgttctaaaattaaattgcaatgatagctgcacaatactgtaaatacactaaacagaactgtacactttaaataggtgaattgtatagtatgtgarttatatctcaataaagctcacctcaataaaccgtttaaaaaaaaaagttggttttctggaggtgaaggcaagacaaaaaaagagggagaatttcctatcatccaggaaagcctgcccagtggggtctatgaacatcatcttaagaccatatgcttcaccaaagttcagtggaaaaatgtctaacatttccatgaccttct

SEQ ID NO: 304 - DNA, 1001 bp, Homo sapiens
taaatatttgtatcctggttgtccaaacttgtcctagctagtggagggatggttggtgtcttggtcctcagttagatcatgggtaattccaagttactgactggtttagggtgtcagtgacattagagcatctttactttgtcccctattaatcaacacatatttattaagcccttgttcttcatgaggcgttggggctatgaagtgtggttcagtctcatcctcaaggaacatcacgcaacctggctgccgtgctgagacggacacagccaagctgcagagctggtgagcaccaggggactgggaatgatgagagggatggtcctgttgagactagaattatggagagaccctcctgaggcctcccagtcacgtgaaactgagggtgagggggtttgccttgaggagcactcattcatccaaacttagttggcagaatgaggacagagctcgatttggaaaggggttgttttactggtgtttggaagagtggccactccrgctctgctttatgtatccttgagcgttgttattctttcttctctctcctgtgttgattttcacctccctcaccctggtctggcctctccgtggccttcctgccgctttcagagatgagcttagactccacacggggctcccaatctgaatgaaatatcccattcctgggaccgctgctccctcacttcattagtgctccttgctgtttataaagccaggagataatatttttaaattccatttggagtttcccgggcagcctctctctaagccacttaggaagtttagaaaagaaggtcatggaaatgttagacatttttccactgaactttggtgaagcatatggtcttaagatgatgttcatagaccccactgggcaggctttcctggatgataggaaattctccctctttttttgtcttgccttcacctccagaaaaccaacttttttttttaaacggtttattgaggtgagctttattgagatataattcacatac

SEQ ID NO: 305 - DNA, 401 bp, Homo sapiens
aacatctttacctttgagaaacttgacaaagagcagcatgaaaaatcatctccacttgggagtttatgtacttcagtttaaggaaaaggaaggccatgtctctttgctatgaagaagagacattctgatcttcaggctatgagcaaatggagaaggcctcagatgttaataagatgtaacttgtagcaagcagagaccatygagagctgcaagtgttaaagcaaggcagctttaatctcagttgcattgggagatataagacttaagccttgtggcattaataggattcaagaattatacaaatataaatacagccattttgaccttttgcttatacaaacaaaacctattttgtttagaattttaaaggatcacttttctcatgtcctcaaatttttagt

SEQ ID NO: 306 - DNA, 401 bp, Homo sapiens
ggcagcactgccaccagcaagtggaaggagagaagggagagagagacagaggaaaaagaattgggatccaggtgggcatggacagagaggccaggaacaatggaaacagatgatcatcgaaagaaagcatgttctctaagaaggccgagcaattcacacacctctgtttatccagctcagactctgtgactgcaaaacttytaggctctctgacaacagccaaaacgggtgtcaggaaatgcaggataggcaaaactatttgcaaggtgaagacctaaagcaacctttcttgggcccattcctagagtttagacttcctgtcggggaataaagtaacccaaaatttatggagaaggcccgggactttccattcaagaacaatagcatctgtacccgcataa

SEQ ID NO: 307 - DNA, 701 bp, Homo sapiens
ttgtaaggagttgttatggatgtgttcccccaaatttagaagttgaaatgtaaaacaccaatgtgataatattaacaggcggaggcattatgaggtgagtaagttgtcagggcaaagccctcaaggatgggactaggaccctttaaaaggacctgaaggaatgggtttggcctcttccctcccttccgccactgaggacacagcgttcatcccctctagagaatgcagcaggaagggtccatcttggaagctgagacgggactctcaccagacacagagactgccaatgccttgatcttgaacattccagcatccagaacggtgagcaataaatttctattctttttgaattacccagtctcaggtattttgttatagcagcactaatggaccaagacaggagtgctataacaaaatacctgaggaaactccagtaattcatttaacctcttaggatctgaatttcctgatattgcaagatggtctttacattgtggtctsactctgaaattctctagcttgtgatgattgaacctagtagcttacagaagccccacagtccaagatgctggaaaaatataggttattttcttctttccttcaatttctgtgacaaccactaagagttatgagcataaataatttccctaaacattatgtttcagcagtctcattcccactttggttttaaatttcttttt

SEQ ID NO: 308 - DNA, 401 bp, Homo sapiens
tgaggagtttttaatacagttacttcaccctcaaattaccaggaatgtcccttaagcccagagtcttatcataggaaattctggcacttggggatatgtagttagcctcttgggcataggtgccttccctgaggtggagcacagtgggccactcctgcccgagcatgttgttctatctcccaaagtctgtggctctgggargaggtgagtgggcagttcctttcctctgtacagcccaaggtgtttcctaaagcccgcatggccaaaggggtcactagtcccccaggaactcctccgcacatcctccttgccggtgagacatcccaggctgggccatgtttagtcaaaactgagagcagcccagcccgctcattcccgccactctcagctgggccagcaca

SEQ ID NO: 309 - DNA, 1001 bp, Homo sapiens
taggatgacattatattatatctgcaacttttatacttataataggctttttatctcagtgtctaaactaagtacatatttgtgtgacatttctttctttctttctttttcttttccttttttttttttttttagatggagtcttgctctgtcacccaggctggagtgtgcaatggcacaatttcagctcactgcaacctccacctcctgggttcaagcgattctcatgccacagcctcctgagtagctgggattacaaggcatgtgccaccacacctggctaattttttttgtatttttagcagagactgggtttcatcatgttggccaggctggtctcaaactcctgacctcaactgatccgcccgcctcagcctcccaaagtgccaggattacaggtgtgagccactgagcccagccatggcatttcattcttagccaaaatattaatctgttttaatttgattatagtacctgtaaatagaattaacatggactggyttttaaatcttatttttcaagtcaatgacacattttgctctgaaatcacaatatcattatttattttaacaaatttctacaatatcgtctttaaggaaattttaatgtcatttgtgttaactttaaataatgacctctatgtgaggaaaaggaggaggagcccttttctggcaacttcttcagccctcgatatgatcttaaactgcaagtcctttggcaatcgctactaagcaaactcgagtgactccttgcctggacttgtcgtgtagtggagtgttggggagtgggcagtttaaacatatttctgatatatattatcgtctaaacctttttctgattctaattttttgtaaaagtaaacggtgcttacatgaacacagaagccattttaaaaagaagaaaaatgtggtaaaaacagctactgaagagagatgtctcaatcatccttaaaatgtgtcttttcccttgaacagaatagctactgagagtttttggttttt

SEQ ID NO: 310 - DNA, 401 bp, Homo sapiens
tgacacattttgctctgaaatcacaatatcattatttattttaacaaatttctacaatatcgtctttaaggaaattttaatgtcatttgtgttaactttaaataatgacctctatgtgaggaaaaggaggaggagcccttttctggcaacttcttcagccctcgatatgatcttaaactgcaagtcctttggcaatcgctrctaagcaaactcgagtgactccttgcctggacttgtcgtgtagtggagtgttggggagtgggcagtttaaacatatttctgatatatattatcgtctaaacctttttctgattctaattttttgtaaaagtaaacggtgcttacatgaacacagaagccattttaaaaagaagaaaaatgtggtaaaaacagctactgaa

SEQ ID NO: 311 - DNA, 401 bp, Homo sapiens
aggtatgtcacccagtaacccaagaaacagataaacagagagaaaccctgcaaaagggattgagcattattgatcttgaaaaaaggagaagggctattaaataacttgttgagagctattttctacattggaagtctgagtgtctagaatgcttgagcaattttctggctgaagggattttccagttagctactggtcatyattacatatcgaacatctctgttgacctaaatactttcgaaagttcattacacactttcataaacttaatactatgcatttaaaaagtcgttcttgaataatctcgaagattaaattcctaggcataccaatcagaggccaaattcttattgttaggaagtgacgctttaacttcactgctttccagtttgtatttgtct

SEQ ID NO: 312 - DNA, 1001 bp, Homo sapiens
tcttaggtctaggaatctaactaagaaaatgccaattctagtctctgaaacctttgaaatactaacaatctacactttctagtcaatcatacttctgtcagaacatcttcctgaagatcaaaggtaatattcaatacactgccttaccataaaagtggccatagcctgtgtacaaatgctatgcctcaaatcctgtattttaccatgaaattcaacaaatgatcacacttggccttaggatgtactcctgagccagaagcatggtaagtactcataaataactgaataaataaataaggattgtgttttacttcgaacctcaaaacaaaaaaagaataagctggaggaataatgtagagtactctttgctttccaagaatggtcgtaatagaggccatggaataagagattgttttccaagtcaaatgcaaagaagggccacgagattaaaaacgtcaactctaatccaatgaatgctgccaatgaaacctctgaagagaytagcattttaaagaattacattacagactcttagcctgtgaagcatgtcagacataatctagagtttagacttggctctggctctaaaggaattctcaacaaaactgagaggcaccataaatagaaagagatattacaagaacaatgagaggggactggatagttgcaataatgcccctttaaaattgaactaaaagataccagctgccttagatctctcaaatccagcaagcaacttcttggactatgtctgattgtgattttcatggtggagtttcatttgttttattacccgaaatgtaaggttccaatttctcagtataatgctaaacagcttgctagcattcttatataaagagggattgtgcaattccagtgaattttggagttggaaaaaattcatcaatcttctcatttatttcaatgaactgagtcctaagaggttacgtgtttagcagtgatcaagaaccctggagttacatactatgggtgaacgtaga

SEQ ID NO: 313 - DNA, 401 bp, Homo sapiens
actgcttgctgcgtgtatggccatgagcaaatttcttaacctcacaatcagtttcctcaactataaaatgcaggtaataatatcaacactttcaggattatagaggaggatcatacaaaacacaaatacttagcagcatgctgtataaatagtaaaaatggtcaataaataataattgttattattgctattttatcagtmgtgcctggcaattagtaagcattagtaaatgcttactaatgtcactaattagtaacactactgttttatattaattacttttttctactgcccaacatggcagaggttatttaagtgttagagctagaacatggatagctaaatctctcatctctttttctaaagacttgtattcaagtcatgaaaacaggattcccttt

SEQ ID NO: 314 - DNA, 401 bp, Homo sapiens
taaagacttgtattcaagtcatgaaaacaggattccctttcataatcataggttgagtagcattagtcaagaattttgcaggagaaaagagccacaatttctgtttaatggtagtctgtttgtaccattgttatgcataaaaccaagaagtaagcatttttcttacagtggagaactaactcattgaaagattgcatagcmcaaatggtgaaatattgcagcttcctgagttaaaccaacatctttttgatataatgtcgatcttttgtggacttacgctttagcaactagatacaaatataaggaagtagtaaagcactgcggaaaatagtgcaagatttcttgtttgttcatttttttcatttttgctttttcatttgtttttgctttttctttagagc

SEQ ID NO: 315 - DNA, 713 bp, Homo sapiens
ctcttctcattgagatggtgaaaaataaaatgagaaaatagagagagaaaatgctttgaaagaagaacactttgcatatgaaagaaattggagattttgtttatgatagctcagatgaatcctgccttgtctcattgcaacagcctgttataatatttcattgttggaactgaaattgcctcataatagacaagtgtcataggacttggatcagtagataaacactacagggaagcctatttcagatcaaaatggtgaagtgcttttgaacatttagagagcttttgaatatttggagccattcaaaaacaaaatgagtgcctggaaagcactgaataagttgaaacagagctataagaccagctagcagagatgctgtagaaaagtttcttgcactggamcagacaacagctaacattctatcccagtaagaatctgggaattcactacaatgatttttaatgctgcttttaaataggtgaagggctgtaatgtagaagaggaagtgttttctttcagattatcagactaagcccagttgatggaaagtataagaagacgaactttggcacaatgcagccaatgcaacaatattcacaatattcatggcatttagaaatgccatataattaattttttcaaagtcgggtagatgtgagaataatctgaccaaagctaatccaccagtgttagacctcaaactttagattctg

SEQ ID NO: 316 - DNA, 610 bp, Homo sapiens
ctggctctgttctatgccacccacagcaatgggctagatacactctctgaatgccaaacttgtgcttcccaggcaccctgctgccaaaatatagctggagaaagcagccagagaaccccatagtcaaggcaagcacaagagcttaactggagacaagactgtggggttgaaagggagggagatgaatcctcttagatgtgtgttgactccttcctaagttcaaagcatttatgcttttaaatcatctctcctccaagtaaatttgtgggacaagctgtattttctccacttaatagacgatgaaattgaggctcagatttgatttggatcatagccagtttgcatagatagcaccagattctattccttggccttctcacttcagggactttttcctaraccacattaccagtagatgtcattctttgaccagcagacaaatgccagagagtagaaattctagccacttggctgaaagttcaggttcagggagtatcttcaagagagggagggactcgagaccagtgtgcccagctccttcgcctctgccccacccagagctgagggcctggacctcatgtgccctccccacacggtgcctactttctct

SEQ ID NO: 317 - DNA, 401 bp, Homo sapiens
tagaccaggtgggttcaaatttcccctattctaattttaatttccacatgatcagaataaacatggctgccttgagatctcattttccagtgctgccagaaatgaaaattccacatagcctagtggaccttcccacctcctttcactggacagcttgctgtttagaggctcctgccattcttaacacggcagctgtcacarcagttagccatggaaagacccattctctcatttgatcccatctccctgccaggacaggatataggccttaaaagtgcttcctggtgtaaggactgagtcggggtttatttatcctaggttacagcaaacattacttcaaaaaacaggaaagagagtctcatcttgttgattatgataccagttatagcaatgaggtggag

SEQ ID NO: 318 - DNA, 501 bp, Homo sapiens
agaagcatcatgaccaatgaccttggataactccactttcttacagcccctgcctcaaacagggattaaggaagaaaataatctctgggatgctaccttccatgaatcagggtctagcaccaacaaatatttgggtatgattcatccagcatcttcactctcattgtcatatttgatgtgtgggacaactatatgaattaggccagtcagataatactactttacagataatacaactgaagctcagaaascaggtgcagttgagagttgagccagatccggtttcaaatcctatctgttttctataaaataatggcagcctcttctgagaatgagaatctgccccattcatgccaccctaaagagatggtttgctttacctgggacttcgagctccacccttgtggcacagatgtcattcgtggaggttaagtgttcttggcgggcagaggtttccatgagagctcatttatgttggctacaagactgttcttctcctag

SEQ ID NO: 319 - DNA, 501 bp, Homo sapiens
cccatggtttttaggatccttagccctgccaatggttatctgagcaggggaagcatatttgttttaagcaactgggagtgtagaagacatgggtgcttccttcctgggatggccaggcaacaagaggcatgtaagaagatttccaaggaagagaaggcaagccatggggctgagtgggagcaagttggtctgctgggaaggagcagaaatactgaccacctcaagtcctgaacacccagtggaggtcatgyctttccatgggtggtctccaaattctgggcatgctttttcttcctgtttccaaatagcttagcaagcttaatccatccacacaacatgtaataagctcttctgtgttccagatatttgataagaactgaaaataaatgataaagcaagattctgttcttaaagagcttatcagaggagtaagtaacaagaaatggtgtgaatttttagcagaagcttgtaaaacatcagacgagaaaaacacgatatgtg

SEQ ID NO: 320 - DNA, 720 bp, Homo sapiens
ttctgttcttaaagagcttatcagaggagtaagtaacaagaaatggtgtgaatttttagcagaagcttgtaaaacatcagacgagaaaaacacgatatgtgtgttctatatggattggcagggtacattattttataccaactcatgacgttccttacccatttgatgtgtgttaaatcctagttccccaagtccataaggagctccttgagggcaggakcaagactcatgtttatttgttcaacgatacctcacccagcattaagcacatcaaaagttgttcactaatctggacaagttcttcccctatctggacatgtggtagaatcccactccctgccctgttgaaattgggagtggtcctaggatgtgctttcactgatgaaattcgaacagggtcacttggcagaaaattagaggaccactgaagagtttcggcctttctgtttgtctctctggcacgtgtcaggtgacagctgcttatcagctagggcccggagtaactctgataccatggaacaaaaccccctgccagcccagtgttcatgcagcatgagtaagatgtgttgcttcaagccactgaggtttggctcttgttaccacagtgtaacctagtccagtctgcctggtacagaagtgttccacaaatatttgctgatctctgtactgatgcctcgattatagcagataggtaaggaagtaaataaagtaagttggtag

SEQ ID NO: 321 - DNA, 501 bp, Homo sapiens
aggccattgacattccatctctttcagcatttcttccactttgaggctgctttgtggctgctcaaactcagatttaagtttgctgtgaaccttagcagtgaatgcctctatctttgcctcaagacttttgtagtcagaataggcaatgcaataagtagtcctagatagagaatggtagacaatttagggaagagttaaatgagagattgtctgaaaaagtgtgcgaagattggaaaggaaaagttccaccragacagagcttcccagggattgcagtcaaaaaccactaggaaattgagatagatggtgatgcctttaggagcttggcctctggcatcaggcaaacccgaccttgaatcccagctattcactcacctactgagtgactgagcaatttactgaacctttctaaccaattcagtttcctcatctgtcaaacaagagtaaggattgagctcagctcttagggccattgaccacataggaaagtaattttcctta

SEQ ID NO: 322 - DNA, 501 bp, Homo sapiens
agtagtcctagatagagaatggtagacaatttagggaagagttaaatgagagattgtctgaaaaagtgtgcgaagattggaaaggaaaagttccaccgagacagagcttcccagggattgcagtcaaaaaccactaggaaattgagatagatggtgatgcctttaggagcttggcctctggcatcaggcaaacccgaccttgaatcccagctattcactcacctactgagtgactgagcaatttactgaamctttctaaccaattcagtttcctcatctgtcaaacaagagtaaggattgagctcagctcttagggccattgaccacataggaaagtaattttccttaataataaggacacatttttatattatgtgcttttaaaaggagccttaaataaagagaagtgagatcattttccagtgcacttagcatagtaacgacaacatagaaagcgttaaaaaaaatgacagcttaagaaagcaaaggatgtggaaacac

SEQ ID NO: 323 - DNA, 501 bp, Homo sapiens
tgaaagagggctctgcctgggctcagcttccaggaaactctcaaactcttgcccagagcatcgtgatgtagccattggaacctcacgcaggcgatgatgatccttttaccagatatcagaacttacctaaccttcagccacttaaaaatgctctctggaaagtattcaacaagggcttgagaaaccaaggagaccctgatggaggagatgtcaaataacgtgagagccttgttctgtctaagctaatttcyggcactttccagagagttagaagtgattggtcttcggtctgctcagctgactttgaagcattggccaaagggctcgggacaagcagggagaagctggaagtcgtctattgcctccacctgggactgcctcaatgtccttttgttccagctggatgtagccccagaaatagcagtaaaggaaaaacatgtgatttgagtttccccatctcccttttctgtgccctctcccttaccaggggatttttcctgt

SEQ ID NO: 324 - DNA, 601 bp, Homo sapiens
tagccccagaaatagcagtaaaggaaaaacatgtgatttgagtttccccatctcccttttctgtgccctctcccttaccaggggatttttcctgtgcccaggcaccccatgtttcttgaagttctgccccagagacaattattccctccagtggagtggagaaaacaagagacttggaattaaaagacacatatccaaatctggatgctttcacatgccagttcttatctgattgcccctgagcctcagtttcctggaaatagcagtaaccaccccacagtaggtaattattttattataytatagtactttaacagatttgggtttgatttgaacagcagagataagaagaattaatttctgctcttgtagatgaagcgaaatttttcaaccaggtaaaattccctaacttgctcactccattaattcctccaaccatccattcactcaataaacatgtattctgagcctactattgtgttaagtagcactaattgacgagagctgaaagagaattcagaccttgggaatgaggctgacagagaaacagatggtaaagcaggagagtggctgcggtgtttaaagcagcccagcagataag

SEQ ID NO: 325 - DNA, 1001 bp, Homo sapiens
cacagaataaatgcccaacaaataatagccataattattcccattcttggtcgaccaccttaataaaagctaccatagaggcagggaatcagtaagaagagatgactaagaggatgcttactgcatgtaggaaaatcagttaatgctcgtgtgactggcttatttccctttgcatactgtccttcaggtccatccatgttgtcacatatggcacgattttcatttttttttaaggccgagtaatattccactgtctgtatctacccattttctttattcgcccattgatgaacatttaggttgtttccacatcttagctcatcttgacagtgctacaatgaacatgagcatgttaatatttctccaagatcatgatttcaattcttttggataaatacctaaaagtggaatggctggatcctatattagttctgttttcctctttttgaggaacctccctactgttttccatagcggctataccattttacattcccaccrtctgcgccagagttcgaatttctccacatcctcaccaacactttttatcttttgttcttttgataacagccatcctcactattgtaaggtgatatctcattatggggaaaaattatatgaaaaggaagcatcaaattaataggcaagaaaaccagtacatagtatttggacagttggcatattacttaaaaattatgtatgaatccaaaaaattaattaactcttactatattagtattctgattgttgacattaacctgtaacaataggagaaaaagttagttcaggaatcacttcccaattacatctgttacaaatgcaaggagaaacaaatacaaggagaaactcctttgcatacaatattttaaagaaaaggacaggtgagttttgggatgcgaggagaggggcaagaaactgtcttctgtgtggagagggatcttgaaacatatcttccaatgggaggccaaatgcaggggggcattgctttcaagaaactaaag

SEQ ID NO: 326 - DNA, 1701 bp, Homo sapiens
ggtcaaatgagcaaaggcaccatcccaggcacagaatgtgcatcctgtggttgttggggggagtctgtcagagtcttattctggactagagtcaggactgggtcccataaggtcagggcagggtgagtgtgaccttggggctacaggcaaggccaggcatccaaggggtctcaactgccccaaacaaccccatcctgccaggccccactccccctgtccctccctcccattgttcagtcccctcaccccctcaccatgggcacctgcagtctcattcagagacaccctcatcttagagtccctgatagtggggagtttggcccctcagaggccttggttgctttggtcaatccataatgcctgggcctgggacccccaccatttcttgttcatcagggacacagcagctgtgaaggcagctgccttcaccagagcagcgatgtagcccagcaagggcagggacagagacgcaaggtctgggggatttttccacaatgctgcagaaagaaagtccctgtggagctcagtctcagccatccctgccccagctgtgagctgaactgaatttcaggcatctcagagtcccttcacctttgcatgacccatttccaggacatgacaggtcaagcccatgggagaggggatcacccaggtctccctcatctccatggacctcctgggaacattgccagggtccactccacccctggacgctgtccccaagcttcaccctctttttataagttgtacatttttattatgaagatctttgaacacaaaaatagggagatgaaagaataataatgtccccaaggttcccatcaccgagtccccataatttttgattttcaaataatgttgactcacccacaacagagtaaacgattccctcagacaatagtctgaagcagatgcgaaagccatcacaaacttaaatggagagaatcaatgatttcttgacacgaaaaaacagttaacgagggtctcaccaaatgtcttgtgaatttcattgtgtatatttttagttgacttcgtggtgcattacgtatttgtggatttaactttagtttctatgtggagtaaatacttgatgttatcagtggtgaatgtgtttttagacccattctatctacagctgtctcccaaatggctgtcaggcttttcctggcaaggcaggagtggcaggagcagagagctggtcctgagaccctcccacagtcaggatgcagccactgcctccctgagcaggaacccagtgcttcctttagcttctcttttcctgaaaaattgttctagcatcaagaggctcagtggggttcaggctggacattggcataactgcttcctaggacatgtggttacttctagcaaagccacccatgttcatcattcttttagtgacrttagctgtgtttgatgatcgataactttgtgcttcagataaaaaggaagacagagggttgaggcttccattcacctcctcgtgagagctgcagtgtgtcgctgaagggagggcccagcagctgtgctatgaacctaggagtgtgcttcctgctttggaaaaaaggaagaaaagtagtttcttcccttttattcaccactttgataatggacgatctggtgctcggccatactcgagggtgaacagaacaacatagagccagagtgagctccagcatgtgaggacatctgacatgtggg

SEQ ID NO: 327 - DNA, 2000 bp, Homo sapiens
ccgccacacttcagcacaaacaggaggaggtggccgtctagagtctggagtccggggagaggaggaccgctcctctcttggagaccaccgctgtcactgacgtgtccaccacccaccactggcagtgcagcccctgataatgccccataactcatccccatctaggatactgcagcacccgatggtgcccacaacctgccccctgccattggcagtgcagcccaggttaatgcccccaaactgctccctgatgttggcagtgcagccacggaaagtgcccccaaccagcctcccgccatgggaagtgactcccgggatagcgcccccaagcagaccctagccttgggcagtgacgcccgggtaggtcgcccaaccgccacccaccccgttgccgagagtgcagcaccagatagcgaccctaacatgccccccatcactggcggtgtagcccaggatagcgccgccaacccctcacttgacgcgacagtgtagcccctgatagtgcacccaatctgccacccactgccggcactgcaaccccggatagtgcacccgacacactccctgctgggcagtgcagccccccaatagcacccaacccgtccctccacccctgccactggcagtccactcccgataatgcccccaacacgttcctggctgtgggcagtgtagtccatagatagcgccccaaaccagcccccagccatgggcagtgacacctcagatatcacacccaaggagttccccaccatgggcactgatgtcccagacagcaccccaactcgagcctcgtgtgaccaatgcagccacagataggcccccaacaagcccccaccccaccactgctgcaggaaatgatgcctgggataacacccaaccattccccaccgtgggcagtgcaacacccagtactgcccctaacacaccccccacacaagatggcgcccccaatccccccctcaccttgggcagtgtagttcacgatagtgcatccaayccttggcccctgagctcactgcccctctccccccgccacaagtccctggatagctcacctactctgccacctttctaccactttggctgtgctgtactctacctcactgccaccagccacagtgaggcgagccatgctgctgcaggctcaagcctccagcatgccaccggtgacaactccttctctaatctggggtcggaacagatgggcgggcagacgtagaagaacctggaatggcaagactctcgcttacaaaggttatgcaaattaggttcctggactacatgttctgattggatgagagaaaaatctctaggtctactatgattgggctttattttcgtgttgtgactggatgagaggaagtcttaggataaccaatcagaacatgataacaaagtccaatcagactaggcctagaggtttctcttgtccaatcagaacatgtagtccaggaacttcatttgcatcaactccacatataaaggatgccaagtgaggcggctcctcattctaggctcttcagtgtccactggtgtagctgctccattccaggcttacaggagaaggaggaggaggcacttgccacgcacgctggagactcgagcctgccttggctccccttgctgctgtggttggtggtggcaaggaagacgacagtgcagccaggatggtaaaaaggtggtgggataggttcgctatcccaggaggtactgcctgaggcatggggggtgggttggggtccctatccagggcgtcactgcccgtgttgaggggctggttgggtgtgctatctggggcatcactgcctgtggaggggagtgggttggggccctatctggggtgtgctgcccgtggctgggggtgggttggggcactatcccaatctgtactgctagcggcagtgggtggttttggggggcactatctggggatgcactgcctgcggccagggggtgagttgggagaactatcgggtgctgcaatgcccttgttgggc

SEQ ID NO: 328 - DNA, 1001 bp, Homo sapiens
  misc_feature (501)..(501): n is a, c, g, or t
gttggaatcatttacttgcagagaggtgtgtgtgtgtgtgtgtgtatttatgtgtgtactcatgtgtataagaataggagaaacactttgtgggcatatcctgctgaggtgagtaacgtgctgattagtgaactccagtctcatcccatttaaacctggaggagaaccacatcaagcacagaagcagccaaagcagcatttcaacaggaaggaaacatctattactggggctttgaagaaacatgccatgaaggtgtactaatatcacaaagggaagggaaggactaaattcagcatgataaacaaagtcccttttttgtaacggaagtgtttgatgatgtttgatcaatggtggatctatctcttgaaaggaaaatgcatttaaaccccaaatggaggattcttatataaggtgcctagcttgtaatgatatattcatgtttataggtagagtgactggtttttagagaagaggtttttttttttccttcatttttgaangaaaacttgtctgtctctaggctttgaaatgtagaattatttacctttccccaaaatgaaatgtttcactgaatctcctacaagcttgtggaggccatgaagcatgttgaataagagcacaggctctggaggccctgccacccacaaagggtgtgctaaggtaaacaactgatagtattttgaaaattagatgacttagaatccattcaataaattttagctatttttattgtcttttttttctaaatctatttggaaaatattgcagataaagtagataatacctttctaaaacacagtgagaccaggcgcagtggctcatgcctgtaatcccagcactttcggaggccgaggtatgcggatcacgaggtcaggagatcgagaccatcctggctaacacggtgaaatcccgtctctactaaaaatacaaaaattagccaggcgtgggggcatgcgcctgtaatcccagctactcaggaggctgaggcaggagaatggcg

SEQ ID NO: 329 - DNA, 1001 bp, Homo sapiens
gatgggaaacaacaggccatgattttatgtttttgttaaaccagtataattctttcaaagcagtgtatatcacaactatttctctgtgttgaagagagtatcaagttcttaaagaaaaatgtaatcccagcactttgggaggctgaggtaggaggagcacgaggtcaggagttggagagcagacaggagaattgcttgaatccgggaggtggaggttgcggtgagcagagatcgcgccactcactccgtcctgggtgacagagtgagactccgtttcaaaaaaaaaaaaaaagaaagaaagaaagaacattttctattctgcaggtgggaggaaatgaagaatgcacctattatttttgtgttagtacaacataaaaaaaatttgcattgtaaagcaaactaccatcatcagctctttaatggacagcagcagacaggaaactgcctccaccctgagacttaaagactgagcaactgagttagatagcaggtgcgcaggcyaatcaagtcaattttctaacacagagtagcatgttgtggaacttgttctattagtcttttttctctgttaaggaagcaaggatctctctgtatggaagcagtgctgctatttctagtttgaggaaaaaaatggtaaagaatttgataattaattgttgttaaaacagcaaattatattttaaacacagattgtccacacctgtaggaggaggaatctcaagaatgcacacaattaataaaagctggttctgaattacccatacaagtgcgcactgcgttcagtaaacaactgatttgcaaactatatcctttctttcccagaaatagcaggaggaagtttttcaaatcaaaaaaaaaatctaactaaaatattttatacgtgaaggcctgcagaattttacttccttttgctgttgaaaaatcacaatagccaagaggagtaatgtattttattttaacttttaaaaagtcatgatggttaagggtagagtggaggtgca

SEQ ID NO: 330 - DNA, 1001 bp, Homo sapiens
tgttgcccaggcttgtctccaactcctgagctcaagagacccacccacttccgcctcgcaaagtgctgggattacaggtgtgagccaccgcacccagtcacattccttttaacacttgggttacatctcctgaactgaatggctaggtaactaaagacatctgagaaagtttcttgcacctatacattaagccctctttaccaagtcatataacctatcactatctattgaatcttcccatatgagctctaaaggctattgttatcacaaaacacaatgccaacttttgagtgattaagtatccttctcatctataagaggatgttgcccagactaatctcaaacttctggtctcccgccttggcctcccaaagtgccaggattacaggcataataaaactccttgatgccatcttcctagaaagatatgcttagcctcattcaatccaaatagttcctgcatttcttttgcatgagatgtaagacattttctgacataamataaaccaaataactcaactacattcatttttataacaacagctttttgaaatataattcacatacaataaattcatccttttaaagcatataattcagtgggtttcagcatattcaaagagttgggcaatcattactatctaattatagaacattttcatcatcaccaaaagaaatctcatacttattaggagtcacctccctcccatccctagcccctagtaataactagccaactttctgtctccttagatttgcctattctggacgttacttaaaattgaaagcatatcatatgtggcctttcttgtgcctctcagattcacctatgtgacagcatttatcaataatccattcctttatactacttaataatatttcactgtatggatataccacaatttgtttattcactcatgacatgatagacatctgggttgtttccattttttaccattattaataatgctgtaatgaacatttggctacaagttttcatg

SEQ ID NO: 331 - DNA, 1001 bp, Homo sapiens
tacacaatataactagtattgacttaagggtactgtgatcaccatgcagtgatcccataaaagatgtgaccaaaatacccacttaaaatttgaacgtcagtcatgtaagaacatgtaaaagatgaagggaatatttcaaaaacgactatctgacgtaatatgatacttactatgactcatatgggctttgttcttcatctcatcttcaaataaaaagttgatgattagaaaaaggagcattagaagggggaagtaacactactcggcaatagagaaaaactccggtcaaaggaagagcatagttacagagctccgaatgtcagggaaaatcaagcatccgtcattcggaattagctctgtatcggtcggtttcttcattacttaattgtacggggggaaactacttcaaagtaagggctcttacgagaggcaacttaagcatttgaaagtgcaggtttatttcctcctagcgagaagtagggggtcactagtgagaaaccyatttcaatctgtgagacgcccccttctactcagcccacgtggctaaagtaaacagaaggtgggccggggcggggagaaacagaactcggtcaatttcccagtttgtcgggtctttaaaaatacaggcccctaaagcactaagggcatgccctcggtgaaacaggggagcgcttctgctgaatgagattaaagcgacagaaaagggaaaggagagcgcgggcaacgggatctaaagggagatagagacgcgggcctctgagggtaaggtgggcgcaagcggaggtgtggtgcggggagaggtgccagtgggtggaggcgggggccagagcgagggcacgtgcgggtacactccggaggaggtgggtgcgcgcgggggcgtgtgcgcgggacctcgaagtggtggtggagtgcagaccagcaaaaagtttcaaagggaaatcttagatgtcacgtctttgtccaggcacccgtgccatcccaacctcccacctcgcccccaa

SEQ ID NO: 332 - DNA, 1001 bp, Homo sapiens
acaaagatgactctttccagcgatttgaaattgctagataagactatgaaattctattaaaacaataacaacaaaaacaatttaacttgcattagaagcaattaaagcataaaaagtagatctaagattttctaaatattagatattctaaaatattgacattatacaatgtctagcatccgtaacttttgaagatattttatttcaaggtaatttcataagaattcataagaatttacctactcagactttgggcaggatggaaaatagagtttctgtgaggtgtgcctatgaatcataagaagggcttcttaatgaggtcagtaattaaggaaatacatttcaatagtgacatttgacttacaacattgtttgggggtggagtcttagaagaattgatagggaacttttaacttcaacaagtgaaactaaaacattaactccagttgttgttacctaatacaagaccagtgcccaataaggactttggaattctttcayaacaactccttggcaggtgcacttcacttgttctggaagtgatattcacttgccaatgtctagtaggaccatgtgccactgcctcaaaatcatatcaattcctccggcttctggcataaactggcacatcagacctaattaaagccttaagaagagtttggcaaatatgacaatttaaacaaagcaagggatttctctcactgcaacttaatttctcattgatgattagttcaataagaaaataagcaaaacaatgtcatagttaagaaaagctatctatcttgttattgtccattatcatgttcctaaaattcaataacccaagacagtcctatggaatttttggagcacctaggtagtatgatcacatatatggtaaagaaagaactgaggttatgtcttttattgtaaactaccccatacttattaaaataatttctcttttccaacaaaggataaagtgactaacatacacatctcttccttataatcactgaaat

SEQ ID NO: 333 - DNA, 1001 bp, Homo sapiens
cagagagtaaagcctaaggggaaagtttgacaggctggttgtatttatgtattcatcctgccacatcctcgaaaaaggtatttattgttaagtaggttcaaaaacatcttcaagaccagaaaatgccttcggacgccactgggctgttgaattccttagttattgattcactaatgtcatcatgaaagaatttatgattttcccaatccagtccaccaggagagggaaggccttgataaggatttagatgataaggagaagaattgccaagattgaagacccagagcaacagcaaagaattttggaaaagaaatttcaccaaagagtaaagttagtgttattttggttatgtggaatattagagtgaattaagtagaggaataaaatcactaataaaattggttagcaaaggcgtcataaaatcacaccaatgagaaacagagtgctaacctagactttgtatatcttcagtttcctttcaagcatttcaaacctccccarttagcttcaagtttatccttaggtagatgtgtacaaaagatttcttcaactactttctagtattcaagatattatttaagggaaaaatcacatttatttattcattagatattttggtaagtattctaggtgctggattaaaagagagaaatggctcacgcctgtaatcctagcactttgggaggccgagatgggcggatcacttgagatcagaagtttgagaccagcctggccaatgtgttgaaaccctgtctctactaaaaatacaaaaattagccggaaatcacctgaacccgggaggtggaggttgcagtgagccgagattgtgtcactgcactctagcttgggcgacagagtgagactctttcttaaaaaaaaaagttaaaaaaataaaatagataacatgtcttatttttcctcaggctctgtttaatggtggtgatgatgacatgatggtcatcactaccatccattgagtacatgcaccaagtcatcatgtt

SEQ ID NO: 334 - DNA, 10187 bp, Homo sapiens
tgactgtcatgtgctaattctaacaatatttgaaagacccctatcaaaataaatataccttttagtagccactttattagaaaatcaactttaagttattcccccatgtttttttctaattgagatataattcacataccataaaatttacccttttaaagtatacaattcagttgtttcagtacattcacaaagctatgcaaatgtcacctctacctagtttcagaacgttttcatcattcccagaaggaaaccctgtatttattaggcagtcacttccccttctccccttcttccttcctctaagtggcaaccacaaataaacattcagtttctctggatttacctattctgggcattttgtattagtgaaatcatgtatttggcctttctctctggcttctttcatgtacctcaatgttttcaagtctcattcattttattaaaaaaaaaaagtaccttttttctttttcttttttttttttttgtccacgtatatattcacaccacattttttgagacagagtctcgctctgttgcccaggctagggtgcaatggtgcaacctcagctcactgcaacctctgtctcccgggttcaagtgattctcatgcctcagcccccaagtagttgggattacagttgtgcaccaccacacccagctaatttttgtatttttagtagagacagggtttcaccatgttggctaggctggtctcaaactcagcctcaagtgatccttctaccttagcctcctaaagtgctgggattacaagcatgagccactgtgcccagccacattttctttttccatttattagttaattgacatttggatcgtttctactttttggcgattataaattatgctgcaatgaacatcggtgtacaagtttttgtgtgaacatgttttcagttaccttgggatatacacctaggagtgacattgttagtaatatggtaactttatgtttaactttttgaagaactgccaaactgttttccaaagtagctttatgcttttacatttctgccaacaatgtatgaaggttccagtgtatctccacatcctcaagaaaatgttattgtctttttaattgtaaccatccaagtgggtatgaagtttatctcgtgattttgatttgcattttcctaatggctgatattgggcatcttttcacgtgtgtattgaccatgtatttttttgagaaaagtctacttatatgtttttaattgtattatttttagagttgtaagaatatgttatgttgatacttgaactttgtcaaatgcctggtttgcagatattttctcctatcccacaggttgtcgcttcactttgataatgtccttaaagtacaaaagttttaaattgattttgatgaaactcaatttctttttaattggcagcttgtgcatttggggtcatatttaagaaatcattgcctcattcaagatctgaaagatttacacctatgctttcttctcagagtattataactttagttcttacatttagatttttaattaatgttgagttaatttgatggtgagagataagagtccaacttcattcctttgcaagtagctgtccagttttctcagcaccatttgttaaaagactgttttttttcaattaactgaccaagatgtatgggtttatttctggactcttaattctgttaatctgcatgacttttcttatgccagtaccacactgtgctgattcctgtagttttgtagtaaattttgaaatcaagacaggtaagtcttccaactttgtacttttgcctaccatgtttcttgggtttccatatgcattttaagatcagcttctccgtttcctttctggatttttttttttttttttttttttttttttttggtggagctggagtcttactatattacccaagctggttttgaactcctggctaaagagatcctccctcctaggcttcccagagagctggggttacaggcatgagccaccacatccaacccccttctgggactttgactggggttctgttgaatctgttggtcaatttggagagtattgatatcttaacattaaagcttccaatttatgaacacaggctatttttccatttattcttaaatttctttcagtaatgttttggatgaaacatgtacaaagtcctgcactttttattttttttaagacagagtcttgctctgctgcccagtccagagtgcagtgctgccatctcagctcactgcaacctccacctccgggttcaagtgattctcctgcctcagctggaactacaggtgcgcgccaccatgcctggctaattgttttgtgtttttggtggagacagggtttcaccatgttggccaggctggtctcaaacacctggcctcaagtgacctgactgccttggcctcccaaagtactgggattacaggcatgagccaccacgcctggcctgtacttctgttaaaattttttctatgtattttttttatcctattgcaaaatcaaattttttgttgataatatatggtcataaatttcatttttatatattggtctcatatcctaccaacttgctgaactagcttattagcactaactttttttggtagattccttaggatttgctgcatacaagattatgtcatctacaagtagagatagttttgtttcttcacttccaatctgggtggctttatgtttttttcttgcctgattacccagttagaacttccagaaaatgtcaggtacaattaacaactgcaaacatccttgtcttattcattttagaaagaaatttttagtttttcaccattaagtatgatactagttgtaggttttgtttaaaaaaagactgtgtcaagttcagaagttcccttctgttgctagtttgttgaataattttatcacgaaagggtgttgaacttttctcaaatgctgtggctacatctaatgaaatgatcatgcgttcttctcctttattctattaatatggtatattatattgattcatttttatacattagattaacattatatttctggaataaatcccacttggcctcagtgtgtattactttttatatattgctggagtctgtttgcaggtatttcattgaggactttcgcatctctgttgataaggtatactgatctttagttctcttgtgatatctttggttttggtgtcagagtaattctgagttcacaaaatgcattgggaaatgttcccttctctatcttttggaagagtttacaaaggattggtttaactcttttttaaatgtttgaggaaattctctacccctgggctttcctttgtgggaatttttaaacatttttaaaatagattatttttaaagcaattttagggtaaaagcacattgaatgaaaggcacagagcttccttaagtacatgctgcccctgtatgtgcatagcctccctcattatcaacatcctttaccagaatggtacatttgttgcagtcaatgaacctgcattgacaattgtcgmtgaaagttcatagtttagagttcacctttggtgttatgtattctgtgagtctggatccatgtttaatgatactcattcaccattacagtatcattcagagtaatttcactgccttaaaagtcctctgtaccctacctatttttctctcctaccccactaacccttagcaaccaatgatctttttatctcaataattttgcctattccagaatgtcatatagttggaatgatacagtatatggagccttttcagactggtttttgtcacttagtaataagcttttaaattttccaccatgtcatgatcgttcatttcttttcagcattgaataatattccattgtctggtttatcacagttgatttatccattcacatagtgaaagacatcttagttgcttccaagttttgacaattatgaataaagctgttataaaagtatgtaggtttttgtgtggacaaaagttttcagctcctttgagtaaataacacagagcacagtagcttgattgacagtaagagtaagaaatattttttctcagtctgtgtcttattttttcattcacttgacagtgccatttgcagaacaaacagaaagttttaattttaatgaagtctaggttatcagttaattcatgaataatgtttttggtattgtatctaaaaagtcaacaccaaggtcatctatatgttctgtgttatcttccagaaattttatagttctgcattttacatttagggctgtgacccattttgcattaattttgcaaaagctataaagactatgtatagattcacttgtttgcatgtggagttgtccagttgttcccgtaccatttcttaaagactatctttgctttattgtattacctttgctactttgtcaaagatcagttgattataattaagtggtctgtttctggactctttattctgttccattgatatatttgtctagactttcaccaataccacactatcttgttaacttaggctttagagtaagtcttgcaatcatgtagtgtcagtcctctgacattgtttttctccttcagtattgagttggctattcttttgcctattactaagtaaaaaaagcagtctgaaaaggctatatatacagtcatttattggtcttttgcctcttgatataaactttaaaattactttgtcagtatcctcaaaatcttgcaggaattttgatagattgcactgcatttctagattgagttagaaatactgccatcttgacaatacacatcttcctatccatgaacatggaacatctctttcttggatatccttcattagaattttgcattttccccatatagaccatgtacatattagatttatacataaatatttcatttgggggggtgctaatggtaatgtatttttatctcagattctgcttgtacattgctggtatgcagaaaagtgatcaacttttgtatattaaacttgtttcctgcaaccatgttatataatcactttagatccagtttttttttttttggtcattctttcatattttctaggtgatcatgtcatctagcaaagacaacttctttctaatctgtataccttttattttcttgtcttaatgtattagctagcatttccagtatgatgttgaaaggcattggtgagaggcaacatacttgccttgttcctgatctcagcaggaaatcttcaattttatgttagctctatggttttgtagatattctttatttacattaaatatgttagctgtatggttttgtatatattctttatcaggttcaggtagttcccctcttttcctagtttactgagaggcttttgaaaatcattaatcagtgttggattttgtaaatactttttttccacctattgatattaccatatgatttttctttagcttattaacgaaatggattacattaattgattttcaaattttgaactagactggcatacctggagcaaatcccacatggttgtgatacattatttatgaatgcattcatggtcatggttgctattagtctgtagttatcttttattgtaaagactttggtgttggtattaaggtaatgctgccctcatagaataagttatgaagtattttctctgcttctgtcttaattgagattgtagagaattcatataatttcttccttaaaactttggtagaaatcagaatgaaccatctgtgtctggtactttgttttgaaaagttattgctgattcaatttctttcatagatataggcctatttagattattattttgcataaatattggtagttgtgtccttcaaggaattggtccatttcaccttgattattaaatgtgtgggcacatttgttcataatatttctttattatcctttgtttttgagacagggtctcactctggttgcccaggctggagtgcagtagtatgatctcagctcactgcagccttgacttcctgggctcaagtgatttacccacctcagcctcccaagtagctcggactacaggcacatgccaccatgcctggctaatttttttattattattagagatggagttttcctatgttgcccagtgtggtcttgaactcctggactcaagcaatctgcctgcctcagcctccaaagagtgatgggattgcaggcatgagccatcacacctagcctgatggcagaactttttaggaacaatagaatggtatatggcattttcaaaaattgttttcccctcctcctatggaagcatgaagggatttttctctagtattcattgtgagaacctcatctggctcctgaatgtagaaaactcacaaaactgtgaggaacctattatgactggatgcctttggagttgttcacactgaacctccagcaattcatcaattatatttcagattttcctatcccaacactggttcctacagaggtttctgctccagtaagctgtaattctttttatccatctgcttccttggttgtgagggcagtgattttccctgtgacctcatttctctgacagatctaagtagtcttgattacatcttttaacctgttgtaggtatattcagattttctatttcttcttcagtcaattttagtagtttgtgtttttctagaagtttgttctctagctctgctttagctccatccaataaaatatgagtatgtcgagttttcatttacaacaaggtattttctaatttctatcatgtttttttgattcctgactgtataggagtatatttttacctattacccaaatttgcttgttattcatgtataattttatcagaaaacacactttgcacaatttttgcagtgttacatttatttagacttgttttataacttgacatacagtccatcctggagaatgtttcacgtgtgcttgagaagaatgtgtatattcagctgttggtgggtggcatgttttatagatgtctgttagacctagttggtttatagtgttttttacaacttctgttttctttttaatcttctatctacttttagccattattgaaagtggattagtaaattatctatttattcctttaattctgccattttttgcttcatgtattttggtgctctgttgcttattacatgtatgtttacatttgttacatcattttaatggcttgaactttttattataaaatgtgtatatcttgtagatatcgtatagttaaatctttttaaaaattgatattgctagtctttgccttttaatttttcaatttatatacatttaacataattattgataaggtaggatttgtctgccattttgtctgtatcttgtctttttttgtgttcaatagatattttctagtgtactgttttaattcccttgtcttttactaaattttttgatgttcttaatggtttccctggggattacaactaacttataacagctagtctgaagtaataccaatttcattacaatataaggaaactttgttcccatatagctacattccctctttttactctgtgctattatacaaattacattttattttatgcccattaacacagattatgttttttcttttaaatcagattgatattgtcatttaaatcaaatatgagaaaaatagttacaaaaaaatacatatatgatttcatatttacctatgtaattatctttactggtgctctttaagttcttaggtgtatttgaggtactgtctagtgtcctttcctttcagcctgaagtatacatttagtattttttgtaggacatgcctgaaaacaataaactcttatttatcagagaatgtcctaatttattatataatacatttctgaaagatagttttgcaaaatacagaattcttggttggcagtctttttcttgtggttctatgtcattctactgccttctggtcttcattgtttctgatcagagatcagctattaatcttattgggaatcctgcatacatgataatcatacagttttcatgattttcttgtgttggctttcagcagtttggttatgatgtttatatgtatgcatatctttgggtttatgttacatggagttagttgagcttcttggacatgtagattgatgttgttcatcaaatttgagaagttttcggccattatttttcaaatattcttcctattctttattcttcatcctctactttggggacctgcattatgtctatgttggtatgctttatggtcttccacagatctctgaggttctgtttatgttttcatttttcagactgaataatctcaattgacttatcttcaagtccctttttcccctccttttcaactctgctattgaacccctctaatttttactgcagttattacactttcagctttagaattctatttaataatatctttttcttgagtttatctcatgtatttaataaaatgctgtagtcttactttagttatttaaatacagttttctttcattatttgggcatacatgaaatagctgacttaaagtctttgtccagtggcctaacatctggactttttcaggaatagcctctattgactactttataggggccatactttgtttctgtttctcttaattgtttagacattttaaactaatgtaatggctgagagcagtggctcgtgcctgtaatcccagcacgttgagaggccaaagcaggagcatcacttaagcccaggagttcaagactagcctgggcagcatagtgagaccctgtctctacaaaaataaaaataaataaaataatataatctggtaaatctgaaaatcagattctaccccctgcccagaatatgttactgtttctggtggttgttgtttatttctttttaactactcctataaagtttgtattgtttctcatagatagccatcgaagtctttgcttggttaacttagaggtcagctaaggattagacagaattccttaggtgcctgagatcaataagtcagtctttgacaaaggggtctgtatgtgtgttggggcatgcattcaacactcagccaggctatttgcagctctggattagcctttattccctgcttgtgcagagtctcaaggttagactgtggtgagagtttagggctttctgaggtcttttgtgggccctacagttgcatgtggctttctaaattcccaggaatatattttcaaagcctcctgtggatcatctcatttcccaggtaatttacttttaagcttttttagttatcttatgttttgctccagttattagctacacctgagtcagtgacaatattcaacagctgcctatgattatttgacaaatgcctctgtggaaaaggtggttcacactaggtgaactccaagttagataaagtaaagataaccttactagtgggatcttccaggaaactaccaaacaggtcaaataatgtaaggtctctgtgaatgggactttagagtatatccaaccagtctagagtatatccaaccaatctggcctcctctagtggcagcctggctgctgcttttcataataaatgtgggctgttttgatttgaaggctaccatagagctgtggggaaagttaaaataccacagagctcactcttctcactgaaatcctgtctttttttcccttgaacaaattctccctatattgctgcaagctttttgctaatttccagatctgaaaaagctgattctgacaatatttatcagtacttttattgcttttatggaggataaaattttcagagatccttattctgccatttttgctgacatgtgtaaagtgatcatttctaattgtaaaattccttttgcatttattagctggaatactttacaggacttttcctcatcaaccgttagttaccatttaatatagtttgtaagaatgatagaataaatgcatggcaagaatctttacttctcaaatttcagagattttgatgggaaattatatttagagatcacaatcagtgtctagatgtgctccctgctatggaggtgtcattacttttaggcttttttaatgggcaaatacatgaagtaattattttttagaaagaaaatctgagattaactcaaatcattaattcatactgatttttcctattcatagttgacagagtattattatcttttgttctgcttctcttgtacactgaaattcttggtttttgatattaacaattatt

SEQ ID NO: 335 - DNA, 3249 bp, Homo sapiens
gcatgagccactgcgcctggacttacaatttcttaaaataagacaacagtgaggtttaccacatcaattgaccctttctttcatgagtgatttctctgtggcatgcaatgctgtttgatagcattttactcacagtagaacttgttttaaaattggagtcaattgtcttcagccctcccactgctttatcaggtaagtttacgaaatattctaaatcatttgttatgactcaagggacattaaaaaaaaaagaaaaacaatcttttattgtcatttcaaccaggttcacagtgtcttttttttttaaattatattttaagttctagggtacatgtgcacaacatgcaggtttgatacaaaggtatacatgtgccatgctggtttgctacacccatcaactcatcatttacattaggtatttctcctaatactatccctcccccagcccccaccgcccgacaggccccggtttgtgatgttccctgccctgtgtccaagtgatctcattgttcaattcccacctttgagtgagaagatgcggtgtttggttttctgtccttgtgatagtttgctgagaatgatggtttccagcctcatccatgtccctgcaaaggacatgaattcatccttttttatggcagcatagtattccatggagtatatgcactacattttcttaatccagtctatcattgatggacatctggtatggttccaagtctttgctattgtgaatagtgctgcaataaacatacatgtgcatgtgtctttatagtagcaggatttataatcctttgggtatatacccagtaatgggattgctgggtcaaatggtaattctagttctagatccttgaggaatcgccacactgtcttccacaatggttgaactactttacactcccaccaacagtgtaaaagtgttcctatttctccacatcctctccagcatctgttgttccctgactttttaatgattgccattctaactggcgtgagatggtatctcattgtggttttgccttgcatttctctgatgaccagcatgttcacagtatctttatcagaagtagattccatctcaagaaacttctttctttgctcatccataagaagcaacttctcatttgttaaaagttttttcgtggattacaacaattcattcacattttcaggctccacttttaattctaattctattgctgttttcaccatatctgcagttacttcctccactaaactcttatacccttcaaggtcatccatgaggtttggaatcaacttttttggaactcctgttgatgttgatattttgacctcttcccgtgagtcatgaatgttctcaatggcatctatgatggtgatttttttctgaaggttttcaatttactttgcccagatgcatcagaggaatcactatctatggctgcttatattgccttacaaaatatatttcttttttttttttttttgagttgttgtcttgctcagttacccaggctggagtgcagtggcgtgatctcggctcactgcaagctccgcctcccaggttcatgccattctcctgtctcagccttccgagtaactgggactacaggtgcccgccaccaggtccggctaattttttttttgtatttttagtagagatggggtttcaccatgttagccgggatggtctcgatctcctgacctcgtgatccacacgcctcggctgggattacagacacaaaatatatttcttaataagacttgaaagtcaaacctattcctggatccatgggctgcagaatggatattgaattagtaggcatgaaaacaacatggatttttttgtacttctccatcagaactcttgtgtggccaggtgcattgttaatgagcagtaacattttgacaggaatctctttttctgagcagtaggtctcaacagtgggcttaaaatattcagtaaaccattctgtaaatagatctgctatcacccaggctttcttgttctattktggagtgcaagcagggagatttagcatcattcttaagggccttgggtttttggaatggaacatcagcactgattggcctcaacttagagtcaccagctgcattagccactaacaagagaggcagcctgtcctttgaagctttgaagcctgccattgacttctccctagctaagaaagtgctagatgacatcttcttccagtaggaggctctttcatctacattgaaaatcagttgtttagtgtagccatcttcatcaatgatcttaactatatcttctggataacttgcttcagcttcttcatcagcacttgctccttcatcttgtacttttacgttatggagacaactttccttaaacctcatgaaccaacgtttggtagcttccaacttcagcttcctcccctctctcagccttgatagaattgaagagagttaaagccttgttctggattaggctttggcatagggaatgtttcattccagaccactaaaactttctgcatctcagggataaagttgtttcactttctcatcattcacatgttcatggaagtagcgcttttaacttccttcaataacttttcctttgcatttgcaattttgctaatttttttgttgcaaaaggcctaatttttagcctgtcttggctttccatgtgcctttctcactaagcttgtttctagcttttgatttaaaatgagagatgtgcgactattccttttacttgaacacttagaggccattgcagggttattaattggcctaatttcaatattgttgtgtctcaagtaatgggcttggtgaaagggagagacagagaggaatggttgtcagtggagcagtgagatcacacacacttttaagtagctaagtttgctgtcttatatgggtgtgattcatggtcccccaaaatagttacaatagtaacatcaaagatcactgatcacgtcaccaaaacagatattataataatgaggaagtttgagatattgtgagaattaccagaatgtggcacagagacaggaagtgagcacatgctgttggaaaaatggcactgatagatttgcttaatgcaaggttgccacaaagcttcaattggcaaaaaatgcaatacctgtgagtataatacaataaaatgaggtatgtcggaacctgattatgtcttagtcataaaacttacaaagaagtaggaggaatattttccatgccaacagaatgtatttaaatgatttgatatgtatttgaggt

SEQ ID NO: 336 - DNA, 1001 bp, Homo sapiens
aagtgtgtttccaccataccttgttggtccaaaacacctctccccagctccagcaactgctgcagctgtgcagggcagtccctctccaggtaggccctgttctgcctggcccgaatcttgtgcctttcccactccagcttggtgggccaggccctgggttctgctgctctccaatccagtgtgtcagggcagaattcaaggtggtcctgcccatcatacccgtacttccagtagccctcggtactgttgtcttcttgcatttcacagcccaggatgacctgcagggtgtgggactctggaaaaatccccagccttgttaactgcaaccaaaggaataggtccctatttccaccatccccaaggaccaaatgatctcaggaagcaaattccttccctcttccctgctcccacaagacctcagacttccagctgtttccttcaagatgcatgaaaagatgaaaagctctgacaacctcaggaaggtgaggccccctctccacrtacccttgctgtggttgtgattttccataatagtccagaagtcaacagtgaacatgtgatcccaccctttcagactctgactcagctgcagccacatctggcttgaaattctactggaaacccatggagttcggggctccacacggcgactctcatgatcatagaacacgaacagctggtcatccacgtagcccaaagcttcaaacaaggaaagaccaaggtcctgctctgaggcacccatgaagaggtagtgcagagagtgtgaacctggagacagagcaacaggccttaaccatgtgtagtaggaggggagcaggatgttgaggctccacacacctgcatcaactcataccatcagctgtgtctggtcctcattttgtgaagggtgagttgcagtcctgtctttcttccatatgacagtcctgggtgctctttccttgtgtgcttttctctgccacacgtggctgccaccccctcactgcccccagatcctattccaa

SEQ ID NO: 337 - DNA, 1001 bp, Homo sapiens
cagagccaccctagccattggtataatagaaataattattattgccactcttataaattactgcaccagccagtctacatcaatcccagatggagatattactgaccctcttcctccaggtcacccagttggtaaatgaaagagatgatatttgttcagaagccagtttgacctgcaaaattttgcttttaaacacctcgcaagagtgcctatttcttggaattatcttccatagctgctactgtctccactagctagtttcaaagcatatggatgatcagatacaaagcttcagcttcctgccacttctccctcacttttgtcagtcttgttaatatggatttttacatttttcatttttatttttatcatatgaggaaacttggggttggggagtatataaaaattgtccattgctatacagaaaagagttttggaggtcttcatctcaataccaagagaagtgacttaccgacttaatgtctgtggaagggcttcaarttgaacccagcgtttcctccaagcttactcccttggactttttggagcagagagatgaggattctttgccaccctagggcttaagttgctaatcattaataaaagtcatcaaactacaaagttgactcagaagggcttcttgccaaataggctttgaagaagcattcggaaatccagcccaatcccctctgcagttctttctgctttttggctgatgtaagcttctccaccttccccttgtgagtgtctcctcaggacctcataggtgtcctctggttcagacacttgcatatagctattttgctttgctttgtggtgtcttcaatgtctttagtcttttttgaaaaggttaaaaagagataaattataattaaagagttcagtatttttgtgttttttactttgctatttttgattttcccccttaattgaaattttgttaatttttttcttctttgaaatatgtgaattgtaatattatgggtaaacttgaacttcat

SEQ ID NO: 338 - DNA, 2131 bp, Homo sapiens
aaaaagtatcagcaagttatgtttggatgccaaattgctctccacttcccttccctgacactggcatttccagaacttagatgctcttacatgtaaaagcctcctctagtgcaccatcgagcttttcaggattggacatcagactttttagttcctggacctctagatatacggcagtctctgacaagaagccctttttctgttttaactttttttttttttaagttttgagacaacgtctgactcgctgtcacccaggctggagtgaggtagcaccatcatagctcactgtatccttaaacgcctgggtgcagggactaagggagcgtgccaaccatgcttgactaatttacttttttgtaaaaccagtagtctccaacctttttgacacaagagaccgttttgtgtaagacaattataccacggaccagggggtgcaggggctgggagcaatgatttccggactaaaactgctccaacctcagatcatcaggcattagattgtcacaaggagcctgaaacctagatcccttgcatgtgccattcacaatacagtttgagcttatgagaatctatctaatgctgcagctaacctgacaggcggtggagctcagttggttaatgttcgctcacccctcagctgtgcggctcaattcataacgtgccatggacagggaccggttaccggtcggtggccggggraatgaggacccctggtatagatggtagtctggctatgttgcccaggatggtcttgaagcctggcctgaattaattctccaatctcaagccttttcaactcagctgcatcacaacttaaacctatagataactgtcacagaaacttgtttccagtgttacgccatcttaaaataatgtgggtggctcttaaaagagcctttgggttctttccaaattggcctcccggaaagctctttacttcttagatgtggcctttctaacattaacttcatgatgttgggtcaattttgacttcgaagcccttgccttcactgggctcttctgctgttgcttacccttggctcctttagcctttctcccgctcctaacagttttaggagttgtcgctctcggcttcttggctctcttattggttttagcagtctttggtgacttggagtccctggataaaaccagcttcttggtcttggcagaaactgactttttagccttgcttctggtagatttaggaatcaccttcttactaagcttaaaggaaccggaagcaccagtacccctggtttgcaccaggattcccttgttcactaagctcttgagggacagtttgatgcggctgttattcttctctacgtcgtagccagcagcggccaatgccttcttgagcgcaaccaaagacatacctactcgttcctgtgacactgaaagggcctcggtgatcaacttggacacagagaggttcggcactttgcgacttgcacttatcaagccagccggcttcctccctcgcttcttggttggaagtttctccatagcggctacaccagcactggcagaagctgcaggcacggtttcagacataacaacagagaaacgcaagatgtaataaccagcgaaaagcatgaaacacccgggcggcctcggggccttatatagggtagggcgcgctgtgattggtgcatcacctaggcaccgcccccgccccttggaggaggagtatttgtgtttgttttacccggaaaagttgagtataacaaaacccctctttacagaatctcccagggtctagtgctgaataatctgcggaaattcatatttgacatgacttttctctttttaatgaaaaatgaccctggatgccaaaactattcgagaaagccctcgattttcaatcaaattcacggagaggaacaaaacttccccttttccttgtaaattaataagtaatctttggcagaagacttatttcatctcttcagagtggtcttccaaatggatagcttcaaatcggtagaggaaagaaattattcacgccatgatttttatttaaaattatttatatatgtgagggaagtaacacagatctcttagctgtctaattgcggagtcagaagatgcttatagaattgtcaaaagactgcagaggatgtct

SEQ ID NO: 339 - DNA, 1001 bp, Homo sapiens
tctctcagacttttgcagaaaaatgagtcattcaacaaatatttgaatcgagatagggaaagtgacgaggaagaagtttgcacttatgaggttttaatttgcaattatttggctacctttttgccttcccaaaacatagggtctttaggagtgaaacttcatagccaaacttataccttgtccagcacagagaaggccatcaaaatgcctggtttaaataaaaatattaaaatgattgggagggtaaatcccttgacctataaatctgacctcctttaaacattatttgtatgttccccaataaactattccgtaatttattagttagcaagtggaaataaaaagaaatgtggaatggggctatgcttagcgtcattaagctgacaggaatacagcgcattcaacttgcaaacacccttccactcccacaaagagcaagctgtcactggccaatcaaaacaatgaaccataatgaaacagtttttcttgctccacccactyggtgaccaaatttgaaaaaaaaaaaaaaccgcgccaactcatgttgttttcaatcaggtccgccaagtttgtatttaaggaactgtttcagttcataccttccactgcgataggaatcatgtctggtcgcggcaaaggcggaaaaggcttggggaagggtggtgctaagcgccatcgtaaggtgctccgggataacatccagggcattacaaaaccggctattcgccgtttggctcggcgcggtggcgtcaagcgcatttccggtcttatctatgaggagactcgaggtgtgcttaaggttttcttagagaacgttattcgagacgccgtcacctatacggagcacgccaagcgcaaaactgtcacagccatggatgtagtatatgccctaaaacgtcaggggcgcactctgtatggcttcggcggctgaatctaagaatacgcggtctcctgagaacttcaaaaaacaaaaacaaaaaaacccaaaggcccttttcagg

SEQ ID NO: 340 - DNA, 1001 bp, Homo sapiens
aatcatttttttataacaacaaaggcatttgcactgagagtcaaggaagtaccgaattattcctgtttttactgaattgtattaaaatataaggaggatataataggaaaacacagcatgtgttcatcaatcacttctcctgagtctcctcacttggtcaaaaatttccggagaaatttttgtttgtacctgatttgaaaagaaaaacaagggagcggttggaggggaagggtggagagatgaggggagggagtgccctagtggaaaccacagcattaacaccacctactacttctacttcactaaaggcactgtcccgattttttcttcagagatcactgttttgcctgctgaattcaaacctccaccccagacacactgatgtcattggaggcatcaggactgggggcccaagttttattatattaaaacgagttcatgctggggtaaattttaagatctttagtggacagaaaggcagttcaaattctttgattttartgacaaaatgctttaaactgacaatgcaacctatcaacaaaaggaccatattgagctgtgtgtgggctgcacagaaatacgccgccccagaactctaagtgctcccggaaaagctcgcaattgttacaacagagaatccaattcttgtggctaaagtatctcctgggggacttattacaaatgtggattctagaacccctcgtgcaatgatcctgactaaagcgatttactatgggtcccaagaatcttaatcttaccaagcaccctcaagtaattctaacttcaatagtctgctaaacggcactcagtgaagggtgctaaagctgtcatggggaatttaaaaactcatgaaataagctcgtagaaaggaagtttagggtctggaggacacagagctgaaatgaaatcctgaagtagggttggaatataattaatttatgtaacaatactgaacacctagtgtgtggcgtgcccctttgtttttcaggtaatcagaggaa

SEQ ID NO: 341 - DNA, 520 bp, Homo sapiens
ccttgaagctacggaattacaattctccttcacaaagacagtcaaaggatgtgatctgatgtgttagattttctctctcctgttcaatatggagttttgcatcttagtttctttgggccgctataagaaaatacactaaactaggtgactaacaaataacaggattttacttcttacagttctaaaggctaggaagtctaagatcaaggagacaccatattctatgtctaatgaggctcactctctgcttcatagatagcatcttcttgctgcaacttcgtayggtacagggggtgaacaagctccctcttttataggggtactaatcccattcatgaggacgccatccttatgacctattcacctcccaaaggccccacctcttaataccaccataatggggattatgcttcaacacaagtatttgtttcttgtttttgttttcaacataaatatttggagggtaaccattcagatcatagtagtaccagtatccaaaactgccaccaaatagtttgtt